European Patent Application EP 4 623 692 A1, published October 1, 2025. Title: Bacteriophages against Erwinia amylovora Fire Blight. Applicant: ENVIROINVEST KÖRNYEZETVÉDELMI ÉS BIOTECHNOLÓGIAI ZÁRTKÖRŰEN MŰKÖDŐ RÉSZVÉNYTÁRSASÁG. The sequence listing filed with the application follows.

SEQUENCE LISTING (20 sequences)

SEQ ID NO: 1 - DNA, 53802 bp, Erwinia amylovora bacteriophage Ea PF 1 DSM 34958
  source 1..53802: mol_type = genomic DNA
gacttaataatacggtcccttaacctttttcttccgaagcctatcggcttcaattcaacaccaaagtagctcctgcttcgcaggcataaggtcaacacaatctagtcaacactgtgctctgtaggtatcatgatgagatagctacgcaaactaaatccgtttcattgggattcggagttgtttgtgggcttagttgattgtgtattcaaaccttggagcttatcatgactaattcaaacgttgttaaatctgttgtcccttctatcacttctgctatctaccgcgctaaagaaacacagagctatatgcagccacagacttgtgccattgccgctcttgctatcttccacatgatgacgtcattcacacgcgacgatgttgtaccagccatggccatggttagtcttgcagaagcctctatcaagaaggccaactccactaacaatgacctgaaacagttccactatgttgacccatccatcaacttgattggactggctaagcacttaggttatgtcagcattgcagaagataagtcattcaccatgactgagcgttggattgagctcgtctcaactaaagagacttgtactccactgacagaagctgtgtcagaactcaatcgtcgcaaaccattcatcaagggtggcaaacgtaagccttctaaactgatgtcagaatgtatcgacttcctgcaatcaactgaataccatgttgatgcaccaatggttgatattgttggtgatgtattgaacatgactcacggcgacattccagctgtgattcaacaagaactccatgtttggaacaatgctcgtaacatggttcgtgaagatgttctgttctcagactacttcgctgataaccgtggtcgtttgtatcacgttgcatgtgctggtccaaatccacagtcttctgactttgctcgttcactctattctcataacatcgagaacattgtgaagaaagacagtgcagcatatcagatgttcatggctgaactttatgatatctctggtggcaaatggactgaagctcgcatgttgactcgtgttgctcagaatccagcaggcgctcttgctcacatgttacgttcaggtgatgctcctaagaaaccattcacctacattcgtctggcattggattggttcaagtttgaaacaactggtgaatgtgattcacgcgttggatttggtttagatgcaaaatgttctggtactcagtatctggcattcattgcaggtaacatgactatggctcaagcaactggtttggttaacagtgagtccaaagcatctgacccatatcaactctcgctggtggaactgatgaaactcttagagaagtcatcaatgaatccatctgatgaaatcaaggcacagtatttcaatccgaaagatggccgtaacttcatcaagactccatacatggcagtacagtatggtggcggtaagaaagcactcactggcaacaaagactttgcaacaactgttgctacaatcttcggtgctgataaagttgacgcatttgctgagcttgctgttgaagctgtgaaagcagcacttggtgagaaaatcaatatgttcatcgctaaggtgatggaagctgttgccaagaaatgtgaagcagaaagcaagttgtacattgattaccgtcacactgatggacaggttgttcataagccttgctacccatctcgtgaaatctgtgatgcattcagcattcgtgttgactccacaactcgtgtaatctttggacagcagaatgaaggtaagccttggatgattcgtgagactcagccaacagcagaagaattcgttcgtaccttcgtagtcaactatatccaaggcattgatgcgctggtggcacgtacagttgctaagtatgcaaagaaagctggacttcgtggtttcacttcaattcacgattgtttccgttgctgcttagcagatgcacctttaatgatggatgtaattcgtcaggcatatgttgaaatctttgtgaagaacaatcagttcgaagcattggctaaacagattggtggcattgatatgttccataccaacatcgttacagaagaactgttaatgagcgaacacgcttattacttctgtcagtaagttccaaatcaattaagggctgcttcggtggcccttttcttttatattaaaaacaaaatccattcctcaacccaaagtgttgttgtaatattgcgacaatattttggctttagttggatgtgaagaaacaaaattctgcatgtcattctgttattggtgtacaacaatattcagcatgtcaacttagtcacagtgaatgttacaggtttagtcaactgtagaactccctgagacggctactcaaagttccagcttccatgactgagtaagaatgagtttcatcgagaagatgatggaccaaatgttccagttgagtttcgaaatttccgagtcctattataatggccctaacacaagccgggactattggaactttggtgcttactttgaatagtgaatccaaaatcgagaagtgagtggcatcctgtcccattagttgcatgtgaatgacaaacaacgagtttatctcacagtttattcgctgaaatttggctgagtaagttgcgagataggctccaacttatcattaggatgtacatatggcactatgctagtcacatggtgcctttcttaatttgattggagatactaaattatggcagtattcgcagcaattacgtacaaaggtcagaattgttccaaagatggcatgttcgattcgtgcgatgatttgattattcacctatggaaagagtattcaaagatttctcaggtcgttctcattgatgacggcgaagatgttgtgttcagcaacgttgatagtgctgtctcttatctggagctatggttcaaatgagatacaaactttggctgtacaaagatggcggcaagctcaatcatcttatagttcaggacacttcaattgcgacccactgtaaaggtggatatatgttgagaagccaatcaatttatcccgaagatggtggtaagttggtgtggaagaatgcagcatacccaataagtgttcatttcgctatcaaagagaatgaaggaatttgtattgcagaagcaatgcatatttcaactctggatgcgaatatgaattggcgagttctggactatctttggaagaattgcaatgagcaggtttgattgtaagaacaaactttatcgaaacattgatggacgtttaatacttcgtcaatggattgaacagcgtcacagttgggaatattatcttcgcgattatggcgataatcagtggtatcgtgctggcaatcaacttcactgtgaatatacgtgcaattatcaagccaaacttattggcatcaacttatcgaatacaggcttatgaaaatcgggtataaatcagcaatgtatgcagtatgttatggcgcaagtttgaagagaactttgaaagtaatgcgcgataacaacaaacgtgtaccggcaagattggtgaaacgtcggtttgtgaaactcatgaaagagatttgccactaaatgaaaacaggcgacaaagttgtaatgcgcaaagttgaagcctgtttagctggcttcacagcatataaaatgtataccgttgtttctggtcatggtgaagtaaatatgtctccggctgcaattcgactgggtacaatgctccatcacagtgagagaactttcaatctggtggacgacaatgggaatactcggttttgtaccgtagctcattttcgtctgttcaatgatgagttaaaaggtttatttcaatgacagctcaaataatgtttggtcatctgaaagatggtgaacgatttgctttcttaggtgaaacgttcatcaaagtgttggaagaatccagcgactataacgccgttaatgcagcaaattcatctgactgtgttaagttcggcaaaatcgaaattgtagagaaggtataaatcatgtcaaatctttgcgcgttttattcagtagtgcatcgtgcagaacaagccgaagaagcgcgtgaaggctttgatgcaactgtaactatccaagttccaacatctgtgattctgtttgcagaaaagcacatcaatatgttggaacaacagcttgcaaaattgcaggcaaaagaagcctcagccgataaagaattggttgaactccgctcaatcgccagtgtagcaaaagttcactacgcaaatcacaaaattgatactggtcatcatccaaaggcatttaatcatgttgaatcgtgacaagtcaggtcgtttaaagaaagctcgtgtgcgtgtgggcgacattgctacaattgataagtccagcaaagtgttgggcttaacagcaggcaaaggttacaaagttgtggcaacagcactgtcaaaagaagacaagcgttcatttgttggcgctcattatcaatgggcgtgtgtaactgaaaaccattttgtcataatcaatgaccgtggtgagaaacacttttgttctctgacaccacgcaatccaaattatgatgtgaaaatgtctaaagcattgtttggtgaatggactgtgtaagtgatttatgggagtgttcaaacgagcactccactaatatcatttaacattaaactggagatttaaaaatgagctattatgtagatgaacacggtgttgtagtattcttcaagtaaggagaaatcatggcctacaaagttattaatggtgagcttgtaaatatcagcaaatatcgtagcaggtatgacagcattgccagcaacaaagcagagcgggccatttctcaggaatggtctaaagattaccgagagtcttctcgccgtgtcaggaaatcaaaatgaacaaaggttcgttaatcgcatgtaagggtgaaatccgtggattcactgttgacaaaatttactccgttcgtgcaggcttgggcgatggaaatatcgctcggactgatggtcgcgttggtggttttattaccaatgtttctcaaatgtgtgttcgcgacgacaacggagaaatccgattaatctcgttcaatgagaattggaaaatggtgcgtgaaactgaaaacaccaatccagttcgtgttcccgtaacccatctgtacaaaccaactcgtacaggtttcgtaggacgttaatatgtcttgggaagaagcaatcaaagccatgctcgatggcaagaaagttcgtaaccagtatttcaccagcgatgaatggttcgaaatgaaaggtggtcgaatctattgcgaaggcggttatccaatggatggctggttcacaggcgacgactggcagttaacaggctggtcaattatttaggccgacaggccataggagctactatgtggtttggttcatcgtacaaaaatggttatggtggtgagtcattcacagtattcaaagcaccaaaaggtggtggctttggatggtggctcgctttggcagtaattctgtatctggtgttttattaatggcaatctatatcagccagtcaaaacgacttcttgcccaaaagcgactcagtgaactttatgagttgcaaggcaggcaatcaaagattcgtgaattctttaaatgtggttggggcggaatgtcattccagaaccgaaccaaattggatttggaaatgtatcgcgtgctggctccacaatatcgtgagcagcatagcagaattgccgaattggagaaacattaacattagttggtcatgattaattcaaagaggattgaacatggccagagtgttaaattattcaaaagtcaaaggtgtgcatagcaatgctgtgtacattggtcgctcaatgaaggacattaaagggaacgagaagttccacaatccatataaaatgtttaaggaagagcaacgtgattacgtttgcgatgaataccgtaagcatttatggaagcaaattaaagctggtgaaatcacaatccaagatttgttggatttggatggaaaggatttggtttgttggtgtgctccagcccgttgtcatggtgatacaatcatgcaagcgattgagtgggcaaagaagcaatagtatgaatacaaggtgcattcgttgagtgcatctcaatattcatgtttaattggatatgaagaacagcaatgacgctggaacttaacccgtaaattacttttatatagagagctaaatcatgtctactaccaaaacttatgacgatacaaataccggcatcatcggcaaaaacgactacaaacagaaggatactcatcctgaccagcgtggccgttgtaatgttgaaggtatctggtattgggtgagcggttgggataaagcagccaacggtcgtactttcacttctctggcattcaccatgatgacccaggccgaagttgatacgatgatggaaaagcgtgcagctaaacaagctccacagcaggcagcacagcagcgccagcagcctcaacagcagcaggcaactccacagcagccacagtcaaacaatccaccagctcagagcaacgagccagcaatggactttgacgacgacattccattctgattatggaaagagattacattaaagcccgggatttagttccgggcgatgttatcttactgcgtggtgactggagacgtgtaactcaaatttggttacatcccagctcaccatacaacaaaatccatacagttcgggagaatgaaagcgacaaggctattgctttgttcgagaagattcctctgagctttgtaatagagagaaagccggtgcaagtaaccaaacaagtccatttctgctcagctattgaagaaatggctaagctggaagccttaattaaggcatacgacgaagcaaatagtttgccagaaagagttcaactgacaaacaccaacttcgaaattgattctgtcatcgtacagcgtcaatgccatgagaatatgatggcatcgttcaatcgcctcaaaaatgctgtaaactcggttcaaaagccatgaaagtaattccaccagcaatagccgcaatcatgtggatttcagcgctggtgttctgttacatgcagggctggaagtgattttgagaagctgttcccgatagggagtggcttcaattaaattaactttaatcaaggtaacactgtgcgtaaaattattttagtattaggcttcgtggcattaagtgctggcgcagtggatttcccacgctccgagcaagaagcatttgcattgcagcattctcctgagtaccaaaccatgccagcaagtcagcgtgcagacgttgaaggtgcatttggtaaatcaagttatgttgctcacaacgacccaactggagaaccagtaaatgtcagaaatcaaacccaagaattgccagttgcaaatcaacggccagccgataaagccgatggacctgtcatcactggagtggagaacaatcccgccaataccagtgaagccaaactgtctgactcgacgggagtggtacagcctgatgtacgagtgcgacccgctcaaagcgacactgcgacagaccgaggaacaaccggagttgcagtatctcgaagctccagtatatcaaatgacccaagctcagttgcggttgacaatgtgtcaagacgagttgcaactaactctgctggaatcgaaagcaatcaccgtgccatcgaatccaatcggcgtcaaattgagacaaatcgtcgcgatatccgaagagttggcgcgactgcgattgcaagcgcaaacctacattacgatgccagtaatagtggatacgccgtttccgtcggagaatatcggggagaaactgctatcgctggtggtttacagtatggaattactgaacactcagctgctacagtacaagtatcctatgacggaaccgggactggtgcgtctgttggattgcattcgtcattctaacgaagcgcgtcttgcgaaccaaattagttgattttgaaaggttcttgttccgacaggaaccttaattaaatcaattagaggtgtaacttggaaataaatgacaaaatatctctgacaagttatgccaacctaatccagattgttgtgtttggtgatgatgatggcattgtagcgaacttgtctacagaagatgctttaaaattggcagcactgcttcaacaccatgcaactcgtattatgttggaggaataaatgtacgtttattacgaacaccatgttttctacaatggttctcggaactataaagggcgtgcaatttactctcatcaaattacagttcacgagaatcaatctccagaacaatatgaagcattgcgtgagaaacactgcaacgccaaagtttcatatagcaaatttgcacgtcgtgtttatgttcgtgttcttgcaagacgagcaaagtggaacaaaatgcagccagagcatccgtggtttaaacggtctggtcaacctcattgggcagaagtgagaaactatctgctaaacattcatttcaggattgattacgatgaagatggcactaaaatattcagcaatattctggattagctttatcacgctgattctgtattcatgcagtcatccagtacatgcagccgacaggcttgctgtatttgaatgtgctggtgaacgaattaatgtaactcagcacaacaagaatcctcttattttgtcaatcaaccgagtcaaaggaacttggatgcaaattgttgccgataagccaacggcagtgattacattctacaacctcgactcaggcaaagttgcgaaaattggtaagaattatgcaggtcaatattatgtgcaattgtacaaagatgctgattatgccaatgcccaccagccagagagaactcttccgtgtcgtctaagttagaactttatcgcgcagccaacaggctcattgaatctatccgttacaaacatctggtaacgggtaaagttgttgctgatggtccaggcgttagtctggaactcgacctgacaacagatgaactgtctgcaatcttacatcaaagagcaaatcgcctctttcatgaaatcaaacaggagcaaccatgtcaggacagcacagtcaatttcaagttgacggaacgcaatatttagttgaaagcgattgcagtcaagctgcattccctcgactggttgataaggtaatccgtcaattggaacgtatcggcaaacatgccgctgcggaaatgtatggccacgaagcagttgtttgtagctatacgaaaatcaatcacgagttagtgaagtgtaagctaaccgtaaatccaaaaggattaccatgcagttaaacgaattaagtgtggcagttgaaaaagctgccagcaactctgcatcgcagaaagtttttgtagaccagttgactgaaaagtttaacgctggcgtcaaaaccattcgtgtgtttgttgaagaaatgaacacatggtctgaggtcgaacttgaacctttctggaatctccagaacgacaagtggattaagctgtcgcaatatcagggcagtcttcaaggcattcagaccagtttgcagacagcgttagaccaggcaatcgaaggtttgaccaatccaccagcagccaaaccggctccagtggaggacgtcaaatgagcaacgttaaattaggcgcagcatctcaggctcgtttgaactctgttcgaatggacttgcgtcgtgtttgtctgaaagcctttgaaacgttgccctttgatgtaactgttatcgaaggcgtccgtgaccagaagcgtcaagctcagttgtttgcggaaggcaaaaccaaagtaatgacctcgcgtcatatgtctggcaatgctgttgacatggctccgtacccagttgattggaacgataccgaacgtttcgttattctcgcgcatcacatgtttgcagcggcgaaggaactcggcatcaccattcgttggggcggtaattggtcgcggattgatgaaaatcagaagccaccatcaagctttgttgacatgcctcacttcgagttgccagcataaccaacacgtaatttcaaatggagaatccatgaaatacgaattaattccaagtgaactcagcgaattaaaaggtcgtgtaaatcgtcgtgacgaacgcatgacctacatccgtcgcaataagtcggacgacaataccgttggtattagaatcggcgacgactatgttcgcattgatgttgacttattactggtagcaattgaaggctccaattcgattgatgacaaacgagtcaagctgcttgaagaagcacatgccactctcgaaaaagtagcaaatgggttgctgccgaaaggctaagcaatgaaagaaatttttcagaaccgtccctttatgaaggtactggattcggagcaaattatggatagtttttcaatcactcgaaaaatcgaggcagttaatcacatccgagacatttgtgttcgattttatggacttaaatcggggacggatatctggcttgatgcagtagagttcatttcatacggcagaaacatggccgagttcctcgaactccactgcgaacttgataaagaagttgccaaacaaattgccgatgctgactacgaagttgtagcggcagaaggtatttgcgaactttgtctcactcagccgaaaggctttgattgggagaagtacgcagaaatctctaatcttcgtgatagccttgatgatgaagttatcattgccggtgttgaattggaaatcccattcgacaaaatcgaagacaagtatttgggcaagtatgattcattcatagactttgttacagagttctttgatgaacattccttgcatgaaatcccggagaaatatcgcaactacatagactatgagaaaatcgcagtcgattgggatgcaggaggcgattatgccaactttaatggttacatcttcagaagttgatgcaagcaagttcgttggtggtgaaatcatttatcacacggacagacagcattattaccagataatcaaccgttgcagtggcaaaggtccgaatggttggttggaaggttggacgtatgtccgcgtgaaagatttgtttggcaatcagacagcatttgaagttgactgtgacccggataaattcaaaatgtatttccgaccagacgaatcttttgattctgactggagcttaattcgtgcggtaattttgtaacagtgtggcgcttcgcgctttcggcattagctggaggtgcgaagcacattgtagccacttggaacatttcggttcctacttggaacgttggtgaatcccaaatcaactaagtgcggaacgtgtttcggagtgtcaaaagcattatacagttttgtgtcaagggttaataaacacattgtgacgataggttagccgccatcgaccactttttctgttaaccagtaaaaccgataataccggcgtgaaactatcgtcaaaacaggttagtcacaaagtctgtttcgagatagcgttatgctatcacacactattttaattcacttgcaacagacgtgagccgaattaaaggagttgtgactacataggcaacgaatcttattattaatttaataggctacatgtgggggtgtatcgttgccgctcttaaaatgagtactgaagcttttggggctaattgaatagagtgggcgtaacagtcggactcatctgtacaatcatttggtggaatatgaaagaatgtttagtatgtggctttaaaaagaagccaaccgaatttattaaattacctatatcaaatgacggtctgtcagacagttgtaactgctgtattctcaaacttagccgtaagagaaataaatcagaaagcacagcaaagtccaaagacaagaataggatgcaggtaagagcaaacaaagttgtgtatgccgccgtaaagggtggaagattgcaacgacttccttgtgaagtttgttctgagccagattcagaagggcaccacgacgattacaattttcctcttattgttcgttggttgtgtcgaaaacatcacgcagaatggcacaagaataacgagcctgtgcgcgctgtcccggcctgagccgcgctttagcattagttggatgtgattatatagggtaagacttgggccgcgcgaaggggcacgggtgaggtaaaatgacgtcaggctgaccaagaaatcgccacctcttaatgtcgcctgtgaggattactggcaggctcaagccttaccctatgcaatcatattgccaacctatacaaacgcctgtgtgtgcggagcatccagcatacagcgggtttcggaacggccttcgccagcaccgggagggccatcagtcacattcatcgctcgtaaattggagagaattcctgtgagcaaatctgtaattcgaaaacactcagcaaaagttatctcgttcgaaatgtctgacggtgacctgcgtcattatgctcgcatcggtggccggtttgtttacatgggccgaaagctgcttggagtcattccagaaatggctgagcctgatgggctctggcgcgaatcaatcgcagtatcgcttgcgcgaggttccaattgccgttcactacgtgaattagttgaactcgtaacttgcttcaactgcggcaccaaaccaaaagctcgtgtgatgatgcgtgagtggacttcaattaattaaggtatcgttcatgatttatggtcgagtaatttcacgtcgaactggcgagtctcttaatgaaggctatacacttgagcaagttgcagaacttgctgaagaatgccacgaaagtgaaatcgaaatttacgaagctactggcgacctcgccattggcccaacaattctgcaagatatggtaagacatatcaaagaactggagagcaaacttggctcgcaaaactcttaagcaaaagctgcgtgcgaaagttcgtatgcagcgtgaaatcattggcttccagcataaccgtctggttgaagaccaccagcatgctggtatgacaatcaactttgaaacacaggtcatgcaatcagttgcaatggcccatggtgtcatggcaagtcttattctggcaaagaacactttcgataaagactctgagcagtacaagtcgtttgaaaaagtgtgccaaggtcgtattgcacagtgtatggcgactttagttggaatgggattgtctggtgaagaagccaacaaccgcattatggcaggtcattaatggctcgtaaaaagcaactctcatttagccgtgaagaagttgaatttgcggccaaatctgtggcctttggtgtgctgcaaactgtacttacgtcactggtaaattccggcgcagcgcctgaccctaaaattggtgcgctgattatgcacttcgccaatggcgtcaatttaatgggcaaggacgtagaattggaaaccaagaaattggtggaatccaccagcaactctgtagcgatggagaaattcgaagtcctacaggagattgtaggtgagcaaatcaaatgagcaagaccgcatcatagctcttgaaaccattaagatgtggttgcaggaacatgatgctgtctatcttgcaaaagaaaatgtgataacgtattgggagcacttttcgcctgactcaaagaaaggtgaatgggttaaattaaaaccatacgaatgttgtcgcatcattaaagccacgcgtgctggctttgatgcaatgaagttgataaagcctgaattaataatgatggctgctcaggaaactgagcgtgcatttaaacagggaatcttctctcgttcaaatgccccaagcgaatattttaacttctgtcgctctcaacatttcaaccggctcgaacttctaactctctgcatgttgcaggaattagttggacgtgggtggaacgttgaagcagtgtgtctcggcaaactaatggttgaagttttctacaaacatggttttgtcgttcccaaccgaacactccgttggaagttgttgcgtgcagtagctgaagaagctggtgttctcattcgcgacaggctcgaccgcctaaccgtttatggtgtaggtcgatttgtctgtgtgcaaattgaaggcatcactgattcaatcaaaacagaattaaccgaagatgagattaattctttaattcgggaaattactctgcgcttcgcgcaaatttgattctgtttttgtttttaattctggagcatttcttcggcattagctgaatgtgaaaggttccatgtaaacttactttttaaatctgatgtaaacacacaatcgttgtgttcatctactccaatataaggattttcccgtggctaaagttgtaaccgtaactcagtacgaagcaaatgatggttctctgttcctgaccgaagcagagtgtaacgcgcatgatttcatgctggaaaacaaagctgaaatcgacgccgctaccgaagcgttcgtaaacaccctgggtgcaatcgaccgttcacgtaacatgaaaatcaatgttgcgtctgaattcctggccttctacatcccttgggtgcaggctggcaaaccagttgttgaacgtaccgttttcgatactccgaaagaaactccggttgttgaaggcgaagctgccgctgaagctgctgatgcagttgcagagccagttgccgaaggcaccgaaggcgaagctccactgttctaagtcgatctggtcggcgtctggtaagcgcgacaacaaagtcatcccacagtggcactgactttgtttaaatacccggaatcccattctgtcaaccacaggccaaatcgcccgagagttgagagtgggcttctggatgattcgaatagcccaatttgtaggacgaccatgcacacaggatttgatgttttattatggcctgagaaaccatcgtatactcaaactccgtgagggagtgcatctacagttggatgaaagacggattggtcactcaacccaaccgctctcttagagaggtcatccagaagtgagtttctgtgagtatattgagtaagtcaaaacgctgtgcagacgtgcaggctaaacgtgtatcaatgtattcacagaagttttcgttcgttagagtcgattatttttacttataaaaataagtgcaaacgataatgaaatgcgagcagccgcttaattaaatttaagtgctctccgtggtctttcgattccatgtaaccaaattcgacgcagtggcccgctgtgattaataatgggcacaattttttcaatggtgttgtattcggttcaagtccgaactcaggcgaaactaaagccacgagatgcagtggaacttacaacatcaacgaaagcattttgagttgcatactggattagacgcgggaggatggccgatgcccgttatgtcatggcccagcagtgtgcaacatcaaaatgaattgaagcaatacattacttaggtaaggctcttgtgcacaaagagtatatacaggttcgagtcctgaatgtgttgtgaacatattgaagatagacgtagatacgggacgtaaacactgttactacgagacaacacatcctccgcgtgtgtcttcaattattagttgcagctaagacctgcggcaagcggcgttaatttaactctggagattacagtggacgagaaagagcaactggtgcttgagtattacgattgcatcatgacttgcgaattgtctgttgcaatggctagaaagtttggtgagtatgaaaacaaggctcttcggtcttgttgcaaaatgctcgcaaagcgcatcaagaatgattctattaaacgcataattaaaggtgtgcagaaagcgaattatcctgttggtgcattggcaaaaatccgtcgcgaatttgatgaggcttgcggttaatggatggtttagacaatattgacttcgatgaaatcgaacgtcgtaatgatgaaaagcttgacgcacaggaagtaatcgaagatgaatctgattgcgatggctgcaaaatttaaaggctggattgctactgcattcctgtttttagttggagttggattggcatatctgtctggtaaaaaggacgagaagcattccaacgaaattgaaaagaaggatgctgaaattgagcaaaccaaagccgtttccagtgctgaagtatcagccgccacggatgcgaaaaaagttactcagtctgttagtaataagtctgatagctctgtcgacgacgagttgcagcgtttcacccgcgactaaaattgttgacacaagttgtacaagttttagtttgattctgttgtccaagaaggaaattcctatcttgactccagaaaccaaacgacaaattctcacgcacaatcttgtgtatgagaaaaaatgtttgccaccaaacagtggtaaacagcctgagtgatattgtgtggcctatcaagccgaggaaacgaaccggagtctgcactgttgttctctctggacacaattgaacgaaagcaagcctcgcagtttacgtggtttaaacctgcgttatcaaaacccgtcacgaattatgcctggttccaatcggtaggtgccctcttttgggctgagacaccgtgaggatttgttggtaatgaacctccgaacaggcaccaaacaatgggactatagtttaatagccatgcagagttgcaaatctgtggacgcgtaaaaacggtgtggagtccaatccacattacgcctgtctggaaacaggagagtcccgccaaatcctaaaccgcaagacgaataccttgcggaagatgtaggtacggccagtaccgaaatacggaagccttagaggtcttggctttcggttaaactatggtccatgtgcaaatgtcagtcactaggttgcgacttcgaataaccacctatgatgtgcaaagtgtcagtcacggggccgccaaacaatggagtcgtagagttaagtaaaccggtagtcgcacagccttggtcggtgtggtgcttctatcattgctggtagcgtaaaccagtcgactccaccaaattcgaaacttacccgacaaagttgtttcgatatcagccctgaacatggatagaactgttcaacatagtcgagtgggatgcgcgactttaaataacgtgaaccctgctcagagcatcctgagaaaataaaactgccgaccgggacgtcgttaaactaccaatgcttggttccgtatgtgatagtactaggtttcgacggagacacgaaactatggtgaaacggtgtgcgcacaacaggttcgattcctgtgaccaagcgccatattccggatgatgcaggctggccaagatatgcgtgcgtacgcaaaacgtatctggcgaggtttgattcctcggtcgtccactctttcaaaatagtcgtgccactattcaaatggcaaaatgtgctctggcatactggagtcaaatccagacggacagcttaataagcgcggtggtaagatttaatacggttgcatcgtattcaggatttatcctgcgacgagccaggctcctcactggcgattggattgtgttgccacacatttctccgagacgtattaatgaaatatgcaaggcagggttttccatgatgatttgttacttgaaatcaactggcaggtgttacgagcctgtgatgttctcccatatacaagaagtgattccgcttggccggtcaggaatcaaaagtcttttcttctgctctttatttaaatttaagcgcagtaactctatatttgtatcggtaacgtagagagcagaataaaagccataagctgagaatccctcgtttttcttacccattgagaagccaaatatgcaacttattgagaaggtcagtggcaagtctcgtttgtcgaactacattgacgtaaacaaaatccaagaagtattgtacgtaacagcaagcccgttccaagtctgtattgtgactgttctttgtactggccgtgctcaactgtacgatattcttagaaacactgtaacccattccggcaaggaagatttcaaatctttgcagcattgggttgagtgtattctgaattcaaaggtggcaggacgtcacgtctttgtctccaccaatatttctgcgaaatacaaaacgttgatgcgtatttcttctgccatgagtctcgacaaggcatacaccgaagcacttgcttcgagtgagcatgccgatgtatatgagattgtgggcaaacttccagtgaagccaaccttcaaccatatgacgcataaattcacaacctctgatggatgtgaactcgtatatgtcgccagccttggttatgtttggatgctgtcaaaatcacagtgttgtggaacaagattcttcaaaactgttggtgaagctgttgaagaaatgcatcaaggtagtctcaatgtttacatggagcctcgaaatgaaacaaaatagtttccctccattccttcctgttgtggaagacattgccactattcgtgatgagtttgcacgaatcattgttggcaaagttattgatgcagatggcttgtctgcaatcatacataaccaagtgtcggcagaagatattgcaaaagcagtttacttcatggctgacgaattaatgaaggctcgtattcccgaacctttaaaagttaatattgattctggtacccattaatgtctaaacaaatctctgccgaagtcgttgactacatgggcaccgaccttgcaacagtcaacgcagcacgcgtcagttatggcgttgttgcaactgaaatgtctgaacgtgatgagcgtctgattgatttcctcgcggaacacagtcacgtaactccattccgtcatgcaactgttacactgcgttgcaaagctccaatctttctggctcgccagcttggtaaacatcaagttggctttagttggaatgaaatctcccgtcgctacaaagatggcgaatcaattgagattgagtgctatgacccggaagtcatatttgctcgacctcagaagctgatgactcaatcagccgtgccaatgtctcaggattttgctgacgacatgcgccactttattgccacaactcaacgtgctgctgtacgtgagtacatggctttaattgatttgggagttgcaccagaacaagctcgcatggttcttccacaaggtatgattaccgaatggatttggaccggttcgctgtatggctgggcaagcctctataaacaacgttccagtgaacacgcgcagtatgaagcccgtttgtttgcggaagaagtaagcaaaatcatgtcacagcttttcccaaaatgttgggctgctctgacaaaataaggactccaacgagatgcaaattaagcagtgtgtacaaaagattaagcacgattccccaacttgtaagtcaaccagcgggaagtcgctgcaagtttggctgaacgagaatgaggatggaacaagaacttattctggctactgctttgcttgtggtgtcttagttccaaatccgtacggtaacaatccaccagacccgaaagaaattcacatcaaaactccagaagaaattcaggaagaacttgatgacatttctacgtgtaagatatttgatttggaccaccgtggtatcgaacctgaatattggggtgctgctcgtgtgcggctgctggtttcagagttcgatggcacgactccaaatgctttggcgcatgggtatactcgtggcggcaaacttgttcgttggaagattaaactcctcaacaagaaagtgatgtggagtgttggcgatacgcaggagaatgacccatacaattgggaagctgccaaagcaattggcggcaagactctgtatatcacagaaggtgaagaagatgccattgcgcttcgtcagattcttcgtactcttaaccgtggcactgattatgaagcacttgattttgcggtaatctcgctgtcagatggttctgattcagtacacaaatgtttggcacgcgttgccgaagaaattaaacaacgttgggaacatgttgttattgttttcgaccaagatgagccaggccgtaaagcagcaaaagaagcatgtcggttaattccgggtgcaatgattgctcagcttccggccaatgatgcaaacgattgtctcaaacgtggtatgttaaagaacacgcgtgatgcagttatcttccgtgcgtctcgtccgcttccaacagcgctggttaataaagacctgctgatgttagaaatggatgaagaacttgctccgggtgcatcaactccttggccgaaaatgactgacagttcgttcggtcaacgtcgtggtgaagtttggacattgggcggtacagaaggtggtggtaaaaccacactggctcgtcaaatgggagagcacaacattcttgagcataagtggaatatcttcacttgctttatggaagaaagccctcagcaaactttacgccgctttgcagcattgcacgacaacttgccatacttcgacccagcgtttgttaagagtgaccctcgttataatcacgagagattcattctaacttgccagaagtttcttccgtatctcgaaatgtgggacaggaagcaacaaggtgaagacccatacgagacatgggaaggaatcaaaactattctgcgtcagattggtccagacattgaccagttcgttctggataacctgaccattttgggcgaaggcatttctgcctctgaacgaaatgatttcttgggtaaggtttatgccgaccaagtcaaacttgcagagcaatatcagttccatattcttgacctgtctcatcttaacccggtggcgaaaggccagcgtcctcatgaagatggtggacgtgttaagaaaggcgactttactggttctcgtgcagccgcgaaatattcacattatatgttcggtttcgaacgtaacatgcaggcagttgaccctaactgttctattattcgtggtatcaaagctcgtgaagcaggtaagttggaagcattcaaaacttattatgacgccgactctggtcgaatcttgcaacgttcttgggacgattcaatgttcgaaaccaaagaagttgtgcaactcactcagaagaaaggtgctcatcaatgagtaaagaaattatcaccgttgtaataaacgagacgttgactgccaatgtgtcttcattgaatggtgtcgcaaccatgtttgtccttaatggagcatgggaaggcagtattgactggatggcaaaagagtatttcgcctctcgctacccaacggatgttcatcgtatcaaagagtggcgaatggctactcgtgaagatattgataactgtcgtagataaccaaggtcttgtcctcctactgttgtgaaacagaagcttggacaaacctcctctcaacttcccagatggagacataatgtgatttatccgtgggaaaatgtattcgccagtgacatagaaactactggtttgctgcaccaaatggctaaacaagaacatccacgtttacacaacatgggtgctattgatgtagtcagtaagaaagaaaattgcatggagtggactggacgtaaaactattcaggattttctggacagtgggccaactctcgtaatgcataatggcgcaacatttgacatggaagcattaatcttccttggatatgatgtgtccaaagtaaccctgattgatacgctttatatcagttggtaccttcaaccacgtcgccacaaccacggtttggcagaatatggtgaagagtttggtgttccaaagccggttattgaggattgggagaatcagactcaggaagaatacaaccatcgcgtgatgcaggactgccgtattcaaactagtttgtgggaacagcaatatacgcagttgctcgcaatctataaaactccatccgaagttcgtcgcttcgttgaatacctgatgagtaaagctcgtcagcaagttattcagcaacgtactcgctggaagttgaacaaagaaaaggctcagaaattccaagaaatgcttgagccaatgattaaggaaaagaccgatgcactcgaagcgtcgatgccaaagattcctgactacactcttaaacaccgtccagccaaatgccacaaacaaaatggcactctgtcagcaactggcgctaagtggaaagcagtctgcgacgcaaataatcttgattggaaagacccgaacttagtaattaaagttctcaagggttacaatgcaccaaacgctggttcgcataaacaaatcaaagattggctgttcagtcttggttgggttccccaaactttcaaattcgacaggaataaagaaacaggtgaaactcgacaaattccgcaaatcactgttaaagacgatgatggcaatcccgacatctgtccgagcctccatgaactcgccgaggccaatccgggccagggtgttgaacaccttatcgggctgggcgtttaccgtaaccgtctcagtattgttaacggctggcttcgtgatgtttctgacgatggctttcttatcgctggttgtggcggtcttacaaatactcttcgacttaagcaccgtggtcttgtcaatattccttctatccgtgtgttcggtggtaaagaactccgtgaaatgttggaagcgtttggcgaagattacgaacaattgggttcggacttatcttcgttagaagaccgttgtaagcaccacttccaatggaagtatgaccctgaatatgttaagaagcagttggcagatgattatgatgcccacttagcaattggcgtaatcggtggattcattaccgaagaacaatcacaagctcataaagacggcattaagaaagtcaaagaacgtccaatgttcaagacaacaaactatgcttgtcagtatggcgctggtgttgcaactgttcaacgtgctgcgaaatgtgatttcaaaacagctgagaagctgcatcaagcatattggaaactcaactggtcaatcaaagaagtagcagccaacacgactgtgaaaactattgatggtcagatgtggcagttgaatccaatcaatggattctggtattcactgcgtaatgagaaagaccgtttctcaactctgtgtcagggtacaggcgcatatgtgtttgacctttggtgtaacaatgtaattgcaatttgcaatgaacgttatggccgtgacccactgttgtctggacaattccacgatgaattgattctgcaagttcgcaaaggtactcgcgaagtttgggaagaaatagttggagttgaggcaatgaagcgtaccaacgaacagctgaaaatgaaccgcgatgttgcgtgtgaagttcagtttggcgacaactactcagagattcactaacatggctcaactggtatatgcgctctatgatgcgcaagaaatgaaattaagccagtttacagccgatgccagcattcttgttaaggatgctgtttccgcttatctggctgagaaagttttaagtgattgcttcgctgatgaagctgcaaaagaccttctcaccgcactgtcaaagtcaaatgatgttcccgaacttttagttgttttggaagcatatgacttcaaactggctatcacgcctattatttcgtaaccaaattattctctcggagaaacaaaatggccttattccaagcaccaaccaaagattccggtaaagctccatccaaagcaccactgctcgaagctggtggttatcctgcacgtctggtacgtctgattgacctcggcaaacagccgggttctggccagtatccagagccgtcatacaaactgttgggtactttcgaattgctcgacgagtatatgaaagaaaccaacgaagctggcgaaatcatcatggttcaagaccctgatggcgaaccaggcgaaatgattggcaaagacctgctggacaagccacgttggtttgatttcgaattcacttacaatcccgatggatttatgggtgaccgttctcacatctacaaattcatgcaggcggttgatgcgtttgaagtcaaaccaaatccagaagctggcgttgccggtcatcctgccaaacagttaaatgaactgttgggcgaaccactggttgttaacctgactcagtacaccaagaaaggtggcaaaaatgctggtcagttggcaaacaaaatctccacctttgcgccaatgaagtcgaaagacaaacgtgatgcaaaagctctggtcaatccaaccatcttctttgatttgggtgcaccagatgtggaagtgtttggcaaactgccgggtggcgatgcagaatgggctgttaagaatcgtattctgaacaaccttgatttcaatggttctgctcttcaagctgcgttaggccagactcctaccaatgtaccggtagagaacaaagcctcagaagcagaagttgacgaagcactgaaagcagaaatggaagctcaggctgctgcgaaagctgctcaggcagaaagtaatggcactgctgatggcggcgtgattcctttctaagtaacacactgcatctacttggagtagatgtaattaccaattggtaaaagggcattccgaatattggagtgccctattttctttggagttttgcaaaagtgattaagaagaaaaaggttctgctgctggtcgatggcgatatggttgccttctcccatgcggctgcggaagagtatggcaaagagcctgaagatatctcttttgcaaagattcaaatgtctatggaatccaagatggatttcatgatgaaacgtattggcgcaactgaaacagttacgttaatctctggtgattcaaacatgcgtcatattatttgtcctgcatacaaggcaaatcgtgatggtgtgtggcgtcctgagaatcttcgcaatgccaaagcaacactgatgacctcatacgatggtttgaagtgtgactatcttgaagctgatgacctcatcggtatcatgtgtcgtaataaagtcgaactcgaaatgggtaaacgtggaaacattaagtctattaagactgtacgtccactgaccaaagacgactacgacgaagtttgggttgcgtctctggacaaagacttaaaacaaattggtggtcgtgaaggtggtccggtaattaaacattatcgttgggaaaccggaagcactggtgaaaagattgagattgtttctggctttggtgaacttcgttgtatcatcaaagacaatggcaaaaccaagaaaaaggaaatcaaaggcaatggtccgaaattctttctctggcagtgtcttactggtgactccacagatggtgtcatgggctgtggaatcagtgaaaccaaaatcttcaagtcgggcgcgaaatgcggccaagaatatcaaaaacgtgttggagttggagcggttgaagcgttcgaacttttagacaagattgataattacgcagacggtttgaaagccgttgccactcagtatgtcatgcgctttgcagacggttggcaagaacaacttctcatcaacggccgattgctctatatgtcaaatacggtggcggaaggaaacaaggttcgactttggcatcataaaggtgtcactgaatatttcgaccttaattctaaacaaatcgtttcggcgtaagtttatacgggcggcattctgcttacacattagtggaatgggaattttgccatgtatggttattgcgggacagaagccaagtttacagcttggctgcaatcggcgctgcgaggcgtttgggcaaagcatccatcaaagctaactctattgcagaagaagcgtgtggcgttgaaggttggtacaagtaagaagccaatcttccacgtccaatgtgagcattgccataagctgttcaagcttaaagaaattgaagtcaaccataaaaataaatgtggtggactgtctgacctatccaaacttaatgagtttgttcacaatcttttactggttcagccagaagatttggaattactttgtcattattgtcatggcatcgtcacgtacatggaacgctacggcgcaaccaaacgtgatgcaatcattgagaagaaggtcatcgcattttcaaaactatctgacaaagaacagatggttaaatgcaaacaagcgggtttcaacccaattccaaaaaccaaaatcggccgtaagaatatggttcgagaatatcttaagaaggttatcccgcaatgactatcaagttattggacgacggaacatcttatacgaaggcgcatgctcatgattgggaagacccaacttgtcaactcaaaggacgttgcgaaatctacatcaagattgatggcatccgagcaattagaaatcgcgctgggcgagtatggtcacggaattccaagccgttaccacatcttgaccacctgcatttcagtgatgctgaaatctttcgcaactcctggaatgaaacatcgtctattcttggaagcgatgcagcgccggtggtggctttaacccaagagaatgtgtacgaattgtctgatggtaacatcgacaaacgtttgtacctcggttgggcagaaagtccaagcaatgaaaagcttcatgaactgatgcagaaaatgttgaagttgaaacatgaaggcctcattgttcgttgcaaagacaagaaaggtaaaatcctctggtggaagattgtaccatacaaatacgctgatgttaagattactggcttcaaagaaggcactaataagaacaaaggtgtttgtggttctattgcttctaactacggctccgctggttcaatggttttcgattgcctgcaagaccatggcatcgaaggtgactacaacattcgcaagtggatttgggctaatcgctcaaaactgctcggcacaatcatgcaagttcgttatcgtgagaggacagagggcggtaaattccggttcccttcacttgtacggttgcgcactgataagtcagaagagagttttgactgatgcgaaatatcaaactcggcgtggtcttaaatggcccgccgggctgtggtaaagacaccatagccaacaaaattgttgaacttggcgcattccgtaaacatcaatttaaggatgcactttatgcgcacactgctaaacattttgaaattgatttggataagttcatccatttcgcctctgaccgtgtacttaaggattcgaagtccttggcgggattgggcggtcgaactcctcgacaagcactcatctatgtcagtgaagaaatcttcaagcctcgttacggcagcgattactttggcaaagttgaggttaaccgtgttgaaacactctgtgggcacatggatagcgatgttaatgtcatctatcccgatggtggttttgcagacgaacttcagtgcattgactcctgctatgatggggttcttgttattcgcttgcatcgagacggctttgatttcaaaggcgattctcgtagctacatcgaactgccagacacagaaaagcgtaaaagcattgatgtggatttgacagacggtgaaataaatatcggggtgcatatcgtgcgctctgcaatcaaacaatacagagagactctgcgataatgtgtcccaataaagttccacacgttaacttcctgctgtgtcatccggcggctcttcttccgtcttatgaaagccgtggcgctgctgctgctgatattcgttctacggacacagcaaacattgctcccggttctactgccattgttggcactggtcttaagccggaaattcccgaaggttacgttgcgctgatttattctcgcagcggtcacggcttcaaaaatgatgttcgtctgtcaaactgtgttggtgttatcgactcagattatcgtggcgaaatcaaagtcaagctggtgaacgaaggcaatcttccattctctgttaatgtgggcgaccgcgttgcacagatgatgattgttcctgccgttcaggcaaccttcgaagttcaggaaaatctgacttcaactgtgcgcggtgaaaacggcttcggctcaaccggcgcgtaattgctcaatggagaatccgagcatgcaattcgaaccaagtaagtacgaccttaatcacgtccagtacacaaacatcattccagagtttaataagttactgtctcacttaaacagtgaagaaaatgacatggctttcgagttcgaagctaaactccaagctctggaaaagaaacttcgcgatgcagacaaacgccttgaaaagctggacgcattagaagcaggtggtgttgataactggtctggttatggtgattgctttgaggatgatgaagatgaataagttaacttgtttttctctgaacctcgatggcaaagttttcaaacgtctccttaaatatctgttcgatgactcattcgaaattgacagtgaatatgccaaacatagtgaatgtcatatcactatgggtgcaactgttgacttggatgtggcagccgatattgttaatacattcaatctcgaaatcaaaccagaagaattagttggtacttgggctgttgaaggttcatccgactacagcaacggtttctattgggattgtgtgaatgaagcacttaaggttgagcaggtaactgaaacaataactgtcaccaaatggaaaccaatccaagatgctcaaccagccacagaagaaagtgtacagccgttccccggttgtaaaaaataatgtcggcgtaaactttgtttacctccggtctactgtcaccacaaatggtggtggaacatatatcactcgtgcattagacgcccgtaataaaactggcgctgatgtaattgtgtttatgattccacgttctgagaacgcagccaggacactggaacgtatcaagcgtggccgtgaagatttaatgtctgctgtaaaaccgcttatcctgcctttcaaaattgtggctgtaatcagcgagaatcagaaagcactcgaagaacatttcgaaggtatgctgtggagtgacgttaaatactaagcgatacgccgatgaattggggaggtctatattggcctccttctctcttggagttcgcttatgcgcactatcacatgtaaggaatgcggctatgcgattggtgaagatgacttctccttaatgctatgtccagtgtgtgattcattcatggaattgaatcgcctgcaaaagaaagctgaaccgtctttagagaaggttattagaatagacgctacaaagcgattaccagaaaggtcgaataatggctgatgacttaggcgacgattataacaacacggttgtattccacctgttgaagttttatggcgacttacttaaagtgagccgtgcccgcttctgtatgcagacccttcctattctgcgtaaatatatcgctgctaaccctgatatcattcgtgattactcagaggcattggatgcagagattgaaggacagggcttaaaagataacgctgtcctgcgctctcttgttgtagcacaacgagaaagattggaagctgctgattcgaaagactcgacagcatatgccagtgaaatcgaaaagattattaaagaaggtaagacagaccgtgttcccggtgcacaactcgaagctgatacagccgagcacaatgcatcagaagaactcattcagcaaatcttagacaatccattggatgttgacccaacagtcattccaaagaaagttgcagacgctgtacggaaaatcttaacttccagttttgagaagtttggtaaatggtcattccatattcaaatgggattcccattccaatctcaggacttccatgatgttatcttcgatgttggtcaacaaatagttgatggtaaaatcgaccgtgtaattattacaattccgcctcgacactcgaagacacaattattatcaatcgcactcccactttattctttctgccataatgtgaccagccataatattattacatcttatgctgaggacgttgtgctggaatcaagcggctatgtgcgtacagtcatgctcgacccattgttccaacgtatattccctaatgttcgtatagacccaaacaaacgttctcttgagcgttggggtactacgaaacaaggtgtaatgcacgctgttccaacaggcggcaagatgactggtaaaggtgctggactgcttgcagagaattactctggctgctttgtggtcgatgacgttatcaaaccaaaggatgcgtattccgatacggttcgtatggaaatcaacgaccgttatgataacacatttatgtcacgtcttgcgaatgacggcgttataactttaccagatggcactctcaagaagtgttcacgaactccgatggttatcatcatgcagcgagtacacgatagcgatttggttggctatctgttacgtggtggttcatctgataaatatcattacctcaacattccggcaatcgttgagaaagatactggctcaaaagagtattatgacaagctgattaagcaacagaactactctcatgccattccaattctgtataacctgaataggaaggaagagaagtctgctctgtggccgtcacgtaaaagtttggaatcgctggaagcaatgcagaaagcaaatccatacacatacaactctcagtatgctggtaatccaactgccaatggtgttggcctcgttaaagaggaatggtggaaagagtatgacccaaacactttcgacagaagcagaattgttcgctcgtttattacagcggatactgcatcaactgcgaaagaatactctgactattccgttctgaaacattggggcgtaacgaaagagcgtgatgtttattgcctcgacattatgttgggcaagttcgaaacgccggaacttaaaacggcgataattggtttttgggaaaagactaacatctttgactcacgatggccttgttgtattccgcgtgccttgtacatggaagacaaatcatctggtcaattcttgaaccaacagtttgttcgtgatgggaatatcaggcttatgcctgtacctcgtgacaaatctggtggtgataaggttgctcgattcttaaataccattccatatttctcaactggcaagatttattatcctgctggacacgaacacattgaccatgtgaagcgtgagatacttggaatgacttcactgggttcaggcactggacacgacgactgttgcgacaacgtttccgacatggttgcaattgaattttccggcaacaacgccaactattctgcgtgggtttaataatgagtgtgattactcgcattgatgcccgaagcaaaaacaatgctggtttcgaaattcgagacgcagcaactggcaaaacgctggtatttgtcgaaactttgggtgctgaaactgaactccgtattagctcaagcgatgctgttgaaatcgtaaaaagcaacggagtcaagctcaaaaggaagaaataaatggcttccaacaaaccacacagcaatcacgttaatactcaaaagacaaagattgctgatggtcttgagaatgttattagtggcatgggtggcgagaaagataagtcggtattcaaccgctggtctttcgccaataagaacgctgactatcgacaactcatggttcgattccgtgaagattgggtaagtcagaaagtttgtaccattgtccctcaagacatgacacgtaactggcgcaaaattaatacgcccgaaggccaacaagctgataaggatttacgaatccgtaagctgtgccgcgaagcgtatcaatgggcacgactctatggaacatcatttattctgcttgacctcaaaggtacaggcaaacttgatactccgttgcgtctggataatttgaagaagggatgtgtcaagtccctgaaaattattgaccggtcacgacttcacgctgctggtagtatcgtccttgatgcactatctccccattatggtctgccagagtactatactctgagtggctatccggggatgatacatcacagtcgtttcttacgtttcgaaggaaccgaacttccgctgttcgagtttcaacgcaacatgtggtattccgattcagtgttgataccgctgatgaataccatagaccaattctatgtcactgctgctgctgctgcacaacttgcacaagaagcaacaattgatgtggttacagtcgccgggttacagtctttactgacgaatcccgaaggcgaacgttcggtcatgaaacgattcagactcatgaagcaagccaagagcttatacaatgtattaattcttgacgagtctgaagagtactcaaccaaaagcattgccttgtcaggcgtaaaagacttaatttgggaatacctgaaaatcgtagcggctgcggttggtattccagcgacacgtttcttatctgcttctccagacggcatgaatgctactggtgaatccgaccttgtaaactatattgacttgcttactggtttacagactgcaatcttcgaacctcgtttagatgttctggatacaatcgttcaagcgcatttcggaattgccccttacacttacgagtggtgcgacatattccctgagtcgaatgctgaaaaggcgaaacgtgctgtagatttatcaacagctttttgctcttattggtgctggtgctattactgctaagaatgcgaatgatattatcgcgcactctcacatgtttggtcattgcccaattgaagctgctccgaagaagccaccaatgccacctaaaggtagtggaaatgcataacaaactggttccagttagctttaacgatgaagaatctgttgctcagccgattgtattatttgctgaccgtcagaccatctcatctgccagagtgctccgtgattctggcgaaatgattgcaccagttacgattgcacgtactggtgacatgctgtacaaagccaaagaacttggccctcaatttgctgaccttcctccagaacaggttgttcgagtttcgactccaccagaagttctgtttgatgaagcaaccattgagttgtgtcgttcaatggcagtaacaatcggccatccgaagtccgatgtaagtttggaaaacaacaaagaattgcagaaaggtttccttgaaggtgctccggtccctgatggtactcatctttgtggtcatgttgtgttaaccgataaagctgctattaatttagttgattcgggagttgaccaaacttcgtggggccatgacgccattgttgagcgtgtggaaaaagatggtgttgtgtctgctgttaagaccaaaatcacttctgtcaaccatctggcaattgttcgccgtggtcgtgctcaaacaactcgcatcggtgattccggtgaagagattgaaattgttgacaaagctcaactggatttggtcgaagctcagcgtgatgagttgaaaaccaaagttgaaactctgacttcaaaattggctgatgctgaatctgcccgtctgtctgatgaagatgtaattaagatggttgaagaacgtgctgcggctcgtcttgaactgcttacccaaattgcaaaactcggtgacgagtatgtgaagatggacttctcaggtaagaccgaaatggaaatcaaacgtatggttgttgcgaaacttcgcgatgccgatatgtctgacaagtctgatgattatgtcacaggccgtttcgaaatcgcgctggaagactctggtgaaatcaccttgtctgatgcgctgtctgcttctcttatgtctcctccagagcagaaagagaagaaacttagtcctcgcgaagaagcacttgctcgtcgccaggctcgttttaataaataggattcagtccatgccaaagcaagattttaacatcaatactggcttcgcagccgctggtgatgtttacggtttagcgttcaccaactcacagcgcttcacttacaaagcagaagccgaaatgagcgcatatgctctggctgttgtgaaaggtgcaacttctgatacctgtaaagttggtaactccgaaggtgaaatcctcggtattaccatgcgtcagaacgtacttgagtctcgtactcgtccgggcgatggtactattaccattccaaaaggtcatcctctggcagtaatgctggaaggtccaattaacgttgttgccaaaactgctgttgctggcgaagatgtttacatcaacgacactactggcgaaattggtggtactgctggtgctggttataccaaagcaaccaacgttaaagctatcaaatatcctgttgctgctggcgatgtattccctgtcatggtaatcatggccgccccaaagtaacaacgccacctccggcaccaagtgtgacagcggtagcagcggcagttactgctgatgcttcaactgccaatgcaactgttacagtagataagttgttcacctttgcaaactcttctgcaagtgattacaactttactgtgactccagcggtgaccggtgtttccgtagatgctacaggcaaagtaacagtcctgaatgcaactactgtggcgacctcagcaacaatcaaagcgactcacaaaactcagacgtctgtaactgcttctaagcagattacaatcacgcctaagacaccgtagtcgtaacggcgcagcaaaagttgcgccttgaagcagccttttaatggaattggaatacaatgccaaagatgattaagctgaacgatggttcagaattcgaactggatgatgcactggttgctatccagaacaacaatgccgtaactctgagcgatgacgatgctgtgttcttccagcgccagcttgagttcatcgaagcgcagacttacgataccctgtatcctgaccttgaagcgcgtgacgctttcggtgttgatacatctggtggtgccggtgttcagactctgacctaccgttcgtacaaccatgttggtggcgcacaggttattaacgcccgtgcaactgacctgccaaaaccaaacatttccggtaaagaatattctatcaccgtgaaatctgttggtactgcgtatgactacgatatcgacgaaatcgcgtctgctgctgtgactggccttcctctggaagctcgtaaagcaatggctgcaactcgtggttacgaacagtacatcaacagtgctgcatggtatggcgattctgcaaatggtttcgttggcctgttccaacagactgatgttactaagaacacagttgctgctggtgcgaacggcaaaactggctggctggatggcaaaactccgaccgaagttctgaaagacctgaccactgctgtttcagcaatgtacagctctactctgaaaatcatgcgtcctgacgaaatctggatgccggttctgcatcaccagtacatcatgaacactgctcgttctgaccagtctgacatgaccatcctgcaattcttcattgcgaacaacgaattcatcaactcgaaagagaaagtgaaagcgatgaacgcaatcaaaggtcagggtacttctggttccgatgtgttcgttgttatctgccgtactgttaacggtctgaaaactttccgtctgcgtgagcctctggctctgacttggcagccggtgcagcttcatggtctggtttatgaaattccaggtcgtggccgctttgcaggcttgcaggtaatgtatcctgctgcaatctctatcaactcaggtatctaagttgatatgtcggcgggtgaaagcccgcctcagtttctgaattaagagaacaacaatgcaattaaaaaataaccgcaaaggcagtgtacaacttatgtatccagttaccaaaaatggtaaaccggatgtagactttgtgcacattccagcgggcgcaactgttgaactggatgacgcaatcttcgaagcactgtgcaaaccactgactactgtttccgtaatggaaatgaaagaagtggaaatcgaaggtgaagttcctgtccagatggataagaagaatgtccgcattaaagagttctatgaaactggcaaaaccaaagtggttaacctgtttaaagagcaaattaaagctggcgacttcactgtcgttacacgtgctgctgtaaccaaagaagcaatgctgaaagtaatcagtcaggccggtgttgataccagcaaaatgactgacgaacagattgttactctttacgacaaactggcgtaaccgatgctcacactcattgatttggtaaaacgctatcctgcgatggctggcattgacccggatagattcgatatcttccagagtgatgccgtccttatcatgggtaacgatgatggacgttggctcaacttttatgaccctgcacaagctgcattgattgcacatcgaattacacaattcggtggcattgatggagaagatggtgcggacatgactgctgggcctgtcactcgaacggacgttgatgatgttcaggttgaatttgctgacaggatttgggataagattccatatcaggaagcggatttgttctctacggcctacggccaagattatgtgcgctggcgtcggatggcttttgctggtccgaggattgcatgattaatcaaaagaaagcattcaaccgattcacaacggcaaagcatttgctggaagtttatcaggaagggcactacgacgaaaagaataactggactggagatacatatcttcccggtaaaatgattcgttgtacgcccattccatacggtgacagggattccggcattggtggtcagaagttaatggctactgatgttggtgaacgtcaaccggcattcatgcgtattcactccagagttattattccaatcaagtcactcatcactatctatggtttgaaatataaaatcattgagaaagatgatgtaactgatgctggctttaacgttgttattgccgcgaaagttctggagaagtaaatggatattaatgataaagaaatccaagcgatgaaagaaattgttgacgtcgctgttgggattccgttgtttacgtatgaaatgcaacagaatgcacctcgcccacaaggtgagtatgcggctgtcaaatgttattcaagttctaatcccggttacgacgaaacacgcattgttgatattaacggtgcggatatgttccgaactcgtgggattagaatcctgacattttatatcctctttagtcgggacggtcaggaatatattgatttcgataattcattttatcgacctgatgtacaagccaaaatgcgtgaacatggtttcgctgcattaggcaaagaggcgctgaacctcgcaacagttcagcttgaaacaaattgggaaccaaggaacggcgttaagatgcagttcaatgttcttcgtgaacaaatctctccaattggttcaatggcgaatgctgttgttggtggtaagtttattgatggcgaccaagtcattgagattaaaggataacaaatgtctattcctatttccgatatcatcaacgttcagattgcggtagctccaaacgcagctgcgactgatggttacggtccaatcgtctttatgacgaaagagttccagccagttatgggtgaaaacaacatccgtatcttcactgggttcaaacaagttcaggatgcatatccttctggcggcgatgaaatcgttaaagctgctgaggcatggtattctcagaagccaactccgaaaactttctgtgttggttcaatctcaaccacttctggtcagcccgcaacttctggcaaattgactggtggtgcggctgctgttcttgcagacctgaaagcaatcactgctggcgcaatggatatcgtcgttgacggtctgcctgctcagaagattactggtctggatttgtcttctgctgccgacctcgctgctgttgcaactttagttgagggtgaacttactggcgttactgtttctcagtctgctggcatcttctccatcacttctgcaactcttggtgcaaaatcagctgtagcagttcctgcggcaactccactggcaactgctctgaaaatcaccacggctgctggcgcaacttcaacgccgggcactgacgcgattggtatcaaaaccgaccttgcgaaaatggctcaggctgctgcgaaagctaaacagttcttcttctatgttgctggcgaacgctctctgcgtgatacctctcgctacattgaaatggctgaatgggcagaagcaagtaacaaagtgtttggtctggcgtcaaacaaaactgatgtgctggttgctggcaatactgccaactacttcgcccaggcaaaagctaagaacttccagcgtaccatttgtgtctatgacgcatcgaatggtggcactgagtatccagagatttcaattctcggtcgtgcatcaactgttaacttcaacgttgcgaatagtgcactggttctggcattcaagaaaggtccgacaatcacaactgccgacctaactcctgaagaattggctggcctacagtctcataacggtaacgcatttatttcggtagatgacaatgttatgttctggaatggtttaatggctgacggcacttggtttgataccgtgcagggtgtttcatggttgtctcagaaagttcaggtgaacgtgttcaacctgttctatcagtcaactaccaagattccttggactgaaactggtgttgcaatggttaaccagcaagttacgctggcactggaattggcccgtaccaacggtctgattgctccgggttatgataatgaaggcgtcttctatccagacggttacaaagtcatttcaaccgacctcgccctgctgcaatctcagaaaggcaaacgcatttgggaaggtacttccttcattgcgattggctctggtgcgctgcaaggtgcgattatctctggcaacttcgttcagtaagggtgcgctaagtgaagcagtattcattctataataccgacctgctgattgatggcgctcgcgtcgatggtttcacagccggtcaagcagttatcactgcgcgtcgaaacgtgcctcagcatcttccagtaatggacgcatacggtaaacttgccgttgcaactactgctgacttgtctggtgcgattacgttcccacttctgcaaacagcggactggaaccagattctgtatgagcgtgctcagctgagtcaggcgactggtctgtctggcaacaaatctctgtggcagccgctacagattcagattgttgacaagatgggtgatgtgctggtcaatggcgtcaatggcgtcatcctgcaacagcctgctatcgttcgtggtgtttctttcacttcgaacctgtgggcaatctacgtcgagcgtctccagattaagactggttcttatccagagattggcgtttaagttttaaaagcgagaaacataaatggcttgtgaattacttacgcgggagtttaaaaactccaagggtgaatctaaactgttcaccactcgccaactggccgcgagtaaagcactggacttgcatgttgagctaatcggtaaagtggggacaagtgtgttcccacttatcgacaacaactacaatttcggtgatttgattacactcatgcgtcaggccgacaataaaattgtcactgatttaatgaagcgtgtaatctgcaatgcgaacgttgaaggaaccgaaatcaaaccggcaaccttcgatattcatttcagcggtgaactcatgttagtttgccaagtgtttgccttcgttctcgaagcaaacttccaagcttttttcaagcaagggctcgaaatgaacgaacagttcaaattggcggaggaggcccgattggagcaggaacggttggcattggaagcgaaccagacgaacccgacgacctaacaagtcaatttccggacattcggtattttctgcatagaccaatcatagaagatagttccctctgttctcttcgtgagttgcaggacggaacttattctttaattgatttactcctcttccacgatatccttgatttaagaaagaaattaaatcctccagttgaaacggaacagtgatggctagcagaaaagaaatgatgggcatggatacggaaactctccgtatgcttggtcttgaggccggattatcttttgagcccggactctcgaagtccaaaatggttatacaactggaaactcatcaagcttccggttggttagatgtgaacagccaacttcttcatgcagatgcggaaggtggctttgaccacatgcagggctttacaggtcacgaagaacaatccatttctgacgctgcaagagttgcacaatcgttggctggtgctggttacactgaaacattccattcaatcatgggtggaggtcgtgaccatcatgttgatgcccttcatcaatacatgcagaaacttggtgtctctgctgatgatgtttggatgcacatgccaaaggcgaatcccaatattacgcctcagaatttcaacatgctgaaaggttatttaaataaccattgggatgattatcaggatattatgcctccacttgaagggcattatgctggtgatatcatgggcgagtatgccacgaataaaggcagtgttgccgattcgtacaaccatcttgcatccatgtatttaaataaagctgcttacaacaatccacatgcctatgaaaaggatgcgtcaattgttgcaacgcgtttggcttcggcaatgggaaatcaattcctcgaagttggctatgctgctgcaactggtgcgaaggttggatatcattccattctcccgcaacttggctctgatgttgttcgtggtactcagtatcctcgcgaacctttgaatgctgctggtttacctttaggtgcaactggttctgctgttcaaggcaaccgcgctcattattctttggttgcttctttgctcggtcgtccagaaggtgctgatgaagcatcaagcgcgattcgtcaggaagtaagctcaacaatgaagtctctggcgtcgtcttataaaggcggtggtgaaacaggaatgaatccttatcgccacgaaacgtcagagcatgacttattgcttgatagtgcgacacgttatgttggtatcgaagaagctcgttcaggttacgcaaacttggatgacacctcatacaatcgcaacaacattcaagcggtaatcgaaaacagttgggacaagatggatgctcagacagcgtctgcaccatctggtgttcccaatccagacctgcgtttaccacgtcgcgcagagattggtactcaatggagtgctgatttaaacgaaccaatgtcttggaatgcagctcgttctcgtagagagagcattgcaatctcagatttggatgctgctcatgcaaactttcgtgatgttgctgatggaaatcgtggttcaaacccgattaagtatcacaacatggaacaaggaagcgatgagtggttcaagttccgtgaacaatatgatattaccggctcaacagttggtggtttcttaggttcaaacagctatacccgtccgtgggcacagttcatggacaaacttggagtgacaaggaacgaaacaagtcctaattcattccaagaaaagatgtttgcaatggggcacaagcgggaagatgaagctcgcatccgtgtttccaaagaactcggtcaggatatccagcaagttggtgcaataaccaacgacatgttccccggaatgatgtattcaccagatggattaattggtgatgacactttatgggaacataaggctcctgaacgtgctggcaagtttgcagatttaaatgcaggcgaacatccagactacatggaccaagttcaattgggcatgttgctttctggacgcaagaaaactttgttctcgcagacgattggacagcaaacacagaatcaatggattgaacaagacccggattggtacaacagaaaccaaactcgtcttgattctgtgctcaaccgtatgcaagctggtcgtgacttcctctcaaaccatgctgaccttcctcaagatgaattgaaagccggtgttcgtaaagctgtaacaggcgaaggaatctggaaagatgttcgtcagaaatcagaccgtggttattctccaaatgctggtacagaagctgacccattcttaacgggcggtcgtcgttcttataatgacgctgctcaaggtggctcagactacgaacctaactttgtgaccagtgccggaaatggccttgtgccagtgggcggtggtggcgctgagacgggtatggcgcttgcggttaagcagggcgtactagcagcaagggaagaggtaaaacgcggcgaggctggcgctggtgcagcaggattcgatgctggcggttcagaagccgatgcggactttgacgatttgggtatgcctcgcggctttagccggggccggttcaacactgcgaacggtggcggtggtggtcgaaatggcggcggtggcggcaacgtgccgggctctgacaacttacctgagtggttgggcggcatggggaactcgctctatggcgggcttcgcagcggcactctgcgcggtgtgcaaaatggcacattggatgcaatcgaacaagtcccgttagttggtggaatcattcgcggcggtattggtgcggcgcaagcggctggtgaaggcattaattcaatgtctaactaccgtggaatggcggaagatgcaggaatggagtctggcgtaggctacgattctatgacgcaaggtttggaaatgatgggcttgaatgcaaatcaagctggtcaggcaaaccaaaacattcactctgcatttaaccggatggcgaatggtgacccaagtgctgctgttcagttatcagttgcaactcgtgggttgttaactcttgcggatgttcgtgcaagtggtggtgacccaactcgtctggctgaaatgttccgtgataaagcgaaagctcgcggatggagtcaggctcgaattgcaggtgctgctgaaatggcagggcttgatgggtttgctcgcgttccaagtcgtagtgattacactatgggccgtgctcgttctaatgtcgatgctcgtatgagcgaagatgttaccagccagaatgttgattgggaatttgcaaacacagaccgtgcatactcttccactgactactcaattcctcgtgttggttttgagaacttgtctggtgctggagccaaagccggtaatgccatgcagtcaacatttgattctgcatcaagtgttggtagcaagtttgccgatttggttcgccaacttgagtccaatggcaaagactttgatgagaatggtaatcctgtaaccagtcgaactggtgctaagtattccatgcaggttcttccgtctactgcacgtgacccaggctatggaatcaagccagctcaaagtgatacaccagaagagtttaatcgtgttggccgtgaacttctcgacaagatgattaacaagtatggcggtgaccacgacaaagctgctgctgcctatactgatggctctggtactgtggatgcagcggttaaacaatggggcggtgattggcttaaacatatgccagcacaagctcagaaacgtgttgccgatttgcataagttgggtgctggcgcaaatggatttgcaggtaattcttctggtccatctgttggaactattaacgttaatgtgaatgcaactgtgaatggcaaacaggcaactgcaactgcaactgtcggtggtcaatctcagacacacactattaatgttggtggcgctgtttctcagaagcgttaagaatgtgcggggcttcggctccgcatttctattcaactttatttgaaattgatttatgaaggtgccattgtgtggattagacgcgttcaggtcatagtaacaaataagaatgacccaagtaagcaaacagtgtttgaaaagcacagtattgaatttgaagttcgttccatcataggatggggtgccgacacagcaacagtgacaatctataacttagatttggatgaagttaaattcttacagaacaaaacattcggagacttgctcattgaaataagagcgggttatgctgatatgttagtagctggaggtgaacgtggacactacaacactaatgatgttaacggtcgtgaagttcgaatcaatgtttccgagccaggcgttttgcctactattttctctggcgtcttaacaaacgctgttggatttaaacgtgctcctgaacatgtgacaacgctcttctgtgtttcgaaagcagcggtcaactcgactgacttcaaagcaatgaaatcaataccgccgggtgcaacattgaaacaagctattctgtctatgacggcagattatggtttcagtgttatctctacgtttggcttgctcgaacaagacttgagcgtggttctcccaactggtcgtgtttttcatgacactttcctaaatgagtttactgctctacttgaagagcacaatcttcgtttctatatttcgacctcggatattcagatatttccggacacgtatggcgaccaagatgcaacaagccgaatggcaaaagatagagagccaatcaagatagatgccaacacagttattggcactccaattgctggcattgctgtctttgatttaaatgtgtttctccgctcggatattcaaccgggcatggtgatggacatttctcctttactcggtactgagttactggcaaacggaatcgttggtgtaactggcggcaagcaattgctgaactacgatgattcagttttccggtacggtatggaagataagtatcttatcgaatccgttatccatcatggggcaactcatggtcgagatttccaatcatctattcatggtgttcttggtggcaacaatgctgctggtttgaatgaagaaaactggcaacagtggtatgcccgaagcggtatgagtatggaaggtgaaggtttctaatgtctgatattattggtgatgttggcagtgccttaactggcgctgtcagtaaagttaaaagtcggttccattacgggccgcatccttctgtcatcatgtggaaggcagggagtgctacacaggttcaagagaaagatgattctattcttggctctgttgaaaatgcaatctctggtgccagaaaagcaatggaggaattaattgtttctccaacgacggaccaattcagttcattcaagtttgatgcaatggtgagcgaaggccaccttgcacaatctacggtgactaaggttccaacctcttctggctttgttgtttctgaacacatcatcaatcacaacagaattttgaagttggaagccgttgctgtcaacatgcagaactcagcactttggacagcgtctgttcaaggcttgtctgtgattagtggtgcaatctttaacaaccctgtacttcctgcaattggtggattgtatggtgttgtgtcttctgcatttgaaacagaagaccgtatccaatcaacgtataatctgtttaacgatttgcgtacatctggaacgaagctgtacatttcaaccattcttggaacttatctcaactgtgttatcacagagattcgggccaagcatgataaacaaacagccgctatgttggctgtagaaataactcttgaagagttgcaagtaatcggaccagatgaactagcagatgcagctaaagcagcaattgcgtcatcatacgattattctgaatttgctaaaatggctcagggtttgggcatcggtattcttggcggtgttccacttccgggactcggttcaatagcgcgtccgacagagcaactgaaaactctgaaaggcaagctgaccaaactgtcgcaacctatctcttctgttaaaggacgtctgctatgacaataagagaagaacgcgatgcactccaagagattgcaaacttacttcctcctggttatgtgaaggtagttccattctctgtatccaaagatatagcatttgagttcaatggcgttacacttaaaatgtctgccttgtacctcaaccgagtgttgaactgttatatgtttgacctttcatggtcatccacggatgcaatttacgggattccaattcgttgtggtttaaatattcttgagcaatttgcaacaccattgcctaatctctatgccaacaaccacgcatatccgggaagtgaaatcacaagctggcaacagcttgacttaatcattattgatgaatcggtgctcgaacgtgggtagtcaaaataacaaccgtgctccagatatcaatacaggatatccagggttcgcatataactttgacgacgaatcccaaacttgtgatgtacagcttgcaatcgaaacactcttcatcggaatgaaagttccttactctttgcagaagaagcaaagattgcagaaggttccggttcaattcatccaaggtggtggatggtcgttaacgcatccggttcccgatggtacgccagtgtatgttcatttcgcccagcgaggaattacacactggctagttgaaggcaaagatagtgctggaatgataaatggaaaacctgctccagcattcagccagttgtttaatatcaacgcagcgacttgtactatcgggaaccaacctattcctaaagcgattaaagggtttaacagcaaggttgctgaatttcgaaacgccgacagaacccaacgagtaactttggcgggcgaaggcttaatagaaattgtttctggctctacatacattcatgtaaaggatggtgaagttgaagtcagcacgcagaagacaactgttaagtcgccggaaatcattctggatggcaacgtcacagttaccaagaagctcacagttaatggtggtgcagcaatctctggtggctctggacaaacattcgaagtcacaggaaacgttgcacacaacggctcttatgtcttgaatggtgtcaaagttgatgggcatgttcatcctaatcctgagggtggcaaagttgggccaatggagagtgcataatggcgggtaacttaaagttagatagtaaccacgacattatccttggtcgtggaatgactcgtgttggtggtgttgaatatgtggcgcagttggttaaatgccgactactcactttgttgggtgaatggcagaacgatacttcacttggattgccttggttcgatggtattctctcaaagggttccagagtatctgatatccaggtcgcgttggcaaatgtcatccgcagcacaaaccatgtaagacaattactttcaattgatgttgacgcggattatcgcacacgtaagttgaatgtttcattcacagccatttctgattatggcgatgtaacggatatcgtagaatggcagctatagtttatggcgttaccgataaaggatttgttcgcaaacctttggcggctgtggttgacagtctcaactcaagattcacggctgcttttggttctacatttgatgtgtctcctgaatctccagatggtcaagtaattggcatcgttggcaatgaagctgcgcttttgtgggaacaatgtcagtatgcgttcaactcctatcgtcccggtgctgttgagggtgttggacttgatgcggtctgtgaacttactcgaaccaaacgatatgtgaacaaaccaactgccgtcactgttgagtgtgaaggctctgctggttctgtcgttcctgctggcctaattgttggtgatggaacatatcagtttgaaaccaaagacgaagtaattcttccgggcgacgtaactggatattgtacaactccgggtgcaatctacattgctccgaacacagtaaccaaaatcatttctggcggaacttcaagccttacttctgtgaacaattcagaagaaggtgatatcggtattgtttatgagtcagacccagcgttgcgagttcgtcgcgacaaaacaacagtttccgatggttcagcaacagcggaagcaatctactctgcactcgctgacctcaatcttgattacgttcgtattcgtgataatgataccggcgctgctattggtgctcagccgtcaggcactatctatgtggtagttgatggcggtactgttaacgatattgccaaacgaatctatcagaataaagctggtggtgttcctacatttggcaatgtcgaagcaacaattaaggacagtaaaggttatccgaaaaagattaagtttagtaggacaaccaaagttcctgttttctttgatatcaaagttaaacgactgccgggtgctaacctgagttcaaatgacgttgaggtttctgtccaggatgctgttcaggcatacgttgattcacttcaaccgggtgctccagttgtgtggtcttatctgattccaccaattctggctgctgttgcaggtattcagattgatgatttggaagttggtaagactgccgaaacagtggctaagaccacagttgaaatggatatcgacgaacgtgcatctaccgttactgcgaacatcaaagtaactgatacaaccaatactccgtaggtttaaaatggctgaaccaaaacgcggtttggggatgttgctttcgcaatacaaacattctccaaaccttaagaagtacattcaatgttttctggatgagttcaaggaaattgaacaaaccatgaaagacgttgtaaagtatcgctaccttgcagattcttttggcgtgatggttgatgacatagcctatatagtcggagcaagccgtatcctctatggtgcggctgctcttggcttctttggctactatgaaaacccggctgctgaaagtacaggtgacgataatcgacccggtgttggtggtattcttcgttctgattctgaccgaaactcaggcgactttattcgcacagatgttcagttaaagaatgccattcgtggtcgtattatcaaaacggttacgaactgctgcatcgacgatttacttttgttctgcgacttggtcgtagggcgggagttggatttggaaatagttgaaggagatttaaaaatggacttcattgttcatgaaactcttccaactacagagcgtgttcttctttcatttatgattcctgatattaaaccagctggcattcaatgtacgctgaaggataattcaggtaacatcgctctggtttattactcaactgactatccggcgaatgtgatatgacaaatagggttagtaatctctcacagatttgggctgaaaatggtgtagctactgaccctgatttggacacaacacatccaatctatcagcccggcaagtatgctaaaggttggattgttgagaaagaaccgcatcagtggcagaactttctataccaagtttcagacctcaagaaccaaatcattgcatctgaacagattcctgaatgggatgcagacacattgtatgctgtggatgctgttgttcgtaagggtgatgatttgtatgtcaacatttcagaaacattgattgacggcgaagacccagcaacgggaacaggctggagcaaaattattggtgcggatgctgatgctgttaatacagcaacacaaacactcgacaccaaaatcacaaaccaccttgctgccgacaatcctcataacgatagcatccatgcaatcggtggttatgagaaggaagaaattgatgacttccttggttcgccaacagacccacgaactattgtctaccatgaaagtataaccggtaaaacagcacatgccgaaactccggcacaagtgggcacacttcctgtggcgggcggcacatttaccggcgatgttgcttttgatggcggcgttaccattgggccgggttcattccaaaaagatggccccgatttaaaaatgagtaatgctggcggttcaatcatcgtggaagcaggtggtgacgttgtttatggcgaggatgcggctggcagtagaagtgaaatcactacagttgcaaacttccaacggcaacaacgtgctgtaaataacttgttcgcacttccacaatcaatcgccgaagttgatttccgcgcaagcagtttaagttgcctggggattggcagatatacaattgatagtggcagcaagactccaaagttctccagcaaaggttgggaaatagaggccggattcttagtcactggtttggaattcaacatgcctcgaactgacttggttgaatactatgccggggatgtgttcagacgtatcttggttgagtcaactgttccacttgctggttcgcttgatttgaaagatatcatgactcgcattgctcccgatgcaactcatgtccagcgaattgttgtttggcctgctctgaacaaatatcagaaatcaacacttcttccaaagtatagctcgctgttcctacagaatgatacttcgaattctccaggaactgcttggtatgtcagcaaagttgacactaacattttcgaaatgcctaatgcaactgctccgaaaggttctcagtatattggtgcattccagtggagtgctgacgatgttcgtggcggtcgtctggattcaactgctgtatggacaacttcagatgacacagtcgttaagattggaagtgtctcaagttcaggtcaggctgtagtcagcatccttaaagctggtgttgctgttctcgttgttaaatggggcggcatggttgccaagctaacaatcactgctaaataggaacttaaatgctccgtccaaaacttgggcgcatttgggctgatggctcaagtgtagctcgtcgcgacccaggcgacacaaaatatgtcactggttggttgtctgagattccaacttatcaggttctcaacttcctccagtggaagaatgatttaatcattcaggctcttgctgaacgtggtgttctggagtggggcggtgatgtaacctataagaaaggtgctgcggtttgggatgaaacaaacaacaaaatgtatgttgctttgttggacaatccagacaaaaccaaagcaccctcaaccaactctgctcagtggactggttcagcacttcaactttctcgttctgcatatgatgcaacggttaagaagattgatgaccacgttgctgatgtaactggtaaccctcacaaacttactccaggacgtttgggaacttatacagtttctcagattgactctttggttgctcagtatcgtgccgaagtacaaacacatgccagccgcaaagataatccccatggagtaactgcaacacagattggcgctgtaccagttgagggcggtacttacactggcgatgttacaatgggtactggtcaactcttcctgtctgccgataagactcgtttaatcaagtctgactcaactggcgtgtacatgaagaatgctgctggtgctattggtattgatgctgctggtaaaggctttgtaaagactggctctgaagccgcatctgagattgtaacaaagtccacttttgcggacaataaagcaactgtggagccaaactacgccattcctcaaccagtgttctatttgccgcttgcgtcagatttgaatatttatattggtggtggtacaacactgtctactcaaaacgatacggcaataaactggaatcctcagatttttaatggcgcgtattttggcacaagtgctggaaacaatccacaatacgacagtaaaataacctacacatacaaaccacttgaaggtcttaaagacatgacggtttgtgttgatatttatctcgacagtgttggttctggcagtttgtgggatttgtatgcctctgctggctcggtaactggttgtggtgttatccaagtaaataaagacaataccgtcaggttctggtctgaggctggttcaaccacaactgtatctgtgcaaaacaattcatggcacagagttgttggggtaagaactgcatcctctttgattctgtatttagatggtgttcgggttgctactgccgctgtaactaatgggccaatcaccggtgatgcatacaacttcatccgtggtaatgtacaatctaccgcaaatcaaagatacattaaagttaagaactttaagttgtgggttggtgccttaacagataatcaagtttcaacattgtaaggtgtaacaatatggccaaaggttggtctttcggtgctctgactgaagcactaaagggtgcggcatttcttgatattggaactgttgcaaattcagttgctgctggcaacgacagccgtattgttggtgctgcccaaaaaagtaggaacttgggtgacctgctcgactatgcagcagcaagaaatcaactcagcgctgcattcgtgaatggcgatggaaatgttgatttttactgtcgtaacaatggggggccgactgctgctgtgaataatcagcgacttgattttaggttgctgtctaaggccgatacagaagggaatgaatttactccattcaaagttggaggtgccacacaaggtgctcaagcagtaagattagaccagttccaaagtggctctaatggtaatggtgcttggactaagattccaaatgggccaatgtggtgcaggcagaacttatctcttgcagcaaatgcaaccacaacttggaatttccctgcacagtttcctggaagtcctgctgtattcttctcatctttcaatggtgagaaccgagcatggtttaacggcatttctgccaatggttgtaacatttacaatccacaaaatgtcgcagtcaacgttaacgtgtatgcgatatggtaattgataagggctacaaagtggatagacaaactatccaagctatctttgttttcatgcaccagtatggaatcttacatggcctgcttgcaggcttagtagcattgattcgtggagcttacgaaagtgaaggacttggaaaagcgctgctcgatgcggccttatgttgtgttattggaacgtttgtcttctcacttccaattctggatggttacttggttaatcacccaaatgctggttttgttgcttgcattgtaattggtgtagttggtgcgaagttaattattacaactattcgtgactcattcacagctgcgattaaacagttgaatccattaacgtggttcaagaaagcaaaataaggaagcctgatgcggaatgttcttctgctcatccttcttctaacggctgtcccggcttcggctgggacttctttcaaatggaatggtccgttattagattatgctgcacaactttatttaaatggtgctgctggcaaagtctccaatgtagactgcatgtccaaagttattttcttcgaagccagaggtgagaaacctgctggaaagattatggttgcaaatgtcgtacacaaccgaactcagtttggcaagccatttgcaaacacgatttgtggtgttgtctaccaaaaaggacagttttcatggactaagaataaatggaaacggaacacagattttcagtctgtagctctaaaatttagtagaaatgaacacgaaagtgttaaagaaagtctcaaaattgcgttatatttcgtactttttgagccgaaaaataccggaaaatgtactcatttttcatcaaaatctgacaagtttggacgaactttgttcataaaacgagttggaaatcacaagttttatcaatatttaggtaacaaataatggatttcttagagaagctggtattcatctggtctgtcatttggggcacaatctttcttgttaactgctgttcaccaagtaaatctccaactgagaagctgtgcaattccatcatgcgagtggtgaatgcagtgttcgtgctcacagttgtagtgtgggtgtattggattagataggcatttgatggtttgatgctgagggaaggtggtcgcgtaagcgaacatcctttccgatgctgataagaacaacataagtttctatattcaattccaaatattgtttcaatattaagtaatatgtggaatggagatagatggtcggtggaacatacttggtcggtcgactgttccaaattagattcgattcgagattcgtatatggttcgaaatttagattcgtaataagattcaaatttttattataattttttttttattcgaccaatcgaaattcgattatgtggctataattttttatttttgaagccgaggaacagaagcccaacaaagtcctgtcg

SEQ ID NO: 2 - DNA, 39879 bp, Erwinia amylovora bacteriophage Ea PF 2 DSM 34959
  source 1..39879: mol_type = genomic DNA
ccagcttccgaatgctctgacttgttgtcgcggttaccttgttgaccttatcgacaccaccttgagcaacgaacgcagcattagccgcagtcttcgtgtaaacatcagaggtgttagccttcttgtcgatgttgccttgtaagccactaactgcgctctcaagctctgggtgagtcacgaagtctccctcggaaccaccagtggtgtactgagcgtcaatctgccagaggccctcagagtcagccacagcgtcctcggaagtaaccttataggccaccagcgtagacgttgagacatcatccagcagcgtcacagtgaccacaccaacggttgccttgtcgagttcggcagaggtcttagtggttcctcgtgagccaatcagggtaaggtccttcggtttgcggccttcaagagacgcacggtcaatgtagatgattccatccagcagaccacgcagtgagtcgatatgccatgagccaccaatagaggcggtgccagcgttccatacagtcttatttactacagccatgatactactcctttcgttgttgtgcgtcattgagtttaccttgcaggactcgcacagtatcttgcagggcttctatccacttgtcaccacgctcggtcacttggataatttctttagcagactctgggtcaagttcggcttcaccattaaactcgcatcgaccactaggtcctgagggttggcttgaggccttgaccttgacgagcaagcgcttgttatcgacacgcaaatcattaataaccctatcagtagaaccttcaagggcctcaatgtcaccctgatacttccgggcgatgtcggacagcgcagactgttgaagtcgctttgcgtcatctttcttgatgtactcattgtgaacctcccggtcccatttagcgttggtctccttgactcctgtggtgtacccaacgaccaccagcagtgccgcgaagaaccacggtaacgctttctgtaaaaacttgagcatagttgccctcctgattcctcagaatccacgtagcgttgtcatcacgtagtgtgtaacaatcataaaggccactacatatagtaatgaccttgagtttgtcacttagtggaagtctccttccgtaaagccatccttgtccaccatctggttgtatgcctccagaccatcagccagaccgcccagaatgtttgcatccggtgccagcttagagatttggaacttgtggcgctccagcagtttgccgatagcgttatacaactgtggggttcgacgctcatcgtcctgaaggtctttcagcatacgctgggccatctcagtatcgagcatctcaaggaatttgatgagagtattatcagacatctttcgtcccctgtttatatttcacgattgtgtcaactaccttggcaccaatctgagccactgtgtaggcgatagccgctacgtaaaaccactcgttaagagacagtccgtagaagtagcgggtcacaacgtcagccgatgccgcccccgcaataggggcagctttcaggacctcgttattgaagtcaatgtttaacatcttgtttatccttgtgaagatacagaacctgcaccgaggttgttcgcaccgtccgcagtgaaccagaaggagcctgtagagaacgccatacgccatgtggtcgtaccgtttccgctaacagcatccgacactaggaccacaccgtaagggtgctctgttgctcgtggaagttctgcgagtgtgtaacgcggggttcgcactgagcctacgagaggctgtagagcaatcaccttgtccaaaccattcatcttgataggcaggtactcactcgcggcctgattcgaggtcttaccctctaacatcaactgaccgtctgtcatgttataaccgagaccaaacgcggagttgttaacgctccagtgcgcaggaacctgtacagcggtaggcacggtcgcaatgtcaatcgcagcgaacaccggggacaggtagaagtgcgcaccgccctcgaagtttgacttatcgttcgtgtggaaggtcgtagcgacaccaccagtgtaacctcgcagttgcacgaagatacgcggacggttattacccagaacgatacgcacatcagagattggagaggcttgctcaccgtaccatgatgcggccattttggtgttgctatctttctgctgaacacgaatgactgctttaccaccaccaaagttggtgccctgtgggcgagcatcagcaacagccgagtcgaagtgacctgtaccaacgagttcaatatcacagctaacaccagtcgcaccagagaaacctaaggttccaatctcgtaccacacagcgttaccagtcatgttggacatcttgtactgagatgactcataaccgtagctcatgctgccagtattgatgaaacctaactggtcccaattggcagtacctcgctcgtacactgagttcacccaagaaggcatcgaaccagacgggtcctgtgaagggtcataaccagacacatcaggactcaagccagcaccctgagcgaagcggcacttaatctgaatcaccttagcgtactgtgcaccagatggcagctttgagttttcctgcgtgacgttcttcagtaaccagccgccctgagagatatcaaacccttggtcgcagtggtcgaaccacacatcttccataacggattgaccagctcgtatacaggaaactgcgtactcgcctgtgtgaccctcgaagttacaatcggtaatcttgattgcagtcgggtggtcccatgctcccggattctcgttagaccaatcggtgcggaagaacgatgccttaccttgagaggagtagcactgtgtcacggcggtgtcgatggtgtcgaacacatggaacactcgacctgtcataccacgagcctgaaccgcatggattcgacagtagtcaccacgagtcacggtgttctctaagaagccacacttggacccggcaccgttcacgtaaaggaacgatacgtccatacggcgggccttgaagcggaacatgtaggccattgaggtcttattgaacgggataatcatcacgctcggtaggcgaccataggagaccgttgggcctttcatcttgaacgctggaatctctgcatcaccgaagtcatacggagagagtgcaatcttaccagaaggcaggacaatgcccggaccaaaggtagcatccacagagcgggaccagttgtgcatcttaacgacagcgtgcatatcatccgtcacaccgtccatcacagcaccgaagtgtgtcacgttcagtgaactgttgtcgtctgtacgtttccagtggtgggtcggaccggaagcaatggtgcctccattatcgactgctgtagtgagatgaccaacgaactcgccgccacccagatacttaccagcaatgtacgactccagcttgacacgttgtccctcaaactgaggcttcgctaggcgcagtgcatcaaacgagatgtagccaccaatagcggagaaaccagcaggggtcgcaaggtaacctaaagtacccttgtcgccagccgcttggattgaatccagaatgccatcccagattttctgagtggaatcacggtaggtcttggactcaccagcacttgctgctgctgcctgagcgaaacgctgtgcgtctgctgtggcttcacgaatctcagtggtaatctcgaagcggccttcctcggcaatgtgaatcgcctgaagctgtgagatgttcagagagttcgcggtcagtaccgaaccgtcccggaagtctaccaaacgggtagccggggtgtgacgcttaacttcaagcaggtcaccaaaagaggagtagtcgccattgagtgtgacttcagtcagacctgtaaagcggtagtcgtccgtcaggcgtagagtcttctcaaacgttacgtcatctacctgcttaatggtaaggaccacagcagagcgcgtaaggtaatcgaaaggaatcgtgacggcacgagttgcggacgttaagggaatctcaacgatagtagattggtcggccatgataataatccttatagttatgaaagtgggaaaccagaggttggtctcccgttagtgagtcttaattaggtcgagcctgttgtttcagctcaacaccctgttgtgcaaacatctgatagagcatctgctgggtcagtgggtcgttcggcaccagttcacgagtggtgttcatcatggaagtcatgaagtcctgctctgtgtacttgttaggtgcgttcagaacgtgagacgcattgtatgcactcatcaccacgttggatgcgaagccagccgctgggacctgctcaacgagtcgggtgtagaagtccttcatcacatcactggaagttgcagcaccacgagaagccttgaggggtttctcatactgtgaatctttcggtgtgatggatgagcggactgtgcggcccatatcgaagcccagaggtgcgcccacgaggttgaatacacccagaggtgcaccagcatgggaagcacgagagaacgctgcgtaggtaatcatgtcctcattcagtgctgacttgaggtagttcgcctgttgctctttcggtagacccgcagccttcatgtgtgcagccatcacgtaatacgctccagccagacccacagaggcactccacgccaacgctgtgtccatcgctcggttgttcttcgtggactcatagagacccttcatgaatcgaccgttgatagagcggatggtgaagttcttgaactgcatgaccatcttcacgccagcaccgtaggaaaccgcatcagtgttagagaccttgtgtggacgtaggattgtttcatctgcgaccttatcagccagacgatagaggtccatagcacgagggtcagcagcgaatgcacgcttgttagccaccttgtacgaaccatcctccccacgaacaacgtggtccttaatcaactgctgaataccagcgaactgctctggggacaccgaggcaccattaaggaaccgagggtcctgccacttggatttcttaccgagcaacgtggagttaaccacttcacccagcatcccctgacgaccagcatcaacgaagtagttggatgtagcgttaaggaacttggtccacggtgagcgtgctgacagctcctgagtggcatacttgaaagtacccacagcctgagcggtcttagagccagtatcagtgtagtcacgtagacggtccacaatgtcctgacggttcggacggattaaatcatccagttccttaccgaacatgaagtggtgaatctcagcgagttcctgtggcttcattgcctgattgcgataagcaaggtcacggaacaccgggatgcctttcagcaacgcacgagtgttacccttcgccaacatgccgccaatctcggtgatgttctgcaagcccatgtaggcattcttagcgaagaacccaaggtcagtcattgcgcgagtagccgtagcgagagcaccctcagggtcacgtcgagagcggcctgtaagaatcttgaccatctctttaagtgccttaacgtctccctgctgtggaccacgagcctcgacagtcttatccagcgcaaccagttcatccttgagttccttagtggtcttcccggttgaacccatgattgcaatgtcaccattgactcggcggtcgtaggcaggcatcaggtgcatcatgtcgtacactcgcaggtcgttcactgagaacggttgaccatcaggtgccgttacgcgcacatcgctgtcaaagagattacgggcttcgaggaagctgttgttctcaataccagtcagagacgtatcggtaagctggtcatcaatcacggaggagttgttaaactggtcagtgtggctcacaccatacgccttatccatcgcgtgcttacggaccatctcttcggtcacctcttgaacatcgagggtctctttcagcatctcatcgacacgagccttcacctctggacgcatacggtaactcgcaagccatgactcagcgaccgcctgttgtagaccatcagaaccaccgaagcgctctgtatggactgccttagcggtacggtcatagacctgtggaacgtatgtacccttgtggcgagagtccgggaagaagtccttggctcggctgtcaccgaacatcgctgggttctccatcatctcacgcttggtgtcgaagtgtgccttgaggatgtccatcactttggcctcacccggcttcaggtcagctctcagttctgggcgctcaatcgcagccacaacacgcttagagatttcttcgcgagcaccctgagcactggtacggaagatacctgttgaccactctgggtcacgcatggcttctttcatagcgtcatagtacctgttgtaaatcgcttggtccgtgaagtggagacgctcgtggatgtccgatgcggttgcaccaaacttacccattgagccatcttgcatcagagtcgctggacgaacaaggtcagcaccaatcccacgcacagcgttgttctcgctacgcagaatcttctgaccaatctcagagaatccacccagagacgcaccgcgaagtgcacgcggagtgtcatcagagaactcagagaaacgctcctgagtcttcgggttgaggatgtttgactcagacaggatagaaccgtccggcaacaccacggaaccttcttgggtcggatggtccgcatactcaatacctgagcggtcatgggtcctgaactctaaaccatcagtgaccatacgggacaggtcctcaccaccagtgttacgcgcagtctctcgggcttccaatcgtgacatcgtagacgcgaagtcattgaagtggtcattacgtcccagacccttagcgaccgtatcggtcagagcggacataccagcaccgaacacgaagccgcctaaagcagcattcgcataatgggcctcaccaccagcaatcgatgtgcggaaaccttcagaggccacgttccatgctccagactgtgcgccaacaatcagcgccttcttcgccaaggagaatcccttagcggcctgtccggcaatcggaatgtagctcgtagggtcaaacgctgcgccaatcacaccagcactaagctgtgcgcccagaccactatcagcagccttagcgtcagtctcatagttctcgttcgccatcttaatgagcgcatccagattctcaggggaaccaccggacaccacgttgatgtagtgcgggtccttaacctgtgagcgaatcttctggagttcctcttcggaccagacgtgagagttccagcgagttggcgtaatggtgtctttgaataggtcgaacccattgttctgacgaccagcacggaaggccatacctgcaacactgttagaggtctcagcctccacggcgttaccgaaaccaaaccacgttgagcggttctcagcttcgtctaaggttgtccccttggcctcccaataggattgaccgaagggcttgttaggcgcaggctgctcgatgccctcagtgttgaaaccgtgggactctggcagagcgccggaatcatccagccctgacttcactgacccttgcttgccgatgcctgtgaaagcatcagaagccggaatccctttaccctttggggtgataccaccgaaagtttctaggtcacccgaacgaggactctgtgcgacatcactcagtcggcgcatgtattccacaccttctgggctgataccggagaagtcacccttgtcgtaagcctgaatctgagcggccccattgcgtccctcaccttggttatacgcgagggctgctttgagttcatcaccatcatacttgcgcacaaggtcggacaggtggcgagcacccgcatcgatagccttggctgggtcataacggtcatcgtcatcaccatcagtggcattcagacccagcgcggacgctgtggctcgagtgaactgcatgatacctttcggcccggtcttagactgagccttagggttgaagctggattcattgaacgataatttacgcagtaagtcataagagacaccatgcgcatctgctgcctgttggtacaacgagtcgtaagcgctcggtacacttttgtcatacttagccatcatgggcctcctattgattatttaataccgcgtgactctcggaactcctgtgaacgctgagcgaggctcttacgcttaccggacttgatgtctgcgcggacttggtttactgcggcgataggtgcacgcttattgatatccttcatggcatcttcctcagcttttgcttgggctttagcctgctggtccttccagaccgaactcagtagctgcttatcatagcgcatgtccagattcccggtagtgtcccggatgtgaaccgtattgccctcagagtacacataaagctgcttattggtgacccaagggttaacgcggacgattccctgcacggctgagtcgatgatgtccttaccctgcttccatgagtccgggtcatcgttcacctgaaggttcacacgagggatgacaccaaacgaaccgcctgcgaggtcatcgctttggaacgtagtggttgactccttgaggaactttgtgacctgctccatcgcaccatcaacgttacctgttgcgtagttgaacgcatcgaacacctgacgcgctgagttgcgtagcgacgaaggcatacgcgcaatctcctcggcagtcgaactgttcaacgtagcggtccacgacttgtcagcctcaattagctggtccttagtcatgccctgtttgttacgctcggcatcaatcataatctgaggtttgactcccagcttatccatcatgtccatcttagcgaacagtcccgcttggtccgggtacagtgctgcaatcaggttcgggtcagcgttacgcagtgcacgcaacttagtcatcgccggggtctcttcaggcatctcaccgttaatcacagcggctcgccattcaccatcagcatcactaatcatggtgccaatctgtgtacggaacggaccctctgcgctatcggctcggagatactgcaacttgagtttgtccttctgctcatcagggacgttcatctggtcaatctgagccagcttccggttcgcaaagttcacagcatcggagtgtttaaactcgcctgtgttctcattggtcggctggtccttgaagtcagtcgaaacgtaatccccattgatgcgcttcaggtaagaagcctccagcaccatgtccttgttctgacccttacgagcatcatcagtggccttagcggtcgctgcggactcctgacgtaaacggtcctgcatctgcatctgagcctgaatcaattgctggcgctctggggtcaactgctcacccggctgaatcttatcgagttcagctttctgtgcctgcaacatggcccacccttggttcaggtcggactgattcaacgctgagttcatatccagattgaacttctcggtgcgcttggcatcgttctggaactctgcgtgctgtgccttgacgaccatgttgttccactgctcatcgcctaacagagccttataggtcgtgtcagcgccatgcagcttaatggtcttgttctcaaggttcatcagcatctgtgcaccacccggacgctgtacgatgccaccgaggttagctgcaaccatctgtgttgcttcatcgtcagacggaatgataccagactctaaacccttcttaatgtacccatcgaagaagtctgcaccttgtggcgagcggagaacgttagggtccttcaaggccccgtcgagttccatcttcgtgttgagcatcgcacccttcttggcttggtcactcagaaacgaatcatgcgcaccgtacaactgaatgttacgctgggtgatgtcacttgagaaaccacgctggaagtccttatcggaatggtccagaccaaactggttggcgaactcaacgcttccatcctgaagacgcttgtggcgataatcttccatttcctgacgagtcttgaactcaccgcgttgcaccttctgtgcgacctcatcatcaagcaggaacgcagcgttacgcccggtcttctccttgagtgccttcatggcgtatgggtcatcttgatacagtaaggtcccgttctgcatagcctgacggcgttgctctggggtcaacttagagatgatttcattagagcgctcatcggcacgcttctgtgccatagcatcgtgttgcatgtatgcgtcagcaccaatctgagccatcttaccgacagtacccagaaggttactctttgattcatacgatgggtctacacctgcttgagcgaccccaacggtcatcgcaccagcgccacgaagacgctccatgccagccgcagggattccactcaaagctgctgagagtttactagccatgagtggcctccttatttattagctttcgctgagtctttattgattgcgctacgagccttgtcaccgtaaaccttctgacccacaacatctgtgagaccatagagtttcgagatgccgatacccagagggtcaacaatctgctccagtgcacccttcactttgccttcagacttctgcatctcctgaaccttgttgatggtatcagtgtgcgtccctagctgttgagcgaagatagccgcgtagtcgcgcttgtagttgtcccgaacaccattagcggcccggatgtaatcaccctcggtgacacgctgaatgcgttccattgagcgaccctcaaggttgccctctccgattgctgccgctacggttcccagagcctgcaccttctccattgatttcaacgagaggtcctgacttgctgagtccaaagtgtcctgagcctgaagtgacatattggcattgttgatgttcattgcgccaatcatgttaatcgcctgacgacgactctggtcattctgagcggctaccgcttggttgccctgagcgccactcattgcctgttgacctaccgccatcgcaataggaatagctgccatccagcacatagttaagtcctcttgattgtgaataattgaaactgcttactctcatcagagaactcatcgtggaacacagcgcctatcgtcttgagaaaccggatgtggtcagtgttgcctacccatacgaaattccacaggaccggataggtctgtaagagtttatcacgatgttctatgatgagttttctaaattgtatacgggattgtaccgtgattcttttaaggaactttgaggtgacgaaccaacattggtcgccatcattaccacctatagccatagcgtgaccgaagtgttcaatcataatgcattcactcgctggtggaaaggctggttgaataccatatgccttagcctcatcaaggtcctgctgtgacgggttgaactctttaaggtgtctttctgtagcaatcctgagtttcatgctttaagtccttcctagtgtggtctctcccgttagtgagtcttaatgcacccgagagagaccgttgagttaaatgcctgtgctacggcgaatatagttaccttcccatccgcaaccaatgattgacagtggggtcgtgtaatcgctcgtaatggtcaccacgttgtactgagcgttacctgcaagagggaatcggaactgtccagactccagaccagcagcgcccagcacggtatcacccatcggcttacctgtcatagcgtaacgataggctcggcccatgttggtcacgtccacgtagaacgccccagactgctcgtagttgacccacgcacggcggtgctgtaatcggcctacatcctcagtggagaacccaccggactcatcctgcttcttaatcaggaacttgctgaactcatagcggaactcacaggcgaacccaatgaatacctccatgccagccatgttgcctgtaatccgcagaaccgggtcagagttccatccgttggctggtggctcaaactggcgcacttcacctacagtgtcactcaccagaatcttaccgcgctgccaccgagtaccaccgaacacgttgttcaggttcactgtggtcatataggtgtcattgttgaatgcatcgccgggaatccggtactgagccttgcagtccatatagagtcggtaaggttccgtgttgaagtccagagtcttcttagtgaagctgattgaacccatccagatatccagaccgttctgcatgatgaggtgcatgtgggaaccaatagagttcgctgccagaatcttcacggtgttcccgaagtcccaatgtgaccacgactgctgctgaatctgctcatcaatgtagaggaacttgtagatgaacaccttgccgggtgcacctgctgacaggaccgaagcgaagttctcagtggacgaacccgcaatgctgaacactccgttcggaatgtagctcggaacgtgcatcgtcatatcctctgcgttcttcactgcgctcacatcctgaaccgcatagtaacggttgattgacgtaaaggtcgcacgaggactcgcaaagtacacaccacgtccaatcccataagggcgagcgccatcggacacatcgaactcagtcgtcaggttcagctccacggacttcgcagagagaacgcccgaagcattgagaacgaactgtgcctcatcggcccacagtaagagttcctcggagaacggtacagcgtacttcaggatggacacacggttgtgactcactgccacgtcgatagggtcatcgtcggacagcacagctacactcgcagggtacatattgaagtacttggcggtacggctcaggatgatattctcaccggacagtagacccagacggttacgatagaagaacacatcggtaatcgcttggcccacaaaggaagggtgggggttggtatcatcgtcaccagcggtacggtctgcccatgtgttaggcttgaagtcgaactgaccatcagcggcacggatgagtgaccaaggcatagtggagtcgttgagtccaacctgaatattccagcctacggtttcctcccagactttgcgggtcaggttgtagcgcacgtaatacttatcggctgaacgagaggtgtcacccacaatcttcacgatataaccatctggcgcattctgtggcaacttagcgaacgtctgcgcgtaatgggtcaccgggctgattagctggtcagcataaccatccttagtctgaaggtcaaggatattgtcagtgttaggcgcaatgatatgcacgaagcctgtaccaacgtttacggcccatcccggattacctgctagtgaagcgcgaatctgcttagctaactcttcagcgatgttctgagcatccacagcagcgacctgttcctcgataggtggcgaggtgccagtaccggaaggtaacttaatggttgcccgagttgagccattgaaggtcacactgagcgtgcgcccatactgaccaccacgaacattgataagagcatcgcgctggtcattgaaggtgccaccattggttaggttcccatcggcctgtacagccttctgacggttcacaacgaacgtgtagtccgcaacggtaacacaacggattgagtcgcgagggttcgctgagttcgcataactggtgtcgccacggacttggtattcataaccatccagaccgaacaccttaatggaacttccagtgaacacaacgtagtactgctcgacctcatcgcggttaatgagatgcacgagaggcgcttcccctaagtagccagcttggcccagcttacgggtgaacaccataggtggacgcttctggagaccctcagtttcagaggaccacccgttcacctgtgactccccttggtccgggaaccgtaggatgttgggctgctgtgagatgccgccctttaggttcttaatgctctggcttactaatcccattgtgcacctccagatatttaatcataccacgcagcttgtcgatacactcgccaacgttgcctatgaccatgttgcagttacggcagagaagctcacgcagcttgccagttgaatggttgtggtccacgcagagaacaccgaacttcgtgtcctcgtgtggtttggcgcagatagcgcacttgtagtcttgggccaccagaagggcctcatagtccagcaggctgataccatacttactcttgaggttctggtccttagtccagcgtttaccctctggagtagccctaaattccttagacccgattttcattgtggtcctccttagtttctattaacgggccagaataccctgtacgaatgcatcgccatccagcatgttaaacttgccgtaatccatctcgtactcgtggcactgcatgtaactctccgcttcctcttcagccagaatctgctcgatagaggtgtcaccgaagtaacgcatattgaactgacgggaagccttggtcacgatatactgacggaagcactgaggcatctcgctgtactctcgcaggcgcgtaaggttcacagagatagacccttggaacacatcggtcagaccagcagtatcatagacgtagccttgtcggttgatgtaggtgttcggtgagtccgctccctgcacacgcagataagacggaaggtatggaattaacccggtgttcacatcagggaccagtacggctccctcttcgatattgaaggtccagcctttcgattgaatcatgcggttcaccttagcgagaatctgttgagcgttcgccacgtcaacgttagcggagtcacccaaggtattgaccggggcctctccgatggacgacaggatgtcattgattgcatcaagttcgtctgctggatttaagaatgagtcagccatgatggcctcctttagtgttgaagcaaaaaacccctcacagtacccgaaggcaccgcaaggggtatcattatgttgtagccttaagcagactcaccgtccgcagcaagtttcgctgccttgttggctgcacgagtacgagcggctttctgcgctggagttaatgtggcttcatcatcaacgacctccgaagaggccatcaacgagttagtcattaagctcccgctttgaaaactaccgcacctgctgcttctggacgcagaccaccatgacccatcgcgtacttagcgataatctggtcagcctgatagtttgcacggcgtgcacgctccagagccaggtccttaagtttcacagtaccaacagccgaacggtgctggaacaggcccacaacgttagccagattgactttaccaccagttgccgggaaggcgtgcttctggttggtcgcagcttcaccatcttcaggacggtcatcaccagcaccaccagcagtcaggtgtggaacttcaaccacctcgaagcccattacgttacggatagaacctttctcagggtcaatcagcgcagcgtagttagcagcgttaggcatcagagccgccagaatcgcagagtagttatctggagtggtgtagaaggtacggtcgttcgcaggaacgtagttcttagtcagaccagcacgagccttggtcagagccgcgatgatttccttaccgagttcaacttggtcagtcagttcagcagcggtcttctgagtggtaatcaactgagcggcacccagacccttgatgttctcgttagaggcatccggcaggttaaccagaccagcaagttcagccagtactgcaccatcagcagccatcgccagagattcacccaactgtgaggtgtactcagagcgcacgtcatagtggttcatcgcgtcttcgatgtcgtaaatcagaacgtcagcagtcagcaggccatcaatgttaatggtcttctcagtgtgcttgatgtccttacgcttatcatcgaggttctcaccagcctgcaagtaagcagctttggtgcgaccgataaccgggaactgtgcggatttaccgcttgaaatggaacgcatcatgtgacgagaagtggtcaccgaggtgcgagcaaacgcagtcagtacttcaccaccaaacaccttcaggaacattgccagcttatctgctgcgctctgacctttaccctgattcgttcccaactgctgtccaccttgcatgttcgccatgatatataccttctgaattaaatttaaagttaagtttgagttagcccgtaacgtgggccaaacgtgctttgcaccaacgagtgaacaacctgactcccaatagggcgactatgcgttcatcactcaagttcaatcgttgagtatttcaaaccgggaacgtgtggtctcccgttagtgagtcttaattaaaagttgctcgcccagacacgctgttccaccgactggcggtaggcattatctgtacgatagcgactgtcactcatggccttcaccatttcgtcacgagaggcaaacccttcggcacgcttcggactagcaggtttagcttgagtggcctgtgtggtcacagtacgtgctgctcgcttaccaaacttagcgctgtaagattggcttgccagattcaggatggccttaacggtcggtaggtcgcgggtctccagcgctttcagcagtgactcagaggcttccttgttggaaacttcgaggtgcttctgtacgactgcaaacttatcgcgaccacctgcgtagtccataacctgattgacatactggtctaccagtgcttcctgacccttgatgtaagagtcaacgaaacctttagagtaaccagccgaagcgagagcctcgtatgatacatcagagataccatcttcttcgtactcagctttaatctgagcgacgacttcaggtgtcaaaccgcgttcagcagcctgtgcgaccatttcctcaaagccagcttcgtgctcgccaatgaggtcagcagatgaactcagctcgtccgggatgtcaccaactggtgcaatctcttcgtcgccttcctgttcaccttctgtgttaacttcttcaccttcgttggtgatttctacttcaggctcttcctgagtttcttccgaatcaccgtcagtgttgatgcgtacttgcatacgaccttcaccatcgtcctcttcggcaaacgggtcgcggtcctgaccgtaagggtcatcattgttggacaagtcaatgcggtcatcgccatcgcgggtttccacatccagactcaacatgttctgttcgtgctcttcttgagtcacgctaccaacaacggcgttagttacaccgaatgacgcataaacgtcagcattagattcagccatgatggcctccattgaaagttaaactaatcggggaaactctgtggtctcccgttagtgagtcttaattactgtgatacatccagacctgcattaccagcagcagccgccatagcttcaggagaagacgtagcgagtgcaccagcaccagcaccaccagatgccgcagcgttctgtgtagcggtctcagtagcgttctgtgccatgatagcttgcttctgttcctgagttaacaggatgccagacgtgtcgataccaatagcattcgcaatgcgcagcttaatgaccgcaatgttgatgtccgggtcttgtgccataggtgccagttggccccacgcagcgatacaccgttccaacttatcgaggtcttgaccacgaccaatcgcatccagaccggtactgatagtcggctcgacggcctccttcggtaactctgggatttgctgtgttgcctgcaactggttcaacagtacgcggacgagaggtaactgaagttcttgtgacagaatggagtagacaccaccgagggtatcttccaattccgaggccacataacgaatctcttcagccgttactcggtcaccagtacgttgcaccgctgagttcaacatgaacgcatacgataggcgtgcttcaatagctgtgctcactgcttgtgccacagagaaatctgcttgcttctccagttggaggaagtcaatgtcttctcgacggcccggtacgaagtcacccgtctgcgcctttgtgagacgacgaggctgagtgatacccgctgggttgaccaatccgattacctttgatgcaatcatgctcatcttgacgatagcttcttgcaggttctctaaggacttcaggtcacccagatactcctcaacgtatgaacgtccataggactcaccgtcgattcgcaccatgcgcacagggatgtacggacagcttgctcgtgggtactgagcgtctgacccggcaacttcggtctcttcgacttcttcgtacttgaagtaatcgccagagtcctcatccagatagacgtgagtgtacacatcaacaagttcatcaggtttcttctcgccacctgcggactccacttgggaccggacatcttctggtagtgcaccaaaagcaatctggtctcgggtcaccacttgcagcatattgccatacgcatcgcgttgcacaacataggccgacagtcggtagactttgagtggggtgtacccttccgggtccggcatgtgaagcaagacgttaccagcaacacaaagctgcttcagggcctcgaagagagacactcggtaactgtttgactcaatgaagttcatgatgatacgttcgaccatagacaggccttcgtccacctttgcgagtccatcagggtcggcaacaagttgcttcgcctcgtactcactaatggtcagcttcatccacgtctgcatcgggaacaacgccagcatcaacttggacgcaaggttattcagaccgcgagcgcccacggcttgccacggtgtggtgtagtcggtagacgagttatcggagtccttcgggaacagggacgggatggtatatgttgcacagttctcggcacgagtcgtatacggctgacggtcattgaccagacggtcatacacggccttagcgccttcctcagcgaatcctgtgcgtgcctgtgaggtagccataggtcacctccagttagacgttcagaccagcgcctgagttgcgtgagacggacagttggcgtttaccaccactgcgtgctttcttgcggtcaccctcggtctcagcacttgagtcctgctcggtgtcaaccttagcaatctcattctctggtgctaccggggcctcagcggctactggtgcctgtgcaggttgattgtccagaccagcgcccttagcgatagccttaagcggtgcgttagtcaccttcttaacggccttcttgattttcttaaacagtcccataattggctcctgcgaatttattacggatagatgtagacgcgctagttgacttctccacttggagagacttgcggccaccctttgacacatcgttgccagtggtatcagcttcgtcctgagaaccaccaaagtctacagaggttggctctgcggtcaatggggctggctcaggggccttcgctgtgtccacttgaggtgtcttaactttggctgagaagcacataaggttaaccctcttggttcatttccttccgtgtctccatctcatccagtacacttgaagccataccgaacccgtcaatgacacctaagatataggactcactgaacccgccagcacgtagcttcttgatgatacccgaatgatttagaaacgaatggttgaatgatgattgaagatattccttgactacacgaggtacatcaggaacgtcattgggattatctaacaggtgcttaatcggtttcaacatttgagtttcctcttagagtgtagctttaagttgtaatcaaataggacccttcccgttagtgagtcttaatgtactcacccgctgaaaggccctatgggaatcaactttctttcttgtactcagcaatctgtttgccagcagcagcaagggaccaaaggccccgagccaccatgccgaccatgagtaccacgagaactatcttcatggcttccacaggtaaatctccttgtcaatccagttgtaatcttcgtgacgaaggatgcgagccatctgtgcctgcttgattaaatcctcttcggacataccagctttcgcagcgatggacaccatgcactcccacagagacttatcgccctgctcacgcttgacccacttggtcacctcttgacccttgttcttaccggacttgaggatagacacctcggtctcagtgaagaacggagcctcaaggaagtccgcagcggtatcgccccagcccggtatgccaccgtagccatccgtaatgtcacccttgatggtctggaacatatgccagtaatcggcctgagacaaatcgtgagacagaatgttaccagttgtgcaccacaggaagtcacagtcagggatggtcttgaagtccttatcgcatgagaccagaacggctttacgataattgaacggtgccgggttagacccgatgatacccatcacgtcatcaccctcaagtgaatcttcacggatgctaatccattcctcatgagcaaacactcgctcaaggaacgcccggtaacctacaggtttacgagatgccttgcggttctccttataggttgggtccaccagcgtcttgcgccagttcaccgtgtccgtaaaggccagcacgatatcagcagttcgccacggtttcttgcgagaagcatacgacttcacggaatctacgaggataccccacgctttcgcatggtcgcactcaagggtccagtggtcatcgccccaatcggtttcaacctcggaggcgctcatcgcttggaaaaccagccagtcaccatcgagtaccagcacaccgggcgcaccctgcttgtctttgcggagggcttcgaacatcgccaatgttaagggtagcttattcattgactgcctccagacccgagaccatcgggaagtgacgctgtgcgaactcaagggccagagagttttcctctgcgttcaggtgtgccagcacgttgaagtaatccttacggaccttcggttccacctgcacgcgacgatagagttcaatctcatcgatagaatcccacccgtagttatacgagatggtcccattctgggtagccagacagcccttgtaggcgctcatcgtggggaacaaggcgattacctcatcgtcgatttcgattgaacgtgttgccgcacagtagtcgtgcttgaggaaatccccacgctccacctcggacacatcgtcgaagtaggacgcgaagtcctctggtagtttgatagtcatacgattgctccatgttcagaaaggaaagctgtaccggacgctgtgatttcccacgctccagcattacgacccgcaccagacaggcacgagatgtgaccacggcttgccgcctcagcaatcagagcggcgttgttacgcacgtagttactctgaaagctcttagggcaagacttaagggtcagcaggaccttgaggtattcgctcatgacaacaccacctgtgctggcgagaagcgacacagcttctgttcctcagagttcaggtcatcgtgcatctctttgataccctgacggagacctgtcttgatgcagaacttagcggctgcttccggtccaccctcaagggccacacggagaagctcacgcttgaatggcgagacggtctcacccttggcgacccggcgtgcaatgcttaggacggtatcatccagagccttctcgctcgctgagtcaatcacgtaggttacgccgaaagatactttacctttgaatatcatagccatgatttaattcctcttgtgcttgagcctgcgctctttgtttgtcttaatggtgtgctctgtaccgtcaatacactcaaggtgttctgggttgatacagccacgattaaggcataaatgattgacctcgtacccttcgggtattggtccattgtgttgttcccacacccagcggtggaacatgaaggagaacttctctcccttgcggtatgaacccatgctgtaccgaaagtaaccatcttggttcctcttatgagagaccgcaacgacacatccagtaggcatagtgtgcaaccggatagtcgctacctttcccataatgaatctccatcagtggcaaacggcccaattaggtccagtcttaccttccgtgtctaaacgacacctaaagttccaatgctcaccgacccagcgcatagcttcctgtgccaactcaatggcatgttcagcaatggcttgtgtccggcaggcaatctgtacttcatcgtgaatccatcccatgtaggcaaagtctccatcgaatccatgtttataaccagcagccagtaggcgcttctcaagttccacaatccacagtttacaaatcagtgcacccgcagattgaagcaatgagttcaatgcagcatgaggagaacgaacgtgaatacgacgaccatcaaggcccttaatccaacggcgtttccatgtgaccctctgttcaccaccgacccatgaggagtccttgatgagggtctgttggattccttcacgcaggttagcgattgctggtgtgttctcaaggaatttcttcttgagtaacttgccgcgctctttacccgccccaacgatttgaccaatcttctcatcgcctgctccatagaggaagccgtagataaacgtcttagcgttgtcacgagttggaagttcagcagcttgctgattgaccgtatgaatgtctccgttgagtataacgtctgcatactctccgttgtcgtaacgagacataaagtgcgcgaggcaccgcaactcaaggccactggcatcaatgcctgcttgaacccacggctctccagtaagtccgtcaagatgatgctctgctccaaaggcagcgcggcaaggttcaccgtaaggactgcgtgttcctgggacctgacccatgttagggaaactgtgggttgcacgtccagtgacggcaccattgggattgactgaaccatgaatctttccatcctctgcgatgtaacggagccacgctttgtcaccttctgccacctgtccgattcgtttctgaatcatcaggtactctttaatcaagtcgatgcaggcttgcttctctgggtctgctacacgaacatgttccagaacctcatcgtcaatcttaggagcgcccttatcggtgaactcagtagggacccagccagcttcctgtagcttcaactgaatgtggtcacgagatgaagggttgaacacaacgaactcaactggtgtgaacggagcgccctcaacgtaatctcgggtgtccagttcgcaaggttccagaccgagacgctgcgctttgttcttcggcttcttatagataccaccctgtttcgggaccttaatcagaggatacttagccagcggtctgccagtgcgcggatgcaggaacggagtgttgccacccttggccctgtaccacgtaccgaaagtatcactcagtctctgcttgagttctgaacggcgtgctgatagttcaacgtaaaggtcatttagcgcctgctcgtttacagggaaaccgttacgctccatcttggcgagcacccacgctgcctcgtgttccaataacacggactcaccacactccgaccagaactcagttgcagacaatgagtaccacggcttgccaatgtcaggaaagtaatgcttctgactgagacacgcttcgagtaactcacgggtaaccacaacgtcttggtcgttatattccatcatgggttcattgaagctgacccactcatcaccatcattgtagtcctcaccctgctcctcaagcatcttgatgaactcgtctttgtactcacccttcatctgaccgaggcggtagccccatgcttccagagcgtgagacccaaagcgacgaccgggcaacttgccggacttcaacaggcccacatctgaatccttgatgttcgcaaacagcaaacgaacgaggaccaatgtgtcaatcacgttacgcatcggtaagtggaactcacggttgagcaacagctttgccaatttggttaacgccggggcatcgtacttgtgaccgttgtggaatacaatcaggtcatcacgagccacagccgcttcaagtgaatcgaggtaagccgcaaagtcaccgggacgaaaccactcgttcgctggtgcacctatgcctgcttcgccaataactccacagtgaaacttggtgactttctccaacaggttgttggcttcaatatcggtgactagcatcataatgctttcctccagttaataaatgataatcataaaggccacccggaggcgaccttgagtctatcactcagctaaacttgacgctgaaaacagggcctgcaagtaatccttacggcgctgctcgtctttgccaatcgcgtgacttgctgctttacccagagccatcgacaggcgtgcaacttgtgcatcatccagtgtcatgcgttgggtgtggtcacgaccatccttagacttccagcggtagaccattgtggtcttgctgttgcgaacgttgatgtgaatacggcgagtccactggtcagcagtgtccggcatacgcagagttgtagtgtgcttaggcatggtgatactccttacttaaagaatttagaaagtgcttgcgcatcggtggcaactttagcggccttgttggtcgcatcgattgatgcctctttggcacggacatgtgctactgcgaactttgaagccagcaggtcttcggccttagccagtttgaccagagcctttgcttcacgctgatacgctttaacaaccagtgagcctacgaacttgatgaatttaaacatgatgtgttcctttggtttcgttgagagggaacggagtgtcccctatagtgggtattaattaaatctgttgctcgcctacagggcacccgcaggtgcacccttcgatatcgcacttagaaatctttgtcatcccaaccttgctctgcgctatcctctcctccgctgcccgtaatgatgctagtcggtttgagccagcccgtgagcttgtcgtaagccatgtgtccagcgataccagtatcaccagtaaacctacacttgagaagacgaagctggacaacattagggctatccccttgctggtcgcgctccaatgcgataatagtatcagacagttgacggagtgcaccactaccacgtaggtcagtaatgctaacaggacgcccttcttcatgtgcttttcctttctctgggttcttaaggtgacaaatcacaaccactacgcagcctttcgatttcgcgaaggacttcaacttggtcatcaatctgtcaatcattttgcgttcgtcggactcctcagagccagacactacgattgagatgtggtccagtaagattaccttacagcccagaccgtcaaccatgtaagccatcttagcgaacagcctgtcctcctgtgactccgcaaaggaatcatagaggtggaacatatcgctatcgaacagtgcatcgtaccacgaatcgaatcgaccatcagccagaatctgctcgcgcatctctttgttctgacggagacggacgttgttgtccaagcccatgaggtcctcaacggtttcctcaacggactcctccagtgcacacaggccgaccttgataccctcacggccccactgtaacatctgttgtctggcgaacgttgacttacccataccggacccggatgtaatcatgatgacttcacctaagcgagcacccagagtcaggtcattcagcgcgggattcccggtgaacaatagcccgacctctttggctgtctgcatggcttcacgcacacggtccttaaggctaatcgctgagactacaccatcaggaacccacggtgctgcattccaaatctggtccatcagtgccttctggttaccgttgagcatacactcattggcatccttgtcgggcaacactgcgaccctgaccttcccgctcggtagcactggcgcacactcttcaatcgctattcgacccggctcatccatatcgaacatcaggataatctcatcgaactggtcgaagtaatcgaagttcgcagccagagttttcttagcggcctttgagccatgacctatcgacaccacagggtacttacagtcctgtagttccatcacggtcagcatatcaatctcaccctcggtgacgacaatcttcttaccgccattccaaaggtgcttaccgaagagggcgtcaggtttatgcgctccagcggtcttgaagtttttatctttatcgcgaatcttttgggacacgatagagccattctggtcacgatagtcagccacttggaacaactgaccgttgaccttagcaacccaatacccagctttgcggcaggtctcttccgagatgcctcgcttggtcagcgcagtgtagcgcccgttgctgtctccgaagttccatacggaaccgctgccaccttcacgcatacttcctcctgaacgtcctcttgatgataacttagccttggcctgttcatctcccggcttccacgcttcacacacgtagcagtactggtgaccgtcagagaacaatgagttaccatcagacgacccacagctctcgcacggaatatgatacaggaagatactgtcttgaccatcctcttgtgaatcaccatagctcatacggttattccttaatcaatttgcgattgaacagagagagaccgttgtggtctcccgttagtgagttctattactttgcagtgaccagctcgttagtcttgagccagcgctgtacgtcgaacgatgggcaagccttagcggcgaactctcggtgaccgtgaatggtcgcgtccgggtattccaccttgaggccagccagtacatctttcagtgactgcatctgctgaggcgtgaagttcgcttgaggtttcccgcttgcgtcaacaccgcctaccagacacacaccgacagacgtatagttcttaccttcgcagtgtgcacctaccgcaccaacgtcacgaccatcttcaatggttccatcgcggcgaatgatgaagtgataccctacgtccagccagcccttctctttgtgccactgacgaatctctcgcagaccaatgttcatacttggcggggttgccgcacagtgaacgattaacagcgtggtctcgttgcgctgcttgaattgtaccttagccattatttttgactcccttagctttgaacttatcgaacggtacggaccgcttaggttccttaagccaatcgataggaattaatttgtcagcgaacttgatgccatgcttctcgcaccactcaccgtaactggtcgggctacccttgtaaatcttagagcggctcgaactgaacacgatgcggatgtcaagctctggatactgttcgcgaatcaataggtgtttctttcggtcatcactatcccacaaccctttggtctcaatgaagattccattaggcaacaggaagtccggggtgtacttatggttactcgccgggatgacgtaagggattgaccactgttcgtaatcgaaagggattcccttaccctcaagctgctttgagactttatcctcaaggccagagcggaaagccccgacctttcggacaccacgcgcagcgtatgcgccagccattagaagtcttcgtcgtcttctacaggctcattaggttcaccttcgttggcgttccatgagtcaccctgaggtgcggcctgacgctggtcagaggaagtaacgtaaccaccttcaacggtctcatcgccccaatcgtcaccaccaccagcgccgaactcaacgaggtcaatcaacatgacaccttcgagttgcagcttgacggaagcgccagcgacctgtgaccagccataaggaatcagcgagaacttcagcttcagcttggaaccaccagagatggcaggaacctgacggattcgaacacccttggcatcaacaacagccagctcaatcggacggttctcaccagttttcttatcggtgaacgagccgtagcatttgaagttgaacgtcacggtgccatcaccattatcgaagaacggcaggtcaccctgatacggcagcagtggtttcttaccgcgtgccacctgaggtgggttctcttcgtgtgcagccagacgttccgcgtagtcagcctctgcggtctcagtgatgaggttcatcatctggacagccttagggtcatcaatcggacaggtcagcgacaccttgtacacaccgcgttcattcttaaagtcaccgtgaccgtagtcaggtttctgtaagtagcagtaaggttcagcggtgccgagagcggagactaagattttacgtttagtgaatgccatgatatgtaccttctaaagtttgattgaatagatgtgaaagttgggaaaccgttatggtctcccgttagtgagtcttattaactcttcaggtgtggacggacgcgggtgaccgcgaagccagccgggacatattctgcctcagctttctcgttggcctcctccagtgtctctgcgtaaacagggacctcgaaggtgtgcgtctgggtctccacctcagcgatgaagcgtttcattttagcttacctttccagtgctccagtagctcaagataattcttagcgtcctgaatgttgtaatcgtccagtgcctcgcggagtttcgctatgcaccactctacctgttccattaggtgccagccttagactgctcgaccagtcgcttaccgaagaactcaaccttctcagcatcatacaggccatcgtcctttgcgccagccttgcggagacccagagttctctgagcggctcgacgccacagcgccttgaacgcattgccttccgcaaagttcatacccaatgcttcgatgatatcgttacactcagcggtgtaaggcatagcgtatggagtggttgtcttggcgatggtcaccttgtagtaatcagatgagccaccagtgtagatggaaccagtgtcatcagcagaacgctgacagccagccacgttgtccacctcagccgtaaccttacctttcacagggaccgggacagccatcgcacagcggcagtcatcgaaacgttcacgacattgacggcattcataatgtgacattagaacacctccttgatgcgctcaatgaacagacgaacacgcgggaacttagtgtgcacaaccagcggggccgggcgggtgcccttctgtgcctcaacgaagacaccacgagggatgatagcgtgaacgctggcaccgaggtcgaaggtcagtccgatgaaaggcaacgtgcgatacactgaacgctttgctgttgctgttaaggtggaacggtctgcgctacgaagcgagaagataccgtttgatttgttgtggtgcagacggatagtcatggtcagtctcctactacagttgagttgtcagcaccagccgaagggccgggcatgttgtcatcgatagccatcaggatgaaggttgcgacgattgcgaacagaaagattaacatacagttatcctcgtgttgataaagtgtgggacctaccgaagccatgctgtgatggtcaagagcggtagtgtgttcccgttagtgagtcttaatctaaatcgcagtcagtccagaccattgagcctatcgctaggcccgctatgaatgctgccagaatccagaatgctgcgcaccagatgtcaatagtatgcatgaggtttctcctcctgatagaacgacgaaaggcccacccgcgaaggtgagccacgctgtgattacatcttggtgaatgggtccgactcggtgcctcggaacttctcgaagctcgggtgacgcagtgagccgtccggggtctcttccatgtagttcacctgacaggcgtaacccatgtagaaatcacggtcagttaccacgttggctgtgaattcatccatcaggacccgcgagatgttcgtggcgttgaccactcgaccgctctctaagagaacctcgaagccaatcaccttgccctcgttagcgagaccttcagtaccccagaccagaccaacgatttcaccgtcagcctcgccctcaggtttaagtttgaaccagccggacttcttgccgcgcttgtagtgcaccagtgggtccttgatgatgagaccttcctgaccatcttcgcgggcctgcttgaacagcggggccagttcgtcgaagtcaaacacgtcttgactgtgggtcatcttccagtcaatcgttgggtacttgtcacgcaggatagccacagcgttagccacatggtactgcatcagcgcggagtcaacagggtaatccttgccggactcgaccgcatcaatgggcaggacagcaatcacgcgggcctcaacgaactcagggtccagcatgaagggaaccttacgtgatttcttcgtggtctcctcagcgtctgggttgcagttgaacgcatagttcttcgtgtcactgtgtgctgtacgcagcaggccggacccggtgttgaagtctacacccttaacgaggaactcacagtcaatcatgaagccatccttaaagggctggcggtcatcggtcagtagctggtgggctggtagtgccacgccgtctaaccaattgagtgccgggatggtcttacccacacgagacaggaaggtcaggccaccgggctggaccaaaacgttaccgcgaacgccatcatacttggtctcgacaatgagcgagccagcggctgcgagtgctttacggattgctttctcgttgaagctgactgctttgaatggattggttttcatggttggttaccttttaatcagaatgtgattgaacagagagaccgttgtggtctcccgttagtgagttctattagtgccacgttcggtaatcgttgaactgcttattcagccacgttgccacggtcacgcagaacacatcaccatgatggatgccggggtacatagtgaagtcccgctcgaagaacacagagttgttcttgtggtccatcagtctcacgttgacctgcatacgcggcagacccatatcgaaacgctcactgagtagaatcaccgggcgaatatccagaccacgccagcggtcctctgcgttgcgtaaggtgttcaggttgccactgtggcagcggtcaaatagttgacgctctaacgaatagtgaatcatggtgcaatcctctcgtgtttgaaatgataatcatgaaggcctccacatgggcgaccttgagtctatcacttatcggcggttccacttctggcgtctctcgaaggccaactggtcgcgcatctgttcggcgtacttggtccccggttcaatgctcactgtttcataacactcctgcacccggcccacgatgtcggtcaacttgtaagtgaacgtcttgtgtgagtggtcagtgtgggtctgcttgattatgaactcgccctcggtgcgtttcaattcgaggcgctcgacagtcttaccgcagcgggccggacccagcgtgaactcgctggttctcatgtgaccctcgggcatgatgcaggtaaacgacaacttggtcaacgccttggtgaccagtggtgcactcagtgattccaagcgtctgaacattgacgactggtcttctcgcaactggttgttgtccttaagtgccacatcacggtgtgtggtgactcgctctaattgacgctcaagttcagcgatacgggaatctttcaggcaaggcgctttgcggaacaggtcgaataagctcatgatgtttctctctttaagttaatcattaagttactgaaatctttaggttttaacttagagtctcttaaggtttcctctaagtgttgtctctttccgttagtgagtcttaatgcaatcgcctatcaagcgaacgcaaagtctgacttcagaatctcttgcaggtcaaggccgcccatcgccggaatctctggcatcttctccagttgtgactcgtgtaactggtccatgaactgctcgcggaactcttccagaacgttgctgttctcataggtctcaacgattgactcgcggaccgccttgaagagtgcgcctgcgtctgccgggttcgtcccgaagctgtcatgaatcaacgcgaagctggtcacaccgtacttctcataggcgtggaccacagtcttacgcaagtgtgacccatcctgactatgcacaaagttaggtgcgatgcctgactcctgcttatgtgcgtcaatgccgctggtcttgtgcgtgttgatggtaggctggatgcggaactgaccgaggaacatcaggttcaaacgggtctgaactggtacgcgatactcctgccacaccgggaagccatctggtgtcacccaatgtacagcgcaacgaccgcgcaacactgtgtcagtcttcttgtccttcacctcagcagccaacagtttagccgcagacttcagccaattcatggcctcaaccgctgccaccaccgtgacactcactgcattccagatgagtttagccatatatccagcagcctgattagcattcaggaacatatcgcccttaccgttgtcaatcgctggttgaatcgtatcgcttaacacttggtccctgaagccgaactccttcgagccgtaggccagagtcattacggaacgcttagtcaccccacggttgaccccatgctccagccaccattgggccatcaccttggtgccatacttggtacgctctgtaatctcgcccgtcttcttatcggtgaccgtttcgagcatcgtgctagtcccattaatcaggtcctgcttgagcacctcgttgaccttatcggacacaatgcggtagatgtcctgcacttcagcagaaggtaacaggttcacagccttgccgcctaccgcatcacgcagcatcgcagagaagtgctgaatgcctgagcacgaaccatcgaacgccagtggtaatgaacagttgtaagacaagccgtgattgaccacgcctgcatactcgaagcagaacgcgaggaaacagaaaggtgaatcctgttcagcccaccatgtgctctcaagcggtgcctttgcgcactccatgatgttcgtgtggttgtcctcaatgaacttgatgcgctgtgggaacgggaccttatcgacacccgctgtgttagcgccgtgcaccttcagccagtagaaaccatcctcaccgattggcttaccttgggcgaaagtcaataggcccttggtcatatcgttgccttgcgggttgaacatcgggaccgcgtagactcgaccgcgccaatccatattctgagggaaccaaatcgccttgtagtttgcaaacttattggcctgcgacaacatgaattccattgacaagcggcgtgacactcgggccttgtccttacggtagaacgctgaggcttctttcttccatgccttaagtgctgcctcgttggtatcaatatcgaacggacgttcaggcatctcgccacggtccatcgccgggacatcctcaaccgggcaatgctgccactgagtaatcgcgttggctacatcaaggaccttcttgttaacgcgccatgcggtattctgagcgatgttgaccgccttgattacctcaggcatagacacctcttcatagcggcgcagagcggctaacgtgcgggtccttaccagttgcaggggcttacgaccagcggcccaataaccaccacccacagcttcagtccaaggcttcggagggacaacacacggttgatacattggggcaatccctgccagtgcacccgctcgcttgctcaatgcgtccgcgtactccttagtgagtcttacggtttcgacatccttcgccgcgttgcctgcgtgtaagcgctccagctccaccagaccagtggactcaatcagcagctctaacatgcgaatgcctgtgttaatggtctcctctttggtccagcgggtccacgtatcctctggcttcaggattcctttctctaacatcttgccctcaatgacctgcatgaaagccttcttatacacctgccccttgcgctggttcagggccttctctacgcgctccttgtagaacttctgctcttggtcccggatgcgtccgaatcgcaactcgtcctcaatggtcatcccaatgttgttgacaacctgagtgaccggacactgcacatccttcgcgagagtcgccagtgcacacttgagggtaatcgctgcggctgactcagcgctcagtccttgcgtcatgttgtaggctactggcttgcggcccttggctgctcgtgcctgctcgtgccattcagtgtacgctgtggcaaacttagggtgcagtgcggacatcaacggctttgctactgcgttatcaccgaactcacccgcttcaatctggcgattcatggccttgatgaaacgcttctcaccttcagtgtacgcttcgtgctcaagttgtaactgagtggctgcgatgcgctcgccgtagttgtctgccagaatgttgaacgggatagctgcgtgttcaatctcagagaagtcctgctttggtgcgttgattacgttggtcattgtgtgcctcattgtgattaaagttttatctattggtgccgccaccttcagacgacacctaagatactactagccccgcagtcgagcgtcaagctccctgtctatccgcaatggttgattcatcaggtgatgcaattggtgctcccttacgcggtcctttaggttgatgcgtgcctgctccagtagactctcacggaccaccagcatcccctcaggcgcttcccacttgaacctgtcggctggcttgcactcgcggtgcttaatgaatctcatctggtgctcagcgtccatcgcatgaatcatgttagcgttgccgccaaacatttgagcgaagcgtgccaccttcccgatgtgtttcagctcatccaaatcaatgttgtcgaggatgttctttccgtgcaccttcggcgctgactgctctggcttcttaccaatcatccggttaactctcagggtcgaggcccggagtggggccatctcctccacattcaggcgctcaatttcaccgcagattgcctcaaagtccacatcttccaagcggttatcagtatatgataccgggtcagtgatgaccagacgaccgtacttgtcaaccattacattaccacgatgcgcatcgaatgaccccacgccatagaagaacttgcggatgccctttgcggtgtgaacaagattgcgctggtactcgttcagggtttcccacactgctggtgcttcccacaagtgcacctcaccatagttaatgatgccccgcacgatttcaaactgcttatccagctcctcagtgcttacagcgtcttgacctgcctcacggaaacaacccgcgaccagctcatccagtaccacgctgtaacagctcttatggcgtgccaaatcgtggatgacaggtaacccaacagttgcaccttgcgagcggcagtaggctgcataggccgcgcctgagtcctctttcttaaagcctatcttaatgaccttgcccggtaacatctcatgcttgaacgttgcggagaaataaccagcgcccaagaacttgtaacctgcatcgcctgccatctctttaagcaactgccagtagtcctgacgctcaacgcccacagccgccgaggtctcgttgccaccgtccgtacagtgattcacgatgtccaccagcagacccaccatcattggctggcgtaatgctagctgtgcgatgggtaactccttgattgacaccagacggttagtgatacgtgccagcattgtcaagtggttagtggtgacggtattgttcattaagatattccttatgggatgattagattgatttcacagattgattacttgatgattaccattgggcctgcgagtgtgaactcagcccacttgatggcgcttgccgcttgccttgcggtcatcttacggccctgcataatgacccgttttgctttacgcttactggtaccatacgccatcatgtacagtgcctgcttaacgtgtttccattcagtgcgttgcaacataccagaaccctaccttgttggccttaaagcgaccgttgcgttcccttacagtgaagcgaggtaatacaccccactgccagtaggccagagtcgccttgtggtgcacaactcctcgcctaaagtctctcgcaatgtacgcaaatatgcaagcgtacacagtcaggatgaatagcagcattagttatccttgcgtgccttgttgtccttgatgatttcccacactaccagagccacaaggccccagcaggtgataccataaatccagccttgtgcatccattagcgaacctcccagacctgcgcaccgcgctccactgagtagcactcaccgattgctacatccactgctgtgtacacgccgatggtctcacgactacgattgattacacggtaagctgtcaagtacacatagaattgattggctggctgtttagtatgaatcattgcgtttcaccttataggctacaccctgcgtatcagagcgtttcacataaggccctcatgctacgaggacactatgtacaccttgtggtgtcacgccttgtgggcatccagattgtgtaaagagcggttcgcgttgttgctgcgagttggtatagcttaaagcgttgttcccgctgagtcaagcattttcgtatgtccgcttgatgactacttgtcaacgctgggtcgtcagaggcggtaactcgtagtctgccgcttgacttgttgacccgttgttgtctcaactggcaactattaaaacataacgattatgaggagtcaacacttgttatcaaaataatgttggatgttctcactatgagtcatccactcaaggttagccctatggttattcagcttgtcgccgtctttatggttaaccagtggtgctccctctctggctggatgataccagaggcaaacgaggcggtgaacgctgtggagcactgaccgaccgttaaggcgcagattgacaaccttatagccgtggttacctatcgcagcctttaagacacggtacgctctccctttgaggcttatcacatcgccacactctgagaccgtgtagccgttctctttaagtgtctctatgtctattggtttagtaatatggttattcatctcttaatcctcttatagttaatctctcctgatagtgagtcttaatagacagtagttgacaatgaccagccattagccctatagtgatggctcacaggtaatctatgagagacagcgactctctgataacacgctaagaagtgatcctatgtgtctctcccttaactgagactgctaaatgataaggaactgtgagcggtaacgatagcagcacattaggatgctggtcattaagagtcattaggtattgactcaaggtgtaacattaggatagtgtaaccactcagggaacacattaggaggtaactcaatgagcattaaacagatagagacacacagaggcccacatatagtatcccttaggtcccacacaccactagatgtagacattgggtccactcaaggtggcattgaaagggaaccataggggtaaccccaccctttgggtgaacgttaggagggcctatgggggtactttgggtgtttactctatgagatactcacaggaatttttgtggtatattcttaaagggtctcattaggttccatcattaggttaccgacatcattaggtgagaccttgagagaccataagacactggatgaccagatacttaaagtgcactcaaggcccttgtgttataggttaactgtagcgatgatgataatcaagcggtagttaacctggtgtccatcttagcgcagcgaagcgttaatcgctacaagtaaccacagagcaaacgagaacttccagttgaccgagttggtcagcatagtgtgcagcgccaaaggccccagcagcaacaatgagaaatcgccatgtaactctgcggcctagtagtttcaatagggtagccatgagttacatcctcctgtggctgttagtgtatggtgatgatatgattaatatcacctctctgtaaggataaacttatagtcactcaaagtgcataaagggactataagtgtattcattcagtatctatatagtgctcttaggggtctctctcccgatagtgagtcttaatgcgaacctgttgatttcattaggttttctccatgagggactatccgtgtccctatgcgtacttatgcaatccttatgcatagacattcagtattaccattcgatgaaccgttcgccgctctcatcatcctcgtagtagatgtcgattgcgcctacagccatcttacggattccatcaccgcccatcacctcacgctccatatgtgcctcaaggaactcagcgaccatctctgattcgccttgtgcgctatccagcatcatcccttgacgaaggaactcaacgcccaacgccaacgcatctaagcggtcatcgtggcgcacagcacccttctcgcgggtcatgcgggtcatctggtagaacagtgagtaaaccactgagtgcttaccgtctttgtctcgggcagtctggtaatcttctctgacaacctcatcacgtacaatcaagcggtgagtagacatcacaggctcaagtgtatcgcagatgcggagttccttcataccacgagcacgaatctcttcaagtgctgccttgtggtgtttcaggaggataggctggaagattttaccgaacataccgtcaccgaagttactctcgaagacaactgtttgcacgtcccactgcttggccttcttagccagcttctcaagggtcggctcggagtacccatcaaggaatcctccagtgtccatcaagtagatataaccattcagtgtgtacagtacgacaaacgtggtttcatccgtaccgcgaccagaggggtcaatgaccataatcttctgctggaactctccggtgcgctctgacgctgtgtgatacgaatggatgtcatcacccttaaggcccacgttaggtaggtcctcgttgcggttctgacggttaggcaaccactggtaactcaaggctgcacgcgctgtatcaatagcagcaacgataaggtccttaaggcgcagtgggtacttctcagcatcggataggttagggttcaacatgaactgcaaggtataaccagctttaccatactcaagctcacgctcacgtaggtcatccgcatcgaatcgaacggcgtcagttggttgtcctgcaagtccttccacttcctcctcgaactcctgtcgaagcatcggggctagacgggaaccataatacatatcctcttgcttgtttcgcggatactgggcgggccagatgattgtggtgtacccacggttatcctcaagctccttgtagagtgtcatctccgtctgaggcgtaccaagatagattacacgagatgtcggcagaggctttaacagagcggcaaactcttgcacaagcgtccacagcttctcgcgtgcaccttgggtggcactgttcgacggaatctctacgtcatccgcaatgatgatatcagcacggctaccagtcaactgaccagtgatacccacagacttcacagacggtgagtggtcaggcttggcagggccaacatcgaaactaatcacagagtccctctggtccggtcccggctttaactcagcaaggaatggcagaaggccgatgatgttcttgatgaatattgagttcgcatccgcacgttccttagaggccgatacgatgagaatcttcagttgagggtcacgccatagagtccacacaacgaacgcacaagtgatgaaggacttgccgataccacggaacgcttgcaggatgaacttcttgttgtcgccgttagcgaggcatttagccatatcaatctggcatcgggttggtggcggcaggttcagagccttccataagacgaacaggaaggccacgaagtcattctttagctgcgccacaatgagcgcattacgcgcccgctgtgtgttatccatgatgttactccttatgctttcattactttaccagtggtcagcgcatcgagtgtgccgttgaagcctgtcagcaggttgctgttggtactgcgtacagccatagacgaatcaatcaagtcattcagcttggtcactacctgctccagcgttgcacctgct

SEQ ID NO: 3 - DNA, 242924 bp, Erwinia amylovora bacteriophage Ea PF 3 DSM 34960
  source 1..242924: mol_type = genomic DNA
gcwtarsgccccggggtttccccgctttaaccgcatcgtaaagattttgtcgcagagactaaaaaaaaaccgccaaagcagccccccgcggaaaaaaaaaaaaaaaagggggggggggaggaggtttggccccccccccagcacgccgttaagcgttgaagtgcaagaacatggtaccggtgaagttagagcatttggtgtcgtccagctccagcagcataacgtggctgtagctctggttcgcaccttcgactggcactttcggatcggtaccggtagcggtgccgtcgtcgtcggtcagaccaacgtatttcacgtccgcccctttcaggttgtagtctttcagggcgtcttctgaaatccacagctctggcacgactttgttcagctcaaccgcaaacgcggtatcgttcgccagtacacccggcgcttgcgcgttcaggaacttggcaattggggaacagtctacgccgtaggagtagatgtacgcctgacctttgccgtctttcggctcgtctgggtacttcagaccatccagctgcgtctgcgtgatgacgaggctcagacgttcaccgacctgtggcttcgcaccgatttttaccgggatgttaccgagataagcgtagcagtcgtctttgaactgcacgacgtggtcaaccgggattgggtctggatcatccggatcagtcagcgcggggttggtaccgtctggaatgctcgccgggatgatgtcatcttcggtgattttcaggccgtactgctcgttcagtttgctcagcagatcaacggtggttttcggctctttgacgtccagatacgcggtcacgttcaggaacaggttttcaccgaccagacggtcataggtgacatcctgcgtaccgatataacccgagttcttacgcgccttcacggtcatacgggtgttgcggtctgctttgtcgtcaccttcgttcacagcaggaacgttcagaacgactttagtcagaggcaggttcgcctgcgggtttttctcgttgatgagatccagaaccagaaggtcggaggttttgtttaaaggtttcattctaacgtcctttaggaggcttattcagggtcgttgtagtggatgtacatacgcccaccgagattgatgcaatacaacgagagttcgataaccagcacgttgtcgtacgacgggttcgttgggtaagcggcactgtttctgccgttgtaggcaatggtcgcttccttcaggttatactcaatcgggttacggtagacaatccagccgtcaccggtcaccgttttcaggatttgcgccatacgggtacgaaacgcgtcagtggcattgatgccaaatttgcgcaactcttccgcgtaatcgtcaaatcgccacgggtagctgtacaccgccccttgtccgaccttggtgttgaaatacggataggagtacggcttcaatgtgtcggcgtcaaagttactcgggattaaagcatcgccgggggtaagcttcacatccaactcaccaatccaccctaaagaatcaggattagctaccagcttaacgacccatgcactccggtcgatatcggtacgggcgacatcagacgtgcgcagcttcaaaccgtaatactggttaatgagtggcacgatgtcgtgggatgtaaacaccgcatccaaacgggcaggaacaacgaggggctgtacgccatctaatccggtgaacatgtcatcgaaggcaaggcggtcgtaaaacaccacggtgtgacccactgcattggcaagcgctgtcgcagtgacccgcaccattgcgttgtgtccgttggcgagggtaacatcttccggctctgtcggtatctggggtaccccaaagacaacgtcagtttctttcaggtcgagtttgttctcgacattcagctccgccagaatgagctgctccgcggtggctaagataggcatgcggcacccttatactggttggaagtgaaggatgaggttgcccgtatagttgctgtctgtatccaactggataatgccgacgcgcgcatacgcgttgtcgtacatgtctttcccggtcggtgtaaccagccctttatacacggcaccaaacagcccgatttgacccggcttcacactggcactcggcgcatagacaaaattcagcggcactacttcgtttaacaggtcgacatccgcagcagttaacgctcgattgtacgcccagtctttcgtcaaggtgtctttgatttctgtccagtcgtaaccgtaggtcacgtactctgcctgaggcttagggccaagggtgaacggtgcaatgatgacactaaggtcaacgtccgtcaccacgtcacgcaggttaggaacgaacttcgcaaaccggagtgtgaacccgccctgccaagccaaacagccagttttgactgccacgtcgagcacccaactttcgcccaagtctttcacagactggtcgacgatgtcgtcaggaatcaacgaaaggccatacttctcattcagaaacggcaacagttcggagagcttaccaacagggtcagtaatcaccaccggcaccacaccgcggaacaacgtcggcatatcgatacggtcgtattcaatcgtgacgttgcctttatatccctgtccgtttaagccgtacagtaaaacacgcgtgttccgttgcgcgccttcagactggacgacttcgggaaaaccggacgcaatttggttccatgtcagggctttgctccccgacagaccattatcccggttaatcgcctctaacaacatttcccgtgagggcttatcgtagatagacacttataccccctagttgttaaagtacaggttcagcgtaccctggaagtttgtacagagtgggcttagctctaaccctaagacgtaatcaaacgccgggttagcaccgaccactttggcggtttctttgtaatacaagtaacccgcctgttgaaggttgtaaggtaccttatcgtttgttccgacccacaattccggcaccaccgttgagaacgctttcgcaaaagcggccatgtcggcattaccggcttgcagtgatggaatccacgatttaagcgaggatgcatcaacgtcatacgagtagagtgaggcttgacccacactcacgtcttggtggtcagggtaaagcaaaccatccaactgcgtatttggtatcacatcggctaacggcaccccaacgacgatattaagggtaacctgcccacgccattcatgggagagcgcttctgcaatgacagtgtgcgcattccctgagacgggcaagtcttccaagtcgtccggaagcagattcaagccgtagcgttgattaagcgcaggaataaagtcgtgtgtcgtaaacacatcttctctatcgaacgtcacatcgcccagtatatagtcgggtaagtcacggcggtgataaaacacctccatttgctcacccgcgtcgcccgataactttgaggtcagaattaccctcgagtcacgaccgtcgactgaaaccacctccggcagagagatatcaacatcatcgaacgtcagctccggggagattttgttctctttgttgatgagttttagcagattctgtttggatttaaaagacatcgcgttaactcggttgtaaggtttacaaaggcccgcgttaccgcaataacgtagaccccctgccagcataataatggtgccgtttgtcatgacaaaaaaagaaagagaagtggggcaccgaagtgccccacgtaaatcaattactcggtagactggtttccaccttgatgtagccttgcgtcacacgctccgttaccgggtcagtgaccttaaccggcaggtagccgttggttaacgcaaaccgcaggagtaactccccgttgccgttccaaccgataccgttcttggcaccaaaactcatgcccgtcaccgcatcgagaattccctcaacggctttcacttcatcgagtgtcatcagtttaccgtcaaactgaacatcgaacggtgtacccgattcaaagcgagacttcgaggtaacttgcacaaacggtgagacgtaacgtgtccagtcgaacaactccacataaatcgtggagttgttcttgaacggcttggtgaacttgacgctcttaaccggacacgcgccttcaccatcccactgcacatccacgtaaccggatgacaccgttttgatactgatggtgccagaaccgtgtgctgaccctgcgccacctacacgaccttcgctggcattaacagagttataaccgcgtgtaccttgcagttgaatctgcacgttctcacctacgccggtcatgcgaacggtgcctaagcagaaccactgactaccggcacggttgttatccagacggaaagcaggcgctgtgtagttcgcagtaaaggaaccgttggcaacgatgccgtggtactctaactgcaagtcccctttctcatagcctgacaggcccggccagttagaggcaccggtacctttatcaaacccgctggttccttgcaggttaatgtggcggcgtgttaagcgggcattctggattaacatcttgcccgagtcttcaatcgagaagttatcaatcgtccaatggccgtcggaaaggtcacctggattctcagtgtgttcaatccaaccgttggtgatttgtgactgcgtagcgcgcggtaaatctaacgcatgtggacccgtacaactctggatgttgaagttgcacagttcaatggcggtttcgtgatcccacacaccccatgactgtccagaccaacgtccttgaataaagctgttggtgtgtttagacacgtagaactggtcgaatttggtgtctagcgcatcaaggatgctaaaagacacaccacccacgtaggaactcgtccagttactcacacggaaatactggccacccggacaagtgttacgcaggaaacctaaggtacctgcaactttcttgtcattcgctgctgtgatatccaccgcgccttcgaagttcagattcgaaatcgcagtacggcgagcgacgatgtcaaagataaaaccgtcttcggtgttgttgccgtataacgtggtgccggtgaagtaaccgaagtctgcttcaatcggtgcacccgccacacgaaaacgggacatctctttcgtgttggtaaaacgtgacaacttaaaggtaccggtcggatactgcacgcccatacccggaatgttcttttgggagaaagccatcatcttcgcaaaggcttctgcggtatcgacgccttttccttctgcaccgaagtgacacacgttcaattcatgcagggagttcagtgcacgcttccaacgggcaccttttggggtgacaacacaataaccaccatcgtccggtgaagatgtatcggtatcgtcgtgaataaagaagcctccaccaaagccggagccttgacggtactctttcaaatccatacgttggccagggaagaccggttcgcttgcgcgtaatgcgccaatcgatgcacaacggtcagaggcagaagcagaaataaccatggtgcatgttcctcaattaagtgaaggggtgaagtccatagcatcttgccgtttatcccgcaagaaaaaagaagagtgtgccaaccacgggcaaaatcaaaaaaaaaataaatgacacgtacgcctcagctgacccccggtttcccgagagtcagcgtattggttgtcgcatcatttacccttagcacatgaacagcatggtgcttttcattttgccgtcagacttacggtcataaacagcttcgactttgttgaccatagggtcgccctttttcatctcagccattaccgcagacagctcatcgccgttcagtttcagcagcaggtccagcatgtcttctttcttgccagcaggtttaacagtttcaacgatagctttgttagtagtgaataagttgcgcatggtgattctccagtatttatattttaagaatgaattagataacccctgcccgattaggcaggggtgtgttgtttagaacagttcagttttcgctttgtccatgaaggcttcttccatccgacggacagaaggactgattgcgtgatatgcttcgcttgcaatgtggtttgcttcaatgcgggcataaagctcatcaatcatttctggaactgtttccgccacgaactcatgattcaatgtggttgccagttccaagatgacggccaactgatttacttggtcgttgtacgcctcatcactttcaaagtcttcacgcaccggcagagcgtgactattggaagccatttggttggcacgttttaccgcagcatctacgtcgttaaggtcgaggttgttaaccctccctgttgcggcatacatgccaatgatggtcagcagatacgttgggctggtacgtgctgcgttacgaatggtttcgttcagtttgattacggtcatgttgtagtcctcgatagtctattaataggatggttaagagaagattattactcaactctcacctaggtaatatatatctgaaatattttttagtacgagtaaacaaaaaaaagaagaaaccctactcccgaaggagtagggcactatctttttaacagccttgtttttctagccagcggtgcaccattaaaccaccgattcgttgcgcgttttcgaccgcttcggcggaaggggtcgggtctttaacaaaacgttcgattagctgctgttcggcgatgttgccaaactctgcaaccagcgactcgatgtccgcagatgcgattttcgattgtctcaactgaacacctttgatttccatgcccgcaatgacagccttggcactgtcggaaactttaggtttcatccacccagctgcgtgctcgctccagttaagctcacgccccatcacgccatcggtcgggatatgaaacttcttatcactagggcggaagtcagaccagaagaattccttcttcatcggataacgttgcttattccgatgcgcaaactccaccaccaaacgaacgacgcggctggcgttaggataacgaaagtctgggtcatgtactaacagaatgccattcatggcgtcctgtgtaagtaccacacgggttttatccgtacggatgatgtatcccccgtctttaccgcgcatgaactgtacacggtttttacgtttcttaggcttgagcattagttactcctgaacgaacctttatcatttcattgaggttcttgatatcaattttcgctacaacgggcgacagacaaaaatgtgtacgtggggtccagtctaaacacaatggtcgttctgttgcataacactcttcacgccacttacgtaacgccaacaattgacgttcccgtaacgtctttgcgataacctttctggctatcttggcgtacacagcggttcgcttatcgcgcccagtaaggaggttagcaaagaactccaccggaatgaaattctctctgtacaccctcgtcttgccgcgatagaagcttacgctctgctcggtaaaagcaatacgtaacttattcatcttcatccttaccgagcagatccggttgttgagaaagtgaatcgaacgtatactgctgcgcgtctggggattctttgcggtgtttcacatagtgggcatatgcatccctcccatctggtgtgctcaagcagagttctttcagacctgacaaatccatcggcatctcggtgtccatgtaaagaacaggctcaccgttacgtaaggcacgagagtacgcatacgggtcgtgaaggtgtggtgtaatcgtacgcgccatcgcaaccgttctggcaaccgcttcatcaccctcgttaatccccgcgatactgcgaactcggtcgtataactctttggttgcaggatcggtagcagccggtgacaataaccccagatagtccagcgtcttcggttgattgagagaaccaaacagaatcagccagtcgaccagagtttctggtgttgggtcatccagtttaccgaagtcttccggcgggagttcagccattgcccgcttacctgccgcacagatagcgtcagtcagttgcggcattaacggcagcttaatcaggtcatcgacaatcgtaaacgtgcctgcggattgcggtaacgtcttgcgcagttccaacatgcggttgatgtgcttacgatcgtcttgacaagtgcgcagctcgttttcgacatctttcaacacatccgacgtatacagcacattcactttggagaagttcagcttacgcaacgcgacgttaacgttgtagtcggccatcgacagcgccacatcacggatacgcacttcgctcgtcagggacattggagggtgggtatacagttcattgacggtgttgtcgagtggatttcctaagcggcggtcgaacgcaccagacaccccagggttattggcaatcttccgagatagtctatcgtcaccgttatggataccgcctttaaacagcacatccatcgaggtctgcataccggcgtcacggttggcattaatcccaatgtggctatagtccggcttgccaaacagtgactcctgcaactcttccatgtacgtattcttggtcttcgcaaccggtttcagtttacgcagaccgtaatatttggtgcccatgccgatggtcgcgcgacagaacatgttctggagctggcggtacatcacacgggtcgttttcggcaggttgaagaccggcaaggtaggcgcgcctaatggccctacaatctcaccgacttctacgccatcgatatagcggacacatttcttgcccagatataccgcaaacccttctgggaatttcaaccctgcaccggcaggataacgggtgacaattgccagagtggtttttgctttacgaggttttaacattttaatactccttttaggttactcttagtgtttcttacggtagtgaacgttccagaggtgcgacgccatattcgacatctggataaacgttcgggcattaggcactttacaataggtatcaatcagcgccagatactcaacagacaggtgcatcaattcatccgacatcaacacaaggtcgtcgggcagttctgccgtacagactgctaagccgtattccgtgccgaccttttgcattcggtcgaggaatcggttaatggcgatatgttcgccgcgggcagacttcacaaactttggtaagatgaactcaccgttctcgctgagaatccacatggattgcgaggtgcgggcatcgcgatggttctgggtgaacttacgcacatcctcaaccgttggctgaactaaactaaccgttaatccatttgacaacgtcagttgatacattaactaatccttctttggcgggatgtaagcgtcgaggtctttaactgtgattaccccgcggatatgtggacgaaaccagtcacggggacgcacgtatacttcgcccggtttcaatgggaagtcgaaaaccggattcgtgtcgtagttaacgtggcgtgttccgtagctcactttattttcttcggtaaacttctgggcataacttgccacatcaggcgaaagtttactcagatgcagaccgtaaacaaaagaccactcgtcacccgcttgcatgtgatggtgcatcgaagccatcgtctttgccagcttctgattacattcatcttcggtatacaccccctcgacggtggtgggttgtaagtggatgaacgctttcagttcggcaatctcacgcagtaatgcccttttagttcgtaaccatccaaacattagaagtgtcccgttccacctgtggcgatatacagcccacagcgctctacagcgtcgttaaagttacgcatcaatagaatcaccccaccgactgtgcgaggcgctctcaatgcttcatattcacgccccggtgtgcgtaccacatactcggttgccaacggcacaatctcgtagtagttatcacgcaggggcaccatcatggtaagtagtcggtcagccgtgtcggtatcatccagaatcttcccaccccttgcgaggtaggaaagtgattgttctggtgacatcccaccgagcgacttggcatcaaaaggtgtcacgtctttcatcagaagtaatccagttctttgattttggtacggtaatcgacaacacgttgttgcagtgtatcggtcgtcaggcgaatggctgcaccgtcactgcgttcaaccgaggctttaatcaccacacagtgcgattccacaacatgggagatttcaagtgccatcttttccagcgttcggacacgcttttcggcttccagcttctgttcttccaaccgaagattgcgttggaagagttcacgctggcgtttattgatcaaggagagcagtcggtctaacatcacttatctccggttcaggtagatgtggttgtggttgtggaatggcccaccaacccagctcagtacccagaagtttttgttgacgtcaaccgagtcccacgttacccacgtcaggcccggtatctcaacccgctgaataatgcggatgatttcagccagctccgtgcgaggacggttccaaatcgcttccagatgcacatctaagcgctctggatgaatcaccgggcgaatggctaccttctcttcgggattcgtctcaaaggccagctgagaaggcgtacggggcacataccacgtccaaccttgcagacgcttgcaagtgttgtaacgggccagctccatcaatgcataggtcaccattttgaccttgcagtaccaatcgttccactccgccacagggtaattcatggcgatttcttctttgagtgggtcaatcttgatttccgggtcgatggccatccccggctgctttaacatcgcgaggtgggtcaactcgcgcttggtgtaaaagttcatttccattttatactccttgtgggggtgacttatttcttcaaaggacgaagaatgatttcgttggtgtaacggtctttactgagatccagtaaagtgtgagcaatggtgttcttgataccattggtaatgagtttaatcaccgcgggtgattgttgagaggcttcggtaagtgccgataactgaatagtcatcttatcgccgtctacggtatacgtatcagaactactttcgctgccttctttcagacgctcgatggccgtagcccaaaccaacgcagagaccgcttgaccaacaatgtggatttcagcttcccatttcccttcgccaagatacgccagattaagactcgccgggccagtaatgatgttgcgatcatcgcctgccaacaacagatttctccccatgttaaaacgtgccatggtttcacgaattgctacctgcatgttttcaggaagcgggacgtgtgagataagagtaacgtttctgttgatggtgttcttaacacgcaggtcacgactaggcagcgtcctgcggagcatgcccggtttattttcaagaacttcttttaagtacatctgcgattcgaggttttggtttgtgatacccaacagcatcgcaggtgttggctccacatgcacacaatcgtccgcgacgataccacaatagacttcgtgtagcagcgcaataattttcagtgcttcttctgaatcggcttcgagctttgtcagcgcacgataagccggacgtacgtacttgtccatcaatacgtaagtgcgtgtttcttcaggtacgctatacccttcaatctgtgggaacttttctttcgccagcgcgtacagtttagttgtggtatcaattaaattctgaatcaggagattgtcagaaacagtaaatctcgaaaacaaaggtacgcggataaattgggcttgcatgatgatactccttgtggggtggtaatttatttattggctaagttattgaccgcggccatggtcagggtcggagagaacttaatcaatgtgtcggttggaattttgtggctgaagatatcgtgccacacattgatgatagctgcgtgcttttgcaactcttctaaggtgacatacggcgtgaatgacgagcgcaacaccagaccgtagttatacagcgctgcccaaccacaaccgctgtcgctgtatgcgcgggtaaagaattccgccggtttctcaaccagctccactttctcaaagcctgccgcttcaaaggcttccttcgctaacgcggtggcgttttcaaagagtgggatttcacgaccgggaatagtaccaacgggaacaatgatgcgcagggtgtcattcttgatatcaaaactcattctatttctccttcgtagattacttcgacattgtgttcttcgcctaaggctttgaactcatcaactaataaaagccggtgacagaacttaccggcggggcaataacacatcaggatgatttcgtcctgaaacaacagcaccaacatcacatcagggtcatcctgtttgagttgttggattctgcttttatattttttcgtgtaggcgtcttccgcctcgggacctttgtcggaattcttgtactccatcagaaagtcccacgttggggccagcgctttgatgccagattttaccgtgatatcaatcagagacactgccggatattgcgacttcgcttttcgccacttcgctatttgcactgtccggattatcagctttctctttttctcgctgtgcgcggtactcggcttgctctcgttcacgttccacctttagcatttcttctacgtggtcaaatttcgttttccactcttcgatgctatacgcttcgatttgcaggttacgatcatcgtgccgcatacgcagtgttgggagatgtttcatttcagacgtcggtagtaattcacttgggaaactccccgcgaagtgattacccggaaggttgtccgtgttgagtcggcggtggaactcgtcatctatcgcgatgcgccacgcggccgttaagttaatcccacgagccagataacgcaccgacttaccgaagtgttgtgggttgcaggaaatgtacagcgcgttctcagacttaacatggtaaatcttaaacatgtaggtcgaacacacggtgatcagttcttgcacgtctaccggaagcgcatcccacatgtccttcttctccatatcccacgcaggggtgagtagcggagaacaacgatagtggtggtcttggaagaacatcagctcgctgtagactttcttcaaacgcagatagtcttcttccgaccactcaccttgcagcgcgctgttttcaatgaagtcggctttgttccaaccggtcagtgctgttgaacccggatggcgagcttgcacagcattcatcagatgtgccagccccagaacggtgttcccctgttgaatcaaacgactctcacttccgtttgagcgaccgatgatacaactggtgaagatttgtgggggtggagagcgccactctagtggctctttataatggtctttgttgtgctttaagagccgcagggcaatttcactgccgagcaaatactcaacgatggccgcaggcgaaccttgatagaaatccatgtagactggatgaataacctcaccaccgtcggccgtcggttgcgcaatgagtttttgtaacacccatgtggaatcaatcccaccggtgaacgctaataaacgtggcatttgatactccttattttacgaaaaaagaaaaaggacactttcatgtcccttttttactgctagaagaaatacttcgcaccggtgtagatggccacgaaaccatagacacaagcttgaacaccaaacgcgatggcacccggtgggcacttacggcgcttttggtttgatgcgatacgccagctcagtaagcatgcgattgtgaagaggattgctgtaacgatataaattttatccatgacggactccttaattattttaatttattgtaattgtaaaccacaccttccttggaactaataatggaaagctcatcaagataatatctatctgagctttttttcattagaacagtgtttgcaacggcaccagatggacaaatgcccaacggtgaatgttccatgcaacgatagcaaacactagctcgacgaacgcacccatcagttcgcctttcaccaaatccttaaccatgccaataacacactgaataaggaaataaccacttaccaccatgacacaccagtagaacagctcgggtacattcattctggtaacatgtcccatgtgatgactttatcgattttaccgtccggtgttgccagcgcacgcatcccgaaggttacgttctgattcgcaccgtccagcaggttacgtaccatcgcggcctgcgggccccacggacgcagttccgcagacacacgctggttcaacttatcgtgacgaatgttttcaattgaagcacagacgttacgttggtcaatggtgcacgggcctgacacagaacggtcgtcagttaccgggaactgaaaacggtaatcgtgatacggatcaacttcacagaagagacgcggcatacgtttaataccacgcaccagatgcgcaaggtcaccgttatactggcgaccacttgcattcattttggtttggtctaacaacacaaccgaataaaacttgccgttgttgtcttcacccttgcccgtgatttcaatcaggttacgttcagttttcttttccatgttcttatccattgttatctaaacattcaacatatgccgtagcgtcttccaacgcatcgcatagctttttcttttcgccttcaaagcagacgatggaatggtacgactccagcacgaaatgccagaggtcatccgtatcagaatagtgcatcgaccaactgacaccgttggctttacacttatccttgaagtacgccagctcacctacaaagacttcgtcctgtacgtcgttgtacacgtacggaacaacatcccaccccgatggtagcaataagtcccatgcaggtacgccggtgattttaccgtctttgtccttgatgaaacgcggaacgataatcagctctttctgctcacgcatatacgtcgccaacttatcaccgtacgggccatagggcaccacgttagttgtgagagtgatatactcaccgttcacatccatacttccgccgagaagcgtagcgcagacgtgttcttcgtgaatcttcgaggtacggaaaagcgattccgggtattggtgattggcgtgccgcaccggcgatgtttcacaacgggcggagcagctgagccagcgtcggaagatctgctgccagtccgcatcatccacaaacgcagacttcggcagacacaacacctgacccgatgcgtggatgctaccttcacttactgttttaccggcctgtgagtaggacttctgtacgcgttccacccgaagcgaatactgattatcttccacgagttaactcccgagattataatagagaggcgcaatgatgttactgtagtagaggtttccgattaacccaccaaacaacaatgccacgatgagcatcacccagaaaggccacttataccgaacggacaacttgccaatcgcgacgcccagtatgttgagaatcagaaagatggcaatgattgacacaacgagcatgaacatcagttcttcctcaggactttacctgtcaggtcgtagcctttctcagtgtacttgttgggctcgtacaacgcatcttggaacaacgcttcaacgatagcagccagacgtcgggcaccgaggttatccacactgttcgcttcgacagtcttctccgcaatgtactcaaaggtgtcaaggtcgtaattgactttcaccccttcgattcgcaggagacgtaccatcgcatggaactcactgctgtccattcgacaaatcgcaatgagggcttccttgtcaagcggttccagttctgcacgcaacgtaaagcgcccttgcagttctggcatcagtttagtgactggggcctctgcgaaagaaccggcaccaacaaacagaatgttcgtggtatcgattccgccgtataaaccaccttcaaccatcttgagcaagctgcgttgtacaccgctgcgagaaacatgcgtacggcccgtggcgtctgtttcaatgagcttgtcaatctcatccaagaacaccaccccgaaattctctacaaagtcacgcccattacagttggccactttgtcgaggtctttcttcgccaacacgttacgtttacctttgggttgtaccacctcaggctcggggactttatagctccacagtttttcatcagcaaagcgggtgaaatcttcacaatcttcgaagacttcttccagcccttccgggtcacgcgctaacatcacacagatgtagagggcaaactcagtcgagtccatcggacgccacgcaatgcccggtggaagatcttccttttcagtctgctcaaacgagtgtgcaacatcgtaccagtcacctgacgacacgcacgcagcaacaggattactgctgagcatctcgacgccgagcgtgatgatggtttccagcacttcgccgtaggccatcagacccatgaattcaccgagcaacgcaggattgttctccatcatatcttcggtgttttcactgaggtcgtcttcgaggtcgtcgatactgttaatcggtttcccggccatcttctcgataagcccgacaactttgttcgccacctcgataagtttctgcccctgaatcatttcaatgtcagcgaagtcgatgacatcgtacggcagattcttcacggcgtgataacccaccaaaaacgcacgcatgtaatagaccatgcgatagtggttgtaggtgtcatcgtcagggaacacgcctaaatctttcagggtttgttcgtgttgctttttagcatcacgcgcagcttgccactgtgcttgtttcgctgaactctctgcttcgtattctttctcttccaacgccttgagttcttcacgagtataacgctgttcgtctttctcaagggtcataccggtacgcatctcaacgtaccagtcggggagcgcaatagaacgggttaaggtttgtaagtccgtgcctaccgtgttgaggttccggcctacatagcccgtctcagaaaagccggtcatatccagctctaaaactggtaaaccaaactgagttttcagtacgcgcatcaacgcggttttaccggagccagttggccccagtaataacagattctgtttgcgaacactgttgcgttcaccgaggggtagcatcgctacccgtacgcggttacgcagagcaatcgccaacatttttttcgccagttcttgaccgtggacataacggttaaaaacattgacgatttccacgggcgttaagttttccataattcaccataagcaggttctgttgcacgacgttaataccttcaatgatgccgacattgaattcactgccgccgccgacaaacgcgatacgtaccgtacgcggattaagcgagtggatgtacgccttgattgaggtgtccactttctcaccacgttgtatctggtaagtttcgaacagttggtgtacgtgtgccattagcgcagtgaggttttcgaaatcgtacttcgccgtgttcggacggaacaacgagacaggctgacgactgaatgcacgcgcagtcagctcatcacgcaattccatacgcatcttttcagggagacgaggtaggatatttgcacgcacgttatcgtcgtttaccgcaaagtacaatgtacgtggtgtcatgccaatcgcatcacagagttccacgacgttgtgattacccgcattgaagtagtcacgcacgatttgggtataacggtcaccgtcggactgggcctcagggacttctttaaacaagcgacaaaaacgctcccagaacttcatttcttactctccgataacttgcttatttgcgacttggtaatcatccccttcgccgcgttggtgtatactgatattggtatcaaacttggcatggtctgccatgagcatgataatcagttcttctttggtaacattcagaacgtgctgtgggagatggttctctttctctaacacacccgacgccatgaagttttcaatcaaacgttcatcggtagtatcgtgtgtgaaatcgtaacgttcatttggtgaagcaaagaaagcgtaacccacgtattctgggttattcatcatgtgttccggcttcatgtgttccaccaacttatccacgttttccgtgaaatcagtcagtgtgtattcatctaaacgaagaacacccgattctacatctactgcgccatctgcattgacggcataatgcgccatccagaccgaccacgtacgtgggtcttcaaacagtgtttcagctaacgcggcactgacggttacacgtaccgggcgactgaccgtgaactgaaaaccgcggccaccgtagggttgaatacgacggttagaggcaccaataaaggagatgcgggctaacgagttttccaccaccatacgggcagtttctgcatgggcttgctgcgggttatattttttgttgcggactttcttctgctttgccatcttctgattctctttgtgattgtcattaaaaggagtggtgctgttataaatctacgcgttcgtatctacgcggtggggtacgtgggaagggtgccaattcacacggcggtaacgcttgaactttcgctttcagctcgtcgaacggcataaacggcacgaagtgatgacagccggggaagcagcctaagatgcgcacaatgcgctcagcagaccacacacccttctcgttatccaaatctggattcatggacaggtgttcaatgaatgttgctacaaacgccgattcagtgtctgaggggaacaccatcacgttggccggttggtgggtgaacgttaggcggtatgcaggtcctgccagtttaatatcgtagaactggccatcgggacggaggacggagccagaatacgatatatcttcgtgacgttcattgtcgttaccactcaccaagatatcagaaatcttaccttgtgagtcgttcgggaaccaccaccccagtttatcgaaacctgcttctgggttgtaagacgccagtaagctcatgccctgaatggtggtgttcacgtaaaccatgccattaacgataaaaccagcaatagaaacggtactcattttcgtaagtcctctctgtaaaccacatcgtagccatgtcccgacatcgggtcgattttctgcaccatcaagataatgttctcaggtgataatccgcatgcccaacctgctcgcgccaactctgcaccagaaccgtaaactaccggcgtctccaacaagtcttcatcgaccgttagtccagtgtggtttgtcggcgcgccgatttcgggtgaccaaccgcgcaggcgagagataccgctaaagattaaggtcttcttgcgggtcatggcgaccagtgtgttactttcaataaatcgcaacagccagatttctgcggctgcatgcgctttctctttgccgaagatgaaatcgtagatgttcttttccagctctttgcgctcgacgggcgtagggtgttctgacccaaagaagtacgcgatacggccacgaacaatacgaatcttcgcgtcttcaaataccatccggtttttcaataccgcacggtctgcggcgatatagttcttacccgcaataaaagtagtcatcgacagtccttaaaaaataaaacagtcctactcccgaaggagtaggacgtactgattagaagtgtttacgcaggatagacacgttcggtgttgcgccacgtttggacttcacagcggtgcgttgcttagccaccggcgcggcaactttcgccagcggtatcttatctgagctaccgcggttgacaatacgcagattgtctgcggagacaatcccgccttcgaactggaagttcacgcctttcttcagctttttgtagtcatagcctgcaaggtcgagcttcagctcaataccgtgctcactgcctacgatccgatactgaatgctggtaccaacacgtttcagcacttcaaagattggcatggccttggaagcagacttgctttccatcttggtgagcttgcgcggttccacatcaccggagtacagaagattctctggctgcactgcgccatcgaacgacaactgcacacctttgcggatacctttataatcgaacccagccaaatccaacgcccgcgcttttgcaggtgggtcagatttaaagacgaaagtgacgacactgcctttacgattcaatacaacgtaattgtacatcagatactccttatagattaaaatgtgggggagaaaagaatcttctcccctagatgatatctatctgaaaagtaatacgttacaggcggatttgcagctgaatcggatcggtgtttcctctgtgggcttctggccaacagaagatacggtggtgcacccgactgatttcaaccgacaggccgatggcaggcacaaacaggaacacgttcagaggcatagtgaaatcgagtttggtttcaaggttcgtgaagtgaacctctttgttatccaccccaataacctgtgcgtacacctgacgcgcttccgttgggccacctaatggtctttgaaacgcggactgcatccgaatgaggtaatcatgcgaagacagctcatcgcggacatcaatgagggatgggctcgacatgatggttggtatccagtacgaaggagttctcaccggtctgtttcgccagtgcccacatccacttgtcagtggacttgtcgtgccatgatgctaaccacacaccgtcgacgataccggaggcatccacttccgggtggaacagcatgtactcgttctcttcggcatcgagaaccacgaactgaccttcttccatgcggtcgaacttcgccagacccacatcgatttgtaccggctcgacattcgggtcaccagtcacgctggtaccgaagtcgacgatttttggtaaatcacggtgaattgcgctaagccacattgcttttaatcctcagggttatttggtttgacatagataggtactattctgtaaaaagacaaaaaaataaacctcacccgaaggtgaggtcatttcattagaactggcactcttcgcggtcatccaccaacacgctggtaatgacgtaacgggccagtcgcatacgcgccgtttcagtttgttcatcagacggcaattgctcaccttcaggggcaaccattgcgtattccgattctgctaactgctgcgcatagtcctctaccgcggtatcaaacggaccacgcaactcagccaccttgtcgagaatctcatcgttaggtacgatagactgtgacaggataccggccgcatccgcaggggataccgtagtgaagttcaactcgttcagcaacgctctgtcctgcgcacgagtggtgatgagaccaacaatcaacttctcaaactcatccaatgaaatatctggatggtcggtgcccatgatcagttcaccgtacttttggaacagcgcgcgcgctttgtcttcgaagccgcaatccatgtcacggacgccgaggtcgaagtcgtgctgtggaagctgttcgaaatcgataacatccattgcgattcctctataacgttagtggtgtcatacaaaggcattgacttgagggggtgaccaaccgtacttctaagtctttgccgttttccaccaactcgcgttcattaaccacacgatggatagaaataccatcacgatgtttcgccttggtgatgagcttatccagtgccaccttttcagatttggtgaattcggtgcccggataaacaacgagcagttcgttgttctcaataatcaccgcgcggaacagggtcttttcgccagagaccacatcgtaaaccacttctttagaacgtgccacagaacgattgatgctagtttgcatgagtagatactccttttaggataatataaataccacgggtcgtggtgttcaacgtttctagtgtttgcaccagcggtgttgggttgtcaaacgtttcacggttcaccacatagtccccgccgtttttctggttagaggcgatgtagttgaagatatccgcgacagtcatctgcgattggaaatcgcttgcccagtgcgttaacagttcagcatgttcatccacgatattgacgagggcaactgcggtacgaccgtgtccaaaatccacacggtgaaatgctgctgtgcccatgccgtacgcttccgcagctttgcgcatactttcgacagtgtccgttgcttctttgaaggacttcgtctcttcatcggtcaacagacaattctctatcatcttcggcggcgggctgataccttcacggtgtggaataatgtacttcaccgcgtgcaggtcaaacccaacgtttttgagcgcttcatccgcagtcgttgtcgagtaggcaaagatagcattaacatctattacatccggcaacagatgcagcggttcatcgacctcaccaaagcggtcaatggaaaccaacagtgctgtttcctgaatacggtgacgtttcaggtagacacgccagcgccccacttcaacaatgtgcttcgtttccatgggactcaactctaagatacgccaatctaatacgccgcgacccagaggcttgtcgtacgtaccatctagtacctctttcgttatctctctcataaccctcctaagctatcgtgtagtgatgggtcactacctcatgtgtgataccatcgtaagtcggtatttctgcattggcgtccagcgagatatacaacgacttcttctccgttccacagagcttcaacaaataacggaagaactccgagaagtcctgcgcgtattgccggtcacgcggatggaacacagaaacatagttagcgactgttaaggcattcggagactgactcacaaacaacaccgacgtaattgtgtcgttctgtttgcgtaccaatacttccataaagccaaaagccacttcctttaagacgtgcttgtaccccggcaatgacttcttcgttatctcacacacacgctccatgtcatccagagaacaattctcctgacgatgaatcatcggggcgcgtgtattgaaacgcgaaacatcaaacggggtaaatttcacacgctttgtcacgaactcaagtcccatggcccggcatatcccatgctcaacgtgagcgctgggttctaataccacatcgaagtgaatgacttcgagttggcgcatgaggtttttccactggtaaaagggcttgttcgtcatcggcaccatattcaggatatggaacacatcaccgtgacgctcgccacttaaaacgagaagcgtctggcgtgtgttagacaccaccagataatgctcctcgtccatcgctaacggatgggtttgtttaatgccttgccaaatacgttcaacgtcaacctgtcgcccgttaaggatgacaggcttctcgtacacaggcggatacgataacaggtgcatggttactccagaacaccaatcagctcattcacacgcccacgggtttctgccttcgaccccaaataccgccccacctctacagtctcccactggaagccgtagtagatgtctttggtgagcagcgtatcagagttcgacaggactacacgacaaccacgaagatgcgcttctttcaggagcttagccagttggcgttggtgttgttggttaaaggaggctttgtggtattgtgcgaacgaagcggttttcgagctggggatgtacggagggtccgcgtatatcagcgaacctttcggtgcactggtaatcgtctcctcaaatccacaacagcgcaactccacttcggactcggtgcagcgtttccagaaagcatgaatttcttctttgggtaaatacggtttggttgggtggtcgccatatggcacgttatacccgcctgcctgattgtaccgacacaatccgttatacccatggcgattcagatagatgaagatggcggcgcggtcaatggtatcttcgacggtgactttctcacggtcgttgagtatcgcgcggcgttcagcgtacacctctggatcgcagccgtttacccagagttcctcacaggcttgaactaagtcgtctggtgcttccattgcagaacggagcaccgcaaccaagtccgggttatagtcggacagtatgtacttcgggaagttggtgttcatgaacaccgaccctgcacccacgaacggctcgacgaaacaatcgacttcaccgaacaccttacgcaggggctggatgattcgcttctttccaccgacccattttaaaatagaacgcatctcaatcccctttgtacaccggcgcaccgtgtccagctgtgacacccagatactttttcgacttcttccaacttaccgcgttttcaaccagttccacaccaattgaccccggcaaagattcccagttcaacaaggtacccagcaggtgattcattggcacgttatcggcgaaggtcgtggccatcagatgttcgtgggacaagcccgctttctgaatggcagcaacaataaggttacggccaatacgtttcccggtatgacaaccatcaacaccgacgccactcaggataatttcaccccactgagcgtattggagttgcgccacgcctaagatatcacccccatccatccagaccagtgttttgtactggctggtgcgcccacgttcaatcaccgattccggtagcacctcgcggaagatttcccgaccgaaagggtcagtctgtccttcccgccagatggtgtggcggactaagccggtgagctgctcaagctgaatgtcgttcaatgtttctaaaccagaaatatccacaatgcgtttatcgattgggagtttctcgtacgacttacaactcaccatccagttattttcaatcagcttaaagcccatacgtttacggaagtcaaagttatccgacgttccatcaacagtcatggcataacgacacccgacatgatccaacaacatcatcatcgacactttattcagagacttagagataatctcctcagcgtgatgaataatgagcgtttcatcacccatggtggtaatgacagagatgtaccccagtggtttatgtcggtcattacgcaaaccgaagacttgatactgtggatttttgagaatcacgttcagtcgcttaatcgcaattgtccgtgacccaaaggcgtggtaatactcgcgtgccttttcgctaccccaagtaaggcgttcgatagtgatattgatttgctgttctgccggttcgaccggcggtttaataatggttgattgcgctatcgattgcatcgatttcccccgcaacaaattcttgttattcacaggaaagggaagttgcgtaaaaaggcaaaaaataagaagggggaaagacccccttttactttacgactagatatgttggtcgatacgacgacgtagcggctccgggatataacgcatatccattccggcatcgcttgtcgcgagtaggcggaggttacgctgttttaccgggtagctctgaacgaagttcgcacggtcgtattcgacgcgatcgaaatgtttcgttccactctcacagtctttgcacagatagatggttggttcggcagggttgctgtcatacggtgaccagcaaatcacttcttccggggccatcggtttacggcaatcgttgcagaggataaagttctgcgcgatttcgttctgtaacgcttcgtggcacgatttacaggtatagaacactgtacggatagggccaatgatttgagcggtgtagtacggcgcaattttccactgatggaggtgtgggcaacattcgtcgtgtggtgagatgatgtgctgggttttaccagcggcataaattgctttcatggtaacctcggttagtgtgcaatacggacggacttagcctggtgactctgccatgcggcgttgagtctcatatattcgtaaccggtttgtacggtcacagtttcggtagccttaccaaagcgtgacgtgacggtaatagaatattccagacgcagggcatcggcgacacgcttaacgacgtcaaatgaaacacggtcgacacgaccgaatttgatgttgctaatgacgttcggtgagacttttgcaacgtgtgcaagttcacgctgagtcacaccatcttcgacgatcttttcaatgatgaaactcatctggttgacgaacttgtttttagcactacgggtagcatcatgaatataacgcattatttgattctccttgtgggtacaatgagacattgatttcaatgtccacctagatgatatctatctgagattttgtggaataaagcataggactacccggtggtgtaaaaaataaaaccctcttacccgaaggtaagagggagtgtttcttattttagtttgttcacgtacgccactgcgatcgcggtcgcgatagtcagcggtgcagtaacttggtcagactgttcgtcaaacttcagccactggaacttatcaccgccctcagtcagaatctggaacgcatagcgataacgatcacgatacgcatcccacgcttctgccgactcaaacatcttaccactgaccgcatcatcccagtccagccctttctctgccagacgtttatcgcgacggagtttggcggtttcgaaaccgacttccatcgaaatgtaaatctgcggagaaccgggttggttacacacaccagagcggaagacttcctgacggccttcatcaccttggttcgcgattgtcacgggtgcccaacggtcaagcaaaaccacgtcgtattgtggtacgacgtattgcagtgtgtattcgaaatcctgacacattgcccgtgcaacctgcgcatctgccacacctgtcactaactgacggcgagcaaactgtcccgtctcggtatctgcacacgggtggttaaccaccttcactcgcagacccagaccttctaagacggcacgaactttctgcaccatcgtagacttaccagcatagtcgtgaccatcgaaggccgcggtaatagctgtcattacgttttccccattaaagcttttaagtgttctgtacacataatgtacatctgctgtaattgaacaaaaaaataaagcaggcaccccgaaggatgcctgagttattagaagtcgatattgtctttgttcagaaccgccttacggagttcttctgaccaactgttttcaatccacgtagtgacgacaggattaacacgacggtcaaggaagaactgttgcaacatcggccactcgtgcagtggataccggagcgtaaacgacagagaacccggtgaggtgctttgcgcgttattaacacgtaacgttggtgacagctcatacgttacacgaacgtcattgagggtggcaactggaccgaacagttctaaacggcgcactaccgacaattcataagcaccgaatttgccacgtaggcgttcttccgacttctgtcggacgaagtagttctggccatcctcaggttttctctgtagacgttctgtcttcatcacgtcggtgaagaaacgattgatggtttcctcaacataaacgtaacgctcacacgcacctttcagagctggtaggtcatgcgctttccacgcctctagcaaatcaggtttacgggctactgttttgaagaacattctcgcggagactaaacgcatctcttcgagcattttcttcaccatatcttcatgtgtccaactgggtgcacagaagaatattctaccaccgaccaacgttgcacccgtctcgctgttcacgagtttgtgggtgataccgcgtggaatgttgttctgggttaaatcgccaagattgtactggaacacatagcgatatttcccatccacggttggcagtgaatagatttctttgatagttggatcttttaataaagtcatggtatttctctcttaggttagttgatgcgttttaaccgacgcactacggcatacttagagtatctgttgtaaaaaagataactattgttatctcacttgaataatatctattcaaaaaataatagagtaaacccaccccgaagggtgggcattacttactggtgttcaaccgtgggtttcgaccagacgccatctgtgcttggcaggttcagcttatccgcagcctcgccgtagacgaccaatgcaggcaggccacgatcagtcaagaagaactgaatacgatatgcctctgcttcggtctccaccacaatcagttcggcagcacgcaataacgacatcgcatgttctgcttcctgcggggtcggctcaacgttcttaccttggataatattccgcagtcgctgtgcacccaacccattaacgttgcaataacccggacgcaggttaacgatgttctcacgatactccacgttaccccctgaggcgcgcgttaatgcatggtacggcgagtgacgacgcttacggtgcatgtcacacatggctttgtgtagaatcccctgaacatgtttgaaattgttcagggttttggggcgcttcatcccggtcactttacacgcaatgtctaagaccttggtaatgtgatacagtcggcttacgccgctgcgccggacgcagatacgcaccggcagtttaccatgtttatcaatgtacgcattggtgatcaggaaaagcgagtctaagatcatctcaggcattgtcgctctctcaaaatccgttaattacggctcgcataaagtcgtatacggtttggcggtgttctgcttctgcgtactcgaacttagaataatcgtcccaccaacgcactttgtgtcgctggccattcgtttcaacgtgacacaataaggtgagcaaaaactccttactgtaacggaaacgcaaatggaaccgcccgtgggggttacgcagaattaattcgagactgcgtgattgcaccccgagggggtcggttttgataacaactacgaggtcttcaaattgagaaaggacgtccgtgacatcatcaaagttactgtcgtgctttagctcgcttctttgcaaagcgtcggtatactgttgaagttctcgatagaacatgcctctttactccgtaggcgtaagtaagggaaaccgatgtcccacggccggtcacgattgaacgggtggaaatagatgttacgactgtaaaacaagaggtacttgtagaacgtcgagaaggtcacatctctgtcggtaacgagcaggtagtcatactgaggggaatcagggcaatgaatgtgcagtccgatgtacttcttaccgtccaacattccttcaacttcacgcacttccgttgggccaacgaagcctcccgtctgaaacgcgttctgccctgtccagtagacaccacgctcggttgcattccgagacttaccaatttcgttacacttgatagaattgaacgaatccttttgctgccaatctgccagtgtgtggaaacgttgtatttgctctaccgagtaatgcttcaacacattaggtggaagttgccagaaactgcccgcaacgcgaaccactttccatccaggacggaaacccaagaagtgccgcttcacaccaaacgtataatgacggccctcctgatggggcacattgcgaacagatgccatttaaatctccttcaccatatcccgatactcggtgcgaaaaccaaacttctggtacatcgcaatcgcttgctggttgttgtccagcacgtagagctgcatgaaaccacagcctttggctttcccatggtcacgcaccgcgttcatcaggaggagtccgacgcctttaccccgttggtcattgttgacaaagaagttgtaaacccacaaccacttactgccaatgtttgaccgcccagtctgaatggagaaagacaggaatcccaccgcacgaccttcatcatcgagcgcaatggctgcctgctgtccatcactccagacttcggtgacatcatcgatttcattaaagccgttacgtccattcaggtctttaagacgggcctgttggtcgttatagagactgttgtgtaaatcggttaactcagcatggtatttctgacccagccgggaagttaacttagaaactaaaacgactttcatgattaacccgccttaatggatgcctgcacccaattgagcaggccatcacccacacgaacgagcgctgttgtaaacgcatcttccacggccatggcattcttgaactgttgggttaccgaacgcagttcgttcccttccagatctttcatgtggtcgcgcagcttctccatgttttcatagataccggtgtagctgaagacaccacgtttggcgctgcggtcttcgagtgcctgtgcgatgcgcttcactgcttccaatgctttttcgcattctgctttagacagggtttcgaacttacccccaatcttcgcttcacgcgcgacagcgaactccactttttctttggcaccaaaaccgcgggtgacaataatcacgttcccggctaatggacgagccttcacatcgttttcggtgaaacgaccgagtaaacctgatgcacggtggatagccgcgtttgacggataaccgattttgtccagtgaaccatcatcgttctttttacggcgatcgacaatcagtccggtttggtccaccttcacggtgtactctttcacggcagcagccatggcttcactgtggttagacagttcgatacacttcgcgaggtcaggcttatcttcgtagcagatgcagctcgcccacgtcagaacacgcacgtcctgcggatgaatctccgccgtgtgcagtttcgattcgagcttttgacggcgcttttccatcatagtcgatttcgacgtcatatccgcaatcttctctttgaagatagggccgtaatgttctgcccactcacggaacttgtccagcagtttagaggacagatgcgcagttcccttaccggccgctttggcacctttcaccgcacctttaccggctaaacgggcggcacccatcccaacacccacagcggctttacccgcgtctttggcgaccttcttcgcgatactgccttgtgcggcaccatcagcaacgacctgtgcccgttccatcatcgcattggactcgcgagcaacagcttcttcccactcagcttctgcttcatccagtacctgccagcgcaacgcaatggaacgcatcatggggttgttcattccaaccccaatggactccaaagcaaccactgtgtcaaaatcctcacacagcgtaataaaatctaaatctggtgacgacatggccacaccccttgtcttaacgcaccttaacggtgtagtaatagttgcggtttggccagcgtacacagatagccactaagtccccatggatatcgtgataatgaatcacacggggttcactccgttccatgaacggaaagatagccgtccatcccggataatcaccgttcagcattgcccaaaactcatcttcctcacgatcgaacgtgaagatgtatttaaccgttctagggtctttctctgggaaaaaggcaaaatataaacgtttccagaatggatagggtttcatagtggcgtcctcaggtatgcggccaggtcataataaacgcacggactccagccacgtacgggcatcgaagccgtggttgtaacaggggattccacactccttcgcatacttcacacccattgcggtacctccggtcggattaccgtgtttatccaatggggccgaataatagaccgcgtctaccggtgtatccagattatcccccataatgatgttcaaattgcgcccgtggagcgcccaggcgaattcttttagcttatcagggtaagagtgtaactttcgtacgatatcgcggtagcgttcgtcctgtgcgattacacggaactccacattaggatgtagacgaggtagccaacccatttttttatcgtcgggtaagtaacagatgaattcatcatcccacacgacctttttgccggtgtcttggtcgtaggtatttgcccactgttgggcgaacttgaactctagctggtctggccctttccaacacccgccactggtgtagataatcttgtagcctttatggtgaagcatgttaaacccacggagtaacgccatgtacatttctgccatggtgacttcttctgtttcccgagaaccgattacagcgacgcgatagattttggtcatgattgacacctcctatagcaatcaccggtgacttaaaaaataaaatgatctctccccgaagggagagaaagccactcagtaactataaagtgggtagcgtgcggtgatgttgtccttgtaagagaaggtcaatatttccgtcacgactgaaagtttatctggaaatggtccagacagtaccacatgtatatccttttggcaggaacccgcatcgacaaactgataagtcttgcgagtcaggttaaccagatagaaaccccctgcggggcatttctctgatcggcctgtattcacgacagcaaacccgccatgttcggctaccgtggtgggattatccaacgcggtaaacttcacacgaacatcccccggattagaaggtttgaacccttccatcacgtacggattaaagtttgcggaaactgtaaacgaaataaccgttaaaataaaagctgctacaatgcgcatcatgtttttttgtcctcttccatatacggtaggagccagtcctgcccctcaagacgcgcaaacatcttgcgggttgcaggtgaccaacgaagttcgtggtcgtactgttttttgaattgatgccagtggtacgtgaaagaatgagtacggtatcccgcctctttaagcacttcttcccaatcgaggttcttaatgaaatcgtcaatgaccaacatcactaactgtttccaagcgcttcgacggtaatgccaataaagtctttgctttagttcggcataacttttacgtttactggaccgcattgccggtatagtcttataaggtttgttctcgcgatgttcgtcgcactgcgtaaacttaaccggcacaccccgaagtgtggacgcaactctgtccaccgccgaggcgggcacgatttcagcgcggcaaaccggctttgattggacatcgtccaagcaccgtgtctcgtacacaacacgtaacattgttataatctcgcggctagaaattaccttccgccatcgataaaaatatcggcacgttcgtcacaaacgtttctaagtgcttttcctccggcggcgtatgtacaacgacgatgttattcgtcatacgatgatagcgtacattatccaatccaatcaccacgccatcaatagcgaagccgcacttgagcaggaaacacaatccatcgacgttcgatgggtggactttcgttgagaccaccgatgacttactttccaacacggcccgtttcagtagtgcggtacccacaccgccccggcgtgactctttcggcacgtagatgtaaagtatctgaccatcggcataggccatgacacccatcgggatatcatcctccaccgccatcactacccgaatggattgactccggtgttcgttctggtcatcaatccatttacgcagggcggggaataaatcggcagagaccttatcaggactcacttcaatgtagagcataagcatctctccaaaaagtcaaggttagtttcactgaggaaatcatccgtagccaccgtttccatcagttctttaattgtccgatcgtagacttttttatccccaaccgtatcttgaacaaaatcgtagtacgaagatacggacatctccttcatgttaatgacgggtcgtaaccagacgacgtggacgtactgtttatagaaacgataagagacaccgtggtcaaatatctgtgggttgtgtggccatccccggtctgcaccgacgtctgtatattccgatggtctacggccatacgacacactcagtgctttgtcgacagcatttgcaaggcaacggtaagcatatgttgcatcgtcgctggaaacgagcttacagagcgttttaagtaagtctcgcgtttgtcctgtgtacggtgtgcgtttcccgctgtaacctgctggtaaggtgcgataatccaaccacgatctttcttcgagcatactgacaaccaacttctgacggtacgcttcgttcaatacaacgttgggtaatttcggtatcgcgttcagcagcccggtacttgggatgagcaccgtgcgtgtacgcatctggagtagattcatgattgtcccctaattgttatcacataaattacaactcgcgtattaaagcaaaaaagaaaaaagacctcgccccgaagggcgagagacttacgacttggtggtggtcgcttttttctggagtttcgcctcaacgactttagctgcaatcgtcatcgaactgtacgccagcgttttgattggccaagtgcagaacactgccaaaccaaacaacggggtgaggcccacgatagccacatccagcgagtccatttctggcgtgtgcatggtgtagtacgcaaggtaccccgcaacagcaacggttgctaacgctaacagaaccacgatgaacttcacaccccgaccgaagttcggccaaagtgtcatcatggtttctttgccgtacttcgcatccagcccctctacagcaccgactgcgcgctgttcgaggttatccgccaactggccaatctgcgcgattaacatcggacgtagagtagcaagaatgacgctggcaggcttagtaacatcgatgatgtctgcgtgcccgagagccgcagccgcgtctttcaccttactggcctcgtcaagactgagcttgttggtgcccgcttgaataaggacatctaacgcttgtgcggtagcatcctgttgagacagtgacatggttaaccccttttccgtttacgccgtcgtttggaaaaggagcctttcggtttcttctctttgggcggcaggagactatttaagttgagcaatgaaagcctcacgaagatgttacacacagcgacggcgtcgttactgtgctcgtccaaggtactgaggtcgacaagagtgtgattcgcgtacagtttttggactgcacgtttcatgtcttccttatcggtacctcgggcttcaacaccaacataagatttcacaataatagggtgataaccgtggatgactttagtcggaaagacgcgccataaggaacggcgtaacatcaattgcagttcaacaccagattcataggcggacagcttgccccgtttcatgaacggggtttctgttgcgaggaacgttggccgagctaaccgaaggaactcctcgaataacgcttcgagttgtatcatgcgggcatcacgtcgtcccaccgtttctccaaacgaggagtcgtgtgtcgggtctttgacgtgcagggtttctgcccacaccacttcagcttgctcggtgccgtattcccaatccagaaccgccagacccagatgtgaggtgccggggtcgacacccacaatccgcaccatgttatccgggagacgcggttcaggtatcaacattacgcctgtcccagatagaacggcgctggttgacccacacgaatcgtcagccctagctggtcgttggtttgtgcaaggttggtaaagagactgatgtgatacagaacctgtaccccaatcgcttcttcatacgcaaacggtgacccggttgcagactcgccgctggcggtgaagtctacgccagaacacagcgcgatttcagacacgatagcagaacctgcatcgcccagcatgatagcggctacgttcaggtattcctgaatgtcgaactctgtccagttgataacaatgtcacaacccgattggacataacgcccatctgggatttcaaccgtactgtcgtcatcatagtcgtagtctggcaggtctttcggaatcgggttcaggtcgctgtctttatagacaaaatcttccgtcttcggcacgccgttttcacggatcgtttcgaggtcggtcgtctgcactgaacgcatatccagacgcttcagataatacgcccaatagttacggccttcgacattaacttgggtacggaacgcgtaatctttacgctgctcatcactcaggtcattatcgagagtacgcaacacgaacggtacatggctgaacatacccgatgcagtaggactttttgcaatcggcacaaaactgtcaatggtttttaccttgacggatttgtgacctgcgtagccgatggacatgtacttcagactggggcgtaccgttggatcaggcagcttaccggtcatcagtttgaaaaactcattgagcgttgagttctgtgggtactttacatccgcaccacaaatcaacgcacttgctaaacgcatggcgctaagtgtcgctgtggacaacttaccgtcatacaccttggtattagccatcgaaaaattctcctacgcggaatccgtcaagtttgtatttcgtgacgaggtcagttaacttacgtggggtcgggtcaacgaacttaatatcaatcgtccctttgaaagcagggtgatgcggttcgatgcgagcgacatacgtggtgaattcacccggtaaaggttcaatcaccaaatcgtacggccccaactgtaaacctaactcgtcaatgatgtaaggaacaaggtagtggctccacgtaatacccatcggaacttctaccacgaccccttccaacagttcggtcaggtcggcacgggtaagatggaactcctgaaagcccattaccccgtttttaaatcgtgccgcgattttagattcgacgccacgcgcgcgtcgttcttctttcgtcagcggccatgcaccacggctgttgaattcaacctggtctggtctataagaagtaccccagacgtagttgatgcgattcaccagtatttcgtggggtggtttcgataggtcgatacgatacggcatacaatttctcgcttatgtcaacagactagaaatactcacctttgatgaagccatcgagggcacgtttcccaatcttatcgctcaagtaggctttgtcttttacgttttcagtaacgtccacgcccactaacggctcagaaatgttaaccacctgatgctgatgcatcgtaacctgaatacccatcgcgatgtccatttggtatcgcaaacgacggggcgcttttaaggcgacgatgtcgggcattaccgcaagcggtgttgaggtggtcatcttcgacttcacagccacatcctgcaccccggtatggggatggtcaaccgacatcgacgcgtgagcagatgcaggtatatccccaagaatcggtgtgataggatcggtaatgtcgtacgagtcagatgccatacgcgccgcaaaatggatggtgtaagatgagagtttactcatcagtcttaccatcgcacgctgaatctcaccctgagacagaaccgctcggttctccatgtttgttgcgatattaaacgcatcggttgcaatgtcctgccatgtctcattcgaaattaacgtgtggtcaattccgtacgttctgaagaactcttcatagtccgtatacggcagagctaaatcgcaacggtagctgcgatacatgtaagtaaacaattgcaaacccgctgcacggtcgggaatcttacgacggttataaacataactgtagcgcttacgtttattatctaacatcgtagaaactgcatcgaacaactcatcgttgctggtcagcgtcccgatgacctcgtactgtgtgtcagcgaaatagtttaccataccatcgtaacgcccaacccagctctctgggtagattgcgttgtgcatctcttccggggtaatccagcgtttaatctggacacccatggcatggaatgccgggatggtggttaactcaatattggagaaccctttgaaccccgcgtacaggtacaacgcaaacagctccttagatgagagctttaacgtgtccccgttggttgggttaaggatgtcgtggtaaatgttatacttgccactggccgttaggtgtagccactcattaaagagaccgtgcatgtattcccaacgctcaatggcttcggggtcgatggcggtcacttcgacgagtttcgtggacaggttcggatactgcgtcagacccagccgagtgtctaagtctgtctggtactcaacttggtgctggctgttttcagaggccagcgacaactctttctggataaggtcagcggttgcgactaaatccaaatcacggccagacgtacgctctgtatagttcagagcttgctggtaccctgttggttttggtgttaagtcatcatccgacccggtggtcgggtcatggattaactggccaacattgtacgctacggcaggcatgctccaaccggtaaggagggtttccaccatccagtcgaagatttctttcttgccggagttgcgctcccaataacggatgttgcggtacaacgtgaacatctgtttctgagtcaggtacggaatgaactcgtgcagctcttggtgcgaagccaagaactcggtgacgtagtagctgtgcgtttcaacagtaaactgcttctcctgtcgcagctgcatgataaaggcaggcagcatagggtagagcatgtcgtagaacgccagcacgaacgcatcgttgtgtacacgccatccttgtgcaaaatatcgtacgtgggtagcacgaatttttgcttctaaatcgtgaatcaatgattgctcttgtgtctcgacatacttcaagtcgtagtacatgatactgcaatcatctagggatatggcccgctccaaactcacaggccaaaagacaccttttatatagaccgcgtagtcgggatacgtcgcgatgaggttttcgatatactcggtgttggaacgatagacgttcgaggttttcttatgaatagccaagttggccaccgtaagctctatttcctcgccgctttcgaccgatttaaatagaatcggtttgtcgatttcatgtcgacgacctgccagatgcaggtagtaccgccacgttgtgcggtcattcgacacataaccgccattctcggttatagccagattcatctgctcagcaatggcttctgatttaaaaatcaaagacatcgccaactggatggactggtctctaaagatattgaacctctgcattttccggagaccccaatggacgatattagtaagttacaggcgcgcgacccagcagttagcgccatcctgcgcaaggcaaccggcccaagcggttcgcaagagcgcggtaagcgcgaggagggaggcaccacaccaactcgctcagaactgacaggtatcgccagttcgcgtattcgtacagcgaagaacgcacagcgtatctatcaggcattgcctgaactcgaaacgattgtcactatcgccacctcttctctgttgtcgtcgaaagacttggtgaacaccagtcttatttacgattgcgtagccgatatgcctcttgacctgcgtcaggagatggtacgcatcgaacgtgagtttcacgacaacaaacgtcagctgccgactaagctgtacaagtggatttacgatgcccttaaattcaaaggtgcaacgccggtacttctgctctccgactcagggtttgataaactgttcgggttggacacaaaggtcgcacaggagtccatcaagaaccaacgtatcgatttcttcaatcagcaacgtggtatcctcggtaagatttctaagccggatgagcgtaaggttgggattgaaagcatactgaatgggcgtacgcgtcctgacggtccgcagaccatcgagattaaactggacgcgttgttcgattcgaagaaagtcagtgacatggcttctatcaaactgacgctgaccgacaaccccaacgttttcttgatgccggaaactgtccgccgtgttgctcgtgagaacgcttctgcgtccttttacgggcagttggaacagactgcatatgaaaagcctcaaacgccaacaggggcaggcaccttcgaagcagacgggttcaaagaaagccaagaccgcaaatacgatggtattaacatcgcggacttaaacgaaacctatcgcaccacaccacagaccatgatgtacggtgagatgcaaaagccaatgatggatgatgtgaaccacgttgagtacaccgagcgtgtgcttccggcggaatccacattaccattggtgttgggtgatgacgtgatgaacccaatcggctatctggcaattgtcgatgaattgggtaacttcatcaatgcgcgctcatctctgtacggtgatgcgaacttcatgaattacctgaacaatgacggaatggtggactctatcattaaccgttctgccatcgggatgggtgaaggtaacgcaaaagtcacaccagagattgctaaccgactgattagtcgtttcggtgagattgcagagaaccagttagcggttgcattgggtgatgcgctcggtggtgctgagctggatatgaacgtctccgaaactttcggtcgtatcatgttgacgcgacacttggcaaaacgccatactcaggttgtgtacattccggctgagaacctctgctacttcgcgactgactttgatgaagacgggtttggtgtgtctatcaccgaacgctctttcattatttcatctgtccgtatggcattgctgttcgccaccatgaacacttctatcctgaactctgcacgtcacatgcagtacgacattcagttgtcaccggatgccatgaacggggaagaaactgttgcccgtatgaaatccgatatcctgaactccttcaaccgtcgccagccgatgtgggggaacatggatgacatctggtcgatggctaccaactcagggattgcgttcaatgttgaggggaacgattactacccgagcagcaaagtgtctgtgtctgacaccacgcccgactacaaagcgccagataaggaactcgacgagcagttactgcgtcgtacctgtcacatcgcggacgttgacccggatttggtactgacaccggataacattgaatttgcgtctcaaatcttctccaagtctctgctggttacgcagaagattatgaagaagcaggagattctgcaaaagccgctgacccgttatgttgtgacgtctacgctgtcttcaccaagcctgcaagccgaactgctgaaagcctgtgtggagtacatcaaagacaaagaaccggacacaccggaagatcagtatgtggcgaaagcctccatgtacatgcgtcagtttatcaacggtatcaaagtcacactcccaccgccagatacctcggcggcctcttcacaaatggaactgttcgacaaacgtacagaattcattgagaagctggcagatttggtagtgaccgacgacatcacacaaatgatgcaagatgcgggtatctcgctggatgcgagcaccattaaaacgatggtgaagaacttctatgtgcgtacgtggctgcgtaaacaaggtatcgagaatgagttcttcgacctgatttacgataaagagaaacgtgcggaaactgtgaagatgatcagtgatgaaatccgtgaagcatcgaataccatcatgcagcttggcaaaacaacgtctggtaagattgagacgttagcgaagcagcgcgacatgggtgatggtggcggcgcaggtgactttggtggtggcggtggggataatccattggatgacaatcctttagacgataatccgctggatgataatcctgacgataacccggacgataaccctgatgacaatccagatgataatccacttgaccctgataaccctgacggcggaaacgacgctgggaataatcctgatgatgtgggtgctcctgatcctctggatattaatccggaagacgaaacggtctaaatagcaaaaaaaaaataagtagcacaactcctaccttcacgggtaggagtttgcttttttttaatcgcccgattgtgcgggtttgccgatttgttctttctcggccaacatgatgccaatcgccagagggtctttctcgtaggcttttaagaatgctgtagtctcctttacctttcctgctgttaaggcgtctgtgagcaccccacgcacgttataatagactgtccagcgacgaccaccatagatggctgtcttggttccccgaaaccgttccatgaacgcagttgtcgctacattgtcaggcagctcgaaccgatgcaacacatcccggtactgatttaactcgattacaagcaacttgaccatcttacacctcagtgtgtatcacgttatctataataatcgtgagtaatgaaggtaaaatgggggtcgagtgtatggagccgcgccagtaggtacgcattacttgtcccacgcaggcaggcgtccaattctttcttgaccatggaataacgcacggtacgcttgttattcacaaccgatgttttgtgtttgtcgcacgcttcggcgaacttagtcatgactacaccattgacgttgagatcaaagtcaaacagtttcttgccttcagaattcagaatgtcgacggttaacattatttttcacctctgataaatttatccatacgtctgaaccaaccaatctcttgaacaatccagagaacagcggccaacgccgccagtacgcaccaacctaccagaaaccattttgtgatcgggtccatgtagcactcctgcaaataaaaaataaaacaaggtgacccgaaggtcacctgtttgtttcagttagtaataaatcggtgcagtgttttcgccggtgctgagcagcagatatgattcatccgctttcaacacgacagacacttccggtttcttacgcgcaaactcttcgaagatagtggtcactgggtcatgtgttgcacccagagaatgtttaccgacgacgttgttgcgtttcagtgttgggtagttacccggaattacaatctctgcgatttcatggcgcacgataagctcaccggaactgtaacgcacattcactttgcgcagggatgaagccaccatcatgaacagctcacggaagaagtccggttctgtggtgtagccgttatcgccaacggttttctggtacaggatgtcggagaagaactccaggtcatccatgttacgctccagctcaatccgtggattggttgggatgttctggcaacggttagtaccgaggctcagtgcgttgtgtaccgcaatggacatagtgcccagtgctacgttggtgaagcgtgccacttcggaagccacgatttctgacgcagcaccttcacgcagcatatcggtgtagaagttgacaatgttttctttcatcttctgtacaaccgaagacaccgcgttgatgattttctcagggtcatccatcccatagagatcatccagacgggccaactgagattcgtgttgagaagtgaactctgcaatacgagattcaaattccgcatctttcgttgggttaaccagatagcgacgtgtgacacggttagcacgcaccagaatatctgcgcccgcgtaatacaccgcattggtttttccagccagtaaatcagccagagcttcaacccagttaccggtggtcaggaactcgttgactttctcattggcatctttcgcactgatggacacacggctacgtggcgtggacagttcatgctctgcgtacgtttccaaatcttctacctcgataatctgtttaaccggagcgtttgacacgggattcacctttggcgcgggttgttgtggtgcagcggctttggcggctgcgggagtttctgcaaacgcctcaagcggcgcggcactaactgcactgagacccggactggatgtcgtcggagttacggggataccatcgccaacctgaatcccacccaaatcaccgataggggaggacgtcactggcgcacttggagcaacggacaaacttgcacccggaattgcggtaccgaccaaaccacccaaagtaccactggatgtttgagcggcggccttaaccatggcccgcacctcttggaagaacttgttcagacgttcatgtaggccagggtcgctttggaatgcgataccggctttctgcaacagctgataagcagcggctttgtacgcagaaatgatgttctctacaatcttgtcttgacccacgcccttagccaggagtatgtcaccaacctgaattgcgatatctaacgcgtcctgtgcagcgatattgcgatcagaaacagcttggttgatggcagtaagcgtcgtgtcattgccagccgctaaacgactttcgatgattttcacgactgcactggatgaaattgccattaaatgattctccttaaagtatacttatcggccgatttgcgcgatgtcaatctcggcggcttcgatttctttcttcagtttcgggttacgcatcatcacaagctggcgactggttaccatgtacgcattgaggatgttggacttgaacggtgcagacttcggaatgaagtgtacgttgccacattcaaggtgcgatgccgaagcatgtttggtacggtcgttaaggttgacggtcttacctttcttaccgcgtttactgtctgtttcagtttgaccaattgcgtgcgtcgagaccgccagtaccatcgattcagtagacgcattgaagaagttgatgcccccattcgacgtgataccacggcagacgaggttcggtacaatcttcttgttcaattcatcacgaatggtttcgtggcaactttcggctgtccggttttccagttgactcaaccgccaacggatgttggagatcgtactggtgaaccctttcggtgcgagcaacagataatcggttacggttaaccgcttgccatacatggatgagaagtcatcctgtttggtcaaacgtgtgcgaaccatcatcttggtggtgtagtacaggaagtcgaacatatccatttctggatcgatgtctgggtccaccgccatgagttcagcacggaacgtgttattcacataacgctcacactccatgaagtggctgttcatgcttcgcagcaaatccacatcagaaggttttgtaccctgaatactacgtcccagaatctccttccagatatccttagagttcaggttggcaatgtcaccatccacatcgaattcgtttatggaggtaaacagtggtgccaatgcgttacgttgctgactccgaccagtgcgacgacctgcgtagaaatgggcagctttgtagaaagccgcacacattgccagtagcatgtgttcgttctgatcccagcgtgacttctcggtgctcggtaaatcttcgcgacggacgacaattgcatactggatacttttacccagctgcggttcacctgattgcacaaccacgtatttattcagatcaatagatttgagattgtacgatggccagatagcaacgcgtgcgcccgtataacgctctacagcctgcttgaagccgtacttaccgaacaaccaatacaacagaggcttctcatcggaatcttgtccctgcgtcgttttagggacgtagaggttcgatgtacccggcaggaagatttcctcctttttcccgttgaccagaatcttcactgactgcttacagaatttcagtgagaccttacgggtgaagtcgaagttaatgaagataccgccatgctctcggcagatacccggttggtgaatcactggtgcaacgtggtacaaagtaccccacgagtacatcaggccaccgcgacgaataaacggcagatacattggacgggcagtaagtcggttctctcccggtatacggatattggccatgatcatgtactgatcggttctggcaatggaaacaggtgcacgaccccgtgcttgacgattgtctgcctttgccaccttaaagataaaggcttcgaatggtgacatgaaacgatattgttgcaccgctaacccgatgggtaaacgtgggttggtttctgcatcgtacgtgagttcgcgcttcagaatcccgtacacccgttcatggataccatcctttgcttgtgcatagccgacgccttctgctaccgcgcggttaaagggaacaatcttacctgacgcctttaactgttttatcgcatctgcaaacacacatactctcctctcacataagcatcgctacgatagccacccccgctgctaatatggctgggatagctttcaatgtttcagacgcgtctttacgtgtctgcgaacggttttcgtaatgttccttacgttcatccgattggtctttcctgacagtcgaccgttcgtcgtaatggtctttacgtaatgtagaccgttcatcaaagctgtcttttcgttcttctgctcgctgtttaaccttcatctccagttccctgaagagggcggcctgttgctcccgttcgattgtcatttcgttaagcttacgtctatgctcaacatctaactgttgtttgtgctgggcatgagacaagtcattggcagcgatttgcgcctcgagtttatttctgagatcggataatgcaggcaccgcatcagaaacccatctaaaacgacgggcaccttcttctgtttcaaatccccgcattggcgacattgggtcgtcgaagtcgaagtgtagcaaccgacttccctctacaatatccccactcatcatcaccagatacattcccggttcgtaaaactttgccttaatcggaactacctgaaccatcgtgttgtagtaccgcacccactttattacgcgagtgtcatcatggcgttgtaccacaacaatacctaacgtcaattccgttgactggccagtacgacgtttcggtgttttatctaactctaatgggcgaaccgagaaggataacccaaggttctctaatacaatagcttctccacgtaaaatgggtacgggatcttccacgatatacatcaacgtggattcaccaaatctatccagttcacggcacagattctgatagacaggcgcaggtaaggtgtctgcgataccaatgagattcgccattcccgccggaatgctgtaagtgacatacaccacgatagcgttcggcgagataacgtttctcttaggctcaatgataatgtacgaccctgttgaatccgtaacgtagactggcgtgccggtgttattctcgtaagtgaaagttttcctgagggcgttatgccgaacaggtttcttcgagatgaccggagcgatatccagattatgtcgtttcattaattacttccagcttcaaaaccaatcgtcaattcacagagataatatctatctcagaatgcgtggattcaaagaggcacataggctatgcctctggtgtaaaaatgttacgggatcaggacttcggcgagtttcaaaagacggcttttgtccatcttagcgacatccaatttacccaatccgagttctaaggtcagcgtatagccatcggttgggaatgttccagtggacgcgatgctatacagacgatcggccatgttgatgatttcgatatctgtctcgacaaccggactatccatttccgcataattgcgctcactgaatcgaccttgcaaatgatgatgtccgtgtggggattcaacgaactctcttcgcaagtatgttaccatcccatgatcggctgaaacgattagctgggtatctgaacccttcgatggtgaaataaccgcaccttcttgtccccacggaagtggttgccaatcgtacgtttcgttcaacatcaaaccgttggctaactccacatagaggtcggctagttgttgtgcacgatgttcacgattgccgtaatccggggagaatagctcagagctaaaacgcacgttgccgagaaccagatagtcggtactaaatccccaaccatcgtttttctccgctttctttttctgttcggcgatataagcgagtaacgaggcgtgcgcatcacaacttagataaataggtgtttcgatatttttcaaattcagccacatccggccgtaagatacgttagcgaactgaacaatataaccgcgaccattaaaaagtggggtaacagatttcacccgatcgaaatcaacaactggcatcagatcaatatccacgataatactccttataaatgaaacgattgtctcttcccttagataatatctatctcaaaaattttagacaaaaaaagaaaagccctactcccgaaggagtagggcattccgcatcagcctaaggcttagcttttcggagcagtggtagaagtaccagcgctctgagtggtagtaccagaggtgttcgcgtcaccagctacagcgcctgcgttaccgcctgcggttgcgccgtcgccactctgagtggtaacaacgttgtaagccagtttctgctcaaccagtttggtgatacctttaacccagatcagaccagtgatcgggcaatggcagatgtgcgcgttacgaggctgcacagcaagttctttgctggtagaaccgttacgctggatgttgatgttggtaaccatgatcggagaccagaagtggttaccccagttcagaacacagtaagaaccatcttcaacaccgtcaactttcagaacccattgcagacgacgagtccaagaaccgtcagcctcgttcttgatgcgccagcggtcatcgttggtggtcacaacttcgtagtcgtaacggtcgcccagcaggcgagtttcaccaacttgcagcagcagcattgcagcagtaggttcgtcagttgcaatcacaactttcggtacagcttgtgggtttgcagtcaacagacgcagagcaggcatgtaacggctatcctggatagcacgagttacctggtcagcgatacgttgcagcagcgcctgacgggcgttgatcagcgcgtctttggtttccagagactggacgatttggtcaacgttgaagtcgacttcttcgaaccatggcgcaacccagtgacgacccagaccacggatagcagttttatcccactgcgtaaccatagtggctttcgcctgcttaaccgcatcggtgtaagacagggtctgagtgatggccagcatttcgttacggatgttaaccgcagaaaccaggtcatccagacgctcagcgtcatcgtactcaacgccaactggctgcttggtcatgatcggagaaccgtattgcagcttgtagttctcttgttcccaaactgggtccagcagcaggccctgagttctccggttctcgttggtacgagtaccgtcgaagcgccagcccagcagttcgattttcaggttgtccatgatggttttaccgataccggaatccatcgacacttctgcaccagttgcgtcaaccagatcttcaacagacaggttggcaccgctgatttcgtactggccggagcgctgaccgttggtgaacaggctcatggtgatgttaatcacgtagcgcagggtgtacttgctctgtttcagggcagacagcgcagggatgtcgtcgcctttataatccagagagtcgccgttcagtgcgaactgagtacgacggaactggaggaccagctcacgaccgtcaccttcaggaggacgctggaagcttgcgaactgcatgtcgcgagtgttcaggatgattttcttaccagccttcacatcgtcgcccggcttacggacagaaaccagcagcgagcccagtgcagcacccggcgcgatttcgtcagtttcgtcgtaaccttcagctacgatacccggatgcgctgccagacggaacaggttgcctttcagcttgctgatgtccagatagttagtcgggtatggcggcacgcggcccagacgcacggtttcgttttcgatgatgtcatcgctcacgaagtattcggcgttgtcaccatcttccatcacgtacggcacgatacggatagcatcgtcttgcagcacggtgtggtcggtcagcgcgttgtgcagcggcttacgatcgtcaatgacgctgtctttcgccagcagcgcgttcagaataccacgggttacggtggtgattttggtacgcacggtgataccaacgtcgttggtgtcaacagtgatggtcgggaacagtttctcagcgaacgcagactgggtttccagcgcgcggacgttcagagtccaagtcagacccaggtttttatccagatctttgttggtgtagtattcggtcgcaaccagcggcgttttaccgtagtcagcgttcagggaagcttggccagggatggcaacttccatgtagttgttccagcgcttgtcagcagattcgcgagcaggcttagacatgaactcttcttcgttgcccatggcagaaagaatcatagcagacgcaacctgcgccgcgtgagacatcttcttaccaccgtacacggcagagtatgcctgcccagcgttgtctacagcggtagagaatgcgtgtgcgttactacgaacagattcgccaactgcaacagttttccacagatccgcagtggtggtgccaactgctgagttagcaaccagagtgttgccttgctcaatcagtcgctccagattggagattcgagtttctttcatttcaagttaccttgtgtgataaatgacatgcgtagagttgcgtcagcacttcatgagcagcaaactgcgtagacgtgctgaatgaatcatccacgacgcgagtcttggtacgcacatatttaaaaagttctgcgcagaacgtcttcttcgcggcgcgttcgtcgctgagggtgaaacccggatgtccggccttcgcttcaactagagacgccactataacatcgttacgttggacgaaagcccagcgtaactgttcggtgaaaggttccccatataaatcggaaagggactctttcgaaccttgtctaaccaagtcaaacacttggtcataatatttaactggaagcagcggaggtgccatcaacgatttgtagatggtttcacgcgagcagtccggcaacagctttgaactgaacgcaatgggagcacagtcatataaccagttaaagaacagcggttggagcaattccaactttttaacgctggctactttatctatgttaggttgaacttcccatgcagggctaaaacgaattcgcattgaaggatgctccatgaatagtaaaatgatgttgataacagccttagccgccttatacgcagagagccttctgtccgagcccgataaagatcatgacgtcataagaaaagtgctcaacgaggtcaaactccccgattacgtcgaagaaggtgacgagcgctcggcgttagctgaaatcaaagacattataacatcagtcatcgacggtggtatggattacaaccacaccaatgtcatgaagcgcttgaaactggctaccacgcaaacacgccctctatacgatgtgattgtgaaattcatggatgctgaggaattgccggaagccgaagaagaacgtgtcgactttctgaacaaatctctctcccaatattatttccaattgcgtcaggcaatccaaggtgtgcagttaaagcaatacctcggtcgtacactcggcgtgctgaatggcacagaaacccgtgttgacctccagacagcgctgaaagatctgacgggatcaatggccacgttcggtgaacgttctcataataagattccttcacaggtgaacaagctgattaccacagacagagcaccgtttgtgaagacgttcagcgacattaaccgtaaggttgccggtaacggtttgaagaccggttggaaagccatcaatcaaatgatggggtgtaacaaagggattaccgaagaattgtggctcatgcctgcgctaccttttaactgtaagtctctctttagtctcttgacggctatctcggttccgctgtttaacacaccggaaaaagtgatggcgaacgtgaagggtaatctggctccactgattctggacttgagtctcgagaacgaactggacgtcaacatcgcttacgcctatcaggctatctacggtcatttcgaaggcactgcgccggtaatgactctgcctgagacggccaccgatgaagaacgtgctgcccacgttcaatccatggcggattacctgattggtaagattcgtgcgaacgggtgggaatactcgtttgagaaacacacgaacaccgacttcaaagtgcattacctgaatgaccttatctccggttacaaaaatgacggcttccacgttgtggggattcgtgctgattatcttggcaccatcaacaaagcaggtcacggtaacggcatcgcaggtagtgacatcaaagagatttaccgtatggcccgaaacattcaggtcgtgcgtaaccatggcttcttgttagcaccgcaccagatttccccagaagggaaacgtctgaaagcggtagacccggttggtttctgtaagaacctgcccggacgtggcttgtacgacaactgtacgagtctggataacgaagccgatggtgaggtgtacttcaacaagcgtgtggtcaatggtcacagcttcttggaagtgcaacgtggaaaacaccgtaccattatcgataccaatgagaaacatcattacactgttataccgtttgcagacgttggcatcctaccatgggattgcgacaaagagatgaccgtaacggcatcctctatcaaccactttaccggtggcatgggcgacgatttattctgagcctaactcagctggagacttcggtctccagcaggggcagttatgtgtcctgccgagacaaaaaaataaagcatcttactatggtgagatactagccggtgctcgatacaccggctaggttaattatttcatcgactatcttttgttgaaaatgatgtcacctcctaaccctttggcgcgtgagcgtggtgcaggggtacgttgaagttccgccacacgttggttgaattgttcgctctgtttcttctgggcgagcaggtgattgacaaagttgttcatattggtcactccggtatgattaaggttactccccgtgcgtggggagtaaccgacttttattttctttgcgaaaataaataaataccccaacctccgaagagattgggggtacagctaggcttcgagacgtgagtcacacaactcgtcggtcgcctttctcaggttcgcgactaattggggaaacacctcatccgcctttttcaatgcggctagataatcagcaatagtttcatggggaacgataaccccgttttccagctccagacctttatggtgagaccgacgaaatggtgagtagagtcttccgtaccagcagtataccctgcggtagcgtaccacacggaacttgtggtcgagtgcctcatcccacagacaacgaggttctgtgaggtggtatttctttgggccatacaggaaatctttaacgcgacccatgcggtgacgacacttaaaaatgttacctttaaacaaaaacgttaatgccagtaacagacgactctttcgcattattcatcttctccttctttctcttcgttaacaggtatggattgcagcgggaattcaaactgcgacataaaattatcaaccttatcacggctgtcttcttcaaaccccacatcgacgtatgcggtcagttcgtaggtaccccctttagcagtcagcttgtagcgaatctcttcgattccccacagggtcaccacgttcagtttgacattctcgtactgggccacgatgccgttgttatcgaatgttgggcaaacatgatacagctcagacaacagcgccaacgcatccagcttgcaatcagacgcgttgtgtgctttgcgcgggtcttcttgcagacgttgggtaatgcgatcatcgttgtagaaatcaaccgtattggtcaggctgtacaacgcaaccattttaccaaccagcagcgcccggtcagcgaacacaggggtggcggccatcagataagatgacgcgtagctcagtgcggtatacgcggcgttacgctcgtcgcgttgattgtcttcatcgcgagggtagtttggtttgctaaaggatacgccggaaatgacttggcctttgtagatgaccacgaaaactttgtcttcaccgttcgggtcttcagatacggcaaggcgaatgtcttccacttccgaaatcagtttagggtcatggcgaagcgttggatagcggggtgacaggtcgaagcgattcaataatagggtcatcttgatagtccttgtgtaaacaaaaaattaaggtagcccgaaggctacctgttggattaaccacgaccggtgcacaggttaacggagtttccgttagcgcggcaggtgtcgtagtcattagaaacggataaatacagtgaaccgaaagccatgatagcaacgatggtcaggatagcgcgtttgtgtttgaacatgatgtattcctcgatagtcgattagagatggttattgattaagaattgcgaaggcgtgccatggcatcggacaggtttttgtctgcggctttaccacgttccatggactggtctaatgctgcggtcgaaacgcgcagttgctcagactgatggccgtgtggattggacggagagattcgagctaagtgtgcagctttaatacgttctaaagtattcataggtaattcctgttgtgtaattagataaagaatattgtacaactctcacctaggtaatatatatctgagattatttttagtgcgactgggccaatcggatgacagaaagcgccacgccgtagtattccggcaaatctaagtgcattcctgttgacccatcccaacctttgaataatgcatcgtgaaaaccgatatcagtgtactgaggataatggttttggacagccgccaattggtttgcccacgcttgccatgcggtgtctgaaatcacattctcatccatccggtaatagataatcgaatggacaatcatctgcatacgcttgcggtgaaggtattcccgaatcttcatgggttcggtttcaaccccttcaataatcagagcgtctgtgtctgcggtgggaataaaggtaaacggctcaaagcggtgcgtggtggggatgttattcttcgcctttcttttactcatctcaattatcacgtttaaacgccctcagaagcattctaagcgcttgtcgcgccaaagacagtaaatgaccagcatttataggcaaacgcctacaaggtcattttaataagaatatccgaccccttgcgaggtcggaacatttttcttttattgccccatcacagtcatcggaggcacgtccatgacctgcacaccttgcagtgcactgatgacgatacgttcatcgctgataacaatcacggcatctttcgcatgaagaccatattctttcgccgcaccgagcgtacactcgttgtcatacggggtcagaatctgacatgggaacggcacgtaagagttgaacgtgatcagtgggccgtattgtagcaccgggaagatttcgttgacgttggtagacagctcacgcgtcgttgaacgagccacacaacggattgctgcgcgcattgccacggtgttctgcgggtcacgggattcgccgaccatctggaagcggaacatgttgaattcgtagtcaccggcatcgacggtatcctgcggggtgatacgctcaacatagcgcggataggttgactggtcaccaacgatgatgtcgttggacagcttctggccgtagaagtagatgtattcgaaatcatactggccacgcagtgcagaccaaaccgggagagtggtcatgcagtgcaggaacagcagttggcccaaggagcctttttcactaatcggcagctgacgacattgctccacaccattttgggtataaatgattgccacgttggcatcaaggctggacgccatgacgtacaacagtgcgatttcgccgtcacgcggtaaaaccttaacgatacgatcccagaggttcgacggtcggctaaagtttttctgttcgtgggcttcaatctcctggataagttggccaggtaggcggagggcgtaaactgagttcattacaaagtccttatggttacgttagcatagaacggcactatgctgtatttttttgtttccctaaccagagcgtgagttctgattgggtattgtggtttgctgtggcgatagatccgccatccagtcccgcttgaaacacttccccaaccacggtgccgtagcggctgtaaatgccgtactcattggcatacacatacttcaccgccattcccggcttaataaggccgtgtgcagagcggttccacgtcactttggtaaatgtgcctgtagaacgggccagtttcgcgcggagcggtttgtcgttgtcggtaaagccttgtttggccaccggcgcattcgtgaccttaccggcataatcgaccgggttggcttgcgagacgaacttatccggcgtggtcatactgacaccacccggtgtaaaggatgaggcacgattatccaatgcgcggatagaacccacgcgataacctgttccatggttcaacgcgttctcatcggttttcacgacagtgtgcgtatcgccaccggtaatcaggtagagcacccccggcgtgatatggatggtcttgtctatctgagcagccttttcacgcggcaagttatagatgaccaccttctcagtcgcagtgttgaacttttcttcgtcccacagttggtacaggtaccaacgacgcagatgctgatagacccccaaccctttgctgtagataccgtagcgttcctgtagcttatcaaacacttccataaaggttgtgctgtcaggcaggatgatgttacggtacagctgctgttcctctttctcgtacgcgagtgacaagacctcgccttcgctcgtcgaggcagggagtgtatccgttaagatagcacgagcaaccgttaacgcgtccgtttcctgatgacgtactttaacgttgcgcaaacgcaagtaccacatggattcgtccatcagttcaaaggtgacaaacgcaatcgccttctcatcggattggccagagaacatggtttgggcttccatgtccgggtcacggttattcaccacgatacctcggtaagcgtacgtggcgagtaaacggttagcactacgcagggtgatttgtaccttcaagtcaccgtcggcattcgctgttgcgatacgcatctgggagaagggcaccaccaaggtcaggtgcgtcagggttgtgaggtcttcgaagaaattcccggagtgtatcagggaatggacacgaattaccgtcaggggaatcccttttacggtaaccaccgcgttgtattcgacgggaggcaatccggccgcttgcgcgatgtggtagtttacaatctgttgaaagcgaccataggccattaccgtttccctccgcgtttacggtacccggcttcgatacgtttaatcagcgtatcgttaaaccggtgctgttgttgcgtgagcttcacttccccgaacaacgatgcgactgcatctgccatcgtggcttccggttttttaaagtaaccataccggtttgccacggggaagagtttgttggccaacacgttgaattcacgcagtcccacaattgggatgggttttggcagcagctgtggcgtctcgatgtgtttaatccagttcgccaaatgctccattatccagccgtacactttaatcccgtcttgtggatcgttgatgtccaacgcacccccggttgccagatactgggcaatctcgaaggggcggtacatcacgaactttttgttcaacaggatagcgcgggctttctgtttgtcctcagggagaaacagaccatactcctgcgtcgcatacgcggtcagggtagaatactccggtatacgccacccgacccacgaatggaacaggtggaatgccgcagtcttgttctgcgtgctcatgccttacctcgcgtatttcagcagtacgtacaccagtggtacgtaatagagttgcgcgttcttcggcagcttgtgaacttgcttagccaaatccaacgccagctttgtggaaagcggttgtttgttcaggtacaactgtaacgcatactccagcccagagctgtacccgccgttatagaacacatcggtcagtaagtacggggtgtacgttagcggtaggaagcccggcacagattcattcgaaccttccagtaatacgtcatcactggtaaagtcatcaaacttcggccactccgcaggcatctggcgaagcggggcgtcatcagagaaataccgggtcacggcaatcttcgaccatcccacattgttgtacgtctgcatggtacggaacgaccggaccgacagccctttgttcttgcggttcacatcttgcaggaacagcggctgttgcgcgataatcaccgtgaacaacgtttcgatatcgcgaatcggtttggtagggtgtgggtagatacgaatatctttgcccaccatccgcagaccgatatcacgcacgaactgtgctaagaacacgtcatacgcgtaaccgtaacggtcatccgggaaaaggatggtttgtgcatcctcattaaagaagcgtcgcaggtacgtttcctcgatccctttgacgtgttcaccgagtgccaagtacgcattgtactcattcggggtcagcagcgtatcgccgcctgtgtaggcgcgctctttaacgtaatagaactcatgtgccgtgcacttgtccagaatcgctttatgggcaggtgtcatttcaaagagcagggtgtactcgatggaatacgtggcaaccttgttgttcgagttacgtgttgttccggtaacgttaaagataccgacacggttgtcacccagagacgcggtgaaaatatcgttctcattcgggacaacagtcgtggccatggtggcactgcccgacatcgtgaaggttttgttactcccgtcttggtcacgcgtcagggggctgttaacccgcagttccagataatggatacagtcgtattgctggactggcgtgtcctgtttcgggtcgaacaacatcttcgggtcgttcttacccattaaccggcgataatacgccagcaacggccacgaggagccttcaacgaccggaagcaggttaacggcaggcgtacgctctaaatcgactaccgtggttctggtgggctctgtgacgatgttggttttttccttgacaccgtcctgagcttggttcaggtattcgggttccgtcttcaccggctcgaatgtggttttgcccttacccttcgcttgcagcattcgatatacctcgtattgcaatgatggtggtgttaaagacagtcagcagcaaatgtttgcggttggtgcctttcccggtttcgtcgttggtggttttgtcctcaatctcctcccacgcactcggcgggagagttggtaagtcccaccaccaatctgggaagtccagattcgggaacaaccatttgatgagtaactcagctgctttcgggtacttctggagtggccacaagtctaatccccgccaatcaaaaagcacggactcggtcaggaagtaggctttatgcacatccatttcacgggttaacgagaactcatcatcctgccagtgatacaggcgcggttctacccgcaaaccatcctcaaacagttcggtgcgaaagaccccggtcatacccgttgggtcgattgtccgacaatgttcgatgtaaggcagcagtaccgggttccactcgtacggcaagtcagtggtagacatcaccactgggtttgacatgttctcttcgccgaagcacacatccgtaccaaacatccgcaggagttttgcttcaagcggagaatgaatgcggtgcagttgttccggtgggcaaagcaagtatggcagacgaatcaactgacggcgttcgttctgccaccacgttccatcaaacgacgtttgtacttcactgcgctctaccccgtcttcgttctccatccatgggggatcgatttgtgggaagtacacatccggcagcggtgtttggttgatgacgtacgggtagacacacccaacctcttcaggacggtcatattcgaaactcgcggtcatcgtggcttcgtaatggttgtcttccttgctccatgctggaggattcacatcgtaaaccatctccacacgggttggggagtaacgcaccatcaaggtttgctgacccccactgtcattagctaccacgccaaccgcatcctcgaagtttgcggccagatactccttgaaggttgggtaaacaggcacgcgtgtttcagaggccacccaacaggcattcaggagattgaacaagggttttggaatcacgaagtacgcttccgattcggtcactaaagaatagcgacccatgtccaacaggctgttcaggcgatttgtccagcgtaacaattcgtcctcagacttggcattacgtcggaaggtgatggtgactttgtatttggtacgaatcggccatgctttgatgttgttggtttcatcgtggaaaaacggcagttcgatccctaatcccactccacggttaatacgcgccatttcgtcacgttcttcatcaacctcaacgtaaacacggtcagtagacgcgtactccacttcggttgcatcaccgagtgttgaaccgggttggtgggcagtgttaaacgagtctaggaagactgcgtcggatttgtccatccccgattcatttaataatcgatagacgatgccgtcaataaccgccttgcggatggtcacatcaagtgacggcacttcgaaatactgttgcatttcatcccctcaggccgtccacatggtggccagtgcttgtgcttatacatatcactgaacgcaaatgcaaaaaaaaaaaacagggagccgaagctccccacttttagaacggttcgtaaaccacgccagcaattaatgtcttgctgcgtacaacagtcatgttgtacgactcacgaatcaccgccgtgtttctgcacaggtcagactttaccatcactttagccgcctgttgtggcgtcaggcgaaggaagttgtacgccattccttcgtagagcgcgatgccacgcaactgcgtatcatacgggtcgctgtttaagcgcgtcaaaagtaccttaacgggcacttcctctttccccgtaatctcacgaaagaaccgctccagcgattcgttcatttcatactcgttcatttctgtcagagcatatccacccatcttaaaccccttctttatcccagatttggtaataccaatcgtgtgtgtgtttgtcaccgtctttcaggtaacgcatcgacatcgtctgttggaacaggttacggtcgatttccgggaagaacgcatctgcgccttcgaccgcaatatctacccgactcaggtagatacggtcaacatccttgatagtctggtgataaatttctgccccgccgatgatgaagacttcttcaacaccttcttcgcggcagcacagcaacgcctctttaatgctgctcatacccacgacctgtttcgggtcaccgccttccacagtcaggtcatccacacggcgggtaatcacatagtggtcacgacccggtagcggtttacggcctaagctgtcccacgtcttacgaccgaggataagcgacttgcccatggtcaaggctttaaagttggcgaggtcagcaggtaagcgccatggcagctcgttgtttttaccgatggcgttattacgatcagccgcaacaataatgctcaacttcatgattgtttatccttgttgatttctttaatgagttcgcgcaagtacgtggtgaatgtcctgcgggagaatgtaaacagctcgacactgtcggtaatgacggcggtagatgcggtgcgacattccacatcgaacacaataccatccattcgactattcgcgtacgtctcctttccgtagaacggagtagccagccgaatggtaatcgggccgcggtaatcacggacacccagttcgatgagtgccgcttctaaatcttccagtacaacgaacagcttaatctgcggacgggtaggcgatttgaataccatcaccggatggagaatggtttccatcttaaaagcaaagctggttgtttccaacatacgtgttcctcgataaacgataaaggtcaaaggcaataaggcagcttgtctgaacgacaagcgccgatcgatcggccaaagacataaaagggcctaccccctcgcataaccaaaaggggatttgtaaaaaataaagagtgccccacccgaaggtggggacgcctttttagaccggcgcattcggaacaggaacacccgaatactcttcaaagattttccggttgttgataccgcggtaggtcggtgagtcagcttcgtctttcgggtagatgatgctgatgtcttccgtaccggtcggtagtgtacggccttcgttgatggtttctttcgcttgatggtacagggctaagccgtcatcgcgcttaatcgatgcaggcagcgtcacacgcagcgcaaataccggacgccatgaatcgactgactcacgcaggtagatgtgctctaagtcgctcccgtaaatgatttcgtcatcccacgtataggttgaagggacatcggttggcatcggcaggaaaccttttgctgcgttcaacaggtcacggatacgctcacgtaccgttaccccatacggcggctcaatctcatagcgggtctcgcgagtaacgaaggccatctgttcctcagcatgatagctgacgcgtgcccacagcaggagtacgtagaactccagatagctacaggtgaattctgctttaccggacgtgaccgacactttgtcttcacggcggttataacggactttcggattctggtatgcgccaacattgacgacagttttcggtgcagttaacatttgatactccttaaaggtgaataggatgaatactcactaggataatatctatctgaaaactttttaaaataaaaaagaaaaaccctactcccgaaggagtagggtattccgcgtcagcacactaacttactttttctcgtaagcagcgataccggcgaccagcaggccgttcagaccagataccaggttcttggtgttagaagcgtctgcacgctcagcagcacccaggaactggttagttgcaccgatcattttacggaccagacggatagacttggagaactcgccgccctgctcatcgattttcacgccgtcaactttcttcagcagtttctcgatggccgcttcgtagcgatcgcgtttctggttagttgcgtgatacgctttaaccttcttctcgatctccacaccgactttgttgaagaaggtgttaaccgtgctcagctgtgcgatagacggagtagagatatcgctctctacgctgtgttccgcttcaacaacggtagtgctcacttcgaagctgtcgccgtcttcagtggcttcagtttcaactttgaacacctggttgcccagcatcggatgttcgcctttcagatcgctggagataacgtcagccagttctttcgccttcttaccagttttggtgaagtcagcttcagaagcattggccagctcatcaacagcattggtcatttcggccagcacttcgtcctgaactttggcgaagtcaccttttttggtgaacacctgatccagagaagcggggttggtaccttcgaacttaccagcgatggtcagatctttgatgaagccaccagacagtttgtctttaccagacttctgcttgctgaggtttttgatctgctcgccgaacttcttagaacgaccctgaacagatttaccctggttgctgaatttcagccagcggtctttgatcttacgaccctgctctttcagccattcccacgcacgcttcaggaaggctttgatgtcttcccacaggctttcacgcgccacgttgcggcggttacggctaccgtagctttcgcgagctacgctggtgcgatggtcgaagccccaacggcggcggatagattcctgcgcaacgtccagcgcttccgctgcttcgtcaggcatgtcttcttccgcttccattttgtcgtcggccggatcagctgctgcgtcgtcagccgcgtcaaccgcgtccagctgcgcatcagtttcgttaccatcttcaatcagcacatcgtgctcagagtcggtggtatcgatatcacgttctttctcagccagctcggccagaataccttcaaccgattctgctggcagctccaggccatccgggacaacagtaccggtgccttcaatggattcgcgagcagcgcgtttttgtgcaaagtttgccattttcacttttcctctaggtggggcagcgtgccccacctcaatgattaacgtcgggtcgtttacgggttaagaaggattacttcttaccgtacgcaccgataccagcaccgatgtagccgttcaggccagcgataacggtgttagcaacgtaagccacagcgcggttcagaacctgatagttcttcacagactggtcagcagcagtacgtgcagattgcagcgcttcgcggttcgcgtcgtcagctttatctacagcaccagatgctttttcagcagcgcgttgcagtttctcaacttcgctatcgaaggtacggaagtcttgcaggactttctcgaagcctttaccgattgcatccagaccctgcgcagccgcagacagtttgcccacttctggagtggcgatctgtttgtcttcagttgcatcaccagtggtcatgaaaccgatagctgcgaaatcaacgccgccagccagtttcttattacccacctgaatgtaggcgttgcccggcagcgcttgcagtttctggtattcgccatcagcgaactcttccagattctgaagtttggttgccgcggtaccgaacagctcgattttgtcgtagctcggtgcatcagacgccagcattacacccggaccagaggcagaagaaccgccagaggctttagatgcagacacttcaccgtcagccgctttaacgacgtaggttgcagctgcatcggcctgtttggtcattgcagcgatagcgcctttggctttgccctgagttacttctttcgcaatgccgatagaaccgtcaacattgaaagaaccttcgatggacagtttgctgatccagctaccgccgatttcatctttggtctttttgctgcccaggtttttgatcgcagcctgatacttcttagcacggctctgcgcggttttacccacgttgatgtacttgagtttcagctctttgatcttgttaacgattgacttgatcagctcaaggaaacgtttccacagatctttcagggtttctttccagccttcctgcgcagcggcagtcatgccacggccacgacggaagctttcgcgcgccagtttggtgcggtcgatgccccaacgacgacggatagactcttgcgccacttcggtgtgggcaatagattcttccgacgcttcttcaccgttatcgattgcgtcttgcgcatcgtcgatagcgtcttcagtacgtgcggtgtccgcgcccagggtatcctgatcgccagccagaccttccagctgtgcatcttccgatgccatttcagccagttgggtatccaggttttctacacccggttctacgttagacaggccgtcgatttcacccggttcggtgttttcgatgctttcacgagcagctctgcgttgtgcaaaatttgccatttgttctagttcctgtttggttataaccgaattacacgcccctagaaaggggcccccttagggacgtgcgattttcaagaatactgccagcgacataatcatatcggacaatccgttagtacgtgtcatccaccgcgcaagcagttcgtggtctgcataagataagaggcgagtatccggttgcatggtttggtgttgcgtgcccatgttacgaactttaccagcctgaccgaaagcggcagacatcatacgcgagcccaagctgcctttctcctgaacgtatttggtgccgtgtacatcattcatgtacgtcgacatcagcacagaccaggtaccgacattggttggacgctttttcccgtctacaacgaacgcaactgtttcattgtaaaacgtattaaacgtaaaaccaatttgtggaaattcgtcatataatacctgttgcaccgactccgcgcctaagaggcggaagtaaggcaggataacggctgccgcggtcagcgtctcatgaatgaggtcatcatcatggacttctgtcgggttctcggtcagtttggccatgtaacgtttaacgagacgctcagccacgttaaagtcggggttgttaatctggttcatcagtctctcctgttgttattcgagaccgttctttttcgccagacgttcgcgtttgcgtttcagggaatccagacgcttctcgtgtttctcgataaggatttccaacgctgcgtcgcctttaccttccgcttgctgtttcttgaacagtaagatacggtactcggctgctttcgccgcttcacacacttcatcgtagttgtccatctgccattcgttccacgacagattaatccgataaatgatagtgagcgggaatggtactgcggagagacccagcggatcggtagctttcgaaccgaaagacttgaccagatcattgtaggtgtcttcatcaaataccgcttccgggatttccgcatagtctgctttgagcttcgactgaggcgtagccagaacacgacaagcgatgccgtacgtcaccatgcgaacatggaggtactgcaaatcgtttggaccgatacctttaactgcaatgttcgaattctccaccgcaccgagttcttcggctgtgatgtagtttacgagcgtaccgctgtaaagaacaaagaagttaatgaggtccagcaattgaaggagcgtggatttgttgaacgtcagtgaagcagtcacaacctgcttaccgatgtcgcggctgatgcactgttcaataaacggacgcagttccagcgtgttacgcatggctgcgatgatgtattccagtgcggacggatcgcgcagacctttgacctcaaggccagagctgcgcaacattttcaccaactcttcgctcagggtttgcaccggcttagagaggaacggtttcccctgttcgctaccgaccaggtcacgcaggttttcaaactgtggcaacagtgattcactgatggcatcgcagttcgcgttcagcgtgtttttcagattcgttgcttcgaagctcggtaagagcaccgatagcatgtttggaataggcattgctaaaccccttaaagaaccggctgtgcgccagagcggtaggcttcgatgattttgttcacatcagccgcaccagatttcgatttggagaagtcagacttatccagttcctgagagccgttcaggccacgagtataaatggtcacacggttccaggtggtgtccactacaacgtaatagacagtcagggtatcttggaacacacgctgacgcacgttgaagtcttcgaagctaccaccgagctgcgcttccagaccatcgatggtttcctgagagaccaccatcacaccggaggcgttgttgatggatggcgacagggtcaacagaccagacagccagttaccgttgcgcttctccatcatcttggtgtagtagcccgtcttatcgcggtagcggttcttacggtactcttccatcaggtcgttagagaaggcgaggtctttcgccgctgccagtttatccagccagcccccgttacgatcacctttatgttgcaggcggatgtaacgctcccagaagtctttctgttcggaagcaaacgcaatcagggtttccataccgtcagtcggtacagatttcacatcgaggcgcagacgcatcggcacttcggttttgttcccgttacgttcaaaggtcgcactgaagactttaccacccgccagaccttcctgctccatcatctgcttcatgaagttggttggcagcgtagaggccactttacccgctttgctgtcgtagttgttggtagtcgagttgaagttctcagtacggctgttgtcgttattgttagtgacctcagtgttaccattgaactggttgttctgattcactggacggctaccacgacggctcgattcgcctacagcaatggcgaggctatcgtatgacggtaaaccaaagcgaccccggcgttcgccgatagccattgtggccagacgggaaccgctgcgggcggcggcatcgagggagttacggcgcgtggagattttgtccagcgttccaataacatccacctcaggcacgccaatcagcagggagatggcagttaattggttagcggccagcagtatctgcaatttatccagaatgcctggcaggtaatcaacgcctaacagcgactgttcaacaagcgtagtgtattcgttatacagaatctggttgaactcttccagcgagtcggcacgctgccgaaacaggtctgggaatttagagagaaacgagatgacactcgtctcaacagttttttctgccattttatactttactccggagtaaaaatttcatgagtgacgagactgaaaagaagaatacagatcccggttacgaccctaatacggatatcgactataccgtcccaaacccgaataattccgatgccgttccctcgttagcgggttacatagacggtcgttcttcatcgacagctcccactcaaaagaagagtttcgatgacgagttatccgtgtgggcagaccgcatccgcttgtcagtcggtctaggtatcgctgcgcagcgtatgaccaaccccttgatggggttcaaccatatgatggccaacaaccccataccggtaaaccgggaatacgggggaatgaccttctttaccagaccggatttcaaccttagctacgacaacatttcgaattcacgccgcatgtcaaacatggcaatgcagccgaagtcgtctctcgactattcgattctggcagccctcgaccctgatttcgaattggggttttccgactcaccgtttacctcaaggggtttaagaaagaaccggttgggaaccccgttcctgcccgatatccccttcgataatttacaggctttcataccattgctttccacgcagctgattagcctgtcgggaatgccggatgagtctgtggacaactggatgtcggatgaagggttgttacgcgaacaatggggaatggttgattccacgaaccttgtgaactatggttacaccatgtcatcgacattaaccaacccgtacggtaatgcgattatgcgcatggccagtgtgtggctggaatacatgtcaggggtgcgtcgtggtcagttcatgccaaagattcgtaattcaatacagcgccgtattgactatcagtcgcgtatctacgggatgaagtatgacccgatggggaacatcacccgcttctggacagcgtgtgtagcttggccaatgaacaacaacgcagggcagcaagcgcaggttgataactccaagccgatgagtaacgatgacaccaacatcacgttacagtggcagtgtatcggtgcccgttacgacgacccgctctacatggagatgttcaacgcgaccgtgtcctattttaacccggatatgtcaccgacgccggagagcctgcaaaccgggaacttcgtgccgaacgcgcgtgaccagttggtgcaggtaattccacagttcctcccactgttcaactattacgggtatccccacatcgatccggttcgccggaaactgacgtggtgggtataccaatctgattaccaacgcattctgaaaagggcaggtctcatctgatggacacttatgataagctggcatcgaatatgttgctgttggcgcataaccccgccgcgatgcagacgctgttattaaagcagctccaaaacgtcagcgacaacgccgcagcgattacccttcgcagtccaactgaccccgtggtcttcttagccgaggccagcgtcatgttggcccactcggcaattgaaggatgtcgggcaaccgtaccaaaaacttacccgtcacaagcccagaccatggacgacctcttccgccatatgtcggatgtggattacgttgatgtgttctcccaaccgtcgggtaccgaactccagctgattatcgacgtggactcgctcttgagcaaagccatgccgttggtctatgctggcgtgcgcaaactggttatccctcgcgataccgtctttaaggtatcgggttataccttctcaattcagtacccgattgagattcgtgtgctgccctacgggacgccggacaacccagcctttgaggtgttgtggattaccgagacacaatcaccgattgcgccggtatcaaccaacgcgctggattgggacttgggttcttcgcccactaccaactccgtgctgctccgtatcaagattccggtgaagcagtacgatgttaagagtcacaccgacaccaccgtggggacgaacgaactgcaaatcacacgcagcttcacgaacagtttcttctacgcccgcgtttggcaacgtgatgccgccggtaccggctgggtagagattccccacacacacagtcgtgatgtctacgacccgaatgtggcaacggccgtgattcaggtcgtgggtcaaaacattcgctgcaccattccctctatttacctgaccaccggtttggtagcgggtgaggtgcgtatggatgtctacaccactatgggtgtgttgaatgttgacttgtcaagctatgctaccgatcagttctcatgggacttccgtgacctgaacggggaatacgatgcgtcctacatcaacccactccgtaacttctccatcttccaggttgtggccgagagtggcgtgggtgttacctctggtggccgcgcggagttaccgttcactgaactgcgtgaccgtgtagtgaacaacgccgtcggcttacgccaagcaccgattacggagaagcagttaacggctgtagcagcagactttaacctgacgctccagaatgccatcgactatgtgaccagccgtacgtatctgatgtcagccccgttgcctgtgtccacgctgaagaacgtcagctcaccgattggttcggtcacgtctgccctgtactttagctgggatgaattgtctagcctgtcgactgttcgaattaacgacaaccgcatgacggtgttaccgaacacgttgtacaggtttgacggcagctcgttgtccgtggaaaccacgatgacggagttgatgaagaccatgcgtaaagaggatctggtgaatgtggggaacagtggttcgtacctcttcacaccgttccattacgtgctggatatcaacaacaactctatcgatgtgcgtatctaccaactcgaccgtccgagcttggtgtcgaagcgttttatcagcaccaacatcacgacagaactgagcgtggtcactgacgactatcagattctgatgaccgaccaaggttacgtgctacggactgtcactaaatcagaatcgccgtaccaagccttggacgacagtcaggtgtttgcgcaaatctcctttcaaccgcgtaactctgagaacctcgcttgggtgcaaggtacgcttgtcggtaaacagggcagtgagcgtgtgtgggagttcttgttggagaccaacctcgacgttgaccgtaacgatgagatgattgttaccaacacccgcactacctcgtcatctacggtgaatatcccggtcagcctgacggaagactttaacatcttctacggctgcacgggctactatccgaagaactacgagcgggcgaacatggacaccctgattgtggctccgtcccgtgacgcgattggtatcacccatgagattttcaaaatcgaactgggcaaagccttgaccgcctactggcgtaaagcccgccctatcaccgacagcatcaactacaagtattacgaagccgatgtgctgaagttctacgacgcggatgtggtgaagacgaatgaacggggtgtgcctgaatacacgtacgatgaatccaaaacaccgccattgcagttgacatacctgcaccgtaaaggtgacccggtactcgacgacgacggtgtgcaggaggtattgcacgagaagggaacgttggtgaaggatgctgacgggaactctgtgattgaccgaccgcgcagtatccggttccgtaatgagatggcggtctttgatgcccgttatctgtttgcggacagtgacgaggtggtggcgtaccgtgagtcagtgattgattacatgatcaatcaaatcacggtgaacatgccgcaactgaccccactgctgctggaacgtaccgatgcgtacttcgtcccaattactaccatgggttacatcgatgcccgtacggagaatggtgctatcacgccaatcccggccgagcaacagttcacagtaagttattacctgactgcggtgaaccgtcagaacgctgacctgattaaagccatccagaagaagacctctgaggttatcagtcagtacctgataagcaacagcaccgtgtctgcggtagcgttgggtgaagctctgcaagatgcgttgaaagataccatcttgggtgtggttgtgggtggtatggggccagaccaagacatgcgtctgttcaccgtcatgtcagatgccacacaggtcacggttggtaagaagatggtgattgaagcaaacggacgtgtcggtctgaaagacgacattgttgcgagctataatcgtcacgatactgcaccggtataaaaaaaagaaagcctactctcccgaaggagagtaggtcttttattttaatttttgcctttgatgaacgggttgttctggctcttactgatgatgttctgcatcccgaccgtacccatgcagatacggcgaacgtagttgaggttcttacgcagaccctgccagaagtcaccgtcacggtctttatagtccgcagacagttcacgacccagattcaggctgtcagaacgttcttccatcatcacgctcagcaacgcctcaccaatggattggatagcagctgccccttcccggttacgtgacattgacttctcccatgattggatacgttcaatcagggccttcacatcgctttccattttactgtatgcgttgaagttggtcactccggtatttgtggataacccatttgccatcacgaccagcgcttgcagtacaccaccggcctcatcatcgttcaaaccacgacgttccgtgtaagaggaaacgaagctgctgttcaggtacgcgccgtactgcgcacaaaccagaatagagttacccacaaactcggtgggctcgtcgtaaccgatcaggttgtcggtgttgttgctaccaacaatggcgatggtcggtgaagtttctgcggtgaacttcccacctttcaccacgggaatgacggtggccagatagtcgttcaggaaacgcatcgcgtgagcaaattcttcacccggcttacggatttcatcgtccttccacttcaccccttcctgcttctgcgacatcacgctcgacagagagtcaaaagctttgcccgcagactggaagaagctgttcagctccggtgcccggttggccatcatgcggaagaccgcttcgtttggaatacgcacacccgcttggcgcatcccgcttggcaacatcccgtacgccttcgctgctgcctgtggactgaagacaccttccgccacgttcatacgcagcaactctgcgacgagaccacccacgctacccgcccctttctcacccgaagcgacatctttcagtaggggtgcgattgggttacggccagagactgccgttacggtgtccacgtaatcgcccgcattggcgttcttaatcagcgcatcgaaacgtagtgcggcggcggttaactgggacaggctacgactggagagttctttggtcgcatcgaggtatgccgacttaacagacgcacaagtcagtgtgtccgccagtgattcatactcgcgcttccaatcatccggtttcacagacttcggagccgcagggggtgtctccgcagctgcttgccatttctcatccgtcttggttttgtattcctcgactttgtctgcggcggttttcgggttggtgttacctttataccctttaccggattccacaatccaactgatgattttcaggatggcggtcagcaccagaataatcaggcccatccgaccggcttctttccatgactctaacgcagccaccgtttcccgttgatgggtaccggtgtagttggaggtcaggattttctgcacgttctttggaatggtgcccggacgagttgattctactgcgacagccaagtcacgcgagataccgtgacggcgaacgtcatcaagaatggcatcaatctgcgcaaggatacgtgtaccatagagcaggtcagcgtcgttacgctgcatgtacaagttcaactggtcgagactgttaatcttgtgactcatgtgctcttggagcaggttacccatttcaccgagacgccactgtggggcggtagcgaccagcccacctacttcggtcatgctggtcatggtttacgccttctgagtggtttcgctgatgtagaagccaacggtttcgaagaaacgctcagcccacagttgcacagttgggtagcaatccacgccgtacgcttcgtcaatgacggctttcggtgagaacgcgtccagtgcacgcttaccaccccagacgttgtcgtaacggttgcagtacaatgcagaagtcaaatccagcacggtgccgaggtcaacgcagtacagctcgttcacatccgagacgatgttcttcatgatgggcacgaggaacgcctgtgcggcttctgtagagccgtatgcgccgttatccggcagacggacagagtacgccagtgtgaaggccaccagagcggtcagtgcttgtgagccctgtacgcctttcccttcgttgtcgcgtttgaagtcgagcacgagggaattcagagaaagtttatgcgtcatggttttacctttcaattaacgagggttaatcccgcgttgctaatcaagtttcgtagcgtgtcgaattgaacttcttcatattcggaaacgccgtgcgtaaaatattcttgggagccttcgtacgtttcttgccacggctgagaacacatctcggggttgatacgataaaggtataacttatcgccattcgttaacgtattccacgttccctgattcgctatcttaaccacatcacccttacgtgtcagctgcattggtgcggcggtactaccggggttgttggaatcaataacgcggttcttttcagcggcatacgccacaccggcatttagggcatcataccgggtacggtaggcagtcaggggcggtgcgtcgaccccataacgaacacctttcaaatcgttatcaatctgctctggggaaagcactgcccactgatagggcagcaccatccacaactcagtcggtgccgacaaagactcccgtgctactttgctccggccagttgtgccatcttcgcagaggccacacgcaggtcgttggacatatagccttcaagggcacgctggtaatcaaccgcggcacgttccttacgacccgcaggcgtcaaggttttcatgatgaatgaatagatgttgtctttgtccttgaccgttttcagaatctggtcaagtgcagcaatcccatccaaacagcgctgacgttgctcgttcgcggctttggtgttcaaccctttgaggacgttcagttcctcaaccagattgcggcgcagcgtctcgaaacgttcctgcggtggatcgtagatggtgttctctgggtcattgatgattaacccgaacgccaccatgaccgacgcatacacaatgccgaatggtgtagtggcacccacaatcagaatcgccatgttgaacagttcaccaaacaagtgcgtatagatgttggtgtacgagttatgacgcagaatccaccactgactcatctccatcttgtagagcgcggacgcaaggtaaggcgcagcacccattcgggcagagaagtcatcggcagcacgttcccagctacggttaccaaaccctttaccgccggtaacgttcgggcgctcaagcagtgtctgggtaacgaggtgcatgtagatgttttcttttttgaacgagtcacagatagtctccggctggttgattttcgtatcgaggatacgttcaacgtctttgactacgcgcagtttctcttgcggtgaatccatctccatcatgcggtttgccgcagcatccgccaacaggttcactatcacgccacgcatcagtgtacgcaggtaatagtagacatgtcccacttcatgcagaatgatggcagcgatttcatacgcggtcagttcagcacggccattgaagatcggcggagtcacgtaaagcggtgaagtgattttcgacaggtcgcctttcagcacggcgttgttatcatcgaactcgccattcagctcgttgtctttgataaacttgctgtacaggtcaaggtctttgttgccctgatacaccacgcggtggaattgcgccactatcgggttattggcatcaatctgcggaggttgaatcgccgcaaacagttcggactccagacccagctccgcgccattggtgaaggtcacaccgatgccgtgattcttctgaatccactctttgataccggaggtgtcgtatgcagcgatggagaaatcccccgccgcttggaacttagcaacgatatcggcgagtgatgccagttttttcttatcttgaaacttaattgactcagcggcaacacgcttgagttctttcacgctttgagcgtgcttagaccagtagcccatatcagacgttcctttaaaaagtttttacgtcaccaccgatcaatatagaggcggatcgatgagagagaaccgatggaaaccaacatgtatttcagtcccgatgacgtcatagcgaaggagtgtaagcacgtcgcttatgccactgacgagagcggggaaaacgacttagtcctcattaaagaggtcatccatactaaggatggacggcttattccgcgtatccaactgcgtgaaaacgtgaagcgtccggtgtacgtaacacaagagccgtatcgtaatcacaaggaaaagaaagagttcgaattgaagtcgcgttgtcaggaattgatgacaaccgatgcgttaatggccaagacattgcaaatgggtttgggtgcccgtttccctgacccgaagaaacgtcttcgtcaggtttgtaccagccccttcgtttatctagccgacttgccggttacgagctggattaaacagaagtacatgcaaaagtataaagattgcaccacaccgaatcgcatctgcgtgtatgacgttgagacccgcgaggaagacaagtcgcgtgacccgtggattatgtcgtttgtactggacgatgaaatccacatgttctgcacgaaagattacgtagcgcgtattgggaagaactgggacaaccgtctgattgccaaggcgcaggaactgctgagcaagattgagttcagagaaaaaaataaaaagacgggcgaaaccgaagtcaagattaagaacgtgatcgcagattacaaaatcttcacgtacgaatgtcttgactcagcacaatgtattgtccgtatgtttgaagagattcacccacgtctgcctgacttgttagtggcatggaaccatgagttcgatatcacacgaatgatggaagcgttagagcgtggttgtgtcgagccggaagatgtgttctgtcacccggatgtaccgaagcagtaccgcaaggtgtggttcaagaaagacatggcgtcgaagaagacggagtccaagtcgcttaccaaagcaccgagtcagcagtggcacgttctgtactgtatggcgtcgttcttctgtgtggatgccatggtgctgttccgctcactgcgtgtgcatgaaggtcagcgacccagctataaactgaatgcgatactggattcagagttggggttgaacaaacttgacataccgggtctgccgtatgaggagaaactggattggcacttaaaagcccagcgagagttcccgctggagtattgtgtctataacatcttcgataacctgatgattgtattgttggataagaaaaccaacgacctctcctcagcgataacgattttggccggttactcgatgtacgatatcttcccgtcgttaccgaagcgtatctgtatcgccttcacctactacttgttagcccaaggctacgtggcaggcagtgtgggggcagagatgcgtaacaactacgacgaagaggttatcgggacggacggttggattgtcacgttaacggcgtgtatgaacgccgagaacggactggacgtgttaaaagaactgccccagttctattcggcgttccgtggtcagactgcggatgcggacttaacacaggcttacccttccgcgaccaacatgatgaaccaatcgcgtgagaccactatctttgaactgctgttcatcaatggggtatccgaggaggttcggcgtcgtaccggtgtgaacctgacagcgggtcgtgtgaatgcgatggatatcgccaacagcttcttcttgttacccgacaaggacgatgtgctggatgcgtttaaccgtcgtgtagcaaacagcgaaccgtctgaagaatacgcacaaggcttttaataaaaagactacctactcccaatggagtaggtagctttatttttttattctgcgaggaaggcagcacgcagcaggctgcgcagttccgggtcagacatacgcgatgccagacggtcgatgttactggtctgggagaacgcgcctttattagcagagcgcgcaaagcgtaccgtgttgttaatgaagatcatgaacacttcacgctcagcctgattgctgaagtctgacaggttttcatttaccagcggcagatagaaaatcccatccgggtatttgttcaccgcagagacgaaacacccaaagccgtcgaggaaggcttgaccgcgcagcttgaacagattacggaacgcgttatgcagctgtccgtacgcttcggctttcttctgtgcactcggtgacttattacggcccacagtgttaccggcagtatccagcatatcagcaatcagtttgacctgactctgttcatcgttgctgtaggctgcactggtaaccgaaagggtttcaggacgcgcagcattttgagtgctcgtgtctttaactggctgagtcatgatatatccttttaagtgatgtgatgtttgggtttgaattcgacgaccacggtatcagaaccgtgcatctttgccattgcgacacccatgacgtttgagaacgcggtagagatatcggcggcaattgcacgcggttccttggctttctcattcgaggcacaagccgcgcagcagtcaacgtgacccatctgacataggatggggcgtcgtaggttaacgattttccccacattggctttcatgaagctgtccgtgatagctgtcagcttaccattaaccatggcgttcatgccgatatagcgcttcacgttcaattccgtgataaacacctgatggacgagtttcgttccgcaatccccttcgacgattttgtggttctggaaaatcatctggatgatacgtacctgctcaccccctttcgcagtttctgcaccacgagagaaagaaccgtcacgaatcgagttgtacttcgccactagattcttgagcccttctttatccacctcaaccaatgcgtttggtatcagggtaaagtcagccccttcttggaaggccgattcaatcccatacatcagcatcagcttacggcgacgcatacgggatttcttcgaggcgtaatactgcaccgattggtcaccggacagccactctttatcgagttcgtccagcgcttgctcaatcttcacaatgaccgctgggttatccagttcgtctttgtgtttctcaagcagggcatcacggattttgtaggtatccgggtgaaccgtccatgaccgaagggtgcccgtaggcgcaatggctttggccagtggggccagttcagctaacccgttaacaaaccggtcaaccatactagggcgaatcgcacccacgttttctgggtcatcatcctcgtagtccacacagcgactgtacatctctttacggatgtccatcgggtggcccgtttccagatacggcatccgtttctcaaaggcataatagatgacaacccagttcaggacataccgtcccacagacgtctctatttcgctctctaagcccggataaccacctaccggtagttggaatcgcatctcaggaacaaacagctcagcgtcctttacagcgtccttaatgggcacccactcccagtggccgttcacttcatcccagtagtgcgccatgccttcaatgaagttcaggtcgtactgctcaggccgttcgtgtgcctcgggaaagatacagacgttgaacaagccaatacgccagacgagtcgacgccacgcctcggcattacacgcagcaatcagatactcaatccggttcatcggtttgctcctctaccccgtagattttcttcaatgcctctaagccgtcacgcaggatgggttcttcgggcgcttcgtcactgttaatcagttcgagcattccttctagtgccccataagcatcgtcgaatgtctcattctcaatgatggacagcccgacggcgtaaatggccaacagctcactttcacccacacccgcttcttcactgaaatcgagtgcactgaccacactattgatatccgaggtgtcgctcaggttcaggaacacatacgcagacgggttctgtgggtagactcgcaggaattgcaccacacgttgggtacgtgggttctctgcatcggcatcttgctgttctgctgaggtggcggccaggaagttacgcatgacgttaatcacacgcggttccaccaccactaccaaatcttcgaagtggatgtcattatccccgtagacataacgtaccatattctcaaggatatacgcaggcggttctcctgacagcagaattccgtacagggtgtccgtgtcttcgaattcttcaaaggctgaagtcaggccatggatgatgcgtactacttctttcggtttacggtaagccacctgtgggttcaacccgacacccaaacgttgggccagcgcgcaggcgcaacggttaaccagcgcttccagtcgcagacactcttcgttcatatccgggatttgaccggtataaatatccatcagcgtcgtatcgtaaccatactcgatagctaacgacactaagtctaacaccggggccaagcggccttcttgtctcaccagaccgagtgtgtcggcatagtcttcgtataagtcagtcatgacggtttcctaaaatgggtctcataacaacaaaaaaaaataaaagggagccgaagctcccttagatgcgtcccttcagttctttctcaagttctggcgggattgcgcctttcttagcattgtctagctcagcacgacgacgttttgcgatttccagatgcttcatcaacttccaacgcggcctatcaagccaggtatcaaggtcgtaaccaaacagctccttgataccttcacgcacgtacgtggtcgcccagatttcatacaagctctggttaatggggttctcgaagtcagagacactgatgttgttctcaccggtctctaacccgagtatcccgtcgtacgtggagagtagctcgtcatgcgcttcttgatacgtgataggtcgactgtctcgccgtttgaacagcgaggtggtgtccagcttcatggcagtgatgatagcttcggctggaacgtcgtcggcgtctatccaatattttcgaattgttgtaagtagactctctgtatctcgaacaccacacgagatagcgcgaaaaaaaccttgtccgggctaatggtaacaataccacggaacggaccgtcttcttcaccctcaccggtcttacagctcggacacgcgtgacccatgtaaccaaacacggccatgcgagattcttcgttgtaagtggacagtgcgttttcaaatgccagcacgtacatgcgatcagaagagagttcttctaacatctcaaagatacggtctggatcttcttcgcgggactcaaccggttcacctttcaccgtctcttcaacgatgatggctttaacgtgtgtcgcataacgcgtcagtcggcggttttccgcagccagacgaatgtattgcgaacgctcggtttcagttgcatggttagccagtgcgttagtggcggagctgttaatcttctctacccacgcattggtgttgtcaatgaactgaccgatagtggaacggccgaactctaccgtaatacccagctgctcgtaatggaagcgagaggctttggacttcggcagctctttacggtattgaaggtattcttcgttaccgataattgcatccggccctttgccgcgctggcgcagccagagtgaacggtgtaggtctgagaacagaccgtcagccatacggatacaacgagccagattcagacgtacttcacgctcatgtccacattcgtggttcggacacagcagcttccacggaataccggctgggaacttcgccatcaacggcccgatgaccagcagccagtagtcatccacatccacgatgtccatcagtgcggtcttaatgtccagaccctgacagtcgtaagtggtgtctaccgcaaagttcagcgagtgttcgatcatgtgctgaagatacacgcccgatgatgaggccaacagcagaccgtacgtgaacatcccgattttcgactgctctgacgtgatacgaatatcgaagtcacacatgtcgttttcatgtggagcacggaagccgacaaagataccggttgcaggcagccagacggaaaccggtgaaccggaaccacgacgacgacgcagagcggccatggcaccttgcgcattcgcgccacggtcagttaccgcagagacgaacttgttgttcggcagcttgatggtctgttgccacgacgtatcatcacgttccagtgccatgtcaaacgcagcacggttattaatcatgataggcggggtcaattccaacgccgtaaagagcttctggtaacgctcctcctcggcggcattgcggaacatcggacgcccttcgcggttacgcggaatactggcaaagaattgcatgacttcctgctcaccggcgagcggcagcgtggtaccaatcagttcatcactttgggtcagtacgcgatggggatcttccgggtccatgctggcaatttcggcacggtgtggttctggcccgaaatcaatctgacgacgtttctctttcgagaggttcggcgtctgctcgtcgcggtctgccggggcatcttctacatccaacgcaggggcaggaaccacatcttctttaaccggtgtagggaacttatccgcaatagccgcaggttctaccggagagtggaactgttggctcgccactgggatttcagcgataggttgtgcacgcggttgtaccgctggcgtaggttcaggctgtggctgtaccggagagaggtcaagtttgaccggctgttccagttggttctcagtgcttctgagtgcggccaacatctccggggtcgcttcgcggtcttcaccgagtggcgtgtcgagtacggcagccacggtgtctaccaccggtggcggagtatcatccaccggcgcattcagaattaccagacttttcgcacgctcagttgcttcggcaaaagaaaaagtgggattgagttttaccagctcgaaggctacctccgccacgtctttgcccaaaagggcttcgcgtgggggaagtcgcacctcagccgtttccggttcggcaccaccgaacgacggacgcggatcgttagacattcgcaggttcctcttgctctgctacaggttcagctgctgcttctgccgcagccagtgcgtcagcggcggcttgagcatccagctcgcgcagcttggtcagtattgcttcatgggaccagttgttgtgcaggcccacgcggacacattcacgacgctgctcataagcagcacccgattcaacgatagacagcagggtttcctgtgctacgttgtctacttgaatgtcaaagtccgccagttccagttcagccacaataacgacgtctttgatttcgtcccacttgtggccatcgatgacctccatcagtttggttgcctttgcatcggcatcagtacgcaccgcgaacagacgcgttttgaagtcttgcatggcacccaagaaggcagcctgagaattctttaaccactccgtcaagtacgctttcaggtcttcacccatcagcgagttgatacgttcaaactcacggtcgattttctcggcgtgggttttcgaatgaccgaggaaaacactctcagtcgtgttcataccgcgcatgatgctacggacacgttcgcgtgctgcttcacgcgggctaaaaccaggctgctttttacgacgagacatcggatattccttattaatgaaagtgactctacacaatatacactaacgctgtaattaagcgttgtgtggtaccgtcacccaatcatgccatttgtccgagaagaggcggtatgccactttcgggttttcatcggtattccctgcggggttgttgttccacagttcgtaagaataaagttcgtacgccgcagtgccacggatactggacgtacgagtgacgaaatacgttaacccacgctgcatgataaagcaggacgtgaagtgttccgtaatcgtgtaatagtgaaaggcccggttaatctccgggtcctgacacaatgccttagcgacgctttctgcgccgggataggcccttagaacctttacgagaaagtctgccaacgtcaatccggcgtagggggctgttggggcggctggagctgggggcgttatcatacgttttccttacaacataaggggaagtcgcaaccttgaatgacaataccgtatcacgcagcgaacgcatacgtgagttcaggtacgtaccgtgtttagcaatgttcatgcaatgcccgaaccacacaatggggttcatgtcccaaccgaacacttcgcgcacaggacgaggacgtccggcaatctgtaagttcagctgttggtcatcaactggcactgtcacgatcatgtggaccatacccggtttgtcaatcgcggtaccggctttgttgggtgtagagacaccgaactccgccatgatgaagtcatcatacgaatcgccaccgttatacttcgccaccatcaactcattgaactcagtacctgctaacttctgatgcaggaactgtgtgaagaactcacacatgtcaacggttgagaacaagatgatgattttctgtcccggttggtaattggacaggaacaccttctcgatcagattccaccacatctcacaatacgaaacgtggaagccttcgcgaatcaacttaccttcaaacaacttgtggttgtacggggacatctttgtcgcccaccacgcgagcttcttatcgtccagcgtgtaatagaacgcacggacatccaccaccttgatgcgttcaaccgacaagcgcatctccatggggaagcgttccagataacgcgagataataaaggtcttcgcaatacccggctcaagagttgctgacatttcaatcgaggcacatgggttcaggataatcccggccagatacaccagatagaaatgctcgtgcacctcatccatcccaatgagtcccacacccaacacatcgtagaaacgctcaatgtcaatccccatcgagtgtccggtgttgatgtactctttcaggaacaattgaagtgataccgttgggaagataatcgcccgaatgtctcgacggtctaattccccactgaggcccatctcgtacgcttcaataattccctgcacaccacgacagaccaacaccttgtctttgtcaattcgcaagcccgttgggtcttcgcaaatatcgaacaaccatttgtccacatacgtcggacgcatgataagtgaggtgcgtacctgtttcttcaccatcaccttcatcagggacttagttttacccctgccggtatcgatggcaaagatggtctggtgccgatcgggttgcagcgctgtctccaccacttcattctggtaatagaagcgggattcaggatcgtccactaacatcggtgtgccgaagttatcaaacgtacagcgatacggttccgaccgttccactttgtggtgcctgacctccacatcaagacggtactcaataaccgcattcttaataatggagaggatttcctcaagatgggctttgtgaaagataaagctacgtgcgccctccatgtgggcgtagtaaccatccccctgttctacggtaatcttgccgcgctcttttcccattttcggggcgtgcagattccgttcggcccatgtcttgatggcaatctcaacgggtcggacaggaacttcaattcgcacccccatggtggtgtgcgtgatgttaatctgctgcataaacccctctacaaaaaaagaggggcatctgcccctctgtattaatgcaaccgtgttttgaatgacccgtcatacaacgacgccggaatcttacgtgtggtatagaaccctacgcggttgagattgtcttgctgaccttggaagaacaacatcggggcagcactacgtatcgcaatcagcgtattgtggtctaagaaccgtttacccataccatcaatggcagtttccttatcgaaccctaccgctgggaacggattgattgggctttccacacgagaaatggcaagcatgataccgatatgtgtcatcggaatccctttcagcttacggttaatgtagcggaaggtatcgaacatcgcaaaggtacattgacgttcagtagacccacccatctccaccaaggtaagcgtcttcactttaccatctttactcattttcaccgtggcatccgtagtgaagtccatcggtgtttcgttcttgtccgcagcaaccgaacgcagcttggtctccagacccgcaacgaactctgccatggattcagaacggttagtataaatgaggaatggcgctttcggcttccagccactcattggaatacgaatctcacctttgcggatgaactggatctcgtcacgcactttcaggaagtacgccaagaacgctttcgagaagttcccgcagacgcccatacggacatccagtgattctccgccacacggttcaccatctgcattcaaacgcacaaacgtaacgtctgtgacatccggcagagaggtttcatcaatgtcttcgatgttgtcgtagtacgccacctgactcagttcagagtgcatcttctcagatacgaccagtgagtattcactccacgtaccgaactccggcttgtcgagtaaacgcagacctttctctgaccctttctcatagccacggaagtagcctttgatgcgcccaccgataaccaacgtaaacagttcacgcaggaagtcgaggtgcttcgttgagagaatcccctgtgtacccttctccgagatggaggtggatgccaagtgacccggtgaggttttctccgacaggttgtaaaccaaatcccccatacagactgcacagataccctgcttcgccatgtggcgacaggtcatcgcagatcggaacaggagcggcttttcaaccacatcatcgaagtggtctttctcgaacacgcgccacggccccgtttcaccgttgaagcggaaacgcatcccgaccatggcgtcgtattgcgttttgctttctttggtgtcacggaaggtgtgttcgtgagcgtgctcggtaccgcagtcatctaaagtgaagtgggtcagcacgtttgcagcgagctggagtttacgggaaccgtattctgcttccgcaatcttatcggtgttatacagatgcgaacgtgatgttgcgcccgattctttcagtcggctgataaccgagttcagaccaccgaagaacccttcccatacctggttcgaatagacacgggaatcgatttcagaggttttaccacgcacataggcttggagtacctgatccatcttgatggttttgtcgagtaccgacatcgccaccgggttgtctgccagctcaggtgaacgaatgatgcgctcgataatctcgtacgcttcgttaaccttatcgaccccttcttcatcataaccacttgggtactgcttagcccattcgtggataacctgataatcaggatggtcgtaaatctgcatcatggtatcaatgtcgatggtcgtacagtatgacagcaagttcttcactgtcaggttgaacgcatcggcatagacgtgctgacttaacagataacgggtatcggccaaatcaatgcccgctttgcgggcgagtacagcagcttcggacatcaggtcgatgtgacgatcatccgttgcccattcacccccacgacgataacacatcgtggaaggtgtcggtacctgcggatagaatcgagagatgccccagtacggccaactaagtttgatgtgtctacccgacatcggttgggttacaccgtcatcaaacgttacatcataacgtccgcgaagacgccatacctgatccgaattcaggttacggagatcacgaacgtgtacttggcgagcatccatcaattatcctcccgagtagggcgcactaacacaaacccttcacagcggtgtatgttgtcaatcatcttatccacttgtgattcacccagcgggtaacgttcacggtcaaccaacacgcccggattactcggtgtgtcagatgcatatttcccttccacaatctgacgatggacatctgggttattggaacggttgtgtgcttcatcgaacagaccttgaccgtagccatcagtcagtcggtgctctgcctcaccaccccatttcttcggactatagttaatgggatacgacccacgcccttggcccgaagcatcaatacaacccagatagttcgtgtgcatcgaagagatagaggagaactcacggccggtcttgtcaagacgtaaggtcatgacattacccacgtagaattcattcttcgtccactccttctcaccttggtagttggtgatctggaggcgggatttcttcggtgcaaattcacccaacgctttggtgataccaatcggggtattgtccaactcgtgcggtagccagatacgaatcgtgaagtcgtagatctctttgaagagttccagacgtttctgatgcgtatcgtgcgtcacgttcagacagttagcccaatcaggattgtaccgtgcgagatagtccatcaggacattccacgattcattcaccttgcctgcatccagcatcggctttaagcgcatcttgagttgctcagatgccgcagaccaatacatgtggaacagtgcagaatacgtcgagcgacgaaccacggcgttcattgaacgaatcgagtggacacgttgtccgaattcgttcagcggcatgtcttcgtcttctttcacttcaccaacgatacctttcgtacctgacaagtccgtaatcttggacgagacagtgactgggatcggatagcgcaccacaagcttaatggtgtacgtgttgatagggtcacgcagtgaacgctccacgggacggttgatgcggttgatgattttggtttccatggtgtctttcttatattcaccacgacgaaccgctgcttcaaccacaccacgaatctcttcgcggaactcttgatacacttcatgagtttcagaggcgaacgctttctctaagaactcacaggctttcggtgaccacaccacatcatctttcacgaggaagtagaagcgaacgatttcgcggtagtagtctttcaacgccacagcatacgagtcgagaacgcgtttgttctcttcggttgctttgatgttgttgttaccgttactaaagctaacatcatcacgccacacctgaatgtcaatcacccgtgaaccgttttcatccgttggattttcatagtgcttcggatcagcatcaacgtattcacagtggtcaaagtgcggcgagacatgctgtagctcaccgatagaagcattgatagccgcgtacaacgggtcaaattgacgcgtggcgattaccaaaccatcatcacggattgcttgtcccacattcgggaaatactgcggcacacgaccgttagggctgtcgtaaccgtatgtatccagcaggaactcatcttcgcgtaatgacacccagatttctttgaacccataggcgtgcattaatgcggcggcggtttttgagatcgtgtaagaatcctcaatgatatccggatgcgacatggtcactgttggcagcgcaacgccgtcaacaaattcaccgttcagcatggagttcatttcggtaaggatttcatccttttccaacacggtagtttcaccacgtaaaatcgcccgaagtttatcggtgatacgcttctcagaggtgaagacattatcatgcgaggtatagtggtttatctcgatgacatccatgacaggcttgttcaacatgccagggctggtttcactgcgacgaaagaaaattgcatgctctagcggagagccactgccgatttgggcgtgacgagtgaacaccgctcttttgtgtgtgccattatcgttatagatacaaacgctacctgaatcttcaacgatgtcgttgaagaggacgtcgtggtagtttgaatccgcaccggtgaaatggaacatcggagttgggtggtcgataggcgcagccgatttcatatggccacctaccatcgacgcacgcgcacccgattggttacgaatcaaatactcacggtcagcgtgggtaccgactaattctacgtgcatgctcattgctttaatactccttcttggttacttcaccgagataatatatattcgtagatcttttcaaggagacctcatgcttatcagctcgatcactctcggtgaagttataccttcgctcgacagtcaacgccgcaaactaatgcaagattacactgaatattttcggaatcatgcagagacgcaagatgtcccaacaaaggcagagtttgcatggccagaaatacatagcttctatgcatactgcaaacttgccgagattcaggataatcaggtttaccccattatgctcattaatgggatatcgaacccgatggatttcacgccggagaaatacccggtgttacgcattccatcgccggtggttgtggagaacgtattgaacaccattaccacctaacaaaaaaagaagggacttcggtcccttccttcttttatttttttaccaatggaacccgtctttcggtttcgttggatcgataccacccagacgtgggccacccgattcgccacccagacctgctaagccacccagacgaggtggtgaatcatccagcaacgagttaccggtgctagacaatccacttgcagtgctggttgacaacagactccgacgatcaatctcagacgtcagacccaatgggttacgtggcgcttgacccatggcttcagacagagacttaccaacaatcgactggtcggatgtaccgttcagatgaccgttctcacgcagcgacttctgttgggctggggtcagcttacggatgtctaatcccgttgaagtaatcgtcttcggcagtgctttgtcgaagaacgcttctaagctaccttgctcagctttgttctgctcagatgctaacaggtcaaccggacgactggttgtggtcggcgttacgctatactcacgcgcggtggtatcacgttccgggtctttggatgaggaaccggtgttatacggcagcgtttgaaccacgttgtcgtactgctggagttcatccagctgaccaatccattcatcactcagtggtttcagcgcacagtgttcacgcagggctttcactacgttgttgtagttcatcacccattgtgcccaaccgcgtgccagacagccgaagtacggacggttgtcattggaaccacacatgctcggataccaaccaaacacagtcatcagcaaacgatgcagaatcaccttatcctgcttacgcggtaacttcaccccgaagtaggttgcagtatcatcgtacgactcttcttcgaagatgtgtttgtagtttgccacacggacatacttcacaccttcaattgacatgtcagaggcgatgaacaagttggtctgcttcttgttctccgtttccatcatgtggttacgcagactgacccatgctgcacgcagcttctcatccagcttcggatctttgatgccctgacagataacatccgtcatgaacttcttgtaagacgcctgcttgatggtcttgccttcggctgcggtatcgagaatcgcatcgatgagatcgaagctgttcatccacagacgcatgcggattgcacgtttgaggaaacggatggtacccgattccccggtcagtaccgattcacacagcggatggaaggcgtgacactctttgccgttcgcatcttccatacccgctttaatcatggcattggtaggaagcaccagacggcgcttctctttgttgtacgtgaaatacgccggggtgccatcgtccgcgtagaccagcaggtcaccgtcacgattgaacccaagcgattccaacatggattgatagaacttaatgatgtgcatgaagaatccttaatctaacaggctattgccggtaccgagacgaatgcctgctgccggtgtatcatcatctaacaacgagttgcccgtacggaacgcgtttggtgatgacggtgcggaagtaatgatgttgctgcgattgctgttggtgctgtggccatggtagcccgtctcgatggctttcatcagcttagaggtatcattcgccagacggccggtataagccaaactggtggtgttaccgttatgcagacgagaagacatgaacgacgcgtaggtgaagaactctttggcggattcaccgtccatgagtacctcaacacgcgtgaccgtacccaacaaagcatgcacgcggattgcgcagcggatatggttgtgcttggtcaccttaacaaacatcgcatggatatcacgttcgaaacgttctgccagtacacgcggtaactgacggtcgctcagtgaataaatagaatcactgtgaacggttaactgcgccggagtcaagaaatcgctgtggcggttatcgaagtcgaaactcacacggctaacgaggttacgcgacagaatcgcacccatttgcatagccagttcgtacgacaccagagaacccatggtggaataaccgttatggccaatccactggtcggtctgttcgatttcacctaagcccaacttacgggcgagatcaagtgatgccacaatctgacgatcgatttcttctgggttcgccaccgcagctttgagatcacccagacggaactgcgcacgagacgaaacgttgtacccgtcagctgaactgcccagtgaattggtcagtgcttggcggaacgctttaatcaggtcgtagttcgagaagttacgcacgacacccagcgcgttgagatcactctcaacattactgccgccggtcccttcgaagaaactctcgacttgtgtcagctcgttgtccatccccatggtacggagataagagttcgagatggcggtcacgaagttctcaggttggctaagctgtcccgcaagcagcgtcggtgcggctgttgcagtcggtgcataaatctcatcctcgttcggcatgaacttctcatccggattgaggttcatcttcttaatcatgtcagcggttttgctgatggtgatggcgttgatgctggactcgtgataaccctgcgtcgctaatgcacgcgagagcaccaagttgtccaccattttaaagccattcggattgataatccgttcacccagaggcgtacggtcatagaccgtttgcatcccatggatttcgttgatgtacaacaccatgtcgtttggcaggttaccgaacaggctctgttctgcctgtgaagtataaccggttacgatataacgcagctcctgagatcgggtgtcgttaatcgggtttgccaccagtaccgccacgaagttatacaaccccgtgtcacggttttcgtactggaatggttgaatgtttttgtcatcgccggagatattgaccaacggacgttcgaaaccgtccggtgtaccatcaaagcccacgatgttactgagtgaatcttggtacgcttgcgtacccgaagcagattggccattctcttcgatgatttcagacaactcgcctaatgcaccggtcgtggcgttaaacgcgatacgacgacggtactgctgtgggatttcacgtactgggaataactgtaagtcgcgtaataacatcttgattctccttatgaattaaaccattttacttcactgactttctggcgagcttgaatcgctaagaactcagttaactgcgtgaggatgcgaccgtgtggtcgatagttcggaatatccggttcacacttcaacagctctgcggcttctggagacgctttgagatggaagtgatacgggttcaggtgattacgcaccaacaactctaacgatgtgcgaacgatactctcctgtgtttcgttacggggtgaacggtatgcctgaggataatatctatctgtagatattttcagttcgctgtcaatcggttcgattggatagccactaatattccctggcaacatctcacaactgagcaactgagccaactgcggcattccgtaatacaggtaaatggcctgagcaagaccaaccccatacgggaacttgtctggatcgatatctttgaatgaccggtggtcagcaaagcgatgcagcgccgcggcggcaagccactcatgcagttcgtacgttggccccgtatggttgacgatttgagaatcaatcagacacttcgcattggcaggcgcaatgtcataaccggacgttttgatgaaacggcgataatccttaaacgtcatccccggacgtacgtattcctttattggtgcagggctacgaccttgtactaagtcgatggcactgaccttccccttttccccattaaacaccacggcagtcggatgttgtttcaagataacctgctggcccgcgatacggtttgcaaagccggattccacttcggtacggataccgaaataaatgctggagacgatagaactgtcttccagtgacccgtctgggaaatcgcaatagcaaggacgcagtgccagtagacgaacaatcgtcaacgacagcaggtattcatccatcatgtctgatccgtaacccataacggatgacaggattgacaggctggtacctgagccacggttactcatctctttctggaacttctctaccagactcggtaagaacaactccagcttctgaacggcttcggactggcggatttcagtatcggacaacaggtcgaacgcgaggttgattttgtacacaaccttacgcttggcttcctgcgagatacctttacctgccacgtacgccccaagcaccgcaaataccggaatgaacggtttgattaacaacgtcaaaatcatcaggtgataatagtccgggacaaagtacgtcatggactccgtatagttcggcgacatgtctgcaattgaagcatgtagcttttgcgggatgaacacgttcttcagtggatacagctctctgaaacgttcggctttgtggtgtttcgcgatgatttccatgaccttcggtgcatgttcgcttataacctcatcgccttctactgccaattccgacaacaatgtataagccccgaacagctcgtcttgttccgcttctgtcagcgtaccccaataacgattcagttcgatgaacagcaaacggtctgctgttaacacgacacctttactatcgcgcggctcgggaccctgccgtttacgctgggttggaatctggtcgaaccgtacttcctccccattgtggctgatagtaataatctctttattctttacaattttcattatcgcgaaaccccgattgttattagcacgacgataaaatctatctaaaaaggaatcgaatgcaaccggaacacataatcgtcctaagcccacgggttgtcccgtgggcattattttagttaaacgtagtcgtcaaaattgtccgttgctgccggagcagactgctggctaccaccgccctgatagttattattgttgttaccgccgccttgacgattgtaaccaccgctaccctgacgaccgctgccgttttgattccattcgcgcttcttgtagctatcatccagccactcttggaacttgtggaagcggccaatgaaggcgcgacacatacgttccgcattttcgagatcagacaccggcgtaccgttgcgcacgataccgtaacctttcggtgtggtgaagaagaatttcttcgtgcggcgctgaccgttaatttcaccgccaatcgccatgaacgggatcaggtcatcaccacggccaacagacagtgtgatggtacctttattaccgccagagaatggcagactgagaacgtctttttcagacttcttcagaatgtcatgcagtgcatcaaccagtacctgacacatggtcgggccgaggttgtaataaacgccttcgcctttgccgaacgagtagctgaacttcagaccttcgcagtcaggcgagtctttaaagaaattcggctcgatacccagcttacgtgtattaccctgattatcaggttcggtctgcgggtagcaccacttgtcgttaaagagttctttgtttaccatggccatgttggcgtccttcaattaaaatgtttgggtatcctcaaaggataccccggtggcgtaaaaagttagtggctcaatttgcgcaagtaatcaataacgtgcggttcgttgaccaacttcaaacagttgtaaatacggtccatcgatgtggtctgatcccagttgtatttctcagctgttttcagtaacacattgcgaatctttctgtcttgtggtgcgaacatgtactggtcaccaaacagagtcaaaaacgctttgttaaacggtatctgcttcggcttgttgtacatcttcgtgtaccactccagttgtttctttaccttcccgctgtgggattcaagcaggcccactttcgggaaccgctctttgtggataagatcagccgggtagtgcgttaacaacagggtgtctttgttgttctttgggaatacatcaaacgccagaaggttttccatccccgtttcttcgttcgtgagcatgtgatacaagtcctgctcaacggaattgaagaacgcctgattcggggtcatcgtttcgtcaccgcctaacgcattgcggaacttcgcgagaggaaactgcttattggccgatttgtacagacagatataagggacacataccaccgcgggggccaccgccgcagcggtggcagtgaattgttctatatcttcttcgacacaagttcttaaaacgtcagcagttaatctttcacgattatcttcgaatgcgtaaaaagcattacggaacaacgtacggagattaagataaatctcttgatactcatggatgggcagcttgcctttccaatcagcatattcgcccgtatggagtaaaccttccatcgccaatgacgtggcgattgacatctgataattcccaaatacgcggtcaacgcttattggggttctcatgcaatgctcctaatgatatcggatacaatctctaagtcgtattgctgaccttcgagtccgttcaacatcacggcctcaacattgtcgggaccgatgcgctcatccgcgatagtttccgtggagaacacagcttcgagtgctttctcttcctcgtcagtgttaatacgcactccctcgatgtggaatgggtattcgcgcttccaacggttgatgtgctcctcgataggagagtcacgatagtattccaccttaaaccggccgatagccgatgagacgtgggtatcgatatactccaacgcagccagacacttggcgtactgcgcctcatggtctaggcttgctgccacagaacactgtggacaggcttcggtgttcacaaggaaatagttccttgcgagcgtcggtgtgaagtcaacaagggtcatccctttgtcttcttcctcaccatgcgacaacctatcaacgcttccggtaacgcgtatcaggtcgttaatcttctcacggtggtcatgcccaatataaataccgagacgtgtccgtggaatccaaaaactttcattgaacgaacgaggtgattccaccggtagttggaacgtaaaacaaccgtgcataaagaagaagtcaaccttctccaatccacgggtcgccatcagttccgccatttcagcttcggtgttcgcagcaatacggtctttgtactcatcctgcacccaacccactgtcgcctgaatcgccgaatcataaaagataccgatgccgtcgagataaagcgcatctgcgccaatcgactcgttcagctcctcaataatcttagactggccgtggtcatgtgacggcgtgccctcgacgatacgcaatgcgatcccattcgccttacagtaatacaacagccacgtcaagaaccccattgcttcttgggaatccgtctggcggagctgtcgtgaatcctcaaaagcatcacctgctatataaatagcgtcgagggtattgccgcatttgatgatgagtgtttttgtcacattcaccaagtgccacgtcggcactcgcttatgtaacaggtgcaaatcgctcaacaccaaaatgcgtttcacatccagtggtttcggtgggatgttataaatcttctcaatggctctcgccagagaggacttagaggtcttcaccatcttcgataccgtcgtctggaataatcggctggcgttgaacaaccgccgcgggtgcagcagctttaccgtcggcttggatcaaatcttccatgcccgcagggtacgcaatctggccattcagtttataacgcttgaatacccagttcagcagatcaatcgtttgcttagcgcgacgacgattggtttcgtacgaggccatctcaataccgtccagcgtattgacaatgagatcgtgtttggcgcgtggccccagaatcggcaggatttccgcacgggacgaaatttccagtgcttcatccgtcagggactgttgtccttccacatgcagcagcgattgtccggtgaagaacaacggtggaatagtgaacatcagtttggtcggatcatcatcctgcacaacctgcaatggcaccatcgctgaaccgatgcaattgatgtacgcgttgtcatcaaaagacccatccagcaacccgctcagaatcggtagcgcctgtcgacggaacatgctctcagtaaagcgagcatacgggtcgaggttatcacgaatctccgcttcgatatccatcgcgcggttaaactcgaagacttcctgtgaccccatcttgttcaaatcgtacatggcattgttttcaaacttaatcggttcgtcagccaccgtaggctcctttatccacattcacataacgcaaggcatcaacccaatcaccacccaccgcaggaagaacccgcaggctgataataagacggtagcgtatgtctgaatcgttaaggtactcgtaagtacattcgacctctactccggctgtaaacacacccccgtataaggtcaccaaatcctgttggaccttggatgctaactcttcggggtcttgcgcgaacgcggcacagcggaaagagaatgatttgatattgccacggtaaatcactgactggctatacccggcttcggtataatggttcatcagctccgtgatcatatcgccggttgtctttgcccaaccccgcgtagaaagtgttccgactgcaacgaccatttttaatctccccagttactaacataggatttgggcgctaacagaagaaaaaaagagagggtgcttatctccctctcttcttctattacatcgaggcgttgaattgggagcaaggatctgcatcttcccaatcaaagtctcgcattctcacgcggttgatatttaactcgaccttcgcgacagcgtctgggcggtactgacgttcttcattggatacccaatgccagatacggtcttcatcgtattcggttgagacgtcagtggtcatctcacgatagttatcgtccgtgtgcatgtatgcattaccacggaagatatccagttcggagaaacctttctcaaagcctgatgccataaattcgttatacggtttacggtactcaggcatggccaccaagaacggttgcagcagtgggttagcgtgttggaactccccaatagtttccaactgacggatgcattctgtgccatcggaatggcgcagtttgcgtacggccgcagtggtcttacggaaaagctccatgttcgctaactcacgacgatgctccaacacactttcacgcatgtcgggggcaatcaggtcgatgttaaatttgctttcaaagaaatcatgaaagccactaccggtttcttgtttcgtaaacgcggtagagatattcttccacatcgacatactcatttgctcctgttataagtcttcgagtgctaaacctacttcgccatcctcttcggcctctaagaggaagctgttctgcatactgataagttcgctatgtaaaatcatgcctctttctacctcattgactttggtagatgacatgaacccgttgtctggacggaaagccatcgccagatcgatttcgatttgatcggtcggacggtaaaccatgagctggtcaccatcaaagtcggcgttagccatcttaatgacgcggtcagaaatacgaatcgagcactggtcaacatccgtgatgatttggtcaatccacaacgcctgtacagacagctgaactaacgttgggttacgcagcggtaggacaaggatacccatgccacccggtgactccgcaatcagctctttgaagatttcatccactaacggatcatactgcatcgccgcttttgcaacaatacgttcacattgacgtgaagtaaagccacgttgtaacagtttcgactcgatgtctacactgagcaacccaactgaccaacgccacggtgccaccaacttccacgcatcatgcggtgaggcaattggtgagattgttgcacgccccgagttacacacatgcgttgaagatactttcgcacgatagtgacccggcttttgttccagcgtctcacgacggaagtcaatatggaagtaggtcaactggcggtttgctttcagtgctttactgataacaaagcgtgattccatactgcgtttacgggtatacagctgcgcaatgtttttcaccgaatcgatagctgcggtgaagatagggtcaatcaccacaccacggcgaccttcctcggacacaatcatcttcgacgaaataatcggcagatgtttggtgagtatcgctttgccttgggtttcgatcagctctatccattgtgtacgcaggatttcactttcactcgcattgttgcgctgcggtggatatatctcacgccagttatcaggccgggtaagaatttcaaaaatctgtttgtagtgaccggtgaaataatgaatcccacgacggacaccatgttcttccatgattcgctttacaactgccgcacgttttgaatcaggttcatccgaacggtagtacgggtcaaggaaccacatcatcagatcagatccgttaccgatggcaactttcgtccgatcaaacttgcgcggtttcttgttgttattaaagaacgcattgaacattgcccagaaacgtgggttgatgaaatactcaatctcatcaggcgcacgcaaccacacatcagattcaatacggttctcggtgacacgatatccacaacatggacattgtttaccgaggttgtaacggtgggcgatcgggttatcgcaagtgatgctacaaattggcgcagagttgagctgttcatcaataatgcggttttgcaccagcaggtcaatctgctcagccactttgatggggtcaccaccaatggccaagtcattgatgatggtcggaggtttgatttgtttcgctccggcctcgataaggaggtcacgcaggtaatgatcctgtgcctctaatcgtcctgagattccataaaactttggtgcctgcatttttacctcaaccaaaaaaagatggtggtagggtgggagcaaaagctcccaccccgactacactacaaacgtattacagtttgtagtcggtaagggttacacccagaccgaatgtgtcgataccaccagtctggccgttacctgacagcacgaacgtttcaccaccctggttgtagaacagggagttgtccagctcgttgttggcgttcacgccgttcacctggaagcttgctttcttacgcagcatatccagtacgcaacgtgcgaataccggatggattgccatatccagagattcgccagtaaagcgcagtgaacggttaccgtacattgcagaagccagcttagccaggtagatgcgctgagcatgaccttccagctcacggttagcgtaagactgggcgtgcatgtaacggtacatttcctgctgtttgtcacccaggtgggtagcaacagaggtcaggtccatatcttgcagagagcggtgcgctgcggtagacgtgtacacgccatccagagtcggcactgcggctgcaacgatgtgggcacaggtgatggtagaaacgttcaactgctgaccgaggtaagtagtgaagttcacgccatcaacatcaccgaacatgctgttcaggacgttcagcagctgacccagggtgttggtgttacgcagagcaatctcagcgaacatgttggacagaccacctacaccgttacccgcacgatgacggacgaccagcgcagcagagcttggtgcgaacacacgcagagcgcggtcaaccagctcacgagagctatccagtttacctaggtcaggagcctgctctgcaccccagctcagatgagaagccagtgcggagaacttacgatcctgtttgttcagggtgttgatgtacaggtcacgccagccgccgttctgtgcgatatccgcgaacgcgccgaatgcgatgaactgacgctccagcggggctttagaacctttcgcctgagagtcaatcagtgacacaacaacttcaccttgcagctgtttcagatcctgtacgccatccactgcctttttcaggccggtgaagcgcaggttcggataaccgcagctacgaacaggtgggtacgcagttgggatgctatcgctcagcagggttggagtatcgctttcctgattggtaggcgtatgctcaacgtacacagcgatgtccgcacggttcgggtgaccgttgacgtcagttgccacaccggtttctggagttgcaacgttcgctacgaagcgatcggttttcttcagcacgatggtgcccaggtaaccaacagcacgaccgaacacgcccagcagcagctggcccatcagagacttcgcccagttgatgtcaaccacattgccagagaagtccggcacgcagttagtgatcatgtagtggacgttatcgataccgtggtcttcacggatagactcagacaccttcgccagcacatctttattgatgaggctagacagggtgaagtaatcttcctgacggttggtggtttcgtagatacggatagactggcccttctcgaagaagaccagaccgtacagccatgcgccgttcagttcgccagcaacgtatgcggcagaacccatttcggcagaaatgccttttaccagaccgtaacggaaacgggacaggtattcatttttctcagcagcttctttcagcagacggacgaagtcgtttgcgcttgaagaagaagaagaccagtcaaaagcttggtcgaaagaatcgacgtggttgccagtgctgtagtcagcagccggggcagctttagtggtgttctgagatacgtttacagtctccgcggcagcagcagcttgagcttcaacgtgagtgtcattttcgccaacaaatttaaccatggttatataatccttgaaagataattagtacgagtaagttcacagtgataatatcaatctgtaaaattgtgggatacagttaagccgtcgcctaatgaataacacataacagaaagaataaccggaaccgtcacaatgataatatacatctgtaatttctttgactacgacctagttcctatgtggtaacacaggagagaatcatgttcagtcaagccgaattaaagcaagtggaaatcaaagggcataacgtcgaccctaccgctatacaattggcagctcttgtaaaaaataaccaccaacgtattcgcaactactttgactcggtacagacccgtgtagaatccggccacctcatcgcgaagttaatctcagccatcggttactcaacagaccccgactacgaaaccgtagagtgggcttgtcgtcgacggttgattggtatcggcaatgccgaacgcttaacctcgatgggtgaatacggaaaagtcttcaacggtatgttcatcgaaggccaagatgagattatctcgctcgtggcccgcccaatcgatcctgagttatcctttcgcgaatacgcaccggcccgctacctgtatcacgagtataccaatctaaactggcaactcgggaatggcaagccgcgtggggtgagtattatcgagatcaatctcgtagagctgctgtggcaacacgttaaagcgtttgcctattacaaccgttccaacgaagtagtgaccagcccgacgtatatctggcgacacgttatcagccgtatgctgccgagctatatggatatctcgttactcaacatccatcgctttgtagcaatgggtcaagatatcgagacggatcaacctttgcgaacgattccggttccgccgctgcgcgatattgctatccgcaacgccacccagacacgtcagtcgcttttgacgggtaatccaataccgggggtcgtattggcacacatcatccagccgttccaattcccattagatggagatcggactgcgattgaccgcatcgttcaccgtgatcccggattaacattccagggctcgtggcatctgacgttggtcaactggcattggatgctgtactgtctccagtacaacaaaggtcacatggatgcgtacctgaaggacgtctcgtatgagatcggtcgctactcagataccaaggtcttaaacaagttgccaaaggcggtctataaccacttccggcaaaccctgattcagcccttgttagaccatgctgaaaaatgagaatttactccctcccccgtaaaccactcaggtttacatataatagggaataacttgtaattgcactcgaaagggtgcaattacctcattttatttttttgactggtagtagctgatgttcaattgagaacacacatgccccacgttgtcgttactaaagcgctggagatggtacttaccgtctggagcaaccaccacaaaatccagctcaacgatgtcgtttggtgcatttagcgtcgggccgcgggtgtcctcaccgaccgacaccttaccctttaaacccggaaagcggttcaggaatccagccagctcagtaacacgacagtgtcccgccaagccgtagtcgagatcaacctcttcgaaatcccagacagcgacgtaacggtactgggcttctttcagcaggcgtttggccagcgtacagttcgggttcatctccacaaccagtgtcgtgcccttgccacccggttggtaaactttgttcgcctgcggcattcgaaaatgtgggataagtttgtcttcatcgagttcacgatgaagggcttcgttatacccggacttttcattggcatcgtcgatgattgcagcgatgcgacccgcgatagcgtgctgtatctgtttcagtttaccaaaacgttttaatttcttcacttcttccagcaaatcgtacttcatactgcgccctatgaaataattggcatggcgtggcagttaatgtcgcgtttcttcttcgggtcgtaagcctgaatgtgaatccgctctcctgctcgccagaccgtgatgttctcgtaccccttttcggtgtactccttgcgtatctccgcgatgcgctcgtttgacgatttgatgtcatgatacacgaccaaccaccttagtgcttagggggaaaccgcttagggtgtcgtgcccgataagcgtcttcctcagccattacctgttcgatacttttatcttgcaggcacaaccctgcccacgtacgcaggataaaatccacctgttcgtgctgcgggtcaatgtctgaagctttaccctcccaaataacaggaggggttacgttttgcctagggtagcaagatgtcgaacctgccggtaccggcccaatggtttggttgggcggtatgataatgttgttaatggttttatacggttggttagaaataaaacgcgccgtgattttattcagcggcatcctcttccccatcttcatcttcttcaccctcttccgcatcgcgttcagacttcttgatgtacttcacatctttcagttccggcaacacttcttcggcatccagagattcaccgtagtagtcggacagcagacgcgtgcgcttcttatcaatcatgaagacgcccaagcactcaagaacgtggtaatacggttctaccgtggcaaacgcagtacggcgtaaatctgccgcggcaatcagctccggtgggataccgtggttctctaccagatactctggcaggattaaggtagcgtacgtacgaccattggtgtcttcaaaccactgcttcgcaccattacggatgaccgggtcttcgatagactcaatccagtccttcatggctgttttagagcctaggttcactggcagtttcaccgcatcgtacggtggttcttcaagatacccatacttcggcccaaagatggcgttatacatgcgatggtagtgataagacttctcatcaccctgatacgcatcacgggatttgatgttagtcgttttcaggtaccctgcattaccggcgcgcagtgagtctacaacgttgtgctcgatagccgccactttctccagcagtggaacgatttcgatacggtcaccgcgtgcaacaatcatacacagttcacgaatcgttttcttgaactccttcatgataaccggcggaatgttagaggtacgcagggacacacccttaacttccagctctgggtctttcttgagctgaccttcctgtccggtaataatggagaagtagtgtttcgctttcgtggtcagcgcaaacgagtcaaacttatactcgttcttcattgcatacaggaacagacgctctttcgctacaccgatgttcgccgacatactggccatcaggtgacgaagatgctgcgtcgcaatgtaaatcatggcgtcagatacacgcgtagcttcacgaccataatgctggccggtataccactgcgcccaccactgcgcggtcatcatcgtggagtccgtatcggataccacacccacacgacgaatcatgtccggcatacgggcaatgttgataggcaggtttttggtggtcaggacgttgcgaatcagacaagcatattcgccgattgtgcgctgcaagtacatcgctgtgctaatcagttctttatacttcgcctgctcactccatggtaaggctttctccgtttcttcgtctttgagtttcacatcaccaaatgatttacccagtggcaccacatcggtacggaactgagcaatcacaatcttcatgtcgccgtcaatggtcttctcagcagctgaccagtcagcgtcagtccaatgggcacaatcgccatattcttcttcggaaatcaaggcaccaatgaagccacgcatgaacttgtcgttgtacttcgccagatggaagaagtcccccatgtagacgaaggctgcacgttcgaggtcactgacccgtgccacgtagtgttcgactttctctgccccgacagctgaacgccagtacaggttagcagagtagttgataacgtccatggtttcttggacggttggaatatgcaggttatacttctcaatacagcgtttgaattctgcgaagtcggtgagcgtaccgatgctgaggaagtgttcgatgacgcgggcaggcgtatcgtaatgtcggttaccacccaacagacgctcgttacctgcgttaccaaacgatgttgcggttcggcaggtggaagtcagtacagagtgtgacgactggttgaaaataacagtgtatggtgaagagaacgcacccgacataccgttgttcagagtcttaacggcgttctgctcgttcttcttgttcgtctttaagatgtcgttaccggcagctgccgcttcgtacatctcgtttttgatgaccgcacgtttacgtacgttctctgcggtgaattccgcgagcttcgaacgcttcacatgctcaggcaaatagaaggtcagagatggtgcagaaataatctgcttatcaatgaccacacgcaggagtttgtccacggttgtgaacttctctttacggtcacccgtttgctggtcgcggacccacagcttacaagtcgggtaagtgtgagccagctcgccatcttccgcaaacatttcattgagttgttcacggataaattctttgctgtacttgtggtcgctttggtgccagatgtacagcgtcagttgttcgaagtacgcatcaatgacatcaatgtcacgattgtactcgtcttttgacagccgaaagggttcgttatattccacgctgtactcctgtgggtcgcgggatcttcatctataacattacccactgacgtgaaaaaagatcaaaaaaaaataacctccccgccgaagcgaggagagtattcagttggtgttgtcaattatttcaaatgtgacatcgttaataccccggtcggccagcgctttggtgattaaatcaatctcctcacggttgtccactgtcgtcgagaaccgcacttgcaggttcttgataaccgagatactgcgaatccacgcatcggcggccacatgggctttaccgtccgcccctttgaacatcaagtagcgatacttcgccacattgttctccggttgggagacgatggttgagaagatattcttctgcttcaccgtcacatcttcaatactacgcgccatttcatagccgcatgttcccaacaccgtcacacgcgtttcgggttgaagcatcggggtatcataaacgatatttacgatgctcccctcctccagactcttcacgtcaaacatcattcctccgacacatcaattattagcctcatacccatgaggttatactgacattgtgggaagtccagtaccacgttcagggactgcacctttccatgatgacatgtcaggaacatctctaccgcgtcacggaactcttccacaatcgccccagcaaagaactgcgccaacgtttcaaccgaataatccaagagtgtcttggtcacggttgccccttcggcgttgtttgctttgtagagcttaatcagcggaaccaaatcttccaacacgccgtcaacggaaccagaatccatttccgtgccaaacttccaacgccgatattctttatcgagcgatttcaggaagttcttaacgtgggattcttcagcccgtgtcatggtgagcatgaaagcttgaaggtaggagggcatggtattgtgcaacgcggcgaagatcgcgtcttcttccagcggacccacgggaagggcaatcttcattttgggaaacgactcaaccgttcgtgtcaccagttctgagaaagcctcactgccggtcagatattctaccacaccgaggtgcatactccaagtgtggtaggctaccactttgtagaccatcgcaactccttaacactccagacacaccaccgtcccttttgggttcgtcaggtcgatgtttatgtgactggcgtcttttattgattcgaacgttttgccctcgcttaacaacgcatggtccacggtagcaatcacattgttaaagcgtaccacgtcgtccatatcgagcgtgtcaaaacacacgcgcaaatcgatgatggtgtcatgcgaccacacactggccatgttcgaaaacacgctggcggccttaacgggtacataagtaacaaagttgtttcctgcggcaccgtcgataatagcccggagcgtataggctgcgtacatcgcagtgaatgcgtaaaacgcttttgccgactcacccttgaagcgattgctttcttggttaacccggtcaagcatggcaggaacgtcacagatgtcattaaggtcaaaatagagtttcatgctcgcaaaccaccactaaccctttaaagtcatcaccgtaatgttcaatatatttccccggacacacagagccaatgacgctggctaggcccattaactctataccggtttcatctaagaacaatgcggcagccatgttgatcgctttttcatgttcctcttgcggacccgaacagccggggaactgcgcaaccatcgacgagacacgcggtaactcatccaccacgatatcttcgaacgtgcggtcaagcagaaacccttgctgtcgaagctcaaggccagaacgatcagtttctaagctgtaactgtcttcatcaccttcggcaaactcatcaaccagatattcaatgaatttaccggcatcccgcgttgtcaccccaatgacataggccatggcgtaacgctgatagaggtgataaagattatcaaccgtttcatcggtcacgtctaattggcaatctgtcagtatcgcggagatgtgttcacggacgtgttcatagaagcgggtagccccaaattccactacccgtgaagacacgtcgtaaaagaccttcataggcgaccccccagattaccaatcagcatgtcaaccactgtcagtaatcgcggcgtaatggcctgatactgctcagtagattcgaactgtggtaacttgtgctggttatgatcaaggtacacatcaacaccaccgatacacgttgggctgtaacgcgctcctacccacttaccgtaacgggtgaaccaataaggggatgaggagatagccaccatgaatgctttaccgacgttctgaatggcattcgcgtaaaccacagtcgagtcattatccagcacaatcccacgcgtagacaattccgtcgccacgtagttgaaagtgttcttcatgctgaactccagcgacccatccaaatggccggactcaacaaacgtgaacgcgcgattgataatcgtgttcatgtcttcgttgacttcgcggagaatggatgcagggtcaaactcggttaatggacccgccacctcttggtaatcggggatgaggcaataggtgttacttaacataaaggttgactcctgaagtaatcattttccacacaccacgctcaacgtgccacatgatgaagtcggggttgggtgtgatggtcatctctttgtctaccgcagcccaaagatccgaagactcaataatgtataactgcaccgtgttattggagaagtagtcgtcagaaatcggccatcgaataatctcgctacgcatccactttttcagggaaccgatatctgcgttaaacaaacgccgatgggtttccatgcggacgagcatctcgatataacaatcgacggtatccggttcatcaaaatagtttttattcgtaaatttatcgattacccgattaatctcacgataggtttcaggaaactcgaagtaaagcgttttcatactcctgatccttatacgggataaagcggataaactcatcggttacattcaaccataaccgataccctttggcggggacgttcagttcttcgcagatagcgcgacgaacgtggcgtgcccagttattggcttggacggctgtggtctttgggcgtgtagaacgcacaatgacagtcaccgcttgcccatcccatgaacctgtagggttaaagccagacaacagatagttgaacaagtcgaggataatatccttgagcaagacctgaacatcgtatccactcagcccctcttcctcagccaatattcggaagtaagctttgcaggtcacgaattttatcatcgttatctgaacagtaccgcccggttgggaaacgttgattgaagtagacatgtcgaatatcttcgcccagttcgagttccaaacaaacaagtttcgcacgaacaccgagacgtggtgtgatggtcacaatcgcgtaacggttgaacttgcgtttgcacatcctgcacgattcttcaatcatcgattcaatctggtcaacgaatctggtgaagatttcaccgaaggccacgtcaatcagttcacggatggttgcatacacaacgcggtcaaccagtcgtgtatcgagaatgtcattgccgaacacggtctctgttacgatacgggttcgcccacgaataatctcgggttcctccatctttttgtcgtgatgcaagagcttgtgcaactgcacttgatcaacgtacttctcaaggtggtcatgtagctgtgcgaaaggcatctcctcaagcgagaggaagatgtgttctaatgcggtatgcaggagctgtactgtcacctcctgtcgttgcatctcagacatgcgtagtgcttgcacatacggtgtcttgtctgcctcaccccaaaagctcacatgcacatcagctggtttgatgtatagcttgaccatgtttctacaaccccgttgtggtaaataaatggatgacggtggttcggacccaacttcgcaatcatgtaccaagcatctgtaccgaagtattcctcggcacgatccaataaaggtttatcgaggttaaacgttcccggatagatgagttcttgaattgcgttgatgataatccagtggggaccgatgtaaccgcgcttggttttcaagttcagttcaaagaacacccgcgtcatgagtagatactccttatggtttcatcacaaagataatatctatgtcaaattaattagactgtggtacgcacataatagccatatagcgtattttttaatgtaacctatcctaccccaccacccatgctatgaaagctgcctaacgccattctggagcccaaaatgaacgtgattgattattgtctccgtaaaatccggcgagacattcccttaccactgctgaaagtcgcctttacgccagagaacctccggatgttaggcgtggccagcagcattgaaaacgaaatcatggataaagtgattcgtgagtatctgattcccgaagtgtcccgcatggggcaatatgctgaacttgacttgcaggggttgccctatgagaatgacacggaagattactactcgcgcatttaccacatcaatgaatttaaaacgggtggccgcgaaatcctcgaagcacacatcgcagtcacgccggtggccggtcaggcgtatacactcccgcctgcgggctcgtatctggatggggccaccaccggtgcgctcgcttcgacgcaattagtcgtcgattcgaactccgcactaccacgtatcagttcacccgaggtacgggtactgggaccgaacaccatcaagatcaaagaccccggtatgtttgtctatgcgacaaagattgcgattatgtataagctcagtgaagaactgaacgaaatcaagacgcctttctatccgcgcgtggctgatttggcggtctttgccactaaacagtacatctataaccaactcatcttcgatatggattcaggtaagattgagaacggtatggagtttggtgcgttccgtaacgtggtggaaagttattcggatgccggtcaaatgttcgatgataccttacctgccatgaagcgggctttggttcacaacgacgacatcggcaaccgttacaactatatgtctggcggtcgtttcaaatcgtagacaaaaaaaagaaagaccaacccctgccgacgcaggggttatcttcttttcttttttacgcctgaaggagcacgttcttcaggtgactggcagtaccatagcaccacgcttcaccgttgcgaacaatctcgtcttgagcgttgcataaacggcgcagtgaaatagtgtgttcagccagaccagcaatgggtacgcgtggaggtaccgttgcttgcgccacgtactctcgcacatcgtcacacccttcacgttccgtccaatcaatcaccacagtgtcagagacatcaagaacgcgcgtgttggaaacctcgtctgggtggagggtaaatccccattctaggctttctaataaccggcggtcaagttctgactgtggtgcgattttgctgagcgtgtcggggtgagcgagaatcacgtccatcggacgcagtgtcgtcttcatggttcatctcctattggaatctatacaggcacagattccctatagggagggactctggcgtaatttttagtgcagactgcccatgttgtggaacatggcatagtcgctggctgaaatggcgtcaagtaacaccgcaaagatttcctcaaacggcagggcgcgtttttcgagggcttcggccatggatgtcaggaatcggaagaacacatccgggtcacgcatcatggcgtttgcttcgtcgcgtgagatgttgtacgacgtggtaatcaccggcacatcatcgcccttacggaaggcggtaccttcttggtaagtcagctttgaagaaaactcacggaacatcggcatgttcatgataatgggaaataccgtatacagtagcaaatcatcataacggcctttcgggatgaacgtatctggcagatagccttcggtcaacgcacgaataatttcaatcggttggtaaaacggaacgatattgaagctgtaggctaaattggatttcatgatgttaccctcctatataaatcaggtagtcaagtaaaaaaataaagcggggttttgctccccgctctaaagttatgctaaaactgctttccattcttcttcactgtgctcattgaaaagcgcagtggggatggttgggatagcagcaacatggccgttgttgttgaaacggtacagtgtttcgtagaagcccatcgggttcatgttggtcagacgtggtgagttgatgatgccgtctttcgtcatgatacgatccgcttcgatgtggaagaaatgcggaggtgtcatgacatcactcggatagattgacgtgcttgagcgaaaacgcaaattcatctcaatcgtagagcgaaccgagtagtagtcctgtccgaattccttatcacgggcatggtataaccgtttcaggtaaacgtacgttgccacccacgcatagtcaatcgttgggtggaacatacggccactttgggtgttaacgaactcttgtgccatcgcaccgtgcagggaagccaacaggatggtttccggtgtgatgagtccagtcggtggcaacgtgagtgtaccgactgggaagttcatccaactgttggtgtgccaactggaatagtcttccgacttggcctgcgcctgcttctcaatttcaaccaagcgggtagcgaccatgcggttcttcatgaccagtgaaccgtcggcattggtgcgtggaaccttcatgcctaagttagcatcgaaatcagtgaacaccgtatcaccaaaatgacgaatgaattctaccatggagaagtcttcgttcaatttctcagagcggtaattaatctttccgttggcttggaagtcaaatgcaccgacactgtagaaacgaccacgctcacgcgcgttatcgttatagtgtttcatacattcgtacgccagccagaactccgcgttcgtcagcggaagggcattgttgatgtcgccgaagcggcgaggaagatagccacgaatacgtttaccttcttctgcgctgtaaccacgagcggcgaaggtttcgtgtgctgacattggggtgaagtgcataagtttatcctcgaaggtctaatgataggttaaagattatagtttaatctcacctaggtaatatatatccaaaaaaatatacgatactaccctctccctatctgggagagggcgtaccgatttacgtcgacttacaaagcgtactacaggagagtcgcccttcaagcacgaggaggccaatcctcagggcgggtattagcgagcatgctaatgctttaacggatggagtctactgtacgaccatgacggttcgtgatgtagacttcatcgccttggtagataaactcgtaggtcatcacagtgaccggaacattgcccgtggttgggtcgggttgttcggagctgccataggcaagtacaccgataacctgttcaatagtgcggtcaccccgacggctggctttgagtaccgcttcttgcggcattgccgtatcgtcgtgataaatgtgctggagttctaccgaggaaatttcggtggcttcaccgccaaacagttcagcggagttatacccatcccacaatgctttgctgttgaacacagcaaacttcaactcatcagcttcgatgaaatcgagtgtagtgtggagggtttcaacagactggcggggaatattttggaactggatttcaaccggtagacctttcgggcatttccagatgatggtttgtccagtgtctttcaggaaggcttcttccagctgaccaaagtcagatgcaaaacgcgcattcgctttgtcaaacatacccggtgcgagttcactaatcaaatcaaccagttcttggttatctttgtcagttgcgctgaatgctttattaaagcgttctacccaaacgtcgatacattcgggtttaccgttaatccacggcttcgcatccattccagaatccatgcaattatgcacgttattagattcggtcagtagcgacatcgcatctttgaacacttgtgactttgaatcgcccaacgttggggactcgtgttcggttggtgtgcggttaccattgattttacgtaagatagtaaacataactactcctgctatttctattactgttgtttctattgctattgttgttagcggcttttcccccgctagggcttcattcgttttgttcccaccaataccgccaggcaattgaaagaaaaaaacaaaacgaacaaaggtggttctcggcccccgcaggggacagctaatgcaggtaagctttatctgcaaggaccgagaatttggttctgtactacccctgaccagtggatgatattttttccggaatgtcattcgggacaagggcagtacaaaatgtggcgactctgacaggtttcgaacctgtgacctgatgattaacagtcatccgctctaccaactgagctacagagtctaaataagggcgagcactggcacgaatcgaacgtgcgaatatccgattatgagtcgggtgttaaccaacttaacagcagtgctcttgctccggtaggactcgaacctacaccacgcgattatacaatcgttggacagctactcaaagcctgtgtttaccgatttcaccacggagccattgtttggtgattcctgtggagttgaaccacgacattacccaacagagccgagagataatgccccaagccgccttggggaaccgaaagggtgaacgctcgccatttaaggcaggtctgattccagagacacagtgtgttggcagcagcagaagaggtgatcaacggcaagggtaagctttcactgtatcggccagaaggccagcgttcgggggaacatcgggcttccgcccaacccgcaaggcacgaaacctttgccggtgtcacagtggacaatgctcccattgttttgttcttgctgtagaagtacccatccacgcagatgtttctaatcctgacaagcaggccgttgccgatagggaattcgggttgcgcccccaaccttctcatccgaagatgagacactctaagctttgagctaatcggcgtttctacgttcgcttctatttcccacagcaagagaacatggcagagaatattggattcgaaccaatggtacactttcgcatacactcccttagcaggggagcaccttaaaccaactcagtcaattctctataaatggtattcccgacgagatttgaactcgtgtaccgacagtgaaagtgtcgtatcctggaccaactagatgacgggaatgtaatgtggcagtgctgatgggatttgaacccacgatctcctacgtgacaggcaggcgtcttaaaccgctcgactacagcactataaattggggtgtatggagagacttgaactctcgacctccgacgtcacaagccggaattctaaccaactgaactacatacaccattgtttggttgcttctactggacttgaaccagtgaccttccgcttatcgggcgactgctctaccaactgagctaagaagcatttgaaaatggcaggactgacgggaatcgaacccgcgacctccgccgtgacagggcggcactctaaccagctgagctacaatcctaaaaaggttctgtgcttcctcgaccatgaatagatttgtcttacgaacgtcttcaggataaggaaacacaagaatgggtggtacccctccgaatctcacggagttctcaaggcgaccctatggcgtatatcgagacatcaacgcacagtccgcagaccgtgggtagacccgaatgacgcacaacaccggggacaaaccttcgcggcaatagcacgctggcaggaatgtgttacccggtaaaagtgggcggccagtcatcatcgcgtaagcctcaagggctgctgtgacaggtaccattgtttggtggaagcatccggtatagcaccgacctggaaggtcacgggtttttcaccatgagtttccgaagcagcgagctttacttccgttgtgtggcaggggcactaggaatcgaacctaggcatacagggatcaaagccctgggccttaccgcttggctataccccaattatttggttctgcttgcatgttgtagcctacaacacactcgggtcaggattgcttcgccccgaccgaacgatactccccgcagacggagggaatcccatcggcgctagaaaaggaggctaatccttaaccgcaggccgacgttcttgtatttggtgcacccaactggtctcgaaccagtgacctcgagtttttcaaactcgcgctctgaccaatctgagctacaggtgcaatttggtggcgtgtggtggactcgaaccaccgaagaccgaagtcaacagatttacagtctgctctcgttgccgcttgagtaacccgccgaataggtgccagaatcccgacctaaccctgcacaccggcaaacgccgcagcgtaacgccctgtgcaacatcaaatcgggtttccgacataatacagtgtagtcttgtaattagactttttatcgtaccggtttcggtagattcgcaggcacaagtatcttggctgcaatggtgtctttgccttcagcaaccgccttcgcaaggcgatgggcaccgtctaatacaatatacaaacttccttcatgcagcacgattatcggataatctgtatctgctttcttaacccgctcatcttcgagcgtagtctcgtttaaaatccattctattctagacactggaatttgaacgaggctatgacgttccgctatatccagcaatgtatccacagagtaatcatgactacggtgagtcaccgtgctttcagggccttcacgatacgttcccatcttcacctcgctttcgcatatataagtaacaacttgtaaaaagggttacttaggtgagaatggggttgatggacttcttcttctgagccagcgtatccgccggtcttagcgcctccaagcaccaacccctttcacattacctttgggataacctagtccacgacggggggttatcgccgacgacacacagtcgccttttcaaatctgggaacttaatcccattatgattttcagattgtattttacaggcgtagctgtccggcttatcgttccggtgcttgacctatgctcacggctgtgaacatactaatgtaaatacgcagtttgcatgtggctctctcgcgagaagccttttcgcctgtaaaccagtaatgggcaagtttccagattcgtagctgcttgataaggcggcgtaagctgcccatcatgtcgagcacaaatcctagaagtccttgcatagattatttgctcacctaatgaaatcgtgaacggtcggttacctaccggggaagcttcacagcttacgcaatagttctttgtgtaaccggctactgtcgacttacgggtatgcgacaggtctcagcgaacgttaccagccttaacgaacaccgcgcaggtagggacatcaaccctacccagcccgaaaagatgcactgggtcagtacatggcttttattttttgtctcccatcactcgtgagttatttttcaggaggatggtagaaacggtttcgagcagatcatcaccggactcggtattggctacaacgagtgtggtggtgcagggcacgtcaactttcttaccgaagaatgcggtcttgtctgtcttggccgtttctttcgtgtagaccgactgcccgttaggcagtttgtcattgacgttccatgtgctcatgtcaatcagttctaaaccagaactgtcttgattgaccgcttcgaggaacttattggttttgcccggcgcagatacccacaggaaagcatcgtattcacccgttgccactttggacaacgaacggataccgcccttggcgtaagtttccgctttggaatactctttcaccaactgttgcaggtattgccaactggcgtatgagccagagtccggttcacccacagcgattttagcgccatcggttaaatctttcgcgtctttgattttgccatctttcttgacagcaacccagacacattcacgcgccagctgaccaacgatgtcaacgttctgcgcttcgttcgggtgcttagcacgccagaactggaaagcatccgcctgcgtaaaaccaatctgggcttcacctgcggctactttgtcgaggttgtctaatgaccccttcgacggaacgacccgtgcgcgggtaccaaactcgctgatagcaccagccagattgacgccatagaccgagttataggtcaggccctgttgccctgtagtaatgattacttcgtctgccgcgactgcggacatgctaaacgtcaacgctgcaagtattccgaaaagcacctttctcatggttatacctatttttagatgagaagaaaagggtggtgcggagggaacgacccccgcaccgaattactacttgcctttcaccttcgcctgcgacttcgccgcaaacttcttgatgacaggccaggccagatacgctactaagccgattacagcgacgtaggcgattaacgtgaaagctcgcccaacgaagttgccaagcagcatcagcagcagcgcggccacgatgtataacttggttttcagcttcatggcttacgcgtcgtaacgcagacccagagcttcagcgatctgtttcaggaccgcttcttcttccggctcgatttcaccatcggctttagcgatagcaatcgctacatccagcacgtcttcacattcacgctggtcacctttcacatcagagatttcacgcagggcagcacgacggccaataccgatgtctgcatccagctgtgcaatgatggtagatgcgatctggttcagttcgccctggaagtttgccagcgttgggttagcgcgcagcacctgttcgattttcgctttctcagaggcttccagttcgccatcagcgtaggcaaccagatacgcggcattgaccacggcttgagccaggtcacgcttttcgaattttttgatatcagtcacagcacggttagcgcgttttttgaacattccgaacatggtaatcaatttcctttaggtgggtgagccagcgcccaggagtagaagaccgtagagtagcaacactccaactggcttcacccccgaaaggctctacgggttttttgtaaagatgacctgtcgggcgagacaggaaatgtggagggacgccgcggaattgaaccgcggtaacaggatttgcaatcctgcgcctaagccactcggccagcgtcccagagtttggtgggccgaagcccacctattcagcctgcgttaaacgattcatgaacaataccgattgggaggtgtgtggttccgatgtttgtgcaggtcagcgtttccgcctcatcccatgcctcaccgtacacccaaccaccccttggacgaattgcgcgcgccacagcttccgaaggagctgcaacgactatggaatcaaactcgtcgtatccgacatcgtctacacgttcaagcaaatacaagttcatgagagttctccagcgattgactatttggtcttccgcggtttctcacattcttgctggctaaatttggcaggggaacagagattcgaactctggacacccggttttggagaccggtgctctgccagctgagctactcccctagaattcaattacgtgcttctcagcatacaacagggtaaacttgtaattagactaccgcgtcgttcaaattgcgcgtttggaggtaagcccaagacttcagtgctgccttgagtgcttcctcgaaagcgttgttgatggactcgattttggttaccgggctatagccttggtaagtattcaccgtagtggcatcgccgtctttcgacagaaccatcacggttaccaaatcggttgcagcccacatgtgaaactggacggtggaaacgacttccgtcaacgccgcgatttttggtacgcgggtattccccagaatcgcgcatgcctcatcgagtggatacgcaaaatcaaacaccagctccggttgaactttttcttcgctcatgtgttactccagcaattgatggacgagacactgtcgttggtgttcacatcgaacttcgatgcgatacggacagcgtcttcggctttggcaccggcagccatggcacccaatgcaaaatctccaccgctaccgacagcaaccggtgcatcggcttgcatcacccacgaacggtcttcgtcggaatacttcccgccaacaaacacggtgcggtcttcggcaatcgcgatgaacgcgaacgtaacgcctttggcaaacgggtcaccggctttgtggccagcgaatgtttccatcgcggcgcgcaggtcgttagcggcgtgcagattaccagccactccgaatgcgacgatgcgcttgttctcgactgaccagtcacggtgaggggctgaaaagatttttaccgcggagttcgacacacggatattcccttgagtcgattggctatcggacgccagtgtttttccatcgtacgcaatcgtggtcatggtttatctccggtgctgtggtttgaacacaggaacacccaagtttgtaaaaaatcacattcagcgacaccctagcgcttcgcagcgtgggggcacccccctctcgtctttccgagccgccaagatgtggatcactctcctgtcggaaggttctccggtgtacacggggctaaaccgtgtacggttatcggccgcaagccgaattcgaaatctggtcacaccccagggagagttcacagcagaccgacggtaagttcgtcgatgacgtatcgggtgacggcccgaaagcggtgagtctcccgtggggctaccacggtaccggtctcgtcggtggcgaccaccgagtctctgaccagaacctgaaacgcgttggggaagtgttaggctgtcccgctggctttgtccagaacccgcatcgtggattctcgaaaaaggcccgaggatgattcgggcaagcgtttggttcgtcgtgcatagaactgggaaaacttgtaattcgactttcccccgatccccggttcccggattcgaactcgtaataaggatcacgcgcgttagttatttaaaacccgtagggtttatatatatttaattattaatattatccctacgggatatatatatttaataatattattaattcttttaaaagatcctgtaggaaatggcgtgcgcgtgcacgcgtataatgaaaggactttttgtctgaaccccagagggggttcaggatcggggtaaagatccaacctaagtgcttgtttttaaaataaaaatttttaaattgagtggatctcgatcccggctagaggccggggagagtgagtggttaaaaaacaaccaaattcagccaaactcacaaagattcgtttgtcctgaattcctgaatttgatcctgaaaacgcgcaagcgcaccccaacgtgtgatcggcatcggcggcgcgcagcggcgaccctccacccggaaaccgatttgcaacccggccaaattcgctctgtacgtttctctgtggcccgaacggggtatggggaacccaagtgtactgggtaggatgaaccctatctcaaaatcgtgttgagtgcgaatttaccccatggttaaaaagtgtacaatctcgccatggacatcggacgatgacaacaaaaaacaaaaaaaaacagggagccgaagctccccgatttctaccctaacgttttcgtcagggtcacattgttcagttcgaagtcaggatggtcatccagcgccatcccccaatccgcagacatcgcttgtactgagaactcacggccttcagcatacgacgccgcagccacttcctcaatcagtttccaaaggggtgggttacgctcctcgtctttcaggataagggcggcacaaccgggggcaatcgcgaccaaggctgaacccagcgcagtatggacatctgctaagcccacttcgggacgcggctcgaaggaatactccccacacagggccagcgctttgttcggcttgtagttgcaggtgaacattgtccagccatcagcacccggcagctggtctttggtaaacacgttaatcaccttaacgtcgctgtacgccattttggcgatgttttccatctcaggcagggatacgttcaagaagaacgggaacgtgatgcaggagccttcctgaagcgccatagcgaccttctcagggcgaccctctttcatcaccacccaactggtgacaatggcatcttcactggccgacttctccacggcgttgatggcatagataaaatccagttcggtgttttctggcatcagtgttttcagggtaggaacgcgaacgaaattagacatgctgtaatcctcgatagtcaatgagttaggttaagattaataggctaatctcacttaggtaatatatatctgaaatattttttgttcagacaaacaaaaaaatagactgtgctacccgaaggtagcacagtcagtcgttacgaacggatactcgagccgtcagtcccaagatagacaggtttgatccacagccccggttccccgaagaggttgatatcatacagctgcatattccggatactgggcggcacgtttacgcctgatctagccagaaaatcccaaacgccattgtagcgatctcgacttacgaagaacaccccgttttcgaatcctgactcaaagtcaaggaagttacctaagcccacttcaaacgaggctgcaccgtcttgcagcagggctaagaaaccaaccgagatatcttctcgactgtcgataaagcgactaaattcggcaaccgtaaggctaccaaagatgcgcttgagtaccgctgcaatggacagcagttcggtggggttacggcgaccatagccacccaatgggttgtaattaatcatggcggtgatgataccttcatcacacagatttgccagtctgttatcctgacaaactacacgcaaaccatttacgttttgggcaatagcggtaggtgtagcaagcatatcggttactcctatgtcatcgttggggtttttgtcctatcaacgtatttgagtctgattccctgtaggcgatatcccgtcgtgtggtaaaggtggttttccacacaacgtacgaacgcatctggatcgagtgcgtctgttgccaaatcagattcgaaacgccaatcctccgactgcccttgtcgttcgagggtagctgcatagcagccgtcctcgacgcccctggtgaagcggaacagttgcagatcggactccccatcgcacccaatgatagaatccctgtcttgcgtaatcctcgcccgtccacatcgagtggctgtcaacagcgcgttgttggatggctggttactaatgaacataaagggaccatcgtatggggggatggcatctggacacaatgtgtccaaatcggtacagcgatacacaatgggtgacttatagttacacagacggttcccgtcagtaaacattgtgtattctaccctcacggtggcaccaatgaggttttcgggcctcaagttcttagccttgagttgcgcctgtatccgtctcgagaccatgttcgttaggaagacgtgattggactgggtacgtaaaacatatccgcgtgacgtacagtcgacaatctttgcttccgtccgacgttctggttccagacggtatacctgttccccatgctccacaaggaattgtgagacagaggggttgcgagaactttgacgaacgtagtcgaggacttcgtaagccgccattgtcgcgggcttaataacgtttacttggaaaggcagcttcttggttggaacctgccccatcgttgaaacggtgagtgtccgcaaatgcgggtcatcctcttccggttctgttgacaaccaccacgtcaaccagcgagacacgttttgtggaatcagtgctgtggtatgaatcgtgatgtcgcccgtgatacccgcctcggtgagtaggcgagccagtaaagtgttggcggcagaatacgtgccattttcaataacgaccattccgcccacgttgcgcagggtgcacaaacaaccgtggtcgagtttccagacaacgaccggtgtggacttgtcgaactcggatgaatggtacttatgattccagtcttgttttctgagtaattttttcatggtttaaaaactccttatggtattatcaaaatgataatatctatccgtaaaaatttagaggaatcgttatgtccgaacttatttttgacttcacgacggggtgttatcgtgatggaaaagagttagcggtcggcgaatcgtctcgtaatcgcattccagatgagtgggacattcctctggataacgggttgatttacgactacggtttaggcgggtatattcctgctgggcagattgtggcctccgaggccgtcaaaaccgaagcactccgcaaagccttcgatggtgtattcaagaacgtcacgattgaccgtcgtctggccaccaaaattcgtctgtatgtctctggtgtcttcaaccgcgaaggaaacgtagagtggtttggttccaaccttctcggtgtgcacaccattcgtttttacgacagtgaccgaaatcgtctgttcgatgaagtgcttgaagtggatgaagatttgctcgaagccgaaatcgcccaaaccaaaacgattaacgccgattgggcagtggccggtaacacgttcaacttgaccatcgcctacatgattcatgcgatgtacccgaaattctccgacaaagagatttacggcgctgcggtggatttggtgaagctgctccagttcaaattttactcgagtatctattaccacttcttcccgaaaccggttgacctgcctgcggccgaagctgcctactccatgctctcattgaagttcgatatacgccgtatggggaactggggactgcacatgaccgatcgtgctgaatactttgtctcgaaggagtgcccgcactacaacgaggtcaaggcgtttaaccaccccgatctgcttatccgctttatcacagacttgaacacccgaaccaaacagacggtgaaagactactacgccgtattggatacggtacgtcgttccaatgctcgtgtcctcagccagtcgtcccgtatcgatttggatggggagtcgattatccgcgataaggtcactgcacttaacaccgccaaacaaaccttgattgatgcgtcttacgacatcaacaacttctacaaagaagagttggcgcgtgtggcgctcgagatggtgccaaaggcatcgcctgtggctatgaagacggttttgttctacatcgcctctctgccgctcgggaagcaacgtgccgaagtagaaagcatcatgaatgacgcactggcccacgcttttgatttgattgtttccaatcgcatcaacttcaaagacgtggccttcctgctaaacaggatgcgtgcgttgtatcagtcttcaaagtccaccaacgaatatgtcctgtcgttgcgtgaccgcttagagaaactggtgaagaaagaaacacacttgacacataccgctgccctcgctgcggtacgtaatgcgttacttctctatttcctcgtgcgggcgattgccagctaaaaaaataaaagaacggcacctactccttttgggggtaggtgcctattcttttttaccgtgccagcagacgggtttacaggaccgagagttggtgtagtgtataaacgtaatgcatccctgatgtcgcgatggcacccagtacaatcattccggtgatagcgaaggcttgcgatcgaagcaagaccatcgtggagagattgttctgaatggcatgttgtttaacaacgccgtgaatgtggtgtatggacacaaacatggcgatccaaactattgctaccgctaaataaaagagttgagtcattacttcatcctctggcggtggataagctctttcaagctttccatcgatgcgacgttgcgcatatcagtgttaagttgagcgatgagggactggaggcgattgcgcagagtcatttggcgtacaggacaagtcacacccacactttgcttcatcacttcttcaatctcacccatcagttgctgttgcttctcctcctcttcgaccatcgcgtcctcgtctccagtaacatctccacctacaaggatattgcgatttcgaatcattagccggttgttggtaatcccatagtggttcaggttcttaccaaataagagcagccacattgccagtaaccaagaaatgaccaagtcatcgtgaccagatttctggtggtcaatacgtccgctgcgctctaccagaccaaggatttggtctatgagttcaccactacgaagtaagtgggctgataagcggagagccatggtgaagacctcaccatataatttccggcgtttatcaccatccgtagtaaagccaatgtacttacggaatttgtcccagaaccgctcagcgtttccgcctgcgggcccacgagcatactccttatacaaatcgtcgttacggctgttggtgtcggttatcctgacgtacagacgacgatgtaaatcacgcacgcgcgactgtaattggaggataatcgcatccgcaactgacgaaccggttgacttacgttcaaggataagcaccgtgttcgggaaccgttccatgaagtcagccaagtgaattgcaaaaccgatgacgttcgtttcgttaacggtcatctttccggcgtactctgccgtcactgagtttacgatagacatcgcaatcgcatctcgaccaacggcttctgacgtatccagaccgatgatgtggcggtcatggagtttggtcgccatttccatttcaccgtaataccagtcggtgatgtagttggccggactgatgtctttgtacgtggcacgcatacgcgaaccgttcatgcggcgcgcatcgtcacctgagaacggtttgttgaatccaccggtagtccattcaccaccgaagtcacggcggatctggtctgggctacccgtggcgttcgcaatcatgtctgcgagcttcgcatcggaggtacccaattgacggtggttgaatttcgcgtagaacatgatacgtggcatcttcgacgtggagttgtgtcgaatcatgtcaatcagctgctgacgggttggaacgtcaatgtagcgctcgtcccagttaatcccagaggtcatcagttcgtacatgtactgaccttctggggtcgccagatcgccaggcgttgtagcaaacacgttaccgtaaggtacaccagattcttcgttgatgttacgggcagccgtaccggatgccagtgcggccggaagaatgatgtggatgttgttggtgaaggggccctcatccgagaacagacgtccggcggttaaaccacggcccacaccgtttgcagattgttcatcgttctgaccaatcgcggtaatcagtttgttaccctgcgccatacacgcaaaggcttctttgttatctgggtcatccgggtggataggccacagatatttaggcaagcagttacgcagctctttcagtttggtgatggtttcttcacgcagcaccggtcctttggtgaccagaatcgtacgcgacttctcaaggaaacgcagcagccagctcaggagcgagcacatcccgacggttttaccgtgctgacgaaggaactcgatagcaacatcgatgttgttgaagaatatccaaaacatcgcgaagttaccgcggtcaatcttaaacggtaccccgtcggtaccatccgcaggaacgcgtaagcattcacggatgtagtaccatgggttacgtgcacattctgcaatcacacgcgcctgttgctcaacagtcaggtgtgggtcgtgcggatctacgccttgcagttccgggtcaagaagtgcaagatgcaaataccaatgctttacaccgagcccttttaaggtatcggcgaaatacataaagtgtttgttcttggtggtgtcatccgctaaagcgcccggataaaaaccccaatcacgttcacgtaatatcatggttcctcctagcctcctccccggtcggggaggaggaaggtgttagctgatgttgtgtgccaacatcggtgagcaagcgagttgtagggtatccgttggtgtacggcgtaaccaacgaatcaccagcgtatcgtcgagcccgactttgtagttcacgactttggcactcatccagtcatccacagccgctgtcaccacttgcccaccaacgtggatttcgaagtgagtcggttccagtggaccggattcgttacggcggtcgtacagcgggtacgatgggtcgtaaagcgctgccagccattcagccttagtagctttaccacaacgcacatcgatttccgagtagttaacgttcgagtatttgaacgtcgcccagataccgtccccgtacttcagcccatcaggcagatattcgaggaagtagttggtgttcagttcggtacccggattaaccagcgtaatggagaaggactgagcctgaataaacgcccggaacttcgaatccactttagagatgtcgcactggacattcagtcgctgtttcacgccgtagagcattgggtcgaatgcttgcccgcctgttaaagtacacgctgctgttgcatcgtagacctgtccacgggtcaggttgtacagataatactggaggcgatagccttggttggcgttcagccactttggcaccacaaacagtttcatcgagtacgccccatcgactgtttccgtcaccgcggtataatctttgaagattgtcccgttgatgaggttctccccgatgtacgtttcccctttggccagcaggtagctgagcgttagcggcagctcgttaccagcgttggttgacaggtaatacgtgtcgtgggagcctgcgttacgaatcccgttgagaatcacacgagaaccatcgatactcagcgttttttcaccgtccgagtatttcacgacgaccgacagcggaatagagtccagcggaatattaatcggcaacgtcaggacagtaccgttgtcatcgacgataaacggcgacaccagtttgatatccagaatctgacgactggcagtatcctgcggcatcacgaggtttgtcttgatgaagtacccggtaccgatttcgatgatatcaccggagtcggcataaacgacaaagctgaacaactcaccgtgcccgacgggtgctaacagactgcccggcagtggcgacttaacaacagtctcgacaccgtccttggagatggtttgcatcggcaggtagttcttgtcaaggcgaccgtttttgtagaagcccgacagaatctccccgttatccgaaatatccgttccacggaagatacgaatcccatctacatccggcccgttgaacgtgatgttgttgtccatcaccatcgtcgcgggatttttggtggtgtcgaaatagatgcggaacttatcagaacggagtggataatgcccaccgttaatcttgtccgtgttcgtcaccgggatggcgttaatcacctccactgtccacgatggggtggagtagttaaccgttaagacacgctcaacgatgttgttgtcatgcacaatccagtcttttggattggggacaaagccggtgcccgtcttctcgtcgtagaggtcgccttccccccagacgcgaaagccgcggtctctgtcgataagatcagtcaataaagtggtcatgctttagaacctttgattttcagatactggttaagttgcacctcacctttcagataccgttgattcacacggtccaagaaagcaaagcccaattcatcaacctctacaacctggtattgcgagtgcgggtgcacacgcacaaaggctttatcgtagccaatgaaagccgggtcgaagttcagaaggtcaatatagccctccatcacgatgtccagctgtgaagtcgaaatccggtattctggatcgtcttctaccaaatggaggtacccttgcttgtaatcccacagcactttgtttaaaagcgggctgtaaagatgataccagctctttaacggtaccggattcaccggcgggggtgttgggtaccacgcggacagatagtcctcagtacgggcgtcaatgtcgcgtgacgcatcacgcagcgcataagtgtcgccagtaatgagtgtgcgcaatggtacggtcggatcatccacagagaacgggaagccgtcgggaaccacgtctacacccactgtgttgtcttcacggaagaccacctcgttacgggtcaggatacggcccccggcaacgatacgaatgaccttatcgtcccgcacatcgaaatggctgttgttggacagcagaccacttgagacgaaaccggttttcggcacatgtaactttccggtaactccacgagcacgcacatccaccacgttctcatctgtgtcactggcccagactttacagacgatgacaatctcaggccagaccacaacgtagtcgataccaaagaccagcggacgtttgtttaaccaaacttccactgtttccatcgttgtccacagcgtacgaatcggctcgctgtttgagcgacccagaattggaatacgcaactgcccttctttgaccttcacggtctgactgaagaacaggtgacggtcatcccgcaccacggtcggccaacgacgtgtccggtcaacgttccagcgaatcgcattaccttcccgcgtgtagtctttccccaataccgcctcggtgtattcgttggtgccgacaccactgaccactttacgaatccacagtgcaacgttctccccttccgcaatcgtgaagtctggggcgttgtcagtgatgttcatcgcggtatccacgtcaccggcgatcccttcgatgtaacgtgctgtggcgttcttcgctgtatacaccgatgtgttccgattcgggtaacagcccagcagtttgcccgacgagtcatactcgtacaccacggagcgtgacgccaacaggtcagggagcgttgctgtccatttaccgttatccaacatcagcttctgtggcgtatcagccgagtagcgagtcacggcattataaccgtaagcatccgtggtaaggtcacgagtgatgttagcctgtttcgccgcagcaactttgttaaaggccgcattctccaacaccttcgctgtccattctggcactgtcgcgtttgcccctaccatcgctgcaatgatgtccttgtcaggcatcttgtacaggtcatggatgtggctggcattgaacaatggttccatcgcgagatagtcttcacggataatgacacggataatcacatcgtccaaatccgtaatcggtttactgaacgcattacgcaactgactcagccgctcggtggggatgctgatgtcattaaacgtgacctgacgaatcgccagatgacgatgacggtgatagtagcgaccttcccgcccattcaagatttgaatctcaacatcgttgttgaaaatccaaagcatgcttgccgttttcgggaaatgcaacaggtacttacgtttcgcatccagcgtcgactggaatgtcggtaaatcaccacaacggaaatccaccacgcgaataccgcgaccatccaccacaatctcaacatcatcccacgttgagatatccgcaggtaccggattgataatcaacgagccgttgacccagaaactcacgtagccgttgttctgaccaaccagtgagttgtaacgatcgatggcatctttgattttgttggcattgggcgtttcaaagaactcgacaaacgtcgggtgcacttgcttggccacaatggtgccggtgtagccgggaaagatacgccagtaaatgtcgtcggtatccagccacttgtaccgatccgtttgtggaatcgctaacaggatttctccggtatcgcggcgcattacgaacgcctttgagaccgggaaggttttcccgttttcgttatacagctgcatgaaggtgctgaacgcattcacacaggctgatacccgcttccagcggtttgggggaatattgaggttcccccagttcatgtggagtttatccaccacgtatgcgtgccaccaacctacgtccggtagagatacagacacaggcccgttacggacaaagccggtcgcgccggtttttggcgtgatacgatacggttcaataatcagtgcccgatcaaggttcgggcgctgccaagcgttgtcaaccgcgtgggcgaccagccagttctccataatggaacctcttaacctttgatgttagtgggtttggtgttctggttcatgatgagttcgtacgtgaacaagaacttgtctttcttcttcgcggtgtccgacttcttaatcgtgccacccaaacgagaacggttgaacatgttgttctccagtgacgcgcgaatcatgaccagcagagaaggcgggtattccagcgcgctggtacacagttgcttctcatagctaaccccgaagaaactggtgttgagcatttgctgtaacgacaacacgctaaagtctttcaagcgtggtgtgatgtctgcgagcttcaccatctccacaaactcttcgatgttacgcgggaagagatagtcggtgtgaccactgatggcctcgaacatctcgaacggcgtacccagttgacgggacaattcttgctgcaaacgcagcatcttcatctcgtcttcgaagttgttgtagaactgacccacagagaacaaagcagccgctgctcggatttgcccgctttgatatggagtgagtgcgtacgcatgcgtaatcgcatcgcctacccatttgctataaatctcatggtggtatggaagctgtgccatcaaagcaccgagccgactattgtttcgtttccacactaattcccaacgagcctgatcgagacgcaaagcgtgttcgattgggtttcgaatttttagctcgttgtttctatccaacgaggtaaacgtgcgtgcatctacatacacgtcgtcgccgataactatcggtaaaggaaacgattttacatcggcagtctcaacaacgtagtgaacctcgtcagattgcgcgacagtttggttgagtttgcgagccagttcgatactggcagcgagtgaattcaggtcaaagctacggaagacgttgcctgtgtaagcgttttcaagtgccatgagttgataccttagtatgaccgtttggtcttaaaagacgaatttatggagatgttccatgagctatattccacgtaacggcgcgcccgtgaactacaaggaagggatggaagataattccgtacccgcacttgtgagggcacctacgggtgacccgattcataagccgctgatcttcacctttggcgcacgctgcgttggtgacgaagcgttcccgttgagtggtgacaacgccctcgacttaatgggccgaggcatcttcgatctccgcggcccatacgcgacgttcaacacaccgtaccaggcgatgttcaatgccaacgccaacgagtgtatgtaccagcgccttatccctgatgatgcgaaaacggccaccatccgtttctacgcagatgtactcgccacgaaagtgccgaagtacgtgcgtgatgcgggcggcaccgtgcagtacgataacaccggtaaagcgaaagtcgaagctcaggttgatggcctgctcatcgtactgcgcagcgtggttattgacagcaacagtccggccatcggcgctgcggtacctatcgacggtacactgaccggtgagggcggcgcgaagtcgaagatgtacccactgttcgatattgaagcgccttacgcgggtgcggatgcgaacggcttcggtttcaaactggtaccgttgagtgagaaatcctctccggcactgggttcggcttaccagacgaaagtcggtggacgtgtttacaacctccagtggtttgaaacactggcgggcgtctcgtctgcggtcatctggaaaaccctgaacagtatgtcaagtgtgaacttcagtttcttacctgacgcatactatcagccgatgagaacgcagctggacttcgaagtggttgttgccgatgcttaccgtaaggttagcccggatgttggcgagctgccaaactacggtccgttcaaaacgttccacgtttatcatgaccaacttgaagccgtgcttgacttggctgcgggtagcatgacgaacgcacctaccgacaaatatctcatcgatatcttcggtggtctggatctgattggccagccgtacgacggtctgcaagtgaaccctgccacggaaaccggtaaagcggtcttcggtagcagcaacattcacttcctgcaaggcggcgctgatggcaccctgggtaacgatgtatacgatgaactcgttcgtcgtgaaatgcttctgttcccatccggtggccaagttcgttacgacaacgaactgaaatattcactgggttgtttctgggactccggtttcagcttcgacaccaaatcggcttgtgtgaactttatcggtaagtcacgcaataccttcctcactctggcgacccacgtttataacgaaggccgtaacgacctccaaacggaggagagtgcgaaggtggccctgattgagatgatcacctccgtgccggagtccgtgaaatacggtaccccagcagcgcgtggtatggtcaccggtcaatctgcattcatccgcggctcctcttacaagaagccggtgccgatgaactacaccctagcgaatatgttctcgcagtatctgggtgcaggcaatggttacgctaaaccggagaaacgtttcggtcgtggcgaactcaccattatcaccgacctgaccgacctgagtatgccgtggaaaggtatggacgtgtacgcttctgactgggacgtgtccctgatcactgcgcgtagctacgactactaccgtgacttcatcccggcaattcagtccatctacaacgaagaacgatctgtcctgaacaacgcgatgttcaacttcatcatggcttacgtctaccgtgtctctgaccgtgtgtgggcggcaatgtcgggtgaagaccgcatgactgatgcggaacgcgcgaagatgctggaagataagattatcgaagcgctggaaggtcgtctggacggtatcgcggatattgtaccgaaagcgtacttcaccgcagaagacaaatcgaacggttactctgtaacgctggatctgcttgcttacggtggcgtgctgctgactcaggtcaacaccactatcaaagtctaccgtcgggagagctgataaatggctatcaaagatcgtttgattcaacccaaccaggggttccactttgacggtggtacttacgacatggttaacccattcgcatcgggccagaacggcccggtcggacaggtcggtaagttcgtcacgaacgcccaccgcctgcgtcgtaacgtcatcgcgcgagttatggaattcccgcgctgggtggactacatgcctaacccgtcactgtggcgtcaggctattaagtccttcatcgaagtccacaccaccatcaccggtctggataaaacactgagccacgaagcggttcagacccaacagggtcgtaacaaccgtattcagtacgaagccggtctggtaacggaagcacagtcctctgtgacccataccagtcctgataagtacggtaaagtgttccagaacatgctggctgcgtggctggtctacgggatctgtgacccacaaaccggtcatccgggtattgtggcaatcaacccgaacgtgccagaccacctgccggatatgtatagcctcactgtgctgtacattgagccggatgcgtatcagcgtaaagcgcagaacgcctggtggttgaccaacatgatccctgaaactgcgggtcaggataccggtgagcgtgatccgaacgccggtcctcagacgaacgaactgtccatcaccttcaccagccagcaatggacgggttggggtccgatgcaggccgctcagtctgaactggaacgtatgaagctctacggcctgcgtcctatgacgcgtaagctgtggctgactccgtctcagcagtacgatggtatcaacccggatgtccaagcgactgcgggtggtttcaactctgtttccgaagaacagaaagcgaaccagctggcctaaggcaaaaaaagataagcttacccactccttcgggagtgggtggcttttttatttttttggttcagacacagcaggcggtttctcaccttccgcttctaagcggatgaccaaccatttaacgtggctgataaacaagaaggtggcgaagacgtcataacgtgaggatggcgcgacatccaccaaggttgggttggcaactgaccacaatgtcaggaggttcttgtcgccaccttcaagtttgtttaagtcggaaccattcagcttgatgtgttccttctcgagaacattcatcacactttcacccaactcataaaccagtgctgatttataacgcaggataaacccggcggttttctgaatgatcgtcgcggtagtttcagataagaatcgctgatagccgttggcggtacaggtcatgatttcaaccgggtactcagcaatctcagtgaattccggtaaggtcagcgaagagagcaaaccacgaatgtggatttcagccagcaaaccaacacgggtaatgatttcttcacgggacaatgtgcagggcagcgccccattggtaatgggactcatcatttcgttcataaagtttctctcaagatcaaaaaaaagaaagctgtcataagacagctctctcttgtaaccctaccgtcgtttccggcgatagagttttgctacgccatccaacggctttggtgttggcgacttgacaacgcggactgttacacccacttcgtcgggtgatgcaatcgtgccgtctttacggattgccgtgaacggaataacgtcagggtgatggtcgatgattatcttaaccattactcttcgtcttcttcgtcctcaccttcttctacttcgaggaagcctttggcgaagtcacgacgcagcgcgccttcgagcgctttgttcttgatggtgctgtagccgaagccgatggcggcagcccattctttctgcgaaggcgcatcgccggttgggcgggcgaacgcagtcgagaaggtggtcttgccgatatccagcgtcacttccatcgcacccagctctgggtctttacgcgcttcttcaccaatcaggtctttggtgatgctaccgaacgcttcatggaagttagcgcgatactgatccatggtatccatgtccgcgatagtcaatttgtgttcacccttttcgttcggggtgactttgatagtcggtgtaccttcttcgaagccacgtaccagattggtaacggactcttcggtcaggcgacgctctaccagctcagttttagcgccagcgttcaggtctgcgatcaggtctttaacagaagtcatcttagccatctttgataatccttacgggttgttattgagtttacgttctaaatcttccaccaagtctggtgtaaagaagtcgatatcgagcatgtcgataatgtcacgacgttcagccagttctctggcgaacatatcgtggtaccagtctggaactttcgcatatgcgttgcgtccaaacttatcctgaatgtgagccaccgcgtggaacttcgcattcgaaatacttttctctaagttgttgcgagcatacaagtagctgcgactgatgtagttagtcacatcatccttagatggaatcccacggtcagctgccgccacaatctcggagacgatgctgttgtagttccctttaaaactgccacggtgttccatcaccgcatacgcgatggtgtagcactcgtcggaggtaagtttgtatttacgcatcagcagaggtttgttgtccagtacccacgtaaaacctttgatgtggtgttctgccctcagctctttggtagagaagatgtcgtgcgcgcccgctgcaataatcgccagcttgagatgctcttgccaaccgttggtgtaacagatacgaatcacgttactgataaccgaacggatatggtcgatgcgatgcgcactgtctgtataacgatagaagtcgtagaagtggcggataacttgctcagtcagtttacgtacgtcttgtggattcatttgttcacagtcccaaaaagttgtttacggatttcagcttcacgtacggtatctttatcgtttacagcgatagccagtttcctgaccagtaccgcacgcacatccatcgtggactgtgcttcgaatgctctgcaggcgtctttagaaccgtcgtgcagtttcaaaaagctgcgtaataattcactcatgatgtaccccttgatagtcgattgaaaaacttaatgttgtaagttcacctaggtaatatatatccaaaaaaatatagaatacgtggccaccttttgagggatggccaccttaacacctaaccggcttgtatctgtaggatggacccacagagcatgttaggatcttctgcaaaagcaccaatgtggcgaatgagatcccgcacattcggttcatctgtgtgaacccaataggcggttccacctttgagtgcccactcgcgacaattgcgtccgtaatcgtcaacaagcagtttccctcgtcccgcatacgccgccttcgcccctgagttttcagttacgatgattttgtctgctggaacaccaaagtgtttatcaaaccagcgctctttgcaatctaccaccaaatcgtgatcatagtggtcttctgacccggaggtaagaatggtccacggtaagcactctttttcaacgaattcaagaacttgaatcattgctttattaggtggaaggttgtagaagaggttaggctcctgttgatacatgtcgcgcatcaacccccggcgtttgagttctggtagtttgttaaactcgtgtgaagtcatcgtcggaaagtatttgggcagtgcgtacaaacgccaaccggcgaacacgccatcgctatccaaataaatcatttcgtgttatccttaaaaagtccccgcacaaaaacatgtaatgctgtatttttttattactgcttcacagtaacaatacggcggtatagctcggtgtgtaagaagaacgtccggctatagtcaatcgtcgcaccggctgtttgcaggtcgagatagaagtttgtgaggtcttgctgtggaatcgccgcgatgacattattgatcttccgcttcgtatccaaccgcacagacaacacttcggctaagacgtttttacccactcttccctgaatcgcatgaagggcaaccgccctcaactcttctggggaaaacatgttaaggctaggaggtatcacaatgtttaccgctttcatgttactgcctccagtgtagtaagtgtgatttgcagaccacgaacttacttaacgggtgacggtatacgcattcaaggcatcgtgatagacatccacaggcaccactttaggttccgtaaagcgaaactctggcgaccatgtcactttgaagtgataagccacatcaggtttcaacgttgtgccgttttcccataccgtgggttcggacaccatgaggacatagtccaattcggtgtaatccttcgccatattggccaggcgcatctcaccaatcacacgaggcttgatttcccagttagccatacggtgtggaacaatccaaacttcccctgcccgattcggttcctttgtgacctcaacggacggctgcacaacactgcgttcatcgaacgcgtagatatacaaccgagggttctcatttgcgaactgaaagttgtggcgagcacccacacagcagttcttgattgtcaacgagcagcaaacgcgtggaatggtctgatcttccccaggtgccgggttgttaggcaaccgcggcgtaaagacacgcaccttaccaccaatgtgtaacggcggtgtctctatcccttttatcgtgagtttcttcgcgacacgaggtagctggttttcaaaccacttatctaaggaagcatcatgttcagccatttaccagctccccttccctaaccccacaacacgcgtatgtgggcgggcctcggaatagttcaggtactcgcgtgcaatctgacgcgctgcgccacgacgagactctgtcgcaatcttagacgtcgcctgcgggttgaaggccatctcttccagcgtacgacgatggataggacggtcaacgaacgtacgggtactttcacgggccactttactgccgcgttcaatcgcagagtatttgttgcagatttgcagaccgtcttcgataacccagtcgaaggtgaccatacggtcaatacgtcgacacagggtaccaccgatacggccttcacgaacgatagcacgcaaggagaagcacacgttctgatgtgggttctctaatgcttcagccagatacgggccgcgatcgcggtttggtttaatccagccccagatttccaccaccggcataccgttacacacttggtcagtcggttttaattcgacctcacggatgtgcatggcaacgtttttggtttcaatccattcgttacgttcaatccattgggcttccgacattcccggctcaaacggcgggtggtcttcttccccaaacaggttaccggcttgtaccttgcgcataaacacgctagaacggtcaaagacatgctttgattcgttgaatgcgtagaagataccttccgagttgaagatgtttaacgcacccagtagaacgtagtaatacccgtccgcgtccttctggagcgtctgccctttgtttacccccgcaagcgctacacagttgtaacgcatggttaaattcgaatccattgtttaccccagttaattgtcggtgaataacggcaccggcgaagatgccgttacccattatctcatgaagagatcctcaagcggttcagcacgtatcggatcgacactgagcgcagaacgaatcccgcgtttcagctcaacgtcagcgagcttcgccagtcgagaggttttgttaagcgaaccatctcgaagcgggatgtactggacgggaccaaacatatcgctgtcttttttcagcgtataacggaagaacgtacgcgggtcacctttcttgcgttgggtgtgtgccgcgtaacagtctgcggtaatctggtcagcaaagacccgaaaaccattccacagcggtgcatcggacagcaactctgcatcatctacgatagtaaaccaaaacggacggttaccaaagtcatagacgtacgaggcgatgttatacaccgggttggaaaccacttgcaacatacggttcgggaatacaaccgtaccggggtcaaagcggaactcgtagtaaggttcgcctgcaacatccacttcttcaaacgaggacggcgtaatctcaataaacgtcgtgacgttcgagacaccgtacgtcttacggtcggtcgaaatggcgaacattcccacgatttcaatcgttgaagaaatgaacgccagttctttcgaggtgtacccaacggggatgtaaagataacacccccctttggtgattgtggctgtaccctcatcgaccaaatcagcatggacctttctcggatcgcggcgtgcggtttcaatggcactcatgccccaccctccgttattcttcgatcagcacaccctgcaacagccaatccagaacgtagttggtaatccacgttgaggccacagcatctggcttctgaccttcaatcataccttcatggatagaaagcatcagattggacagctcatactcgccaaatacttcacagcacgcagtacgaataatgaatgcggtgatgtctgaggtgctacgggtgaacaggtggtcgatagatgacgcacatgccagtttcgcttcctgcggggtcagctttttgctttcgccgatagacgacaggtaatccggatcgagggtatcgattgacagattgaatgcggtcttcatcgcctgacggttagtggtcagccagtcagtatccgctgccatacggcgaatggaactgcgacgatcccacgcggccacatacgcatcctgtttatccaacagcgactgcttgttggtggaggcagtggtatcaccgtcatccagcagatacaacgcacccagcagcgcttcaacggtaccgttgtcgttcaggtagctatccagcgcttcctgacagatgtacaccttcttgtcgttggcatcgtaagaataaacgatgttgccgagtttggtgcgcaccacgaccgcttccgcgtacaggtacacccaaccacaatagctgtagtgggctttggtgaactgggacttccagcggtcaatactgacgccagagtttgcccacgggttctccaggaagtaagcactgagcaacaggaacagaacattctgcttcatgtagtgcggagcctgtgcagagtttggcactaccgcattacccgcacacagtgtacgcattgcttcggacatggacagacccagctcagtcaggagcttgctcaccaactggtcgaaggtcttacggccagtttccggcacgtcaatcacatccggtacgcttacgtccaatgcttcatgcgagaagcccataccggtcgggttgtccagtttgttaatcaacgcctgcacaatcggctcgttgatgcatgggtcagtgtcaaccggcactaactgccaatcttccttcacttcttgcaccggctgaatttggttgttcttcaacacatcctgcacgaacggctgaatcacgttacgggagaagtccagcatacccgcacaacgctgactgatcatacgcttcagttcatacagcgtcggttcgtggtcttccacacggatagactcagcgcctgcggcggtgtccaccacaacgttgtcttcgcctgtaccgtgtgcgggctgacgcagcgcagtaatctgcggcagggtttggaagaactgctcatcggtaatggcagagtcaaacaccgagccttggttcgtggctttgttcagcagcgcaatcggtgaaccttcgtccgcacttaaacgcaggtttgcttgtttgagcaaacgcatggcgttggtagtagcgttaacagagtacagattaatcattggttgttccccttcacggtgctgataacatcctgcacacgacctgccagacgaccgccgaccatgtcggcaatatcacgcttgagcagacgttgctcaccgacatggctgtcaaggccgttgttcccacgcatcaacccgtggataacttccgtggtcagttccacggcatttgccagtgtaatcgcattcatgcgttgcaccggggagaagctgtccgtctcttgcgactgcacattgcctgaaaccggcaaattgtggcgcatacggatttgttctaaaattgacataccttactccggagtttgactgggcggtagcgacccgcccagagtgttatttgattttagcagggagttcaggaacggcctcaccgtctaaaatcttcccgacacaaagaccaccgtggaaaccggcggcgttacatgttccgatgcgcatcagtgaacctacgatacgggcatctaccgagttacggccaaagatgatgtccagctcctctccacgttcagtgtagttctcgccacgcatcaactcttgtaccgttgttttcaactggttagcgataaccattttgtcggcggctgccatgtcaacccggtgcgtgatatagaacttcacacacatcgtgttatacgccagcggcacaccgtctacacggtaatccccatttacgcttcccgacgtaggaatatccttgccgagtgcgttagccagtttacgacgttgacggtctttcccattcaccaacgttttcagcgatggagtcaggtcttctggatcaccatggtaaaccacttcgattttgtcgacgtgtccccgcacaccggcttgcggtgagaacgaactgagttcgtacagggtctgggctgcctctttactgaagccgctcatatcgtcgttcaggttgtcgctgaaggtgcatagaattgactccacgtcaacgtggtcgccttctttcaccatttccaacatgttctggttaaagccaatcgtgacttctttgattttggtaacatcagactgtgctttcgcagcgaaccgctcactaattgcattcgagtcttcaattacctcttccgcttcaatcaacgcgacgttagccagaatggattctttcaaacaaacctgagtgggatcgtagagatccggttcaaagtgatcaccgttaaaggtgatgatagagcccgcagggagtttgtcaccctgcttccatttactgataaccgtgtgcgggtaatacgtaccctcatgtgccccataccagcgacctagtgggaacgtttcttcttccccgtcttcgtacttgatacggataaactcatccgtcttcatcacaattttacccggcttatcgataccacgggcgtgcttcacagacgtacgatgtgcagccgctttctcctgttcagtacgataaggtggtaccattgcccccacgaccgttgtggtcgaaccgtattggatacctacgaagttttgacgcttcgcatcatccatcaacgtatccggtacgagaccatcgataaacgacagcacttcacccggcttgtgatcctcaccctctttactgcgaatgaaggtggtgccgtcaaccgtatcaaagcgtgggttattggtcaggaaggcggtaataccgacgtccccgttatcaaccgtgttacccgacacgatacccaagtcagattcttggaactcacgcgtatggtacaccatcgtcttacggttacgaccacctgtcccgcccatggtaacaacgtctttttctttggtgcactgtatcgggtttgcacccggtgccagcaacacacttgggtcagagttaatagcgccccacaccatatcctgactcaattcaaagcgacggttactacccggtgcgttttgatagttacgcattgctctcaccatcgccgtgtagacgtgatatgcaatacgttggttgccgacgaacatcatttcatcgccgttgatttccggtttcgtgtagtcattcagcagcatttcgttcgcgcgttctaacaacccgataaaggtttccggttcccccatcttcctgaggatacgagcgtgcatgtcatcgacgaacgcggtccgcattaatcgaagctcattgatgtaccgtggtgtcaggccatctgcatcccgaatcaagttcaggtaaatgtcttcacgatcgacttccgattccgtgtaggtggtcaggagtttcaaatacttatccagaccattgacaatcatccgctgcttgtcattgtcacaaatcacaacaatcttcgagtctgctaagcgaataacagaatcgtacaacgttttatcgatgcggttacccggtggcagcacttcgtaacgaatcccgaagtgtttcagcatcccggtcaacccgaggtagtaggagaaaatgaagcccagtgtcagcgatgtccccatcagtgacaactcggtcatctcgcgtggggatttagctgcatccacccctaagaagtcggctaggtcgccctgcggttccatcttgtcaccgtcgactttatagagttgcgagttttcatccatcccgatgaacttaccgccacgcattttcgcaaccggtaatagctctttcgcttcaaggttcttcacgccctcttccccgaagaactcgttgagtttcttcgaatcaaagttccactgataacccatggcgttaaagccggatacccgacgcgctaccatggtgtattgccgtggtagtgtattgagtgggtcgaacacgtttgccaacttggcatcggtgacgttggtgttcttcgggtctactgcctgaatgataatggcgttcgttaaccaacgaccgtaatcgttcgctaccttatcgctacgccttacaaagtttttaccgtaggcagtggttaaagcgaccgtgtcgaaatcaactttacgaatcggtaaatcaacacgctgacgacgcatggtgtactcggtaccatttgccatccacgttccatcttcggtcaatgcaggagtctggaaacggaccgttactggctccccgccgattggttgaagacgaatcgtgtggtgttcgatattcccggtaacggaaatctctttctccactttgtggtcatgaattgccatccccaaacgctgggacgacgcaacagcagataggatgtctttcggcaacacgacgctgttgtactgcttgtccatggcatcaacagttgactgcgtccagtcttcggttgtgacaaggggtttaaccagcgtcttcttcggcttgacttcaatgtctttgaccgaataggttaacgcttgctcgtacgtctcttttggattgtacgggttcggcaattggttgaagcgttggttggattcgtttaagaacttgtatgctttcgcagtgacacgtccggcttcggccaacttctcgacttcttgcttaatcactgccgcatgatcaatggttttctcaacgacgatggtggtcggtttgatgtcttctttcggggcttcaatcaccaagtcttcgttggtgtcaaagtccacaacatcatcattcacgaccggttcttcgttgacgatatcttcgtcggtgatgtcatcagacccttcaacgatgtcgtcgttttcaacatcgtgcatgacggtctgttcttccccttccggcgtaacaaactcagtttcgaacttgtcagacggttgggtggtcatcacctgaatcagggtacgatagaagtggcgtgacatgacatcgtcagtcaggcggccaccggcagatttacgcatacgctccaccacacccatgttcatcgacgtaaagccgctgttgtgggtgaagatgaagttcatgcgggacagttgggtcatgtccatacctgcgaacaaagtatctttctggtcaccacgcgcccaaccgaacaggtcgagtagccacagcagctcgatagactggaagtgctccagtttgttcttgatacggttgttgtaggtggttttgaacttatcaaacgacggcagtgtagaaccgagattaacgacgatatagttctgacgcagatactctgcggtgtcgtacttaaactggttagcgattaacacctgaatgttacgcaaacgatcgtaccatgacatcagggtgtcagggtaacggtagtgcggcaacatcggggtgtagttctcgatgagcagcacttttggatcgcggcgaactaaggtgtcatccgtcaaacgacggaaacgacggttcgcacggtgataggccagaatctgacgttcctgaccttgtaccggtaccggaataggcttaccggaaatcccatcttccggcagacgataatggtggcgaatctgagcaggcttctccagctcttggaaatacggtgtggtcaccggcggtgccagcaccacttggtcaaggtcgaccgtatggaaaacagacccgcgtgggatctggagtttctcaagcgggatgatgcgcggtttcccgaactcatccgtgcggcgcacagagaaacgctggttgaattgtttgatgagaagcattggtagtccttaaagagacgttacaacaacagcgcgttaatcgaccgttctatcacgtcatttataggctgcactttaaaactgccatccgtcgagaaccaatagttcttggagcttacccaacgacggttttcctctaatgcttcaattgagaacggcacgttgcctgaacccatatcgccatcgtagtccccgttcaaccctttcagtcgtgaagggtgcggtgccatagattcgacccacgtcgcaacgcggttgtcggggaaggagattgcccctttcttcttgggcgttaaccagtcatcttccagctcgtggatatagagggaagagatggtggtctccaatcttatggtcgaggagtacgtcgaaccgcgcccgataatcggatagcgcgtaacgaacatgaagtagtcattccagaggtcataccctgacaggtatagcagttcacctaaactgatgccccgaacgtttttacggtcgaaggcttctggcaaatcgtcgatgtcgaagaacactttgaaatgtttgttgtcctgataaatcagcgcaacatagtggtctttgtcaatcatcaacggttggtggcgagcctcagtcacttctagtcggttaatcaaccgctcaataccgtcatcggtggtaaacaggtcgtagacctttccgcgcacttcgaggagttcgcgtttgagcgttttggtgttgatgccataaaggttgccatcaccggcacggatttgggacagataacgttcgcgaatgttatactgcgccaccggcaagagtgatttcaaaccttggtataaaccgatacgggtgtctgtggctcgcacttggtcttcacgacccatgaccttcgacccggtcgagaacgaggacaacacgttacgtgtgccgttctgcaacttacgagaggttaccttgcgtcgagcaaagccacctttcccatcgaggatgttaaagaagtacatccagatgtcgttgtacgcttgctggagtttccagcgaaccgggtcagtcaattcggtacggacgttgcggtcaggaactgcacgcgccaacgaaatgagtcggcgatacatccccccaatctcttcttcttggtcgcgaccgtcttcgcgcacaatcaggtcacgcagacctgcgggcagaaccagcacataacggctgagactaacgtcgcggaatttgaagaagaagtccagtgagtcatcacggcgtaacgagtcgttacgggcgggggccagatccttgtagtgggacaagaagaaattataaccggtgtctgcgcctttatcactgggcagggccggttcgaaatctttttctttctcattccataccgcaaaacgtttgcctgcgcaaatgtcctcatagagtttctttaggccaaacagccctaagcaaaccgttggagaaatgatgtctaatttaacatcgatgtatgcccagcttgcgtcacgttgctcgctacctgtcaggccgaagatttcggttgagtaaagtccttccgggtggaagtttttcgtcatgccctggaacgtgtcggtagtagtaatttgtcttagctgagacaccagggacttgttgacgtttaacaagtaaatgtcaacccagtttagcttcttcacgttaagctcctgaattggaagtaaatacaatggcaaaaaagaaaaatggtgtcgatgattttaacttcgacaaccttgatcttgattggaatgactttgacgagccgcctcggaacaaagacaaaaaacgtaacccaatcatggagaccggtcggacgattaagcgttccgcgctgtcagcaatttggccagaaggcaaacgtgaccaggtcattttaaagggtatgcccgattctgctaccgatgcgtacaaaggctatcaggacgccaaatcggtcgcaaaagatgtttacgctcataccaaagacgagctggtcaagactgagcgtgtaattaagaaccaagcccgtcaacttggcccaacaatgaagaaatatttacccgatgcgattacgcgtcgtgtagataagtgggcacgcagtgacgagattcagggtggtagatacgaccctgagcaggcgggcttagaccgcatgatggcggaagtctttaacggtcaaggtggtggcggtgacgccccaatgaccgcacaagaacaacgcgatgcccaacagcaagccaccgaagatcgtattcgtgatggcgtgaaggacatgaagtccgacgcgatgctcaatgcggtactgagtattgcccgtgatacgaacacgactactgcattaacacgcggtgtgttgctgaacgttgaacgtaaacaactcgaactcggttaccgtactctgtttgcgttgcaagatttatccaaactcaaacaaactgagtttgaccgtaataccccagcgttagaagccatcgtcaaaaacaccgcactgcctgactacgccaaagaggacttctcagaagttcgctgggcacatgtacgccgtcaagcggctgactggatgaaccccctgcgttatgccgaagggttcatggattccattcgtcagaaagccacgaagaaaatctcaggtgccttctcagacggacgtgggattctcgaaacgataatggggatgggtgtcgaagatgactttgggatggaagacagttcctccttatcacccgacgcccgtaagaagaacggtaaagacaaggccatgggttgggcaaccaagttcctcgccaaaaagctgttgggtccactggttgaaaaaggccaagggaaatccaaagcgtggctggaagataacccacaggcaatgtccgcaattgagcgtgcaaaattcttagcacgcggggcgaccgacggttcgattgcgaactcggcgattgccggagaaagcgaaggattcttggctaacctgttccgcatgggtaatgctgtgggggtagttgacccactgaagcgtgagagtgtgttccttgacgagcgtaacgttgagaacttgaaccgttcggcgaagtttgaccgtaagttctatctcaccgtggtggaatcactccccgcgttactgtctgaaatcaacaaatcgattcgtcgtggttatggcgaacatgcagatgttgaatacgacatgaccacgcgtggtatcaccagtcgtcgggatttggctgaccgtgtccgtaaaggattggcggatgacaaaggtcgtcaaaagacacaagagtccatcaacagtgttgtggattacatcgaccagaagaagacgcttgaacctaaggagcgtcagcagctggcggactacatcgagtcgcgtgcggcgaccggtaagtccatggacgtcgatgcaattatcaaagaccaatcccaacttttccgctacatgggcggtaacacggcgcgtaaggtggtcgatgccctgaaacatgtggcggctggcaccgcaggggaaaactggggactgtcgaacgaactgcatgaccgcatctcgtcggtgcaggtgcattacaaacgtcgtcaggaagcagttgaccaagcggcgaccatttacggggaacgtatcctccgtgatgcaggtatctttaactacgacaagaagaacaatgtttttggcgtggataaagactttgttgacccgtacacgatgttcaacgacacccgcatgggcaagacccgttctggtcgtgctttgacccgtgagcaggagctgcaacgtaaactgcaaaatggttccgcaaccgccgattacattcgtcggaagttcggtgaagaaggcggggtggaagacaccttatcagccggttctgcattaaacgacgtggcgggcggaaaagggcgttacggtggtgggattacagcacgtcaaatggcgcgtgtgctctacggagagaccgagacgaacttagtcgacctgttaggtggtcaagaccgtaaaaacgcgtcaggagagactgacaggcttatagaggctattcgtgcaacgaacgtaaccacctacgtccaagagattctcaaacatgtcaagaacatggatgaggaaggggtattactggcctccttggaaggtggtagcggccctgacggtgccggtgcaggcggtggggatggtgatggtccgtctccacgcggaggtggtccacgccgccgtcgtatcgtgctcggtgaatcgggactgttgcgtcgctggggtgggattctgtttgatacggccagcggtggcttcaatatggccaaacgcggcgtcatgggtgccaaagaccgcttagggaagttcggcagttgggcaaagggcaagttctccacgggcgacggtccgggaatcttctccaaactcaaaggtctggcgactggcggtatttcgggtgcctttggttctgcggtggaattcgggaaaggtctgcttggtgtacgcgatgtgtacgatgagcgaggcaaggtagtgttgcaaggtaagcgtttagaagccggggaatactggcaactgagcgaagacggcaaccacttacacaatccgaagacgctggatgagattcagttggggatggatatcctcgataacgccggtaacgtgattctctctgcggctgatttagcagcagcgggtaaactcagttactacaaaggcgggaaactccaatcgctgttcaaagccatgtcccacaaatcaggtaaccttctgcgtaagatcatcggcgcaccgaagaaagtgcttgaccggttagccccaaaagccaagagtatcaaggagtggttcaccaccgcaccagacatctatgtgaaaggggaaaccttcccacgtatgacgtccatgctgatgcgtcaaggcaagtacctgttgaaagccacgaagaccccggtcttctccgtgaaagatatcactgggccaatcgtggatgatgcaggtaatgacattattaccgcacaagagatgcagaacccagacttcaaactggtggacaagtggggtcgtgatatcaagtcaccgcttcaacgtatcatcggtcgtgtgggtagcctgctatctcgtggtaaagatttggtcatgggtatcccggacatgctccgcaagggcgcggggaaactcaagcatctggcaaccaacaacccaattgccaactggtttaaagggaagggtggtggagacttcttcagcaacaactccctgttcggtggcttgaacaccaccggcaagaaaaccaaccatatcctcatccgtatctacaaactcttgaaccgacgtatgccgggggaacccgaggatgaaggttggactgaggagatggagaaaggtactgggggtggtaagggtgtgaaggacgcactcaaatctgcacaacgtttcgggcgtggggtgaaagcccgtctgaatcgccgttggggtcgtcgtttccgtaacggccgtgccagtgtgtctgattggttccgtggtaagcgcgatggcctcgcgggttgggcaggtggtgtccgtgaccgcttcaacaacttttccgattccatgcgtgagtctgaacatgacatcggtacccgttatgaagtggaacgtcgcttagcgggccgtgacgatgagaccgctgatttctaccgcagtcgtctgcaccgtaaaggcaagttcagccggaacaagtttaaagatgcaatccacgacgatatctccgcagccggtgaagccggttcagaggcgctcaatgcggccaaaggcaaagcccagtctatcgggtcgaagctcttagaccgtatgaaccggatggtgaacctgcaagaagtgagctggttcaacaccatgcgttcgtcgctggaagagaacggggcacaggaaggcttcattcgtggcatgtacgccaagttctcgcgtcgtatgaagttcaaagaggggggtgagaagcgtgactacctccaatggttccgccgtaaacgtaccgaccacgagggagcgactgcttcgggtggacggtcaggtggaaaagccaaagggattatggacctgttcaagtctatcccggtcattgggccattggtaagtattctgggcacggttgcgtcagtcatgggtaccattgcgaaatggggcattatgaaaccggcgaaactgttaggtcagggtgcgtggtggttagcgaagggtggtgctcgtatgctcgggggtgctgcgatgcgtgggcttatcatgccggttgcaacagcagcaggtgcggtggtcaccgcagtgggctggccagtgattctggcggtgggcgcagtagtcggtctaacttgggctgcctttaagattgctaccacaacctacacggaatacctcgatacgttacgtctggcacagtacggtttccaagactacgataagtggtcatcggacgacggtgccaaagctcgctaccttgagaaacagttgaagcaatacgtgagcttcaatgaaacgggacaggccacttgtcgtggtttaggcgcgaaagaggtgcaggagttagccgttgggttcggtgtggccgaggatgacaagtccggtatgctcgccttccaagcgatgatgctccagcgtttcatcccgatttatctgcgttggttgtctgcactctacgcacaagagcgcgatatccagttagcggatgttgggaacgcaaacaaagtcagcaagtccgagatgaagtctatcttcaataaagtccaactcaccaaagatgccccacatctgcgtgcgttgactgaccctcgtaatgttgaccggagtttgtggcagaagtttaaggatgcggtgacattcacctcacctgacttactcgacgccgatgatgtcatggacattcaggaagatgtgctccgtggtattaaccgccgtatggaagacaagaagaaccggaagttcaacaagggcgcaatggaagcccgtgggattgaagagtcgggtgtgaaagaagccttcggtgctctggcagccaacgacaaagaaacccgtgagaacgccccacgtccaaacgggtgggaggatggtacggagcagattcagattcaggtcgataattttgcggtcttgaatcagaaagatgtggatgcccttgaatccctgcgtttcaaaacgtatggtttgaaggaactcgaccccgcgattgtgggccagctgaaaatgctggaacgtttcgtgttgccgaacatcgacattaagaatgcgtcgtacaaagggaaatggactgaggcgatggacgtcatcgaacctcagggatggaaagacccgcaccgcagcgagaaactgcgtctgtggttcaccagtcgtttcctgccgacctttatgttctacgtctgtggcttccatcggttcgtaccaacgggcgacccgttaaacctgaagctgaccggtgggtatctgtttgagctgggcttactgaccagccgtgcttacaacatgaaagccgatattcgtcagtctgtctgggaagtggcgattaacccgttcggtcaagaccccaacatggaccctggttctgtctctaaagaactggaaaccttgaaggtgctctcgaaagaggctgaccttgcggtgcgtaacttactcaacgacaaaaagccgatgggtaaacgtgcgaagtgggcagagaaaaacaccaacacgagcttctaccaaaccaaggatgatggtgagtcaacgtcgtttacggcggaagaccagaaggctgcaaaagcggcaggtggtttcggtggtggtacctttacgggcacgcctaccgacatcaatcaagctgtggatgcaatgggtggtgcgaagaactacgcagctatctctacgggcagtgtcggtattaagctcggggatgtgcaagcgggtgactacaaacagttggcagagaagtacccgattggctcactgaacagtgaggagcgcgtcaagcagatgattgcggacgtggcgaaatccatgggggtaccaccgagtgtggcgttggggatggcgtatgccgagtcgaagttcaactacaaggcgaaaaacccttacgcgtctgctgctggcctcttccagttcattaactccacttgggattcccagttggggcagtatggacgacagttcggtattcctggacaattgatggcaagttcaggggggcaattcgatcctcatgctaacaccattctgggcgtgcagttcattcgtgataatatcatgaaagcccagaaggatttgggtggtaaagcaccaccgcctgcggtggcgtatctctaccacttcttaggtcccggtggtggacgtcagttcatgcaagcatgggcgaagaacccgaacgcacctgcgaccgctgcacctccggttacacggaaagtgctggcaggtaataagagtgtgttcttcaccaaacaagggagacttcgtacgctggatgaggtcattcgtgaattgaatggccgtatgggtgcggtaaccgcgaatgagatgacggctgacccgtccaagacaaaacaagcagtcagtggtttgtcgccggatgcaccatcctcatcaagtcctgcggtttcctcgggtgctgctgcaaacgacccgtccatggaaggtactgcggccggtgcaggccaaaacctgccagccgataacgaaaaccgccgagacggggcactggagacaaaaggggcaatggccgcagacaatgcagtcgccaccatgtcatctggccctgcactgccgggcggtacggcgtcgggcagttccgatatgtcaaatgttgccgacgatgttgcgaagcaagctgctgcggatgggctctctccgaaggatgtggagaaagtgaaagccggggcggcgcagcgtgctgcacaaacaggcggtggtggtcaagtgccattatcgtctgatatgtcgccagccgctggcggattctctaacgccacggttgcggatcagcaactgcaagtcacgaaggacatcaaagcgattctggaagacatgcggaaactgatgcagacgggtacaccgatggggccatccagcccgccgagtggcccggcaccgaaagcaacgcagacatacccacaaccagccccaagtctgaacgtctcacgtaagacgggctaacaacgggggagggaaacctcccccatttccataagtgaggttaacgtggatacacgatcgctcaacgacacaacgtgggtgaacggattgtttggcagtatgaagttgccacgggatacccgtttctacaacacacgcacgtactccgatgccttgctgtcattcagtgacaccacggtgggcggtaacgccgcgttaaatgcaccaccccaatttacgttctttgctgacccacccattaccggtgcgttagcggtacccaaagacgcccccggcccgcagagtaaccgtcggtggtttgagtcgttctccgcacaagggtcgtatcgcctaggcgcgtattattacgaatccattgagcagaacgccttctatctgcactgtcgtttcggtaaaccacgctatctgggtgtggccgccttctttgccaacatgtacgattcgaaactcgcttatctcgcccgcacgggtgactatccgggtgtcattcgttcactggcctcgtataccgctgctgccgccatttgggcaacggtcggtacagttgcgttcgcgcttatcttgattaccccacgaatcatgaaagccgttctcgacaaacagtcttcgaagtattactacgtgaagccgaccatgcacctgtacttacgtgctgtgcagaacatcgtcaacacgcagctgctttatcgtcgtctggtaccaaccaacatattggcatcgttcggcttggctaagaatgacgaagacaaaaataaagaattcaacgcaaacaaggaagacatctacgcgggtctgccggatatctggaagtctaacggcgagttcgatatctatcgaatgatcaaccgttaccagacactcgcaaacttccaagcgaagacgattgcagaaatcaaagccacctcgaacaccgaagctgagatggccacgaagattcagtcgttctacaagaccatgacgtacagccgccagtatctggataaagctgcctcgtttgaagtctcgctgtcaacacttgaacaactcgcacgtaccagtgccggttataaaggtgttgaaaacccggacatgaatgaagaccaagtgttggataacatgaccgcgaagtttgctgatgcagataatgccggtggtggtgaacaacagttcttgaaatcggcagacgttgcccaacagcaactccaagcccaaaccatggcggaaagcaatggcgcggacgataacggggaagcgttggcgaaggataccggtaagattgagaactggatgcgtgagggtgagaagagtacctttggtacaatgttcggggagttctcgaagattaccgatggtattgttcagcaggctggtgatgaactcagtaacggttcccagtgggtgacatggaagattaatggccgtgatactaccacccgcacattcagtaactccaccaaagaaccggagatttcgggtactgtgaactccgcgacccagaaagcccgttcgcttgaagtgagtctggctggcgggaaaaccggtattgatggcgtcgacggtttaatcaccggtctgaagtctgcgttcgcaggcgcattggacttccttcatctgtcagggattatgtcgctgtacaactcgtcagtgattgatttcccggaggtgtgggattcatccgatacgtcaggtgatgatatctcgttcactatcccgtgtcgttgttggtcaggtggggacttagacgtcttccaagacctgattttgcctgtggccttctggttagccgcagtctgcccattagccactggtaagcagtcgttcacacacccgttctatctggaagcctactctcgaggtcgctactcgatgcgtaatgccatggtgacgaacgtgagtctgaacttcggtgtcggtggtttgggttggcgtaccgacggtgtcccactgtcttgcgacatcaacgttaccattcgtgacatgtctcgcactatgtacatgccgattgttaccgataccggcgtgtgggatgacgataacaagttctctgacttcatggcggtgttaggttctgcaaccttacaccaacgtaccagtggttgggcgaaagccacgcagaatgcgaacgtgcagttccagtcatggaagtctgccttctcgcagggtgcgattatgaacaagttcttcgacctccctccggctcgtatggtggcgaacgtctttaccgcattcaccggtaccgcgcgtggtgacctgtaagcaaaaaaaaataaagctacctactccttcgggagtaggtagtctttttttatttagcgcatctgatggagcatcgtccactggaattcgctgtttggctccgcatggtcatacgagaagaagaagaccagtgcatcttcctcgatatcagcgggtaccttgttcagcaacggcacggccgtgccatacttctggctggacgtcagggcaaaatgctggttcgtaaatccaccgcggtagttttcctcacccaacacttttgccacgatcatattcggaatggcgctatacatttcgatagcgtggaagtcctgccatgcgccgtacgtaatgggggtatcaatgacaacgaaatccaacccatcaaaacgtgcagaacgattagccagtcgctccaatacccaagcggccaaaccaaggttcccccagttctttccgtttacgctgatagtctgactatccgcattaaaggtcagacggttctttttcttcgacatcgtcattctccggcatttcgataaacatcagttcgatgaaggcttcacctgtgcgggtattgcggtcgggatggataaggataaacggcacacctttcgggtacacgtcatcttcgtcaagccacatgctttgtgattcaacaatctcctcagcaccctgccgtaacgtacgcatgatggtcgggtcaatctctacccagcccacatggttatcatgatcgagatggtcgtacgtgtaaatcacctcgttgaggaacgtacgcatctcagcttccgtgatgcggaacttgcacagacgcaatggttcttcaccaaaggagacgccaacatcgcaactaacgaaaaccttatccggttgtgtgcaacaccgccagaagttagcgcgcgtttcatcgcaaaccgcaatcgttttaccgtttaactggactgcaaacaaaccgtcgccagaatcgacgatgttgatatcaaacatgctactctcccgcgttcagggtgtggcagttggtacctgcaatcggctttagactctcttccgcaatagtgcggtcgagtgtgatgacctgcggaagcgacattacccacaacaccagtttactggaatcggtaactgttagcttctgacccggatagtagcagatgcccgtattcacgctattacggtcaccaccttccgtgaagaaagattgcagttcatgcaacagttcttccgtgcgcttgttctggtacgccaattccgtattacggataatcaacgagcggaacagcagcacatcttcacaaccaaacaggttaatgtattcggtggtaaagacctcaccttttggaacttcggtgtatgccgacggagagtgaaccgtgtagatctgaatcgatgtggcttcattcgtcacacccacttcttcaatgaccgttggtaccttggtcttgagtgtgctacgaatcagcacaatacgtggatgttctttgctggcgaagcatttgacgatcgcacccggcaccggcggatggatattctgcgtcggctgaataccaccgtgtaattcaacctcaataaactcgtcacggagtttatattcatcgaggctgagtaccgggaagcggttacgtcgtccgtactcgaacgaaattattccctcggcaggggcttcaatcttacccactgcaaaagctaccgcagcctgcacctcgctcatggcgaggtttgtgcattgctgagcaacaatccagcgtgctgccgcctctgtcggggcaactaccgtggcatgaaacgattcatccacattagatttggtgaagtcgttcgtgatgagaaataattggtattccattgtcctactcctgcattgttagtggacgtgaattaagcgtcggcttctttgatgaacacgccgtcagcgttcaggaaacctttacggtctttgatttcatcccacgccagagagaaacactcatccagcgagtagtcgtaatgacgcgccagttggttggcgtggtgaatcgcttgctgtgcgtggcccagcatctgttgacgttcgtcatgcgttaagcggccgagttccactttcttcggcgagtcgatagcttcacattcgtaaaccacatcaaccacttcggtcaggttcttacgcattttgtggaaatggtagtgtgggttatccactacggttttggtgtcgcgtaccaattgataaatgtgtgcgatttccgcagagtcgatactggtcagttccagtacattgaccagcacaaccagcgcatcgccgatgccgtcgataatcagacgctttttgtttttacctacaccggtagccgcttcaccatcttcttcatagagcttagtgccctgtgaatcccaacgcccgttttccagaataccacgatcggttgaccagccgataactttggccacacactgcgatactcggaacagtggaacgatacggttgtgaaatactgggtctttgtggaaatccagactggtgtggtaacgcaatggtgcatggaactccgcaggttcaccttcaaaggtatagccgttaaccagcgtcatcggggattcggtgctgagcgccaggcgggtaatgcgagacatccgtttacctaccgccgccaactgaggcataacgaaatccaaaatagcagcattcaggataatagatttgtgctcaattggcagttcgaaagtctgttgcatttctgatagtccttaaaaaatgaaataggggtgtccataaggacacccgctcatgttaaattttgcaggcaccgcctgcacagttgtcgtcttcagcgccagcatcgacaccgccttcaactactgcgttctcatctacgcccggaatatcaccaccgaacagatcgtccagagacccggtgtcttccttggtgataacttgcttctctttttctacttgtgacattacagacctcagttaattaggtgaatcaccacatcgtcagataccaccggtacgagcgaccggtagattttgtcgaagctgaacttattgaagaagaagccggtttcgtcgatgataaccgtgtcgtacgtttcgccttgccagttttcaggtaaatacccgaccactactgtgacaccttcacggataccggctgcctctagacgttgaatcagctcatcacgcaacggagcgctatgcacgaaataaagagtcttccctttgttcgttgccgcagtcttaacagcatgtgctgtcacaccacgttgacgcccagagccataacggatagtacggaactccgctaaggcaaggtggggaagcaaattcatacagagcgcaatatcgtcttctttcccaaccagccctttggaaagttcttgcactactaaatcgtaattgattagagtcttagacactttattcacctttcagttaagttattctgcggcttcgtccgcagattcagatcccgccagttcttcagcgaggttttctggcagtggttctttcggcatggattcaaccagcttcgcaaccgctgccacaatcaggttctgccaatctggattcaaccagaagcgaatgacgtgcgcactttcgttctgaccgtagacttcgttcacttcttcccagccatcaaccggagtggcgctatacgctgctgcacgcgctgtaccagcgataacgtaccagtcttctggggtcaggccatgttgttccaacaagtccagtaacagccactcaggcgtcagaacacggtctacgttttcgtggtaggtgtattcttcactctcaccgagtttggtgaagttaacatcgtcgttgccggtgatggaaccgtcgccctgtgcagacaacatgatcggtacggtgttcgggaagtctgggtgtttcaccatgatacgccacaggtcgctcccggtgctggtacagccacccggaatacgcagacagcgagtgaagtccacttccagattgctgcaatcaataccctgcattttcgaaatggtttcacgcaggtacttcacacgctcagaaacatccacaccgtcgttcagcttccacagctcggcagtaacggttttagcgacgctatcggtgcgcgggtcgatgtggcgaatttcttcagcgcacagaacctgaccactcacgtcggttttacccaacggcaaaccatcgaccagctcggtgcccaacatcagcttagcttcggcggtgtccttagcagccacgataccaaagctgtagctgtcacccggcatggtgtagaaacgatcagagaagaaaaacagggtattttgtttgtcagtcattatggcattccacgaaattaatgatgaaccggtcagggttcgttgttggggacatgaaaatccccatcgtataatcgatttccaaatcgtcagctaacaccattaaagcgttgtcatggactaattcgtaatcgtcatcattcaggtgaccgtcaagagacaggacgtgggtgtaagacgccactttaagaatctctatcagggtccggcggtcaatcgtcaactcacacgaggtcttacgtttcgtgtaggattgattctgccagccgtaaggttcggagtaaaagtaaaagacgttttcgaaatacggattggtggccgccacctgctcgtatatcgctgcccaccagtacatatcacacaccggtactgtaaatgcacccaccttcccgtcgcgggtatgaataggaaagtgggcacggtgttcgcggggtgcgacaacgaccggatgtgcgttaggcttaccgggaaacttcagtacgttgtcagacatacgcgttccttagatggcaacaggtgccttaatcaccgggtggctttcgtaacccacgatttcgaaatcttcgaacttgtagtcaaagatagaatcaggtttacgtttgatgacaagtttcggcagatcgtgcggcacacgagaaagttgcaacgtagcctgttccagatgattcgaatatagatgggtatcaccacctgtccagacgaaatcacccgccaccataccgacttgctgcgccaccatgtgaaccaataacgcgtaagaagcaatgttgaacggtacgccgaggaagacatccgcactacgttgataaagctggcaggatagaacacgttctggtacaccacttgctgtcagtacattatgctcatctttatcgtcttcgtattcttcgcacttagagaactggtaagcttctgggtcgttatcagctaaccacgtcttacgctctttcagcgtcatctcacgcgtgtagaattggaagaaggaatggcacggcgctaatgccatatcatccaactcaccgacgttccaagcggagacaatgatgcggcgattatcgggatcgttacgcaactggtcaataatcgtctgaatttggtcaaagcgcttggtaaacaccgccagcgttttagctgggtcgccacggttaatagacccgctgaactgataaccacgttcgtacaacactttcttggacgcatcgtcccagtgattgacgagtttagtgtctgcccattcacgccactgtttaccatagacaggaccaaggtcaccgttttcgtcactccactcgtcccagatactgacgttgttgtctttcagatactggatgttcgtgtcaccgttcaggaaccacagcagctcgtgaatgatagaacggaggtggagttttttggtggtgaccagcgggaaccctttacgcaggtcaaaacgcatctggtgaccaaagatagagatggtacccgtaccggtacggtcagccttttcgtggccttcgtttaacaccgtatggattagctctaaatactgtttcatttaccgcaccttctctaattcaagaaataaccattgtaagtcattgttcggattgatgttcagcgcttcgccattacctacaaccacgacccccggcttacggtcatggaggagatgtttccatttcgggctggaagtaatgtgcttttccagaagcgcctgtaacgctcggttcatctcatcccgcacaaccggagtcgggtcaaccagactggcctcgtgttggaaacgctgaaccaatactgcgaactgttctttcagaccgttgacgatgaaatgcttttgaagaacgccacgttcatccagcgcaccgataagcgggtcgtcggtgtagtccggttggaagataccgaactcatccaacttacctttcttcttgtacagcgtggtagccgcattaatcacactgcgatcgaagactaacccgccgcggtgtgccaaacctttcagtctggcgaagagttcggtaatctggtattcagtaataccggcatcaacatcattttcagggtcggtctccagacgcatcagggcgcgagtcaaatcaaccagcgtctttgcaacgtcgttaacgtggtatgctggattgacacgggcaacacgcacgccggacgcatcgcacagttcagccagacgctttggggtgatgcccccaaacgagacagcaccaacgagcgatacgactaacttaccgatgccagaagagacttcgagattgtgcatcttctgcacaccttctgagatttcacccagatggcggaacaacttcaacgtttgttgcaagagcgtaccgtgcttataaatgtccgactgaatgttccatgcgtgaacactttcgaaacttggcagtaccggatattgtacatcagacatctgcactctccacttcggaatagctaatcatgaaatccaaacccgacgcgtgttcgtgattggaatgaacaaggaggataatctcaccgctttgtaaaacagacggcgtcatgccttgaccaacgtgtttatcagatacgcgacggagagaaccgagtaaacggaacgcgtacacaccgctgctaaattcaccatgtcgcaacagagcagccgcagcatcttggcttgggcggaagccatacatcggacctaaagccgccacgttgccattcagggcaatctcgttggtgactttcaggttgaccttacgccccaccccgatacgacgatagagcttctcaaaatggtggttattggtatccggtaccagatggccgttaacgcttaaccctttacccgcttcgaaagacagtgtattcattttagttattccttaggatttctacatagttagccatcatggcgtaaaaagaaaaaagaaaaccactcccgaaggagtggtcatctattacagacgtgtatcaacgtcccagtacgccctcaggaattcaacatcttcgggattggttgggcgagacgggatgacttcttcaaccgcaaacgggatatgttcacgaattgattccagcgcaaaccgttccacttccaactccaccttcacccactcgccgtacgaactaccctgcttcatggtattgagcagcgtatcgtagtcgtctgcattcagcagttgtggatgaccaccggcacggtagaacacatcaatgtcccagtgcttgccacctttggtttctaactcacccgcgggtaaatggatgcgtttaaccaaatgcgacacgaagtcgtcctgatagaaggtcagcgccgtatcaaacccaatatcagagttctcttcgacacaaccctcgtcagcaaaacgcttcacggtcagcacggctttatggtcttcggttaaccgcacacgacgcttgccccggttaatgggcatcagggtatcaatgtacatcgatccctcttgctcacgtaaccagttccaaccttcttcggtcggcttcacccaaagacaatactctttctcactttcgaccgagatagattcccgtgccactttcatgacaccttcttcttcaccccgttccagttcatcaatggtgtcaagaaatgacatatcgatttaccccagttgtttgatgacgtcctctgggtcgaagtccacggcatacgggtcgatgttttccacaatccgcgtatacagaccgggtaaccagtccgcatgatttggaatgtgaatcttcccgttcatcacgtagtagtgctcaaacggaataccttgctgatgaatctccgccatgatattcccgagacacacgccatccagtttaagtttatgcaacttgtgcacgaccgccttcataaaacagcgctcgacgtgctcagagaatgcacccggacggtaacgtgacccaccgtaaacagctttcttcaacaaccgccctgcccgaatcccttctgccccatcaacctcacgcattctgtcaatctcagggaatttcatgctgaaacattccaagataaacaggtcacgttgaaccgggtcgttgtcaaactgatgaaggggataatcggaaatctcctcctcagtatcaaggtgcagaaagtaatccagtacacgcagaacgtggtaataaccttccagtgtacggtacgggccatgtggcgtgtcgaagtacgacccatcaggactggaggcaaagttacttgccaattgacccaccgggttgcgagactgcgaataaatgttgtaatggttaagtccgtctgtagacggaatggtgtctgtggccaagctccgataaccgactgagcgtaaacgacgcacaatcttctcacggaattgtggattagcagacaggtaggaaagttccccatcaaaccagattggatcgaaccggccgattttctcgaccaacgataatcccagcgacgtcgccagtctactcgctaacgttctatccattacgattgagtcaaatcctgccacccgttcttcgagtggtagggacttgttgaacgcatgtacccagtttggcccttggagctgagccagtattaaccgagccacaatgcgatcacgtacagcgggttcccagtccgaactgcgcaccagagcaatcaagtcacgcagttctctcatttcaacgtttgtcataatcttttaccttcaggctgccgggaagaactgattgaccaacacatccgcgcgttgcagacgacggctacccgccgcacagacatacttgcgcttgtcagtcgttaacagtgcctgcaatgcgttgatattgcagtacgtgtaattcagcagctcggtacgcaccggggcgactttcgtcttgtcccaattcggatcgagggaattacagatgctcaacaagcgtgtgccgtaggtttttaaccctacgcctgtatcgacttgcaagctcccgaacaatttctggataacatcattcgccagttctaacccttgaccgggttcgagtttggtcagatagaactccacggtatcgatgttcccaacactggctgcttgtaccagtaactcgccatacatggcgcgtttggcaaccgggtcagtaattgcatcgaccatggacacggttttctccggcagaccgtactcagacagtttgctggataagccgtagatgaggccagaagttgtaccaatgtcaaaattggccagactgttactgcccttgaaactttcgatgaaactgtcaatcgccagataatcatcaaagtctttgaaggacttaaaggtttgggttgccccgtcaatcaccgcggtgatttcattgcgtgcttggttcaccgtagagacgtaggaattaatctcttgctgcacctcacccggtaaacgggctatttgacctgcgacttgcatggtcgattcgatacgcttcttaatcgaagcatagtcggtgcccaccgcattcagtgcactgtcacgcaacgcggtaagtttactgaacccttgtgacagcagactgcctgccttgccgggtttcagataatctaacaccccattagcggcttcgttcttgggtttgaacggttccgccacttcacggttaagtgggttgatactcggcagggtttctttcggatcggttgagaagcctgcgatacgactccccggcgaagtacccgactcagctgaccccggtgccttgaccgcgttagaagtggctaagtcgctacccccaaacagattgccgagcttatccttaacggtactgaccccgttagtcagactgtcgtaggctttcccagctttgtccacgctgtcgttgtagaggttctgggccgtttgaataccacgctccgcaccgtctaccgtatcctgtacgcggttggccgcgctcacgaccccgctttggacgcgatcagcagcattgcttacgttactgatctggttagaaaacccgtctaatttattcagactcattgcggttactccagaaaacgagttgggttaggtcaacgacgatttctgtctcgaaggactggttcttgtcgttggtacacaagaacgcacaacggaactcacgaacatcaatcgctttcagcgcctcaaggaacttcttccacgaaatcttcttcgtgtaacgaatcgcggattgcaggttgtgtcgtttgtcgttgcgtcggttagacagtgccggacagttcttcgggttattaacataagccgttgacagtttgcgccacatctcagagtcgatgttgtattcaacaaagaaactccataacactttgagtaagatgtgctccatgacctgcgtcgctgtgcgctgccggtctttgaagaacgcgtttaacgtttgactcgccgaccctttcaggtcttcgtccgcctctccgttaacaatccgtagcaattcttgtttgggactgcatgagccgtgtacgactttctctgccccaaacttaccacgggttgccttcgcagttaacgttaacgtttcgatgcgcaacatcaccaaactttcaatgaaccgcacccaagtgaagtcaacactgacaccccttaccgaaccaccggttaaggcgttaatcagtcgactctcacgctcctttggctctgctgttgaacgacccacgaagcgctcatccgccacgtacgctttcaacaacaccatccagtccaccggagctaaacgcatttcgtctttcacgatattccagtacgctgttcgaaggtatatcccaatcggggtatcgtccgggacgccttctgccagcaactttttcaacttgctattcttcttactcatagttcgcccttgttccaaggagatgaacggattagaggtagtgttccactatggtctctaactcacgaacgagatggcgtgtcaagttaaacagcacatcctgctctgggttggttttactgctatacacgtctcgataagtctctaacaattcgtacgttcgacgtaacttctgccgtacgacatccgcgctactggtaccgaaatactcatcgaaccaacgcagcaacggtttatcctgttgtggatcaatcaccgcaggatagggactccagtctggattgcgtccagtggtgttcagcacccgatcgtattcacgcagcagaaatgcaaaccgctgatgaacaatatcgtagcttttacaccggagttccagattacccatcaggtcaatactacggtaagtattaccgttatactccagaggttctgtaagcaacgctaagcctattaggaccctctgataagtattctgggtattcttatggaactcggcctctaaatagcttctacgccgcttatgtgcgtatcgctttaaaggaaacgtgagccattcgaacaacataagttgatccttagttgagataatctcatcaagataatatctgtctgagttcttttttaaaaagaggaatacccatgagcgaagaagtgaagtaccaagccttcgacggagatgttgatgacgaagagtcgcttctccgccaaacccgtcaagcccgtattcgcgtggctaacctcattatggaagacgacaatgtccacaaggacaaagacctcgtcaattcccttgagaaaatgctgtctggtgtggacagacaaatcctcggcaaacgtcgtgcagaagccgcccagaaaaccgccggtgctgcacaagacgttgcaaatgccttgaactcggttgttcttggccgtccgggtgtacgtatccaacgccacgacgataacagcgaagaaaacaccgggtaccaacccgcacttcctaacgttcctaaacaggaacacaaagaaggcgagctggcacccgttggcgaaaagattgatgtgaatgccattatggctgtggcgtttgctcgtccggggagttcaggggacgaagaatagaatacagccgggcatctaccgggtcgatagtgaccagttcttccatgaaccgtgtcagtgcgctgaacggattaaccccatcgcgctctatcgcttcaatcgcctcagtcgtaagtccgtccgtcagcaacgctggcgggtggattttaaactggggtatttttttcgcaaaatttcccgcatggacagtgacccaattaaaccagtcgaacatgtaccagacgtcccatatgctgtcgagacgaccgggtgagagatctttgtgatcgatatagaccatgtccaccttaacctcgttgtacagctgacggaagttctgcaagaacgtatccgactgttcagccgtgaggtcggtgtaaggccacatgttaatcgtaatggtcggtcggtcaataggcgacgacattactaatgtggtcaagtcaacgagcacctgattcttcaaacccaacagaaactctgtcgggtctgacatgaacaacgcgcgcttgtcacgttgtttgagttgttcagaccatttttggataccaatcgcttctgcccagatatcggtgtggcgcttacgaaaagcatctaactcgagcttctctaacgcctcaggtgcaatgaccttcgcccaacctaagcgggtgtcgaaaagtgtatctatatctaccagatagcgacgtcctgttctcattgcggggaacctatgttgttaccgatacccatggctttgtaataggcactccacgtacgagtggctttactggaggtgcgttcggcaccgggtatcttgatacggccttggccagtttgtcggatggattggtagaacgcacgttgcagtgcttcattacctccacgcgcatgcaagaactcttccaagctgttgtccagaccatccgagaacataatgtacgactcagggaacgataccccggacgctttggatggaccgaccacttggccagagagtttgtcgcgaacacggtcgttcttcgcaacagcaatcttcttttctcgcatctgcgtctgtctgcgtaccggaaggggtacgacaatatgcggccaacgagttcggtgcactaagcccgtcttcggttccgtaaagtacagacgctggcacaactctaaccccaacgcacgacagatttcgacgttacgcatgtggtcgatttgcaccttactgcccgccgggttataaatcggaatgccgtggcgtagcttgttaaagtcttcgtcgctcaaccccggaatcgacgctttcgcggcttcggtgttaatccctgacgggtcgatgagtgttaacagctgatagataaacgcttcggccttcttacggcgtgcaggatctaatttcattgcattgcccccgcgacacgcaggacaggaagaacagcagattccagatcttcaatccagaacgggatggcgtccgtattctcaggaatactgaacgcgtgttggttagcgccgttagtaccgagcagtttggtgtagaattgattcgtacactgtgcaaaatcgctgaggttgtggtggggtttactcagctcattaaccagctgatcactcacctcacgatttactgctgcaataccttgacgcaaccgctcgacaatatcattttgataacgcatgggttgctcctcaagtggcggggtttccccgccacaacagattactttttcttggttaagaacttcggttccagaccatccaccgccattgccagcagagacatcgctgtcagtgtgcgtttaccacctttgacttcctggtctttgaacatccaatactcaacggtgttatccagaatctcgtcccagtcccacttctcgttgatcttctcatacaattcctgaggagagatatggtacttcatttccagccgatggtagttgttctgcatgtatgccaatgcggcagtaatttccagcgcacgacgcagacgaacattctcatcgcaaaggtcacgaatggtggtacggccgaatttgagacccggcagaatcgccagctctttgatagcgccaccggaaccagcactggtgtaaccgtattcggttttcagtaccttatcgaggtaatgccataaagagaggtgatacagcagacccatctcctgagagaacaccatacggaatttcacaccggtatggccacccttcgcgcgatactgcgtgaagacgatttctttcaggtcgttcaccgaggcgttcatcgccttcgaacgtttggttgggtacaactcttcgttgacaccggtcttcgcgtcgtaactaccttcgtgctttaactcacccgatttggtggctaccagcagggagttagtcaggaaggaaatctgacgacgtgggataccggcgaatttcagatcatcgcctgcatcatcgagcagcttggcatttgccggtttcgcacctttaccaccttgtgacattgctttaccggaatcgtcggcaagctgtgcaacgaaggccaggaagaaaccaccacgggccagtgctgatggccagcgagacatcatgttggatttctccaaagagtcacgcatgttcagggcgttctgttcggagtcaccgactttggtttcagagtgcttgtcttcgattttagacgagtgccactcggacagggagtcgatagaataataccacgggtcattcatggtcttattgcgtttacgtactgggtcagggaatggcgtctcacgcacgcccttgccgcccatatacgctttgaaacgaccttctacttcatcacggatgtacgaggcgtaatactcttcacccggcatgacgtcagaacccacaaggttgtaacgttcttcttcgatgagactcagaacagaagaaccgtcgtggataccgttggcattctgtgcagagagataaccctgctctaaacgatcgagtgcagcggaaacctcggtatcgaatttcgatccccatgctgcccgataacgtatcatcatctggaagatacagaaatccatcagcgtcgatttgaaggtgttaccacgacccgcaaagcccatgatgtgggcaaaaccaccgttcaggtagtacatgccgtcttcacctttcacatacgtaccgagcgcatgatccataatggtgtagacgttaaagcgtgggcgaatcacttcacccataacttgttttgctggacctgccatgtcgtaactccgttaagcgcgttttttggtaggcagcatcagacgacgcttattattcagttcgaaatactgttcaacccaggcttcttcgccgatgtctttgaaacggtttttgttacgatcatcaatttcaatcgtcagctgacgcttaccatcagtcaacgtttcagatttcaggatacgaccaaccacaacacgattgccttcattatccttacgcagcggggtgaaataaatttcaggttcgaatttcgcggacagggcacgcgtgaacattttgatttgcatcttcaattcctcaggggttagtcgtctacataacacagggcttaaccgtaaaaagacttagtatgtagcctacccttccaccgaggtgaaaatgaacctgaacccgattgccgcgctttctacttttgcctcgaaagtgtcggctgtgcttcctaaaacgtttaatggaagcgaacaagaaatcaaaccggcaaattacgatgacatgtcggcaatgtccaaatggatgcagcaagagaaattcctgcatttctctggaatgctcgtcaccgtaccaccaggtctgaacgtgtacatgattgaccacatccaacgtctggaatcggtttggtctgtactggacaatctgattgatggtgtactggaaccggtgaaccgtcaactggccgcgttcacacacgacaaaggtatgttgaccgtacctgtcggtttccgcttcaaagatttgaagtacccactcaaaaacgtggacccgaaagacctcgtcaagaaattggccgcgtcttacaccaccacgtcggtcgaccaacgtccgattgagaaggtcttccacaacgccggtgagattgatgtggcgttcaaccgcagcaaagcgttgagcaaagaagtcactgaaaaactcaagcgtaacatcgataaactgattgtaagcatcggtgccagtaccgatgaattagccgaaacgccggtacacccacagtgtgccgctgaaatcgtcaagatgctggatatggcatctgattgggttgagctgtttggtctgttcatgaaacagaacaacgagctgattcaagcattaagccagaccggggatagactgaaagccttaaaggccaattcaaaataaaaaaaataaagctacctactccttcgggagtaggtaggctttttatttctttcgacgcagctctatctgttcattgacaaagacttccatgtacccaatcaactccatgacaaactcatccagatgttcaaaaaggatagcttcaattttttggcagacggtatcccggtcgaataacactggcaacgtcctgatgttccacgcctttttcgtttccgctaccgattcttcgatggaccggttgataagttttcggtacgcttcatcatcaagctcgaaggtatactctggcgcatctaagtcctccttctcgataactgcacgaaacaccgcatcgtgttgtctgtagaacacccgataagtgggccgcaataacgtttgtgccagaacaaccgattccgtgtgcgaacactcaagcatttgatttcgcaggtactcttgcaaatcgatacggatactgtcgaacgcatcaacccacatctgtcggatatgcgaatcgtcgtaatcgaaatacacgttcatgattaagccggttcgtcagggatatcctgaatcatatctgaaatccgacctaccatctgcttaccgccgtcggttgcaaccattaccggtcgcggacgaaagcggaacgagatttcgatgatttcagccgtcagttgtgcaaacagaacatcgagcagcgaggagatatggcgatgaaccaacgcaaccaaatcgtcgcgcaacgtactgcgagtttcatccgtccacgtttgtacccacgcattaagcgtttcgttcgctgtggtcgtctctttgtggaacttcaacagctccacgttcaactcatcacgaatgtcttccagcacgctgtcgagtttagtatcgagggtgataatctcgatgttcttctcgatacgtttgtctttgacatcggtattatcaaattcaaacgtcagcatggagttggacaaccgtgacaccggatcgaacaacgttgaccagagcgtcacagtgaggagtttgttgtcctcaaccgacagctcattgtgatcatgaagaaacgcatccatcgactcacggatttgcatcatcatttccggccagtgtttttcaaagttaccgggggtcaggttaatgtggagtttcaccaagcagctccctttaagagtttttcctgaatgtagacaatctctttgatgcagatatcgctgactttaaggctcgtgtctttgagtatcttatcaattgcctgcgcattggccgtgttcagcacatcgtgcagtgacaccatctcaaagttgttcccgccctctttcatggggacagtcacgtacacttcggtagcatcacccagcgccatactttccatgttcgctgcgcccttttcaaaggcatcgcgtatcaggtcaagcacatcggccccatcgtcccagtgcgccaccataacaggtatcggggtactgagcacattacggactttgtcgatcatcgcggccaccgtggcattaacaatcccctcggcatcgaccagacaataagtatcgcccgtttccacttttagcgaccgctcgtattccgcgagcgcattgtggacttcaaactccaacgacttcttcatcgctaacagaaccgcatcgagttttgctcgtgattcggttaacgagaagtctaataatactttcatgcaacacctctggatatggctgcgaaattaacttggtagcgacaacgaacaacatctaacggcgtgtaagacacaccgacccaaaccagattaagttcgcgtgacacattaaccatctcatcgcgtattttcttcacgatgatggcagtgcgttcatcacccaactcaacaagcgctgcatggaacagatgcttgcgatgttggaacatagctgcgggatacatggaatccaacttctccatgagcatcgcttggcgtcgttcgctgggcaggataaggccgttcttcgcacactctaacaggtacgaggtcacgagcacgtattcccaccccgacaccccaacaatactttccgtgagtttcggccaccatgcttggaacatcatcagtgcgtagctgtgtacagttcgcatcggtcttcatcctcggaacacagacgctccttcgccatcacatagagcttatccaaactaagaatcgagatgttcttccaaaacgcttcgatgtcgtagccttcgtcaaacagacgttctggaataatcggttcgtgatcttgtcgccacaggtacttattggatgggtaggtagtaaccagcgcttcccattcacccatactgcgcacaccatggcaccacaactcatgcatatcgacatcatccatttccccggtaaaccagatacggaaacgcagcaggtcgtaatcggtagaaaaaagaatgggggcgtcgagatgattggccgtctcacgaagcgaatccaagatggtactttggatattgacctcggtcgtcaggccaccggtggtcgcgtagtaatcgttcgtcacccgttcgattaacttgactacccgtgctgaattgtcgataaaagattcatcccgaacatcgtcgtagacccagacgtatgatacggcacggctgagttcatcggaatagacgcatgctttcaaacgttcacacacgtccgttaacaaccacttgtgacgggagcgtaagtcagaccgcgcgatttctcgcgcaatcatcagatacgctatcttcgcgatatgacgcgcctcaccgagacgcatcaaatgatcgtgaagtgccgtcagtaggtataacctgactggccgcatatccatacttacagctccgtgaaagccacgccttccggcaaggtgtcgagtgcacgccatttgacaggcaccaacatacggtcaccctctgcgtcattttgcacaacttctaacaccacatcagcttccacatccaacttgcccggccaaccttgggcacagactaccggttgaacatgaacaacgcgcgcttcaatagcatcctgacgcagcttacgcagcgtcgcacgctcaggttcaccgatgccgtcattttcatacaccactgcaaaggtcttcgggttatgctcaagtaactgagcttcgttggtaaagcgcagcaggaacagaccatggcggtcgaattgggtaacatagttctggatagcttgttcaagtttcatttagatactccttaaaggtcaatgatagtttgtgctttttcggtcaggcgacacaacgtcaccatttccccgaatgggatatggtcaagcgattgcccgtcttggataagcgacccattaaataaataaaattcattaccatcgccaacagtggcgtggtaaaagagtgtgcccgcacgagcaccttgccactcggcatacagctcagcgtcgtaatccccttcctgtacagcccagacgtggtcacgtccagagtccatatgcaactgaccttgacagggctcgtaccagaagcccacaatgtcgcgttgccccacgagttccgttaaggcttcccatgttggtgtcaagcgcttcgttgcagcatctaagaactcctgtgaaaccagttggttaatcacgaagtggaagaagtcgaacattttattttcaatcttttcttggtcgtctatccccaaatcacattcatagttgtaattgtccatgtaccatgaaaaatcaaacgtgatgtaattgaagtctaaaggacgacgcaaatttgcagcttgtaccacttcctcaacacagcggctgaatacatccagcgtaatctgcgacgagtcaagaaagaagtcaccccgatagcgatgccaccacgggtcagaattcatctcctctctaaagtaccgttcccacatcttgtcgaacaacccctcgacaagcgaggggttaaagagaaggagttcgggggtgttaacacgaagcattttgatactccttatagactactcaccaagataatatctatctcagagttttttgattttatcaatcgcttccggcttaatggtatatagttccacacccggttcttcttccgagtcttggtcttcggcagacaagatataagtagggatactttcttgtagcacacggatatcaccctgcatcacaaaagagtacggccattgaaatatctcatcgcgcagttctgaaatatcatccgcttccgccgcgaactcgtaatcaccgtgttcgagcaaggcaagacagacacgatcttccagtatctgccggattaacacctcacgctgcgtgaagataaccgcctttccttcccaacccaattggtcgtcgccgccaaacatctcgtaaatctctttcacgaaacgggtgacgtaccatttcatcgcaccgacaactaattcagacgcagggagttcacgacagtgggcgtcaaacatctcttcgatggtaaacatcccgcagtttcctgactctcgccatgccttatacttagccgttggaatacgaggaatcattaagcgttggtggaaatcgtatccagtgttactgttgatggaggcaattgcatctatcaataactgggccactacctccgccatcgccttacgactgattgccgcgcaatcgaaattcggtattgcgtcgccaatccccacttctgcacgccctttgatgtaggtcatgtatgcgtaatcacacaaccccttcatcaggcagtcagtgtgcatcgttaagatttcactgaataccttgcgcattacacttcctcttctttcaggatacgcttgttagcataatagccacaccacagtccatggtattccttaccgatgtagaccacagcaaattccacgcaacgtttctggggacgacgacagaccacgtaccacttaccacccggctccataatgcggttcatgtccgtacgatccggcatgtcgatcgaacgcgtcagaatgatcggtatctgcttgtcgctttctgggtaattcaccttcacgttgaaactgacatcaacattacgataaaacgtctttatcggtttgtctttctcatcaaacaacagatgagtgatatcgtttaccacaacgcttgggcgaccctctacggtgtcacgcaaaaaggcagccagttcgtcacgaatctctaacgcacggtaagagagtaacgctgggcgcactacgcgggttatggcgaggtcatcgtacaaccagaggttaccatcctcactgaatttcatcaggttggctggtagaccctcttttgttgcgtcttggaacttcttacgacgcaaatgggtgttgtagacaatcgcaatcggatcgtaacgcttcatcggtggtacattatcccacgccagttcgttgtgtttatttaccaactgatagatgttatcccagccgtctttgcttaggaacaccgcaaactgcgcatcgggtatcatcttaccgatgaacacgatatcttccttgttctttgcgtggttcccaccgaacatgtatttccagctttcaccgttaatggtcatggtcgggtgttcttcattcaccagtggataacagaacttggtgttggtgacttttggcatgtcatgcagaccaccgtcacctgccaatatttcgggttcaggttctggtggcaattcacccgaaacgctccacagtgggcggtactccaccccttgtcccgcagccacgagagatgacgctttacgtgccatcatatcggcacgttcgttgccgtagaacccagcgtgacctttgattttaatcacgcggatagaacgcccttcctgacgcagacgggatttaatctcatcaatcttcttgataagctccacatttgcaatcggggtaccgtccgcttttgtccagccgcgtttacgccatccatccatccattcgttccacgcgttaaccacgtaagacgcatcgatgtagacggtgtagttcttggcaaggataggtgagttttcaaagagactgataaatgccatcagttctgccacatccgaccaaaattctgccgggacgggaatcacacagtcaaagaaatcaactgtttcaggcaccgtgggcttcttaatgtccttcgggaacttcttgtacccgttggtcgtgacacactcctctacgtccggtaagctgtaaggggtgttttcatttaacaccccactgttgaatgcgtatccgtgaataccgccccccgttccgttcggggggccaacacgactaccgtccgtatagacgacgacatgatcgtactctttaacgtccattatttctctctcagataatccatcgccgtatattcaccggtcatcagttggttgtgcgcttccagcatacggtcaaagccgtgcagacgcgccaccatggctaagtggtaaatacgggcagtaatgtaaccttcacgcgccgcatcgaagcaggcgtggtggagataggcatctttgccgcgtgtccagttgtgtgactccgcacggtaatccggcgtcaggttgaacgcgtgcataatgcgctcagcggtacggtcagagtccagcatcgagaagcgtttcagcaaactcgttgggacatcgcactgggaaaaggcgttcatcagaatcggttggtcaaactctggcccacgcatagacagtgcaaccttatgggttttgaacttctcaaagaagtggtacaacccccacagggcttctggcatcggcatggtgccagagaatgcttcggcaaacgcttcacgcgatggtgcatagtcggggttatctccctcaccacgccaccatgccatggtatacggatcttcgtggaagatagctttcgctttctcatcgttcgggtcaatggtctgataatgggtggcaatcagacgcatcgtagcaatatcccatgcgcccgccccgatggaaaccggatacgcatctgcccgagtggatttggtttcaacatcaacaccgataatgatggtcgggatatggatatccggcgcatcgaagatattcggcgtgcgtttggttggggtgacttcggtcatggttaaactctcctgtgggtatacattagatgggtgggttgtgtaaaaataaagcgacacctacccccgaaggaataggtgtcgtgattagttaaggcatgtgctaaggtgggcttcgtatgctttctggaaagacttacgatcttcacggtagttcaatagaatacgcttgagttgcgtggccaaatcgcgtgagatatcctcaggacgacgagcctgttcgtctaaggaaatgcgctgcgggatggggtgaaccacccacaaatcaaacttctcacagataggtgcaacttgcggtggccgccacccatgaaccttggcgtaatcattgagattacgggcgtacacgaacacgtagtacgcatacgcattaacgtctgccacccacgcccgataacgcgggtcttccagacttacaaccccctgcggatagacagggggttgtccaagttcacgtactgaccactccgtattgacagtggccggtttgacgggtgcccagctgctacacgctgcgagcaacagcgataagcaaattagcatgaccctcattttcactcctcgtttaagttcctgagcagctcttgacggaactggctcatatctactacacctacgggcttcgcagcagcttcccgcttgctgtcaggccctttggtttcagtgtgaaccggtgtttggggcaccgctactggggcaggtggtggtacactcgctgcccccttcgcgccatcatatggtcgattgctcaagcattcgaaaatgcggctgtagagcgttcttaactcatctgcctgcgttttgatggtctccccacgctcgtcgttctggcgagcgacgtactggtcgtgttctcgaatctgaaccaatttatgaaactggtcaacgtaggcgtaagacacaaagagtgaatacgtcagaagtaaaacgattgcgagtgctgtgattttattggctcgggttaccttttctccatcccccggcttgaatgcttctaaaagcaactggagaaaaggaagcagtttaataattgcagctatcatgctcacctcggagtttatttttatgttcaatttacaaggcttcatcgaaataccggcactaatcgataacgctcctgaaggtgcagttgctccagtaggtgagttatccgatcaaagttggtcttttgcgaagaataaacaaaaattcgcgaaagctaaccttcaggttgaattagtggcgttcacgtacctccgtgatgaaacgaaggtaaaggtaccggcactctttactgaccacgtcctcgcgctgacccagtggatttacaaccaagcgattctgggtaacacgaaaaatgacgagtcagaatttcagcgtttgttagtgggacaattccaaaccacaatcagcaatgtgcagacgggtgccatgattcaggcaaacggtaactggttcccacgctgggtgagctggaaattcgaaaccacggcggacaaagtagaaagtccgtcggatgttgataaccaaattatggtttggttctcagacgctgattttgatcaagactatctcggctgggaaattgaagtgcagatgcccatcatgccggttgacactttccaagctgtcaagacggtcgtcgcaaaagcgatggaatctttcaacttacctgaccatgatgataaagtcaacgttctcgctgacggttatccatttacggcgcgtttaacgcacaactatacctggcacgatcgtgaagactatgaggctacgctggtcattccaatgaccctcataatctacggtcgggcaggtttgaacccaactcgccagaaacaagcgttacgcgattacattctggcaaactcggattatggtaataaggattgggtgccggtcttcccggaaatcttcaccaccaccaaattcaccatcattcccggctggtccatccgagggattccaaaccaagaagatgtcgcggcattatacttgcccctcttcccatatgatctccaggtaaaagccatttccaaattcggtgaatggcgtgcgctcactgcggctgagaaaaataacggtactatcccgttaccgaccacggaagtttctgacctgccgagcatttataagtcgctcaatgctatcgctatcgctggtcctgagaatgataagaagaaagcatccttgatggatatcattccagactacgcgctgattggtagcagcaatccagatatctcccgcgtgtcaaaaccgaccaccgaatggttgagcttatacctcgaagcacttattgcggctgaggagtaccatccatataactcatccctgaacgtggtgaaaatggaagacgaagaccacgagggtttaaccttctgggtctttgaatttgataacgtggagttccgtgttttggcacgtagcgctgtttggcaataaggagtcttaaatgcggatacctttatcgccagaggtaaacttagctgggttgttcacggcgaataacccgtatgagtttccgaacaacgtggtcttcaaactggaggccatccgtacgttccctgagttgttacgtgacggagaagatgtctatctcaagtattacgagccgtatgggttggcacgacaagactacctcgatgatgcggatgttaaggctgcaatcttaacgttcaaatcgaccgacggtgaagtccgttatgtccctaacacattcttagctgattaccccggacaaaactcgattgcgtatacccgtaatgtgtatgtgttcgatttgggactgacgccgagttatgtggacgcgagtaagctaaatgatgacatcgttgcgttgattaaatcgcaagtgggtgtggaaaccaccggtgagttgaccgtcatgcagtatgagggtgttgtcaccgaagaagaccatatcaagatggaagcacgacgcaaagccaccatccgccaaacggaaccgctgacggagcagttagcggcagcattactccgggcgaatgaattgcaggtgatgaatgacaacatgttgaaaatcatcaaagacgcgggcttaacaaactaaaaaaataaagctacctaccccgtcggggtaggtaggctttttatttatttgtcttgggcgaggaacgccgccacgatgccacgcacttgggcacgcgtacgtttcttggcagggagttgcttgagctgctcgacgatcgcgtcgatacccagctctttgtgaatcttcgctacgatggccatctgttcttcgtcgatttccaccttcacggtttcaccctcgaccttaatcagacggtcaaccagttcgagtacggagttaccgtacggcccaatttccagaccacgttcttccagtaggttaacgtcaacaaaggtggttttcaggtcatcttcggaaccgagaagcgttggcctctcttcgacccgttggcgttggcgacggaagatgcccatttcaaagaactcagaggagcccatgattttagacacgtcaatccagttgcgaatttcccagataacttgaccgcgggacatcagcatgttgtcctgcgtgatagccccgatggatgctgcacattctgcgtaatcaaacggaatagacagctcaccacgcggaatgtggtacgggtcggcggatgcaatcagctgataaacaccggcctcgtctttaacaacgatagaccacgatgggtacggctgccacgacaccttcaacgcttcatcatcaggaatatggaacttatgaccattgatagccactgtgttttcaatcccatcaacggcgatttggatggcgggtagtggaaacgttttttccagttcgcaacctagtaaacattcaagctcggctttcgtgaccgcgttctgcccggcattacgtttaaccagcaaattactgagggcgctcagcgcgttcagcggataggcgaaatcgcgagactggatacgttgtacgagtgctttgattacagaagcgtgaaacatgataatattccttgtgggttagacagtcatttaatgggtagtttacgtaaaattaataacggccgtagaacggcttataaatattcgggtagtagaacattgcattgacggcttcttgcggtaaggaatcccaaccaccttcgcgtaccatggcacaaagaataccgcctaagacagcttcctgcgggaactcacggtcaaaacgtggtgggctagagtaacctacttgtgaaccaactttgggttcagggttagatgcggatgaacagatttgtggccatgacatacgcttgccgtatttacgtattaaccatgtgccgtaagagacaagctcgtatacatcatcggtagtgagtgtggatttctgtatccaacgacgcttgagatagcccgtgatggaaagcgtaatcaggatgggaatcacaagcgattcaaatgccagcaaatcgaaggcttcccatgttgtcatggccgaaagaatcacggacgagataaggcacattactacaagtacgacataagtggaaagaaaccgccagcgtgtgagaacgtagaggcggaatggatgtactggcttcctgatttctgccagtttaatcagcgatgtattactcattattatttttccttaaatgtaattaatgatgtgccataacttcgggttgaacgaaatgaaatccgtggcttcctcgcaaaccttgaccggtttttttcgcttgctctgtgcccagacaacagccatggtcgcgtagtccatgtcaaagttcggtatctctcgatgaatccgctttgctgcgtttttcaagtctgtccaatcggcggtcttgtataacccccgcacttcttcccccgccagaagctgtagccagcccaactcttcaagagtatgacccgactgctctacccagcgttctatcatggtcaatcggtaaaggatagccataatgctgcaacagaagacccacatcccgatgtagacaaacaggaaagcaccggccgggtcttggttaagtgcgaaaactccgtaggcgtaaaagaaggtacaaacgaccagtgagtttaacatgaagtaggcatagggatcgttgtgtccccagcgttgataacgtgcaaacataaagaatctccttgtaggggcaaaataaattaaaacagccagaccccgaaaggtctggcgttttcggttacactaacggctggttaggcaccacttggtactccagcacaaacagatgctctggggccgtttcactgcgccagattttgtgcgtctgcttgagcttttccagaatggtcaggaacgaacgttgaacgtacgctgactcaccccagaaaatgttttgtaacgcaacggacgcttccatatacgcttcggtgaagctcaggccgcgattgtacggttggttctgtcgccatgtcagcacatgaccgatttcggtttcgtcaacatacgggcgcatgccacatatccacatgaccgcttggtttgcgttccagtcgaattctgcatcttcggtatcaccgaaggcattttcaaacgcgtcccagaagttgtggcgctccgagaattcttctcgggtaaatggttttgcagggtcgatggtgtcggcccctaacgcaattgacagaatgtcttcggctgtcaactgtgccgctttacataaagcgggataccatggttgttggacgatgttcaagcggtgctcctatagtcaatgtagaggccagtaacgtggtgcgagttaccggcgcgtatgtgccgtacaaggtgtgccaaatctcttggagttcagcgactttctcactgtcgtcaggtttcactgcggcagtttgttttaccggttcagatgcatcgataggcttaaccaacgcgccataaaaggccgcatcccgtttgtaggagcgaagctcacgagccgcccgagacggtttcttcttgagcatagcgatagcacccgcagggccgaatttgtagcccagataaatttctccattagacacaggtcgcttcaagcgtctggtcatatcgttttcgacatggttaagataggccgaggctaatttaatggccacgcgcgaattatggatgtctgcatttcgtgcaagaccaagctgcttaccgtacattttgagcatcgcacgcttggtggggtcagtcataccgacgagcccttttgcggtactgccttgtttattcaccgccatgcggttgaatgtggattccttataaatcagtgtggtcatgagaccggtgtgtacaccttgctcgttactgattttcacaatgagagggcggactttttcgaagcgtccctcaatcatcttgaactctgttgcgtagtccttctttggacttgaagtgatggctgctgcgttgaacgacagcactgtcgccagacaaataagaatgaaacgtaacatcgtcgtatactccgttggtgttctttatacttttccgttactcggcatgaataacggcgcggacagcaatgactccttggtacgtgcccatgtgataatatctatttaagaaagtttagattaaggctttctttgcctcagtgattaatgccaaaggcaagtatacgcgatagttcgtttctccaggttgcagccggttgtagaggtggtggtaaacctctacacgttctttccacttcatccacccattgaccatgcccagaggcgggatggcaatagaatcgtttaagtcacgaccaaggtcagccaacgcatcaatcccggttgtgacgaatgacaactcagaccgcatcttaaaatgggtcttggttggcagcaggataatcttctcctcttcgtagaggtaaacgtgcccgatggtaatctcaccagcacgacaacgcgtgcgatagttttcatacaaatcggggtaacgttcacgacacgccaatgcaatacctttgcccattgccccaacacagtttatcgtgatgactttgtacgtctctggggcattaaacaaatcaccgtctacatggcgttcatcacgaaagacgagcatagctaccaatcccatcccagacagaacgtaattccttttcagtctgcacgataattttggttgtcattatcccgtccaatacagaacgtgtggcgggttgtggccggtctgcaatgaactcggcttcagtacggattgtttgtggccacttcaaggcacacgccacacaaatcgccgctaaggactttggattccatgagcggggtgcttcaacaaaaccttcacgacgaaactggggcatgttagataacctcatcatgatgcgtaaagacggcagtccgtgggaactcttctttacgggtatagtagaaggtacgtttgtatccctccctgaccggttggatatctttttcgtaccaccgtaatgcaatggccagcccggaatgcagatacaagcgctcgctttccgtgcagctgctgataagcggtcggtgaatccccgacaactcttttaaggcgacggagacgtgctccggtatcactttattcatttatttttccttacccaggaagcaaatgcggcttccaacccttcgtggtgaattccactgcggcgaaggcaagacacaagattgatggttgatgtaatttgttcgcatttctgcgggttcatcatagtaggccagaccttccgcacatcgacaccaacatgggtcaacattttgacttcacggaacaaagacggtcgaaggtacttcggtgtgatgttggccgcttcaataaccggctccatacgcagcaggaaattaaggcgtgtcaacatggtattgccgatttgggtgcacttccaacgcagcatcatttcatgcgccaactgcgacaggcgtgcgacttctgcttcgtctttataaacggtttgaatggcgggtctgaaagtcatggcctgttatccttagtcaatttctttacaagggctacggtaaataaccacctgcttatcttttcgatagcgctgccacaccagagaaggttcacccaactcttttgtcgcaaccgtacgtaaatgcgcgtcacctaacatgacggccaaccgacctttccgtcggtactcctctatcgtgtctaccatcttggtttcacgtaagaagaaactccggcttacattgaccgcaaagccgtttttatctttaatgtcctttgcaaagacgtcatcatcccataggtcaataccgatagccggtacgccaagctttaatgccagttctaacccgcgtggcgaaatactccacatccggtctttgatggcttgcttgatgtctttgggtgtgtgccatgcgtaagggcctaactcttcgcacagcaggaactgatagggcttacggcggtgattgtcgaggatagcccactcaacacggttccgctcatctacggtgtgttcctcaccgtaaatatccaccagactcacagctacacctgaggatgaactttggcaacataaacgtctttgccgttaagcaacgcatcttcaaccagctccagcacgctcgcgttcatcacattcaacggttgctgaggtttgactgaaatggtatcccacagcgtcgtcgacttcggtaatgttcccagtgcacctgagatgcacgcagagatcccagaacgctgatggtcaacgtgaccaatcgtacccacattcacatgcttaggctgtgccataagtgtgtcctttaagaagggaaccacccgcgcgtattcttgcgcacagacgacttccgggatgaacgaaattttagggtttaacataaatagctctcctcacgtaaaaacacttcactcatagtgaggtgattcgtgaggagagctacagtctttaaacaacagctgattgtgtggtcttgttattagccaaactggcatgtttatcaaagaacaggtttaaccagccgtcaagctcactggccacgtacccaagacgtgtaaagaaattgtacgcaggtctgcatttttggtgcacggttagctgtgcgttggagtagacctcgcgggcgttaatcaactcaatcaaggcagacatcttaccggaacgacggtattcttcagccacaaagagcgtacgcagtttcagcaccccggagattacccggtagatgcaatagcccaccacacgacctgcttccaatgcaaccgcaacgcggttaccccggaacagtgtggcaatggccagctcagggacgtcaattttgacgcctaatacactacgttggtagtttaaaaacgcataatgtaaacctaacaactgtttctgctgatctgttgtcagctcagtcgagtctttaagaatcgctgcatcaatcatcttattatcctgagtgagtccgccaaaaagacggttagtgaagtcggttgcgtggtacgcatagcatggttgctattaacgtcgttgacttttccaaagtcgcgtttttgcagcatgtttccccacatgccgatcgtggcctctctggtttccccgccagtcttccccgaaacgccgctccaacttcacattctctaattttatttcctgagcgaaattatcgacaggtaacgaatgataacctattggcattcccagaccaatgattactattttacgcacccgttcgtcgataccatccccctcagatggattttcattattcatgctatcgtcctatatcagaacaatcccatgcacaaggcatacaccgccccaaaggcaaatgcgcttgtacccgtaacgaagtaaagaatggagcaaaaaagattttttattagtttcattattttaccgccagaacagaagcggtttgaaatacgacgggttacgtccccagcgcattccgagtacaaacatttccagcgagacgatggccatcgtgaaccaatcccacttcaaaaaaaggactatcaacaacatcccgacaatgcccaacccatcccaccacgtaatggtgcattcacccatcggttttctagacttcatcgaaggctcctttaaatttagcacgcttcagcacccagttcagagaacgtgcaacaagatacaaacaacccaacgtaaacaacacatcgaacatcatggcttatcccctttgtattttgcttttactcgcttagcaaaccggagcggcatcggccacgcaatcatgaacagcgaagcggtcgcgattccgaccgcccaacctgccccaaagacgatgtagaacaccgtccaaataaaacccactactgacactaaggcattgtacattactgacctgcgtatttgattttcacgcccacgttgtaaaccgggggtaatgtcacgcccgttggttcaacaacacagtacgtcgcttcgttcaacttggaatgcacctctggctcgtgggagaccacgatgacctgagagaattcccccgattccgacaacatcttaataaaggccacgagcgcttgcttgtgttcttcatccatcccttcagacggctcatccaatagcaaaggatactgacgtaagttcagtcccttgtacgcggtcaaacggtagctcaggttaaagatgttcttctgtgctttggagcctttgacaacatccaccacagggtccgggttgttttttagcgtgtacgggaacgtgtaatccaaatcgccttcactgacatcacacggcaggacattcatcgggtattgccaaactgccccgatatatcggttcatcatctcagtaatgcgcacaatcgagttatagatgtactttttcagtacacccttctcgggtgaccatgcggtaatcatgagacgaatgtttttctgtcggtgttgcaactctttctgctccgactccaacgatgccaaggtatgcagctcactgtccatttgacggaagcgatcgcgggccactgcataggtgtccagcaacgactgtcgtttggtttgcaagcagtttaccatcacgttggtagtcgacgtttcaatcatggtgtccagaaccgtaaatgcccggctcaggaactccacagtcgtgcgtacatcattcaaacggtgtaactcttcacgccatttcacaacttcacgttgcgcgtctgagcgcttctgagaggattctgctaacaacgcacgaatacggtcaatcttggcactcaatgcactgtcaatattcccgacagcattaaccgcttcatcccaatccttcttcgccttcaccaggtcttcaaacacccgacggtattcaattgcctgcttcagttcttcaaagaattgaacggacaacatagcgtaacggtcacggttaatggtaaagacctcttccgcaatcagccgcttgaagaacaaaccaactaccggatctttcgtgtacgtcatgatgatgtcacggatacgacgtttggccatcacgtccgtttcgatgtcaccgcgcgaagacatatgagtttcaatcttcgtccgcagtgctttacacacatcgacttcccgacgaatagcggcttcgatattctctaagctgtcattgataccagggcggaagacgtgtgtgcaacgtggacaggttacttcctgcgtgtcgatgaaatgtgtgcgatcatgctctaacccgctcagcacattctcagcccgctggagctgttcacgcaatcccgcggagatagcgtcatgttccgctaaacgttcctcagtctcacgcagacgcgacgaatgattaatttcatctaatgacccagataatgagtacgtccactgagagaggtcattctgcgcgtttatgagcatctgggaactgagtgacccttcctcgattaactctggccaagcggtgatgtgcctgaccatgctgtttaacagcgcagactggttctcaatcgtctctttgaggccagaatggtttttcatcaggtattcctgacgtgtcgactcatccatcagaatcgacaactctcgactataagcatcagtcgttgcatccgcagatgccgctgactctttccacaccgaaagcgtttgttcagccacactgacttccaaatctgttggcagtgtacgttcgttcagaactttcgccacttggctctcgaggcttttcaagaaggcgacaatcttctctttgttcgatgacccatcaaagttaggcaggatgttaatggcctcgtcaagctgacgtaactcagattccatttcagccaaacgggcactgagcattttgcgttcttcatcatcgtgcaacacccgcacttgtaaatctgcaatcttcttggcggtgtggtcgattgccccgttcatcagactggcttgtttacgcagctttttgtaaaagtctaacgcatagctcaaatccgacgtggacatgcgggtgaaccatttacgccgttggtcggtgttcccgctggtcagtaatgattccccattgatgagttctttgacttctttatcaatcccggtcagttcataaacgcgggagttatacactttggcgttggcatgatccaacagcacgaaatctttggtcaggtttttgataaagcaaaccagactgttaccgtcacgtttcactttgaactcgtaacggtcgtcaccacacagggcaatattagtgtacatccccccatcgatgaaatcagttttaggtggggctatcgggaagaagacattcagcaaacttgttttcccgcaaccgttaccccctaagataatggtcacgtcggacataagggtgaaatcaaaggtttcgatttcgtgcaatcccatgcccgtaaaaccttttaaaataatgcgttcaaccttcagcatcgtgaggtcctaatgaattagttgtagttctttcataatcactaatactcacgtaaaaaaattaaaggaggtggcccgaaggccaccacgtcaggcgttagcgtccaaagaacgctccgccaaaatgttactccatgccacaccttcaacagactgtaacagctccaatgtaacctgagtcatcatgaccgcaaggtcgtgggtgtagagcggtgctttatcacccaagaataccggaacgatatatggcgaggacggattctggaaatcatagagggttccagcaggcccgactttctggtaacccgcaggattacgaatcaccacaacgcgcgatttaccgctaccccaatccgggaactcgcacgtaatcgccgactcgctgttggataccagcatgacacgcaccggcatttctgaattggttagataacggaacgggtcttcatggatgttacgttcttccacgggttcctcaaagtacgcatcaatggctgccagcgtatggggatacttctgttctaaccacgggccaatggtcgggtgttgacggaacatatcgaaacttccttttgaacaccccatcatgaacgcactggtgccgttcttcagggactcttgaatctccagcacacggatggcggttaacagctcttgatcaaacatagtggttcctttttggacaaaaaaagagggtgggcaatagcccccaccctctgcgacttagactgtcggccaatatccgctcacgacattgtacgacggtccacactcacggcgagtaaaatcgaagataggtaaacgacgcttgccaatttgcagcacaccgtttgcctttttgtgcatttccgagcgcacgaaatccggtaacgccatttctgaattggtcaggttcagaatcttaggcgttgaagttgcgggaggtaagaccagaatgtgttggcaatactcatcggtcgcgtattgattttgcgacacgtcgaagtgatgtccagatgcgtaaatccacgactgtaccgcaaggaacgtttccttgtgctcggcaaacaggctagaacccagcgtcttagtaaaccaatggtgactgatactttctgccaactccaccgctttgtcgtcaccgtcgcgtttaatggcgtcggataaggtcagcagcttgtgggcagttgacaccattgactgaaaacggaaccggtcaatgttgtacgcagttttcacttcgaagaaacgacgagcagtattcacagcagtagtaatggaagcaatcatgatataaacctcgatagtcaagaataaaaaggaccctgcaatcaggataacatcttagggggaaaacattgcagggccaaactgttagcggtcgagcggaactgtacctgagactttaccaaacagggcgagttcaattgcacgactgctgtgtgcgaatccgattttcaaagaagggtcacaggtcggtgcgatgaccggctcaatcacaccttctttggcgttcaggatgaaataatatccggcagggcaatgggtgccaccgtcagcatgaacgagcgtgaactcgtctttcttgccgacttctttacacgccacggtaccttttgtacacacaccgaaatcgggcgggttatactgatactgaatctcctgcaagatagcaccgatatccgttgacgcggaagcggtaggaataagcgaaacggctaaggcgaaaacgaaactggtgataactgcaactgcgtggcgcatgtgactttccttagttcaggggaacggtagtgattgcccaattggctttaacgtcgacgacctgcaaacctattttgccatcggccatccgtacaaactgcggacgggtctgggttttgcaccctccgtcgtaatcaatatcgcgtgctttaccagtgcgcatgttcacgataccgattggggtatcctcacacgccgtacccggtgtgccggtgacggacacccattcttcatccggggtcatggagaccacgtcacaatcaccggccttgatatcctcacgctgacaccagaaagagactttcgtcttttcgtaagtgatgtggtcggggtaccgtggtgcggtgtttgcgtaagacagattggcaaaactaaacagggttgcaaccaacagcgtaaggatgagtttcatgatattactcctgagctttaattgtgatccgcccgacggcgacagttttactgtagaagtttaacatctgatacccttctagttcagaaggggcaaaggacacatggtcgatgtctgggtcacacccgatatcttcgagacgctggtagaagcgggtattaccatttgcaagggccactccgcggcagctaccatctgtacccaccaacttgtacacgtagatgtctccttgaaatcgaagcatctcagcatgttcatcgggagccatcggataggtatcgtccgccggtttgaatttgtcgaacgtgacatcgttcgcttccactactttagacagacctgccagtacaaaacatacaaccgcgatagtcgataggagcttgcgcatttttattctcttaaaaaagttaatgttgcggtgaccacgagggccaccacatggaatcagaaaacagtaaagaacaggcgagcgtctttgttgaagttgtaccctgctgcgatcatccctgccagttcgtcataggtgacttcgacacggttctcgatgccactcagttcttcactgaatttaatgaagacactgtcaccgacacgttcaacaacacaatggagatagttttcaatatcaacatcgttttcggacatctcgagccgaccaacaacatcaactgcgcggtgtgctgcccagtcgcaaaacacgtccatgacctgtacacgcattgccaacggcaggtgcaaggcaaaggccacttcctgagaagccgcagtgaattgacgcttgtcatcgttagcttcacgcactaccttccacaggtcgtccaacttatctttgaaactttcaaagtgtgcaatgactttgttacggtttgccagcactttacgaacggcaatgacggatgctttatccacgatgttaatccttgtaaacggtaaaataaaagaaaggcaagagttaatagctaactctcacctaggtaatatatatctgagattatttctactgcgagagttggtaaatgaacttacgtgaaataaagccgagtttgatcaacccgcgaagattgtttcccacatccctgatggctttacgggccacaaagatttccatccgctcgcggcgttcattgatttccaacttcgctaatgcttcgtctacgaatccaggctctagaatacgcatctcatcgggcacgcccggcgcttggcgaacatgacgataaaccacccaatctgggaagtcgtccgacagacacgcggaggaagggatgtgtatttcggcgctggcaaaacgatttgactccagatggtgatagagtgcatctgagggcaactcatttactgaacaataagccgacagtattttgcgaacgtttttggcttcaccttttggcaacgacacaagggcagctttcacatcccaagaacgcgcacaacggaataccatgagtaccccgtccccattgctcatgcatttctgaatactgcctaacgataacccaacaggaagcttcccttcgcgttgtagacgttccaattcagcggtatcaaaatagctgtgcatttgtagcatgatgttatcctaaaaatatagattgctgttgtaaaaaagtggggacaatgtccccgtggcttataccaccgcctcttcactcccataacgaataccggctgtgttcagagggtagtaaattacttccccttctgcttcgccactaccgccatagatgaagccgtcgtaacccattgaagataccatgttccgcatcgcgccatcttcggctatcgcacagatttctaaaggtaatgtcaagaagtcttgcaggcttcggtcgtaaagtgaggtcaaggtgagtgccgtcccgtgactggcttcgagttcctgccagcgactggtgttgactaaaaagtgctcaaaccgtcctgcaatggcgagtaccttataggctgggaagaactcatagaaccaatcgagtgtaatacgtgaggcttctggtgcgttaataaacggacgagacaacgacagggtgactggaatgatggtaacactgccgtatcccttggcaatcttttgcgccccttcacgggtcgctgcgtagaatgtcggacgcatctcaacgagggtggtgccctccattgctttcagtgactcaatgaaggtagaaggtttgcagatgtgaaacgcttcatagcgcatgtcttgctccttagaatgaataaatgtgttttgctacacaatagttgtgatgctccgccaagtggcgcagcgttttcgtacgttcgacagcactggaatagcagaccgccacattgcgaccttctacaccgtccagtaacttgtcaatgtctttcaatgagaagtggtgcgcatctgttaaaatcaatgcgtcgctaatccctttatagccgctctccccgtcgagtgcgcagatagagccggttggctccataccgtctaccgaaagtgatagtgggaggacaaagatgacagccaactgttttgccccaccgggacaaaacgcgcagagttcacgcacgggcaattcacttttggtggtaaagattgactctagcagaaggacacgcgatgctgccattgatgcgtatttaaagataacggccggtttgtgttcgtcttcgaatacaatgtattccccggtgataggtaatttttgtacggtagggaactccttaccgtaattgaacatgatttcgccgctgttcagttgttttacaatcattttatttttcatccgattaagcatacctggttgccagcatggacagaactcttccagccgtaagttgttgctaactctgctacgacccacgcacggtgttcttttggaatgagatgatgaactatccctttcagctcgtccgcgtcgtaaagtcgcatgggtttgttggcgctcacatcgtttggtgttgggaactggtcatgactaacggccagccatgattccttccacgaattagaaaacacaaggttaatcgcgttagtgccgaggaagtcagccccatcggttgacttgaagtagatagtcacgccgggtacggttcgacggcggcgaccatcaacctttatcatcgcagcgacaatttcaacgcgcccatgtggccaaagtacattgtcaactaatgcgctatacaggtcacctaacagattccgtgaaaagtctgaagagagagcttgaatgcgagtaatacggataacgtcgtctttgtcgaccacagtgaaaagttgctgcgtggtttcgggtaagaaacgttctaactccgaatactccacatcagcttcattgttgtaaatctcattcagtatatctttgaggtcgggaaattggcacatgatgatattccttgatagtctatagttggtaagtaacgttagcgaagttgaatccggcgtcgacgaaataatccaccaaatcttcttttggtgaccactgcattacaagctcttgaccttctttcaaacttgcgattgtatccagttgcgttttggcgattttctcactcatcactgtggtgagatgttccatagtcgacaactctttggggatggtgaacccgtaatagagagcagggatggaaacatcgcgcccttctggtttacagacaacctgatagttgaacttgtgaatgttgatgtatccgttcagtaacattctcaaactgctgagtacgcccggagtgactctgtccacgtagatgtagaatatgcccccaatgcaggtgagcggctgtacgtgaaccggtacgttgttctccagcgtgaccaagaacggaaggtctttcaaatacaaggtgtgctgaaagctcacagggaaacgatactcgttcgcttctttgcagtcgtggtacatttcgttggtgagaatctctttgtgagattgaagaatgaacatacgttgctccttgacagtcggttaaaagattaccaatgtaatctcactcaggtaatatatatctgagaaaaaatttaatcgaagtggggccgaagccccacacggttaaccgatagacagtttcgctatcagcaacacttgacccccgtagaacttcacttcgctccagcccgcccagcgggccattacgtagatacgctctggattctcttttgcaccgaccccgaagacggttttaacgttcgcagcctgcaccagatagaccggcgagttaatactacgttcagccacgtcgggaatacgttcttcatcggtaccaaaatcggttgtgccagtcgggtacgggtcacgttccattccagcttcaaacacaaagcattctgtaaacggcttcacaccctgcggatggccatcgttaatgttaccacttacccacagttccaacacaactgccgtgttggagttaccgtggcgacggatagtcaacgtaggtgccgttgtactaaccaacacgctcttaccagtcgcagcgtatgctgtcgtgagcatcttcgcgtagttcatctctaactgacgcaggtattcgttattgttgagttcgagaatcaccgcgcccccttcgcggtcttcgcacggttttacgggaaccaaatcgcgaatattgtaatacggggaggcgatagcacgtaagccggactccgacaagagtttcccaaacttctcacgccaatgggaattcggagtccgcaggacattgtcttctaacagcttagcgcctaacttaaaatcgaagttgtaattgattttgctcatttctaatacctctgaaaaaggaagaaggataaccgacggttccttattcgggaaacgtacacggtatccgtatggctcattgccatacgactgtttgctaatgtaaaaaagaataagtcaagatcaagacaaaaagaataaagggtgtcggtagcagggacgctacctccgttgatctatgcaatcctcacacagatcccccctttcccccgacggtttcccttcgacacaacaaagagatcaactgtaaaaaaggggtaatatgagaaccgaggaggtaaacgtggaaaagtctcaagtccatttctattctctgggtatcgtcgccgaagacaaagcgcgcaagacggatatcgtgagaatcattcccattgaagtcagcttcatggaaccgaccaaggttgctgtccaagagatggaaacagaaaaatcccactccacgggcaccgcaactgataacctgaaagtcaaagaggggaacaccattaccgcacggtggtggaagttcaactcgaaccgggtcaactccccgaacgtccgtaaagaagaccaagtgttaatctatcaactgggcgaaacggacatcttcttttgggttgacctgaacaccgcaaacgtgaagcggttagaggatgccatctttgcgttttctgctgacccgaacaacatgatggctgatgacctgtcgaatgcgtacgtggtgaactattcaccgatggacggacatatcacgctgcgtacgtcaatgatgaacggggaaaaggcagcatacattcaccagttcaacacccgtgacggtacatggatctgtcgtgaccatctcggcaaccagtattacatgaactcactggaatatgacctcgggtttgaaaatgccatgctatcgaaaatcaacatgaacaaagaagacatcttcatgttctcgaagaaatcgataaacatggaaaccaaaaccatcaaagggaaatgtgaggtgtgggatgtaacagccggtaagtctgccacgttcaaaacgcaagactggctcgtcgattcaccgaagtcgaagttcaccggtaatgtcgaagtcgtaaaagacttcttgtacggcggaacaggtgaaggtaaaggactattcacggttactgatgcgaagattgcgaacatcacgttctctgtccatacgcacaccgagcaaggggatgggaaagacgtgtcagccccgcactaaggaaacgataatgggtatcaaagatagaatgattattcttacaggtcaaaccggccttgtcgacgtaacgaaaggtggtcaaatcggctacgttggaccagtgggtcgcggagaattagtcttcgtgctggacgttccgttctgggcctcgaaagaagccaaagagaagaatcgtaaccagccgggttttgttgactatccggtattgaccccagctaaacgcgatatggtattccacaccaagcggaatgaacagaaacattaattacaagacgactgtctattatgacaaacgtcaagctgtcgaatactcgacgacattaaaccccgtcttgttaagcagccacttttttcagcgctaatttgaagatgttcacaataggcatgacagacctcggtctaaattaaagtcatgggaaagccctactcttcggagtagggtacttttcttttttacataccggcacgttaatatgctagatggcattgtgcctttaatcagaaagaggatttttctaatgagtattaaagagtttgcaagcgcagaaaccattccgtccaactacaagaaaatcggtaacgtcagtgctaccggttcgactgttgatgacgtaactgccgcgctggctaagaaagccgaagaagcaggcggcgacgcgttcaaagtgattggtatttccggtaacaatacccagcacggtgacgctatcgtctacaaagctgaataagcaaaaaagtaaaaccactacctctcccgttaaggagaggtagaccggttatttttttcgtgctttaacgcgcttcatcgacgcattgataacacgatacggctgatagctgtgaatcgggatagcgtcattcaccagattctgactctgccacttgctgtgattgaacagccagttaggacgtgtcagttccccggtgtggaatgtccactcaccctcttcccatgttggccaataaccaacacatttgccgaactgattaaacagtgggccgagcggtttttcactgtcaatgtcattcgggtcacgcaaatggaaacggccgtaagatgccccgtggttcagccccagttcttcaaactccagatacgggttatccactaacacgataaaactcgattcgtgttggagtaatgctttgaagttctcggggttcttgagcgcattcacggatgtcggtgttgacaaatcacccagacctattttctcccagtcgtaatactcgcgggtttccatcatggtcttaatcaggctcatgttcggtagactcagcatgattgccttgtcactgaaatagaactccggttttaaccagtgcaggataccaccgatgacgtaaccgacggtcttgcccgtaatactcaccgacaatgatagcatcagtgtagaatggtaatcacgggttgtgtcgagcttggtgagcgtcaggtcttttattggataggtttccaccgaaccaatgtcgtcaaagaaccaacacccgatgtcggattggccgctatggcggacaatgtttcctgcgccggacaagcgtacgcccacactatcctgcttgtgcggtacccactgaccgttcacgttgtacaatacattggtggctaatattgtccggttatcacccgtcgccagtaccaccatgtcactggcatcgtccagtgcaaagtcttgactatagtgatagttcggtgggcacagataggcttctggcccgatgggcgcgttcaggcactggtagtggccttcaacaaattcgagtttaggcaaaccatcttttaacagagcaagacttatccccgctttggtgtttaaccagtcttgcagcgtatctgagcgctgctggagttcgcctaagtaatacagactgaataaggtgaactcgtgtccgagggattctaatcccacttcgaaagtgtggtaatccgcacagagtgtttttaatggctgggaaacgtcgatggcaacccaagtccgggtgtctctggagaagccaaatgcacagtcgccccgcacttgataaatagcatccacaagcgattcctctaagggttcaggtcatagtatgaactcgacgacttggatattaaggagtagaaaatggctgtcgtctttgacccgcatcaaaaattaccgggtaatgaaattaccggtgagccgggaaccgtcattggtacgaagtaccgcatgctggtcccgaagaatggccctttttacaccggttcattggtcgtcaaaagtgctggtaaagttttaaagctggcctcggactacgtcatcacccatccctacatgacctctatgcagcggacgggccgtgccactcacggcatggtgtggataattaaccccgattacacgcagagcttcacactggattaccacgcggtaggtatcggtgtcagtagcactgcgcaggtgagtgccgagcgtgaccggaataaagatgtgttcccgtccgactgtcagtgggaaatggtaattggggatgtgtacttcccaccagtcgatattcagttcgattgggaaaactggaaaggtgagcgtgaactgatgacggccatcgctgccatcggtaccaaaattgcgcaattacccccaatctctgacccgtatttgaataatccgtttgcaccaacgttcccagacatcttcatgaataatggccgttctctggtgacgtacgataatcaaggcgggttttcaggtattaatgctggggttgcctcggtctatttatcttccaacgattacctgctttacaactacaagctggaaaccacgtttaatttagcgggttacgcaacgaacgctaatgccacatcgtgggcgatgatggtcagtgcgtattggggtgtcggtttccaaaacatcacattgaagtgggatagcgccagcttgttaatgcggtttgtgctcactatcaaagacgttgaacacgtcgtggcctcgtttactgcgaacaaagccttcatggctggtaagttccgcgtcgtcgttgatcgtaactacgacaacgataaagtacacgttgtggtgtatggcgcagccggtgaagtgaaaatggatgctacacttgatctgcgtaatcccccggcagactttgttgcagacatggcggcgaacgccacacttgccctgctgcaccgtggtaccgattgccggatgatctggtatgttaccgctggtagtagctggcgacacagtgtcttcccagggatgatcgttcctgacggcagtgacgttttaaccatcctcaagaagtatcacgagttggttgatagtctgtaccgtaactcaccggctatcgcacacgttaccgataagaacaatcctcacggagacgattcctacgggcgtatgcgggtaattgagaccaacggtatcgctgacgatgcaacgctcgtctacggtcgtacacaggcgcaattagccacgtatgtgaatggtcttagtgcgaaagcctcagacttcacagacaagatgttgcgcacgggggctgaccgaacgattaccggcacctttaccatgttgccgggcctgtcatctataacctcatcaaaagacgctgagtcaaatggtgtgggtacgaatttgcaggtcgatgataaagcggtgcgggcgctggcgcgtgacaacatccgtgtgtctgccggtaaccagccgattacgtttaccgctggggcgaatacgtttgtgctctaccctgactcgcgtggtctgcggtggaacaacaaaatcttactcgacccgacgacagttggtcagtacctgccggggaacagcgggggtggtgatggtatctattacggtgccaatacaccaacggttagtattaccggtaacgggattgaaacccagccgtttatcttgaccttcctcccgccgtctgattccgatgtgaacacgctggcaatgcgcctgcttaccagtgagtttggtgactcgcaatcgttggctgcgaccccggctttgattaagaagctggcacaaacctttaccgggaaactggagaaggcgcgcgcgtatatcaacggggtatcgttggcatcgtctgtgaccatcgacaagtacacattgaatctgggtagtgtagagaacatcagcgatgatgcgctgccggtctcgaccgcacaggctaccgagtttgcgaagtatgctcaagtcggccacacccatgacgctgcggcgtttggtatcggttcagccaccacagccaaagcgggccttattcgctacggtgggttggtgaatgacgccacactcgccctcgacggttcttacgtgcttcaacagctgaaagatgtggcgaagctcgaagcggtgcaggataacagtgacccgaatgcggtgattgatatcttgcgttatggtgagagtggtaacggtgcgattcaagcggctgtaaccatcacgggttggatggtgtccatcaaagcgaacaactatttcgttggtcgcgattacacggtgcctctgaccacgttcaacgtcgcagaactgttcccggcaagtcatgaagacaccacctttggtatatttgtagacatcgttgataatgctgcggtttacgtcattaaggacagtaccaatctcgccgaatcggaaacgatgacacgaattggcgacatcgtgactgacgaagacagtgtcatttctgccagtgtccgtaacgtaacgcgtttgggcgattaccgcgagttgtctgaccacgcggcaaatgttagtgcccatacgccacgcgccatcacacaggcggcgtttgggtacacttatggaaaagaaggtgtttcgtgggccggtgggtcaggctcggtaaacaccgtagggagtgattggcgagagttcgctatcgatggtctcaccgcattagcggcaggctaccccattgatggtggtttccaagtcaccacgaccaatcgtgccggatgggtgaacctgacaccaatctcaaacgttgatggtgtgggtgttaacttcacaccggacgagacaaccgtttcgggtgatggactcttacacctcttggcgtacaagaaaggtgccgccttccgcaccttgtccttggctgttaccacttcaggtgtcaacagtcctgctggtaaccgtgtcaatctggcattgtgtggcaactggggcgcagcgggcccaatcccgtcgttcacgttaggtatcgacgagtcgcgttacgcgatagcatcatcgtttgacaggctcaacccacgattgacgtatggtctgaatcgggggcctagcatcgtcattaccggcacggtgaaacttctgaactacaccatcaagtacacgttgacgctctccactgtggcgtcaacgatggcgattgaacgggtagagactggggagaaaagcacggccgatatcacaagccgtttggcggccgcggacattgacgttgccatgcttctcagcacccctgaaaagccgatttatttcggtgttggggccgcgttgaacaagacggtaaaaatcatggtgagttacaccgacggacagttcaacgcacaacaccggtacgctacggcactcgattacctgaacaactacagtgagttgggtcgggtacgggtttacgaaggggtggctggaaactcgcaagcgattgacctcaagaagtccgttatcgccaacagcattgctgcggcgaaatggggtgaaggtctgccgagcgcgattaactacgtggggatggacttgcaactcgtaggcagtaactacaaggccatcgtatttagagattaaggagaagcaaatggtttcgtatccttacgactggaagggtactagccccgcaaatgcgttcacggaagaacgcatcatcacaaatgagaagaccgatgaccgggtggtgattctgaaaaatcgcccgttcttcgaagtcagcttagtggtgactgcgtccggcagtacgaccccgcttacccgtggggtcgattatgaaataacctaccagatgccagaactgaatgagtcggtggccacacctgttgcgtgcggtgtccaactcatcaatccgaaaatcggtgggtctttgacctttaaaggtcaagcgttgggggatacgttctattcgccgttcattgacattctcgatgagctgattaaatacctgaataaccctgtggatgcagattggtttaaggttgataatcgcccgacgttcttcccccctaaaccggctgccacttcatggcatgacctgctgaataaaaagtacgtggcgtctgccgttcatgacgttgagctggactctgaggcggcgaacaatgccgttaaggcaaagcttgccgcattgaaagtcaccgtcgccggattagcgaaggaaatcaccacctttaactaccccgcgcacattgctgcacacaatccccacgggacgacgcccgcgcaagcgaacgcccatcctgcgaacctgaagaccccagacacgttcttagcttacgggaagaccttacgtaccctgacggctgaaatccgcgccttgggactccagcagagcgacatcgataaatatatcgagaagtgggcatgcaaagatgtctccggtgtctttattcagcaactcgctgccaaccggtcactgtttaagtcgaaaagcgggacatcggaaatcacatttaccgatacggcctttacgattaaaagcaacggggcggttatcctcgccgcaggctacgacgccaacgacaccaccacccgtttcatggagtggacgtcggggacgaacaccctgcgtatcgagtcatcaggtaatgcccttggaatggacaagctgaccctgaacgggaaggtgttgctcacgaccacgttactgatgaaataccaaccgactgagggtggacaaaccagcgacccggacgaccaaaagatttacgttcagggacgtggcggtatttcagtcaccggtaaagggtcgaaagccgatccggtcaaagcttctctggcgctgccgtctgccaccaccaccgtaaaaggtaccgcggtgttaaagtcgggtgtgggcgatgaagtcagtggcgttgcctcgaccccggattcgttgcagccgtatgaaggtaaggcgtcgggctatgtggcgaaaaccaccatgctcaactccaaaccgatggacgacggtgcgcgtgtgttgaccaggtcagatatcgggctaagtcaggcggataacaccgctgacgttaacaaaccggtctctgttgaccagtctaccgcgatggatgggttaagtgataaaggacacaagcacacgtttgcctccttaaacttgccgctggcaacgaacgccactgagggtctgggacggtacaccgatttggacgatggattgtccgctggtaaaggtgtgacaccgaatgtcctgaaacgcctgagcgatcgtctggatgtgattagcgatgcgttgaagtcggtgaagacgggggtgtcaaccgacttctccattatcgatgcctcaacgtggtcggttgcttctggccgtatcctgcaagtcaaagacctccagtatttctatctgcgggggaatgaccgggctgagggtaaagtgagtgggtcgattaacctcgaaaccaccccgatgttcaactggttcagtccgaacaacacgatggagcgtaactggacgcccgcggtcaagaataccgccgcgaactttgacttctccgccatttcctccaaacccaacttcgccttaaaagcgacgcctatcggcttgagcgccaatgggatgggtaacctgtccgttatctccctgctgtccaaactacgcttaaaatcgtacacaggcacgctgaggttgtatatcgtggcgggtggcaaggtgacggtctatctggacggccaacaggtggggacggggaactcgccgttcttcttggaagtcgatgtggactccgcaaaacaatctgcctgcttggggattcgtgcggattgcaatgacgcgaccaaagccgcggcgatggcctttgaggtttacgacgaatcgctgccaatttaccgcagtgatgttggtacaccgattgcccagcttggggagttcatgaccccgacgtttggtaaccgccacttcctgtacctgaacatggtcacccaatccatgtacagccgtgctgaaccgcaactgactaatgaggtttcaccagaaaccgcgttgattggcgtggttgatgtccctgcgggtggcatcactaccccgaccgtcagtttcccgatgatgcacgattatgggatttccaatgacgcgtctgaccacattgccagtttgcagcagcatattccgaccgcccgtgattggacactgacggataatctggtgatgctgccgattggtaagctgcggttcaattcaccttctgctctttatggtgaagtcaccgctggcgctgagacggtttacggtctggcccagatgtcacgcaacagcaccacgaaaaaagcgtacatgctgctggagaccacggagcaatcaccgcaatggtggtttaccccgtccaacccgaaggcaaacgggacacccaccttccaaggcgggttagtgtacgaagagtaccaaaccaacgggttgttcgcacaaccgttaccggtcttggtgtttgccagcccaacgcttgggagtgtgcctgcggattatcgaaaccgttatctgcgtgtaccactcgatggtgcgacagagccggactacggctacgttaacgccattgcaacccatgcaggtgtcaatacgacattgccaacgtttgaatctaacgtcctgtattccaagacgacgtcacttcggaagaacgaagcgtccgcggtcttgggggtgatggatttgaccactctgaaagcaggctctccgagattggcggtgcgttactcgtacaatgtcacccttcggaaactgtcggtgttcagcgtgtacttcgcgggcaatccaaacgacacggacgggaccttgctcattaatgagttggagattcagttcgatgttgatgttcgtggtctgatgggtggcttcgtcgggcttgaactgccgccattgggcggtggcacaagtatctgtagcctgctgggctctgtggcaccactggacgggattgggtttgctgaagatacctaccagtaccttcgttcgctgttcgagtcgtatgccgattccggtgtgctgccaaacacgtcggttaagaatgcgaccgtggtgttacctgcgggggtgttcgtaccagacgtacggtataccgaataccagttagtcccgatggggtgccgttctttccatgcgtcacacgcaggttacctgccgttggcgtttaaccgggatgcgctgcttcagtcggttcactctgtcgtcacgaacggcaactggttcggaaaacccggcagctctgacggcacgaacttccttatctcgggcatgctcgttgagtacaatctcccgcagtcctccaaagtggccaaactgaaaatcgtcaaaggcacacaagccaatgcggtacgtcagcttgccatcggtggacaggtgataaatgtggcgtacgcttcatctcttggcggtgaactcggcgttccggttccggcacgtcgtggggatttgaaactccagctggcatacttgccggggtacacatccgatccgttgaaactggagttcacgtacgaactctacgatgcgggcggtacactgctcaccacgataacggaaagtaccgtagcggatgcgatgtggtttatcgctgaccgttatacagcgaaaaggataaacccgctgcacatgaccacgaagttgtggaaagtgttgcaggataaaatggacgctgaacgcaccacagatggaactgacttcggtcagtgggtataaaggggtacacgcttgcgggcgtgctacccgcaagctaccgcccgaaagggcggtaaccttttatcaatacgtaggagtgttttttcatggcgagcacgaacgtagccaaatttaccggtacgctactgacgaccacgtatccgaacaaatacaatgtggtcatccctcctgaggggccgttcttccgtaccgggcttgagctgaaaaacagcgcaggcgtgaagctcattgagggtctggattactacctcggctactattataaagaagccgctgtcgcgatgaaagaccaaatctacggcggggtcatgttgattaacggggacacctccgttgactacacgatctattcgattggtcgcgagtaccgcgtaccacagaccgagattggcaagttcttggtgaaagaggacatcaaagacccgcgtaacaccgactggtctgaactgatgcgttatgcaccagtggtgcctgcaattgacccgcctgccaacttagatgaagccctgcttcgcgatgaggtcgtgaaggcactggacgatatccgtcaaggtttgattaagcgcgcaggcgacatggatgcggcatacgccgaagtcaccgatttgatttttgccaacggtaaaaagattttcgatgacaacatgtacagtcaccaccgtatcaaaaacgcacaccaatacactgcggacgagattggggcgttaaaggtattgaccaaagcggtagactcgacgaaggcattcggtaaaacgctggatgaattagtcactatcatgaaagcaaacggcattcagcaagctcacatcgacaccctgatgcctgtggtgcttggtgaattgcgcggacgcctcaaggtgctgaataacggtgcgttgacattccgtactgccgactccagccatgtcattaccctgcaaggtgataagttcctcattaccaccacccgtgctatcaacatcacggcggatgcggacagtaacgaacggggcgtgggggttgagttgggttcggggctgaacacggcttacgtcctcaacggcgcagtggcacctatctttaacggcgcgtatctggtcacaccggacatggtctcgttgtacctgtccgaagtaaaactcttaccggggaacgcttacttttcgccaaccgataccatcaaggtgttcggtaccgcgaagcagacttctccattgaccatgaacgcgcaactgcccacggcaaccgacaaagtaccggggctgtttgctatcaccaacctgtctgcaaatatttcttcgggtactgcgatttcgcagtatgccgttaacgtcctgaaaaagacgctggatgattacgtggacaacacgtacaccattaacgggaagaagttcattgatgatggcacgaaacagtcccttaccttaacgacggccgatttgggtgtgggtaacatcaacaataccgcgcctgctgagaaaccgctgaccaacgccattcgtgcggtgttggcaaacaagtcgctgtctaaccacacgcacacgtttgctgacctgacgggtgtacctacggcgtctgatacggatgcgggtctgttacagttgtgggatgcgattgataacaccacgaataaagtggtgacgtcaaagcagggctacaacgtacaacagcgcctgaacgagtacaaaggcgtgctggatggactgatgccgtcgtggacgaccggcggtgccgcttacggtaaccccggctatctgcctatcccggccgttgggaactacgctgggttcgccaagcgtgtcaccccaccacagtccttgggtgtgattaagcaggaagcggatacggtgtattccttacggaacgccaatgatggcttaccgaatacggaccacatctattactcctacgcccagattgacagcgcagggaaaatggttaaacgccagcaaacctccaacgtttaccaaccggcaggtatgagtgcattccctggggtgcaactggtggcaatcgttgtgtgtggcgaagacgcgattgtgtgtctgggaacggacaacaaatactacaccgtcatgtttgacggaacgcttaaccagaagaagcacctgcgtgtctggcaaacaacgttcccgaccgatttacccggttcaggttcgacgtttaactacacaccgaatcagctgacggatcatgtcgtggtctacaaagaccgcgtgcatatcctgcgcatggaactcagcaacaactactaccgcacctttatgttacggggcacggtagacaccaacaaggcgatggtgtttgcgtctgtggcactgactggcggtaccagccgtcaaggtgtgttcgttaacctgcgccaaccgattgaccccggctcaaccaccgttgtggccaatggtctgtcgactgtaacggccgcgggactggcgaaatggcaaacgcgtaacattgcacatggcccacaaacccatgtcggggcggcactgaaaaacgcgacgttgcgtgtgggggttgtcgggacgatttatttggcgaatgccgacgggtcgtatccgtttaccgtgtggccgacgtcgtatgtggtggatatggactcgcttgcggttacgcttgagaaccctgaaatcttcccattaaagattgatgttgatgggttgtatctggcgaccggtgaggagctgcgtaccaaagggtaccaagcaaaatggacgaacgggtttgccaacaaccgtacgcacatttaccccatcgaagacagtccgtatttttggacgtactttgacccaggcgatgcagtgaccgcgaccgggatttcccgctgtaagataggggatgatacccgtacgctgtttgaccatctggaggcccattccaattatggcatgaacgctgtggatacgtggtcgtttgatgggggtgtgggttcggtactgaaagtggggtacagtggtgcggtatacctcggcaacaacgcctacctgctggcaccgattaccgaggccagtgcagtgtatgtcgaagctgacccggattcccgatactcgccagactttggtggcttaggcccgtccaacgttcgccgtgcgtttgacctcacgaagtattacaagttggggaacatgacgtggtgtgcatcaggtagcctgcaaaacgggaaaccacaaggtgcctattggacagcgccgggcagccagaactatcaggctgtgggtgacagtccaaccgctgacgtgctgacaattagtcagagtgactggaacacgcttatcagcaccattaagacacaagcgccgtccggggcggctaacgcatacgcgagcgaatacatcaacgcaggggccgatcctcagttctctgtgtgggccattcgtccgaaagatgccaagccgatttggttagcgcaggtggcggtgaaaagcgaccgtaacagtagccgttttgtcgactactacctgttccagatttaccctaccgtgtcaggttcaacggtatctttcccaatctccactctggatttggtgtacggtaccaacattgctgagccgtccattacggcgatgagtatcacgtactaccattaccacacccagcgttacacgcaacctatcttctacgagaaaggggacggcacaggcttcctgcatttgccaaacgtgtatcagtacaacgtggttggtggggcgtcgtcgaaacactttgagatggtcttctccttaaacgggtcgaagctcgtcaaaacgagtgcgacgatgttgacgtcggcgtattactacaatccgacgcagttgacgattgtcggtaataaactcgcccgtacgaaccaaggtttcgtttcagcggcgtaccttgcgggcccggcggcgacccctgaagactacatgacaaatggtgcgggttgggtaccgaccgcgacgccgttcgagattgtggctggggtgaaaacggcagaagggtgggagttgtacatcaccgagtctgagagcttacggtttggctccggctattacacgttggatgcgtataaccagaacctcaagacgttgttccccggtgcgtaccaaaaccgtacgttctacatgcacgctgcggtggttaacggacaaccggaataccagcttctgacgcagaaaatgccagatactgattcccggctgtttatcggtacagtggtcacagacagtcagcgtatcctttcctcggagttcacgaaagtgaaacgcttgggtgaattgaaacagttgacggaacacaccgacacggtctacagccacgatgtgaatgtggacagtgaagcgcgcctttcgcgtctggggttattgcgtaagcaacccctttctgctccggcggctaccggcgatgggtatctggatgtgtcgcagattggcccggtctttacgtctcaaagccacaaggttcccatcgagttgctgcgagatgcgcaggtcgctaccttgcctaaagactacaagaagttcacgatgaaaggtgccaactttggtcaggcttctgatgtagacaatgggtatttggtgggtattccggggatgtcagcagtcgtctcgattgcgtggaaaatgattgtggagattaccccgtcgaccccgacggtgaaaatcaaattgaagagtggttactctttgggctccggcaccatcggatgtaccaacgccaacctcgatgtttccgcaacgttttcttctacgctggctgaggccacacttgctgccgaggtgggggtcaaaaacacattcgtgtttaatggtatcaccgggggtcaggccaccgcgttcgctgcgttcagtgtctccaatgtggataacggcacagcgacagtgttctatatctccgatgctgctaccgtggccattcgtgccacaacgaacgtacagggtgcggcggggcgtatcactggtggtgtgcttgatgtttataaagtcgccatgccagcaggcgtttctattgatgattatttcccgattgttcatggggatgtcatcttccgccaaccgattcccatgcttattgccgacaacgcgttgtacatcggcaacggggtcaactattacggcggaacggtcaccccgtcaaaactgacggtcaatcttatgcctaagttgccgtaaccatctaacacgtcgagacaaggacgtctcactaagggagtttggccatgccagatattctatttcaatacccacttgacctgacaggggctgcgtccagtaacgcggtcaatgtcccggttgtgttaggtggggggaaggtcaaccgtgcgttcgctttcccagcagggccgttctatgcggacacgttccgtatgcggcctgccaatcagcccaacaccatttataaacgcggtaccgactacgagctgatttacatccatccggcgtacatgaagcttgctaagaaccgcgaaatctgtatgggtgtggtcgtcactaacccggctatcccaactgatatcgtctgtcttgcacaggtcgtcggtggtccacagtcggcggttatctctgcgattaaacaggcgttggctgatgccaaccttgaagaccgcaaagttgactttgctgacctgcgtaatgtcccggatacctttgcagccgccccggcctttaaagacctcggtgacctgtttggtttcgaatacatcatcacgcaactcgcgttgatgaccgatgcgattaactccggtaacgaagttcagctccaacagattctggcagccatgtctgacatgcaaacccagatgatggcagcgctacaatcgcacatcgatgccaagggtaacgttcacgcgctggatattcatcaggcgaatggtctcactgaaaccgaaattcgtgcgctgattcaaacggttcagactgctatcaacgctgtccttgcggacatcggcaatttgaaagcggcggacacggcactcggtgcgcgtatcgacgcggtggtcagtgcactcggttcgtggaacgaccagctgaactcggtggcgctgaactaccaaaaggcggcgctacaacaggccgacctgaactctctggtgttacaactccagaagatggtcaatgaccagaaccaagtcatcaatgggctcaagcagcgcatcagtgatttggaagccgcagggtctgatacccagcagcagattcaggatctctccggccagctcaacgcactgaaacaacaagttgccgggttgcagaactctatcaacacgttgtctcagaacctgcaaaaccacatcaacgcggacaacccacacccgaactacctccacaagcagtatggtggtgtgattcaggcagccgtacacgtcaacagcagtctgacttctcgtgacgatgtacaagctgaagcgggtacaagataacacttattacatgaggggctgtcattatggcagcgtcctcatttttttattgacaaaggaaacgtatggcgatttcaatgaaaaacatacgcgaccgcgttaacaatgtggaagcaaactatgctaccggacctcgtgtagacgggcaggtagcatcgaaggcttacaacgctgcggactctttcagcgggtggtctccctcccgtctggattgtggcggcagttgtagctggtcgtgttctaacgggtgttctgcaagctgtactagctgtgcaggaacttgtacttctacgtgcgtgggtagctgttcttctaactgcggcggtgggtgttcgggttgttcgggttgttcaggtacctgtgcgtcatcgtgcagtggtaagtgtggcggcggttgcgccgggtcatgttcttctagctgcaccggctgctccggctgctctggtccaatgtagggagaaactatggctatcaacttacgaaacctcgctgatcgcatcgcggtgatcgaagcgaactccttaaaaacggaaggtggggtacaaacctacatccgtggtaaggcaaccaataacgtcgacttattcggcggccaaggacgtgttcattacgattgcggcggaacctgtagctggggttgttctagctgttcaggtggctgttccggttcggcatcagggagctgcggttcctcatgttcgtcgagctgtactgctggttgtaccagtgggtgctcaggatgttctggttcgtgttcgggcgggtgctccggttgttcgggtacatgctccggtaactgttccggttcctgtagttccagttgtacgggatgctctggctgttcaggcagtcgatagaaatctatcgagtgaggacctatggctatctcattgaaaaacattcgcgatcgggtgcagaacgtcgagggctacatcacgaccgcacaggccaataactatatcgccacacgcggcacggtcagttcgaccaacaaccttgctgggcttccattgacgcactataactgcggcggtagctgtagctggacgtgtagcggtgggtgcagttacggcgcgggtaaccgataaagtaaggataaagacaccatgaagaacgacctccatttggcgtatcgcacgacgcaaaatttcccgttacatatttcgtcgtacgacagtgtgaaagcacatatcgcggatgaagtacgccttatctcgatgctgccaggcgaatggcctaaggtacgtgggcgggacatcgtgcgtcagcagtacaccgaagagaatacctactccatcggtaagcacactgttcagcatgtgaagtttaatgaaagcgagctgaactccagtggccgcctgattgacggtaagtatttctttactgatgcagtcctgaaccactcgatggatttggaaatgatcttcacgccgtttgcggatttggacgtcattcccatggttcgtcgcgaatggagctgggactatccgtcgtctaacccgttctggtacaccttagtaccaaccggcacgacggaatataaaggtgtggaaaaataccaccacatcctaggttatgaaacgctcggtattcattgtctggccgacttgctggcatacagctacaagttccgctggaatgcggtagatgagcagttcgaagcgattaccgacccacacgaaatcagtcgccgtatccgcaaaccgtggatgcagttcttggttcagtggcgttacggtgaagcgccgggcacagaggctgacctgagcaagctggtgagtttccttctgacgaaggtctcgttaacggctgacgaagaaaaggcagtttcaaacatcaagtcgcgaatcgtgaccctcgatgaccttaaacgggttaacggacgtcatgcgattctgaatcagattctcgaagcctaccattctgactttcttctggatgtgggcgcgaagtttgaggacgaccctcttttcgcgatctattaaaaactggagcaatctgcaatgaccgatgcaccacaaatacgtccccctaccgagctgtcgatagtgacgacgtccaagtgtaatttggattgtagtttctgcggcggagcgtattacatggacacaaaagatgttggtcgggaaattcagcgtgaagcgctgtttgagcaactggagaagtacccgactttacaagggatgaattggacgggtggtgagcctttgatggcgacccgcaagattgaacctttgttggcagaggtcaaagcccgctatccacatctcacacacgagctgtacacgaacggactgaaaatgcgtctggaacatctcccgatgttgcaacagtttaaccgtatctgtgtatcgttcgatggatacaaagcgagcgagcgtccgctctggcgtgtcgttgaagatggtgcattcgaagcctttgaagtgatggcagcgctgaacaacgtccatacgtgggctgtggtcacacgcgaacagttagccgacaaatattggcacactgatctgctggacttacaccgtgcactgtaccactacggtttcaaagacatgacgctgctgttggacaaccgcatgaaaaaacctctgaaccaagatttggtgatgaacttcatgttcggttacaacaagatggaagaccagattgaacggttgaatgtcatgaacaatggctctaccgggttctccatcagcaagttctttgagcagtcgtgcaacgcgtgcagtggtctggttcgtctggactctgatgcgtctgtcggctacacgatggatgtggacatggaaatcgatagcggctgtaacatgctggcgaaagtcattgggcaagatgcctaccgttacatcaaccgcacgatccaagctcgcaaacatcgcaatgaggtaatcaaatgagcgaagaacgatctacatcgcagacgcgtaaacagcgccccacactcacgtatcaggttgtaactaacctgtcatgtaatctcgactgctcgtactgctacgagcgtaagtatccacgtaacaacaaagtggatgacgccgtcgattttatccatgcgtgttttgaccgcgaccgtcacatcgaagatgccgaaatcattatcgacatcatcgggggtgagccgtttatgcagccgaagattctgaaagccgtctttgagacagcagaagaattagcggcgcgcgacaaccgccagtacgtattctctatctctaccaacggcaccttgttcgaccgtcccatcagcaaagaaattattgaacgctggaaagaccgtctatcgattggtgtgtccatcgatggtctgccagaagtacacgaccgctatcgtatcttcaccacttcgcgtgaaggctcgtacgagcaagcgatgcgcggctaccaatacctgaaatctgtcggtattgcagaactcggtatcaaagccacctttaccggtgaaactctgccgcgctacggcgagagcatgattcacctgattaaagaaacgggcggtggtaccatctccggtaacgtcacgtacgaagacatcctgacgcgcgatatgtctctgggcattgcgaaccagatgatggacgttatcgattattgggttgacaacggctatcacacgtcaccacgtaacatcctgacccacatcattcctgatgggctggatttcatggcgacatgggacccggactggcgtcagaagttgctggacgatgaagcaacccgtctgcacccagaccgcgtacgtccttactgcggtacgctgacccacatgacctgtctcggcttcgaccgtaagatttacggctgtaatcgcttcatgtcaaccgtaaccacccgttcggctgttgcggaactgcgtggtcgtgagattgtgaacatcgacggtcacaagctcctgaacgaaatccagacgcagtacactaactacccgtctacctgcttaggttgcccgatgaaacactcgtgcggtagctgtgcagccgcttcttacgagaacggtgatggtgagctggaagcgcgtaaagagtaccacgctgagcgtcgccagtgtggttggactaccgcgaaactgttggtgtccgaatactggtatcagaaaactggtaccacgaattccgcagacctgcatgacaagtccatgtgttattgcgcgagctgtgtacgtgaacgtatgcaggcagaaaaacttaaattagaactcggagcctcgaatgaagtcattgctgattcacaattttactcggcgtaacgtccaccttgtcgatgcgtttctgcgcaaacacaagctgtacaacatccacgcgatcgtgccgggtgaagatttcaacgatgacaccattcgtctgttgaaccgttatggcctgaacgtcatcctgcctttacagggcgtggaagatgaccaccagtctgttgtcgaaatcgagaaacgtaatcccggtttcgaagaacgtgtggtggctttcccaaaacacaagttgcaggttatgcgtcgctctactggcgaagctgacccaaccaacgtagtgggactggccctgaacttccccggtgtgaccgttcgcgctctgcgtggtacgcatctgacagacgccttctaccacgagtttgaagtggcacgcaagacgttggaagagatgggtgacgaagcagaagaggccaaactgctctggggtgaagagttggaaaatgatttccagttcattgacttcggtctgctggttgaccttgggattgcaggagaatccggatgcttagtaacgacgaaataaaagcccgctatttcgaacggggcacacgtatcgaccgctacggtaactacgtggaagaataccaagaccagatggaaaaccgcattgggttctgcctgctgctgcactaccatctgattaacggtatgagcgacaagaaagcccgcgagaaactcaaaggcttcgacctgtctccggtcgaaattgaattcctgatgaagaagaccaaagagtttattgccgacgtactggggattgatttagatcaagtacgtaaagcactgacctcaacggacaactacctctatcaggaagtcaatgcgatttatccaaagctgaacgacaagtataacgcagaacgctatgcacctattgcgttccgtgacaagacgttccaagccgatgagaagtcgcgcgcatcgatgcaaagctacatgcagtctggggttgacccgatgtactggatgacgctgaacaacgagcctatcgagccgtggacggtggaggacgtgaaagccctctatgcggaaatcatcacgcgtgacaatgacctgcacatggtcatgtctgtgttgaaacaacgcatccgtatcctcacggaacaaaaagacttcactgcaatcaagcagcttgctgcggataatggtgtagcctaagccgtacccactccttcgggggtgggtcgcttttctttttttcttacggttgttatgactgttgttctttattagaggaaacgttatgacaactgtagaccgttggagtatggaaggtatcattgctgccaaagtaaacatcgaggccggttatgtgaataacccaaacgatttgggtggcccaaccaacttcggcattactcaagcaaccgcgcgtgaaaacggttacaccggtgacatgcgtaacctgacgcgtcagatggcactggacatctacaagaaagggtggtgggaccgtatgcgccttgaccgtattctcgcatggaatccactcttggctgaccgtatgttcgacttcggtatcaacgccggtcgtgcaaactgcattaagtctctccagcgtattctgaacgtgttaaatcgtcagggtaaactgtacgccgatatttccgctgatggcggtatcgggcctgctaccatgactgcgctggaaggtttcctgaaagcccgtgggctggatgggttcaaccgtttgatgttcgcactgacatctcatcaggtagcttactacaccgagatttcagagaagcgcgtacagaacgaagagttcacttacggctggtatgaccgtgtgtaccgtgagatgggcgactacgccatcaaagtgggcgtctgcggaaaataagggggttggcgtgctcaaggaattgaagtacaaagtcttaggtaatccgtggtttgtgttaacggaagactatttcctcccctttaccttgcgggttttgtatagcggtcaccccgaattggacaagatggttcacttgacgggtgtgcatcctgacacgctgatgtacatagtggcccccagaggctttgtaacggacttagcgagcatccccgatgcactgaggccgatactccaccctgatggcccgtgggccttagcggcctgtatgcacgacctcctgtaccaacgtaaagcgtcgacagtcccatacccggatactccagcggggaatctgtcgcgtaccacggacaagacgtttgcggatttgatgtttctgcgtatcatggaagcatcgaatgtcgataagttcattcgggaatcgttctacaaagccgtgaaggagtttggttggccgagctacgcagatgacaatctgagtttggtgtaccagaccccggtgaaggaaacgttacagtataaccgaaactacctcttcttccgggaagcgggcgaggagcggttacccgcaatccctgatggtgagcgtgtggagttagttcacggtactccggtgaatctcggctaccaaaacatcaaacggccgtttattgcgttgttagattaaaaaagaaaaagcctactaccctaagggtagtaggtcttttattgttttaattaaaatcgtccagctcaccgttggtggtgctcaggtcagttttctgaacttcttcagtgacggtgtaagacgccacttggcccggcaggtatttgatgtggccagctttgatgctgatatcaattaccttggcaccattgtcgccatcgctacgggtaatggtcaggtcagacagcgcgaactcatcgctggttttaccggcggtgataacatccgcgttcagtttcgccagcacttcttcgtcggtgtcccaatcagcctgatcggcagtgactgcttttggaccgataataccagaactcagacgagtaaagtgtagctctttctcaccggtgaagtgggtgttgtcagccaccgcagtgatggtcagtttggagttacgggtgtcactaccgtcgccgggtgcataatctgcaaccgcaccgaaagtgacgtcagcaacagccagagcctgtgccaggcttgagttttttgcattgaacagggcaaccagttgcgcctgtggggtgatgatggccatcgggtgttcctcttagagttaacaggtggtgcatagaaaatagagcaccgctgcactttcttacgaacgtggcttgttatatgacgtttgtcactaataaaatcgaaattgtgaaaggtagggaaaagatgcgtaaacttcaaatgatgctcgtcgcgctgattatgctggttgcgggctgtgcgatagcaccaaattcaacgggccaattcggcacgattcctgtggcttcaacggacttctcggtttaccagtgtagtgcggcaaaagagacgtttgtgaagtatcagccgcagattggtaaacttgaactgatgccattctcagttacggtagtcgataacggggccacatggcacgccagttatccgggcggtgatgtgcagtcgcctcaattgtttaaagacctgctcggtaaaatcgacggcagtgtcgatcctcttaccggtacccgctattatcgtttacacggtagccaaggtaagaatgccacctattcgtattccactgtcgaccccagcaccggaaatggcgaagggatgacgttcttccaatgtgtgacggaaggccaaccctcgttgaatacaaccggtttactggtcacgaaataaaaaagtcctactctcccttacgggagagtagggtccttatttttttgtctacggtatcacgagttccaaaacgtggaaaattgacgcagcgctactcacgttcaacgttgacacgttttggggggctgttccataaacaaaataacatacgtttgcgccgtactgctgtgcaaacatcgtgcttcccaatccgttaaggctggctgccgtgtccgcaagcgccatgtctccccacttttctccgccattgttgattaacaacagacgcaccatggtgttaagccattcgccatcagccagataatttgcagcgttcaatccggaggcttgcttgattgtataagccgcgttgtacgggaaccgtattacaaattcccggccgtttttctgcacagtccgccgttggttacgcgacaccgaacccgtagggactgccccgccatcatccgtaccaaataccagaccgctgttgtactgttgattgtacgtcatgctggcggttcgggtttcggggatgaataatatccgaccccggaacatgaacttgtggtactgcgcaggtgtgtactgcgcagccgttatccccaactgtccattgatttccagatgggtcaacagttcactgacctccaccggcccaaaatacccctcccaccatgtaccgaacttgatatccgtgggtcctggcccgacatcaaggtagtacgcttcaatcagtcgagaaccgaagacgcgctcgccgtttttcaccgatgcaacccagtaactgtacaccgtgttttttgcaaccgatgtatcctcgtagcgggtagcatctggaccaagtgttaccagtggggcaggaagtgcgttacgattcaacacggcgacctgacctgcgaggcgatagatttcaatcgcctcaatgcccttcgcagtctggctgggccacttcaatacaatacccatcagtagttctccaccagttcaattaccggacagtacaggccatttttgttaacatggttaacgtaattgatttgcgtgatatttgtaaccgacgacgaacctaagttggttaatccgcgcgtgaggcaccgatttgagttggtgtcgtgctccatgcagatgtggccatcttggtaccctgtcgaccctgaggatggcgggtaagcataacgccatcctgacacgcgtcgtttcttagggaagtacagctgtgtcgaataaaagagatcgttgaattcactgaacccggtcaaatcggtatcatcgtgcgacacaccgttgtacttctcatcaaacggccacgctttagggtcagagtcgtccgacaacccccgcaggacacgcaaccgataggtatcccctttccactggcactttgcgtcctgaatggcgtccggcaagtcaccgtgcccaccttccggcccagtatcatcggtaccataaaccatcccggcggcgtacaggtcagcccatgacatctgattggtaagatagcccgccgctggaatgtagagaattttaccgttacgaatgaatttgacgaggttcaatcggtaggccgcattccatgcggtacttctggcaagaaacacatcctgcaccttttgctggaattgacccaatgggaattggtcatcgtaatccagtggcccgaaataccccagctggtcggttccgtagaccagctcatttggccccacgccccgccgttgttgtttggtgtaaacggtgttgattccgtttaccgtgcggttggtggcagggtccgttaccgtcgtgaagtagttgtaggccacaccatacagcgcagtggtgtcatcccacgacgtttccccattacttaacactgctaagggttctgggagtgaggcaggggagatgggcgaggtgtcgcggtagatgcgcacgaccaccggttttttattgtcgttccgccagcgtaatgtgaaagccattttcgcggcactccttatcagttaaaggtatccaattcaccgtctgcttcatcgagagggaatttcgaatttggtgtacggattgtcgccgtggctaccgcaggcgtgaaacgtatcgagtcggtaggcgcaggtacaatcggcataatactttccgtgctttcaacggacaccgcaggtggcgtgagtagcaactcagccgtcgtgatcggtgcaatcggaaccaagtcattcacagacggttcccgtacggcaaatacaggtgtattcggcattgtgtattgcacggtaaagtcagccacgcctatcagtgcttggcttgggtctaccagttccaacaccggaacgtaattgtattttgacgttttatccatatccatgaaaccgctaccgcggaagttgaatatgatgtaccgtgtatcgtttcccggtatacggtgttgcgacatccaatagttaccgaacaatgcgataccgggctctgttccccactcacccccattgagtcgtgaaaccaatgcgtaatcttccccaaaggtcagaagattcgaaccaattttttgatcaatgacatcggagccgcgtgggagacggtggtgaaaatagaatgtccggtttttggtgtcggtgtatgaaaacaccttgtcttgcggaacaacaactttatcggtgccggggttaacaaggtagttcgggtcgtcttgactgtagagcgaacccgccttgtagtagtcattccacgttacgcccgccatgttcgttttggggataaagacgattttgcctttgtaaaagaacttcatccagcctacggttgtcccgccgctcgccggtggggtaatggtcgtgcccgccaccacaccgtttgcgatttgtgtaccgttaggcatatcgatagctgagacaataccaaagtaacccaaatcttcgttaccgatacgcagttcttgcggccccggtccggaatttggatagacaccaaccggtttccttgtccaactcacgtttaggctgccggtgtagaggggcgaggtgttcttgatggcaaaggagagatttgtgggactgataccgcccgacaacaccgtctttggtgcagtgaaatcatccgccatcaagttaagcccgagcgcgtcgttaatgtccggtatcgcatcttctaatgttacagcgtcacctgcaacagagaccggaagatacttttggttcgtaaaactcaggaggttgatacggtcgtaatggaggtcaattttaccggctaaccctttaccgggcacacccacgaaattcgcgagtgtattacgacccccaaaattacgggccgaaaccggcccgtgtataacgacagaatctggcgagataagtcccgccatgtcagggttatcaatgacgacttgtttgcacaataactccagtgcagtaccgttgtagaaacccatgggctttccccgttatggcatgatcagctcaagcacaatggcagtggatacagcggtggtaatagccgtcacgcctaacgtcgccggtgatgccgcttgcgcaaacgctgcctgtgttgccgaatatagatgttggcccaacatgagtggtaacgacgtcatgtcaccgaaacgacgtaacgcacccgcttgtgtttcaaccgtcgcgcgcagcatacgggttaacgtcgaacggtattcgctggcgatggtatcatcttgcaccgtcaggtatttacccaagtcgatgtcagagagcttggccaagcgtgcgatgtattgcaacccgttgatttccacgatacgtttctggttaaccgaacccggtacccccgacggcgttttcccaaaatcatcggtaccgaacaccatgcctgcgtcgtagaaacggctccacgaggcggtgaacagtgcgacatctgggaagaacagaatcttccctttgtacgcaaacttgaaccagttagccggttgtccggggttaccagtgtaaaccagacccgtcagttttgcggccaagtcgtttccggtaataaacgaagcactcggcacacgatccataaagcctgcgttccaacttccccgcgcaagggtggcgttacccggcccggtctccgagaaatacgcggtcaactggttggtaccaaaagaccgctcagaccctttcttcgctgccagacagtagtagtaaaggtttttgttgaccgccgtgaaatcttcatacgacgtcaggctcggatcgagcgtcgccaatggcgtacccggattctgcgggtcaatcttggttttgctacgatacacctcgaccgcatccaaccctttacccgcttggctatcccaactgattttaacacccatttttgtttacctcttcgccacaacagcggtatcttcaaccaactctaataccgggaaccagaagcagctcaagttacccgcgttgtacgccatcgccgaaatgtaatccgccgtatagggatacgtcgtaccgccgtacactgcaacacgcattccacgcacgacggaggttgacgccgcagaattcgcgttaggtgcacgctcttgacaccaaatacggttagtcaacgtcaggttgcccgcagtggttctgtcgtaggagttccacggcgtgcccaagaacaagtccggcgcgtcttcaaagatgttcggtagacgctggtacttcagtggcactggccacaccaacggatagaacaaatcgttgaattcgttatcctcagctaccgtgagctgttcttggttgctcttttgagcattccacaggtcgagcgtcaatggacggtcagtgatgccacgcagcagtcgaactttgtatttgtagcccttaaagtcgatgacgcggttctggttcgttagtgttaacccggccaagactgcgtcggcaggtccgtttgcatcgacaccgtacaccaaacccgcttgataaatagatgaccactggcacacgccgaaagtacggtctggaacataaatgattttacccttgcggataaacttgttccacgacggtgtgactgtgccacccggcagacccgatgttgtcgcagccgcggcaaggatgtgggttgagttcacgaagtcagaagacaacacttgcccgaagaagcccaagctgtcatcacccaacatcaatgtggagggaccgataccccggttgtccgccaccagaatcttctggttaggtgtcagcacctcatccacatcggttttgctgccgagaatgtaatagtacgtgttaccgaacattgcgtcgttatccacccactcggtaatcccagcggccaatgttaccaatggtgcaggcaagttcgcgttgtcaagtggtgcatcgccacggtaaatcgttgtcttggtggtgacaacgttggggttatcccattttaatcttaaagccatgatttcacctattgaaattcagggagttcgccgtcaaggctactgagcggaatcttcgaattgacatccacggtaattttcatgtaccggaaactgccgttcggaattgccgcagccacattgattggaggacgtaccgtgtcctgtggtgtcgtacttggcagttgcattgcaggcgcactgatcgtccgcatatacgtgcccaagacattgatcatacgcaccggcatcttcggatcgcgtgattggtcaatgctcatcgcaggcgggataattcgcccaaatgattcccctttaacattacgcagcggtataacgaccgtcttaccttgcaccaacttcaacatgggtcgccagttgtacgccacgttatccttaatgctggttacggtggcttggttcatctggctggtaaagatggagtttgttgtaccgtcgtcgtaatggttcatccacatgaacaaggtgtttaaatcaaaggacaggttatcccactctttggtgccgtatgcgttaccgtgcagcttattaaagatgcgggcagagacactcccagcttcgttacgcactggccccatagggtcagcagaattcgagcgtggtaatgccaaatcaacaaacgtgttattcccgtcaccggttttcaccacccacgggtatttgctgtcgcccttcaccgcaccgatggcattcaacgcattccacgttaccccggtcatcagcgtgctgcttgggaagtaatagatttccccatccaacgcaatcttaatccagaagagattcgcattcagcaccggtgtaaagttacccagcgtgtcacggtcactgtcaaagaggtcggacgcagacataaactcggcttgagttactgtaccaaaatagcctaccgacatatctccaatcaacatggtctttgaaccggggccagaatccgggtaatagccggaaggtttacgtgaccacgttaccgacaacgagccggtgtaagcaagtgatgatgacgcaactgtaatcggtacaaccgttggctggtatgcgtatgacaacgccgcagtcccattcgagatgtccgacgcctctaaccccagtccgtactgttcatttaaagccggtaacaaatctgcaaccgtcgcagctttgccgtccgcttcaaacaccaccgtgatacccgtaaagagttttgacaggtcaagcctgtcgtagaaaaactctctgcgccccgtaaacccagcaccggctttcccgtttaagacaaggcgggtttttcgcccgctcgtcccaaggttcgtagtgaaaggtccgccgagcacaaggatattatctttggtcagcggaaaggggagatcagggttgtcacggaggatttgctggcacaccaaacttaatgagtttgccgcataaagccccatgttgatactccgttatggtaagacaagttcaaagacgtaccgcatgtacatactggacatcacaccggtgttggatgtaaaggccatcgggcgatacgcatacgcgtaatagaagcccgatgtggaatacagcggaatcagacctactgcaccgatgtcagtattggaactggagttagacaataccggcaagtcgttccagaaaggctgactgacgcctagctcggcaaccaaaccgtcaaccgcgttaccacccgaaccgccgaacatacgacccatggtattaaaccactcacccttcggaccccagccgtttgtttcacccggcgtgttaccccacggcatacgtacaatgtactgacggccgtctttctggacccgagcgttttggggaacagcagcaacgccaccgggggttatcgacagaacatcagcgcccgacatcaaaccggtagcatacacggaggcgtaggtcgaataaccctggtgtgtttcaggaaagaacagaattttcccacggtagataaacttatgccaatactgaggttcgtattgataattgctttgttgcgcgggcgttaactgtggtaacacttcctgacggttaaagaactcttctttcgtcaggcggccaaagtagccgcatacccaatccccacgtatcggcacttgagaacccggtcccgtatccagatagaacgcttgcgtaatcttcgacccgattaaacgctcatccccttttaccgccgccacccaatacgagtagatggttttctcggtcaagtctttgtcgtcttcagtgaaagatgtcgccccagcatcaagtaccttatagggcgtcccaggattcaccatatcgagcgtagcattccaacccaccttacggtatagctcgatgctagtaaggcccttagaagcctgtgacggccatttgatttggatggtcatatcagctcctattcctgcaactcaatgatggggatataacgacaaccctgcgttggtgcaacgtaggtaatcttctgcatgacgtcgagggcggtatacgcggtaccagaagtaaacagtccccgcgccagtgcccgcttggttaacgtatcacgttcttgacatgccacaccgccgttgtaagcagcattagcagaagagaacgaaacgttactgatgttaatcgtggagttagggcgattgactggcgcacgacggttagccgggaaacccagtacctgcgtataaatcaaatcgttaaattcgttatattcaggttgcgggaccagcttgtcgtggtttgttctgtccagcgcattatcaaacgggaacatcagggattctgagaacgtccgcagaccacggggaacacgcaagcgatagatgtcgctgttgtgaataatcttcccgccttggtcggtcggttgggaatcaccccaacaaccatctggtcccggaccatcaacaccatagattagcccaccggtgtacaacgtgttccacggcacgtcagcagggtaaatagggttgcggtcaatcagatagagaatcttaccgcggtaagagaacttcatcatcgggatgcggtctgtgaacggtgtgctattaatcgcattaaaagaagccgggaactgcgactgatccatctgctcggcatacggcaccagacccatgtagccgtattcgtcattaccccacaagaaggtcgtcggaccaatacctcgcttcacctcgatggtgtaactttgctgtgcaccgtagactgtcttgccgtttgcggtaaccgaaagcaggtagtagtacgtaccgccttttaatgcggtagtatcccgccactgcgtttccccgttcgtgagcgtggcaattggtgcgggcaatgaacccgacaccaatgcttttgtgtcccggtagatgtttactgtagtggcgagcttgttagggttcgtccaacgtaagataaacgccatgtgtattacctcttaaaacccatccaattcgccattggcatcagaaaggtcagttttcgaaatggtgcgattcgctgccttggccacaatcggtttataatcgactgttttcggaagacccatcacgaccggatggagttctgataatattgcagactgtgcagtgactggttggaactcaatcgttttcggcacgcctagggtcggcggtgtcaatccttcggttaacgtactgacggcaggcagtgtaaccagcgtgttttcaagtttcccgtttaacgattcgagtggcaccacggtgttgttgaggtcaaccaattctaagacaggccaccaacactgcgttgtccctaacccagtttttgatccaaccgtccagttagtgccagtcatcgttgataagcggaagttgttcgcggtgttgttactaatggtgtcttgcatcatacaccattggccccattgcgaaccgttttcgttaccccacaacccgcccgtaaacaggcgagtcatgagatctaattctgacccggcgtaattaccacttccaggtcgccctacaaagtagctatccggttcggttaacgacgctctcggcgtacgcagccggaaatagctcgtcacacctgcctttttcaaactgacttgtcttgattggctgaccggtgtcgccgttgggtatttccctactccctctatcccgtacatgtaacccaagttatacaaatcgttccaacttaggttgctggctgtcgggccctgcggcatgaaaattacgttgcctttatagaagaatttgaaccatccctccacaaaaagctgccggattgcagttgttcctttccccaagaatgtggcattccacagttctaagttagtgaacatctccgtggtatcgacttttccaaagtagccaaagttctcatcacctaagagcaaatacttcgaacccggaccagaccatccatagaacgtcccacgttccaactggtagctgaagtgcaatggaccgatgtaggctggggaagtgttcgcgataccaatcgaaatatctgttggtgtgctcgatggcgcaagtaccgtcgttggtgtggctaagtcctcaaccgataacgtaatcccgagtgtgctgttaatgtagggcaacgcggcttgtagcgtggtgactgtcttcggtaaatagatggttggacgaagtgtcgtgacgaacatgtacggcagttgaacacgatcaaagtacatcgcggatttaccgtaatatcctttacccggtttccccacgaccgttatcgtactgttgcgcccagacgtattggcggattttacagtaccattgatggccaccgtggtatcgttaattggtacagggaggttagggttatcgcggttcacctgacggtagataagctgcaacgccgcttcggaatagaattgcataatgactcctaagaaccaccgcgaacaaaaaaagaagggccatttggcccttccgttttagttgttgtagtggtagtacgcgacaccttttgccccggtttcgtcgataccggtctgaatcaccacgcggtcatagtccttattggcgtactgtgcagacgtggttgggacatcggatacgtagttactgttcagcggcgcagaatacgccggaacacctaacgaatccaataccgcacgtaaaccaccccagttcggcaaccctgccgaggtaacatttaacaggtttttgtacgccgtgaagtcgatgccaaaggtgtgtaagtccacacacttcttatcggtcaacggaatcgggtggtttaactcattgagcgcgtccaccgtaattgaagtatccaataccggcaagccacgcattaaccagcccgtagacgacccgacataagccggtgacgtggggaggatactgatgttgtagttgtacgcctgattcggctgactcacatacggcagggaaccgttgttgatgtctttcggctggaggttaatcccgtacttgtcaaggaacgacggcagcaactcgtggatggttgatgcggtgaagttcgtgataccgcacgcaacacgggtggtgctgccgagtttccaccacggcagaatacgatcgatgttgatacgatcgtaatacagtgtgatggtatcacggaagcctgcggtttgctgaccacgcagccgggccgacgtgttacggttgttgtttgccgcgttcggtgtgacctgcgtaatcttctcaatgataacgttgttcgcattgattgggtacggcaggtcagggttgtcgcggttaatcaaatcaaaaaccagaaggtcagagactttaccatagttcaaagacatggattacacctcattcgggtcatcaggtttattgaattgcagatacatggtacccacgaccgcggtattggtagccggaactttcagcttcaacactttctggtacttgctgttggtcggcattgtggttgcgtcgtttgcaccgatggacagaatctcggcaccagacagtccccacgttgcaccgttggtggtatcccacgttcctttcgtgacaccgttcaggatattcacgagggtcgacaacgtatcgcccgttgcaacacccaccgacagtgcaatcagcgcgtcgtgtgactgtgtgaagtcgaacggatacgagtacacttctgccatggtagcattcacggcctcggaacccatctgaccgttcgggtacttcagaccggacaggacgttcgtagtcactttcgacggcagggattcatcacctttcaggactttgaagtcagcctgaccgtaccatccgagggaagtcggattcgcacgcagacggacagtaccctcagttacatcgtcgttccattcgataggtgcatcgataaagtctgcttcttcaaacacaaacccatagcgcaggttaagtgccggaatcgccacgaacagggatttgttcgacgggccgatgtagatgctgtcacccagcagaaccaacaagtcggccagattacggcggttgtagtacacgtttttcttacccgaccacgttgagcctaccacaccgtctgctgtcaccttgatttgggtgttacggttggtggtcatgcctttgtcggtcccactgatgtctttgggcgcactgtacacaatgtcagtggctttcaccttaatggagttctggccgttgatagccgccaacagaacgtccttagagggttgataaattgccatgatttattcctagttgttgtagtgcagcagccaatcgccacccacagaaccgtcggtataccctgtgataacaagcacattatcgaaggcagtattcgcacggctttcggccgttgtttttagacgtgtaatcgtggctttcgtgtagtcgaacgccggaagaccccgactggttaacaacgtaatcaggttgtcggaggcaccactggtgaagtttgccccaatatccatacgcccgttaacaaacgcctgcataacctgcggttcttcggtgaagtcaaagccgtacgaaagcaacgttgcacaaagcttgccgtctttcgccggaatcggatggttcatctcatttaggatgtcatccagaatggcttcttccagactgttcttgccgcgtaccgattcgaaggagaaccctccggtgtactgcacacaggtcttcaacacattcacggtgttcttttggttcaggtacacgtacacatcaggaatatcacccgactcaagatttaacccgtagcgcgcgttcacgttttggacaaacgctaacttcttcgcttccgtggtcaagtagccataagcgttaggggatgtaacctgtggtacgatgttcttgaacaagtcattcaacgacaggcgagtgtagcggtaagtttgaccgccaacgtaaccacgaccttgacgtccccgcagggtaatctcggtattggcaccaccattcactgtcggtgtaatcgcccgcggttccccaatcagggcgttagcaaacccggcaggcgtaatggccccagggttctccgcgttaatcgcatcgtacagatattgtcgctgagactgactataaatcgccatagcagactcctcggcagataaaaaagaaaacggagctgggaggaggattggcctcctcccagcacgccgttaagcgttgaagtgcaagaacatggtaccggtgaagttagagcatttggtgtcgtccagctccagcagcataacgtggctgtagctctggttcgcaccttcgactggcactttcggatcggtaccggtagcggtgccgtcgtcgtcggtcagaccaacgtatttcacgtccgcccstttcaggg

SEQ ID NO: 4 - DNA, 75270 bp, Erwinia amylovora bacteriophage Ea PF 8 DSM 34961
  source 1..75270: mol_type = genomic DNA
cggtcagttgggatcggtgcagtcacttgcgtgatgcccggtttaccaccagactcaacactggaacggctcatgttgtagattactttctcgccaccgtgttcagagatgacacggaaggagtcggtataagcaaacggcgatttacatcccagaccaaagccaccagtaacagcgttattggttgacttggtagaagcaccatatgtgccgtaaatctctccgatcttgtcgtgaggaataccattaccactatcggtaattaccagatcgaaatcatcggtaatggtgacaagtcccggaatgtgagtcgtgcctgcttcaatatgagcatcccagaagttacacagcgtttcacgaatgaacgctaacttctggttggaatacaggtttgctgacatcatctggaagaatgatgcatcctgagttattgaaaactcagttgtcttttgtgcaccaagcgtgattgaagtcgcttgctgctggttatcggctactaacatttttacctcggatgtttgggttgatggaatgtttacagcgaggctgacagccctcttcgagtaaccgggccacagtcacgctaaaggtttggccctgccaacctctctgtaaacacaccaaataaaaaagcccaccgttcctgatgggcaaagactacacagcaataagaaggtggggtatctatctctcagggtgaaagcctgattgcctttgctacgggggtgctttggctgagatagatccccgattcggtttaaccgggaatgttttcgtaaggcagcattttgcggtattggttccagccatgcagattaccatgcaggcttgggttcaaccatgattcaataccatactgactgtctcgcagaaaatctggagacgcctgatgttcagcaggtgaagcatgtaacggcgaactgccaagcagcttgccatacagcttcagatcttcagcaacagttgtctcacgaccggaatgcagcagatagctggcacgagcacagcgagccacggagcacttgataagcacatcgtgaatctctttctcacttggctcatcacgagtgattcgaccgtatttgcagtgttgatacgcagcaacggtgtcagtgactttgttgatgtacggcagatgccactcacctgatttcagcagaacgggcgtagacttgctcatttccacttggatcagatcagacagcacacgaatttctggctgtgcatcttcatggctacgcagatggaagaagttcttccagtcggtagcagtcaccactacgttgatatgactccacggctccagcagacggttaacgatctgcttgtggtagccagcattgtcaaaaccttctgcgatcttgaccacacggtcacgggcaataagccatgcctgctctttcgatacctctacagtatccgtcagacccagaggaataatgactttatcgtcaagctcctcgtgagcctgcattcccggaatgtttttgccccagtgcatcgggatcgccggatcttccatgatgtcagcgataatacgcttcacaggaatagcacggctgcttgatgcattgcggctgaacttacgatgagtcatgaactcagcgtgtataaaacggggataacgaagctgaagtgtggtcaggcgaatgccatgatcaccgatgctgtcagccagcacttttacagtgattgtcattgcacacctacctttttcagctcatcgaataacgctttacgcagattaaacgtatccggttcctcatcgtcaggatgacaatccgggttctgcaccatacgcttcaacgcttctgcttcagcaggcgttagcgtgatggtcagcgttaccagttgctcggtatgagccttaacgtgggccattggttaatcgctccatagcaattttcatgtccttcttggctccaatagcgagccagaaagagatgacgaaatagatcagtgacgcgaaacagacgattacgttgatccaagcagaaatgcttccatcaaaatcccagttcactgtcaccagaaagcagaggatcgcccagacttgatgaagctccagcatgatccacttgaattgtgcatcagcgtaagctctcatcgtccaccatccagatagatgatttgtgcactggtgattacctcacgcaccacgaaacgtggcggggcatctactgccagccattgaccgtttttagagagttcgtactcttcgatcttcacggaagtatcggagacttcaagtgtgccacgtacatggtcaggcagacccaatatagacacgctaacgtgaaactcacgagaggcgttaccacgctcctcagtgcctttaagtgcttgtgcgagaacatccatctaatatctccggttggaaccaagatagaatggcaacgggtgcttgctattcttggttcgatgattggttttaatctgtggtttattttttacagcttccttttcaggttcaggctgaacatataattcatcacagataacgagagttgcttttgcaccacggagtttacctccggcatgtaaagcaattaacttttcttccagcttcgccatatcaggattgaatgactgaatgaaagacaactggcgttcattgaacaccagcttataaaattcttcacgggtaagagagcctaccttaccattgtgcattaccatcatttacagcacctcagatattcaaggtggcaatgatttctttagcagccatcacaccaccgatagaacgtggagcaaccaaagatgttatcttgaattgcttgtaaagttcatagctcactttggatccagaattactggcaacaataggaatgccgtactgtcccagatccagtaatgcttcagccagttgacgctgctcaggtaggccaaagcctttcggagcatagttaacaaagctggacgttgcagacaggggaatatacggagggtctatatagaccacatcaccacgttttacttgctgcaatgtttccagccaaccagcgtgcataaatgtcgccagtggtgctttatcattgaaagcgagtatttcctcttccgggaaataaggtgatggataacgaccatacggcacgttatataaaccatcgttgttgtaacggcataagccattaaaaccatgacggttcagatacaggaatatagcagaccgacgaatagaaggagtcaggttagtattgaactcatcacgcagaatataataacgagtctctgtgttatggttctgaaataataccttggcttcatcaattaatgattcagggtaatctgctacatgctgatggaagttaatcagatcctgattaacgtcaccgaccagataacgatcatagtcagtgttcatcatgacagaacaggaaccaccaaagggttcgacaagacgattacctaacggcaaatgttctttcagtctgtcaatgattcgggattttgatcccacccactttaatacagtgcgcatgtaacctctttggttgttgctgttaaacgaaaaaggcgagcattatgctcgcctaatcctgcttcacgccagcttattcagcagcttcagcttttgcgcccagagcttttttcacgtagccacgtacagaacggcctgactctttcacgtcatacgtgtcacgagtggtgacaacggtagttgcctgaccttcgccgttgtcgaggattgcaacaacgtggttagcattcagttcaatacgcacgccagatggggaagttactttgatcagtgacataatactctcgcttgttaattagctcttacgagcagggattggtttatcctcttggttctggtacttaccatcgtaatggacgggtactgtcacctcgtggaatacaacttgggcaatgccggaaccagccggaatgattaattcctctaccccgtggtagaccagttccaaggtcaagaaacctttccagcccggctcaattacagtattgaacacggacaggccacgccttgcccaagtggatttgtcatgcacgatgcccagcaggtcatcgggcatttgaaactcttccattgcagaggcgagtgcaaacgcaccattgctgtactctgcatccaccttgacgaaggagccacggtggaacacgacatcctgtttaatacgaatgtcatagccagcttcagacaggccataggacacaccatgctcagagagtttggtttgctccatgtctttgatcggagccttacggagtagagcagaagcgtttacaatcacggttaacctcttatatgaatgagttttccgaaaggaaccgttttactcggatttcggatacatacccataaaatgggcaagtcgtagtccagaggttccattggttccacttcgagatctgtaaagatgattgcggcagtgggcttgtgttcgtggatgaactcacggacaggagccagattcgtaccgccacggccacggattttaatttcatcgaagctatctccagcgttaaattcaatgacttcctgaataacgtcatcgaacagaacaatggtcattttgtcagggcagaaggtatcccagacgtatttcacttcggagttgaagcgtaccacctgtggcctgtcaatggagccagatacatccagaaagtagatcaggtgacgcagcttgccttcatcgacatagcgactcggcagatacacgtctcttgatcgacgatttggtctggcccacgaataccccacctctgcgagatcggtcatccacttttgcaattcaatttcccaaggcactactggggtcagaaatgccttcagtatttcttcaacctctcccggcataccaccggagcaaccagctaatttcgattggtgttgtgcagtcaagacaatctgaaccaattcagaaataggaacttgtggctccagcatatctgcttcgtagtcttccgggatgggtgcatcctctggttccccagagacagcacgagctagaagatgatcgtaaatatcctcttctgcccagccacggtaatactgatccttgaaaggacgggtgcctgtgaacacaaagccagcatcttccagatcattattgatccgaatgtcgcaggcatagttccacaggcgatgatcacgggtgcctttgcgtatgtggtgcatacgggcaacgtgccagagttcgtggacgaggacagtacagcgtacttctggtatcaggttctggaaccacacaggattccagtagagtccgacaccatcagttgcagcagtctcctgcccgtcatcccacacgaagaacatcgagcacatcaccgaaccaaggaaaggagcgtttctccccatgaaaaccgcagctttcaccttgtccagttcacgagttagccccagttcatcgaacgatacggcttccatgttttctccttggatcaagacagatatttagccagctccagcattgcagtgctgaaggttggagtgtggcgaatctcctgaccgcagccaatcatggcaaagcgatagtagagaatacgcatatccagaggcagacggttggcatacacagccagatgctcaaacgattctgcgttggtgtgctgctgcattgaggatacaacagcccaacgaccgttaacgtcaccgggaataggagcattagccggatctttcatgatggtcttaatgtccaccagatccttgaagactttcgtaaagctcacgaagtcagcagcaacaccagatgtgattgtgcctgcatacattggcaaccactcattcatctcgtattcttctgtctcgaagccgttgatagtcttcttcttgtagccatatacctcgcccttgatctgatcgttcatgaagctccatgtacgaggacaacagaaagttctgtcgttgtgatcaggacggaagtccatcagcttcttcggattggcgttcaggaaggcgatgatgcggggatcccattgctgagggatagccacgtcttccatgaactcttcaaagttgatagacatttccagatggatcaggcgagactgcattgccgtagacaatgtattggtgatggcacggtctgtcatcaggttgccagcacagaccaccacgcattgtgggtgcagcttaaactggcccactttacgatccagaatgatcttgtaagcagcagcttgcacatccttgggtgctgagttgaactcatccaagaacaggatccagccgtcagtaccttcaggtggagtcataccttctaccgggaagatgtccgtaaacggagccataacagcccagccttgctcggtgaaacgaggcaagcctgacatgtcttcaggagcagatgtggacaggcgatggtcaattaagtacaaattgtactcttttgccaacgccgcaataatgcttgatttgccaacgcccggtgaaccctgaatgtacggcacaagccgttttttcatacagtgctctacgaactttttaacctgtcttggcgtacaggtatacatcagaatgtctgacataccctctccagttaatagcgaacagtcagaaaaagaaaagccccttaaaggggcttctcattagactgcacgatgaactttcttggcatgtcccatacgggaagctagaccaagattggcgttcttagccatcttcttcacagcatgtttcgctgtgacttggctaatctcgaacatgaaacggttggtgttgatttcaccacgttcaaaacgttcgaggatttcacgtacttcctgagcatgtgtcatttggccttttccttctggatcatgttttgcacataatcttcgagttgatgatcaatatccgtactgtcccagccagttgctttagacaactcagctttgagccagaggacggtataatacgaggacttccaccactggtcactgcctacagtgccgtgatttatccacagaaaatggaagacctgtgcttttgcttcagaacggctgcatcctaggatgtcagcaatgtcctgataagggtcttttctttctggatcaaagaagtagccgaggtgaattttaatcgcctcatctacgtcttttgtgtacatgaataactgagacatacttttctccacagacttaatcacaaaaagaaaagcccctcatttagaggggcatttccgattacgctccgacttcggagtgaatctcgccgacttgcttggtcaggtcgttcaactgttcagttggcaacacagacagcagggctttaccgatcacttcattgaaggtcggttctaccactttacgctcagacatatccgccagcagcttgacctgatcctgaatggtcagtgcagcttcgtagatagcatcgccagtgatagattccactttggttcctggctcttgcagacccagttgaaccagcttcgcacgcttaaccacttcagcgattaccgctggaatggtgccagccagcatcgtaccagcacgcttcagatcttcgtcggcagcgatggtatctttgccgtacagacggatcaggcgctcaacagcatcggcgtcaggtgcgttcacgttaatgatcgcatccagacgacccggacgcagcatcgctgggttgatgttttccagatggttggtggtcagcacagtgatgattttgctggatttggtgtcgataccgtcgaggatgttcagaatgtcatccatctcaacagaacgctcaccagttacagcgcggtcaatatcttcacagaagataacagccgcagtgcggtcatactgcttggcaaactcaatggcataagccagttcgtcgctgtgcggcacgtagatgtaggtgatacccgcatcaactgccagacggcttgcaactgtcgcagccatagttttaccggtgccgtatggcccacccagcagaacgccacgcttaacagggataccgttagcgatgcagtcgttcatgcgagtgatcggagtgaacaggttggtttcgatagctttctcaacttcggcgctatacaccagcatatcgcgggagatgaaggaagtatcgaggaacttcggttctggcatatccagcagattgccattgtcgtcgaggaagcggatcttgatcgctttgccagcgtagatgcttttcgttttcaggaactcagcaacgccatccagcagacgctcgatgtttgcttcgtctttacgcttcacttcgccacggatagcgaatgcaatgcgaccatctttgcggctcactgaggtttcaatgtagcctttgatgcccggcagtgagaagcgaccccacggcacacgacgagttttaccgaagtcggtttcgatggtcagcatctgtggtggacgtgaaccaaagaagcccggggtggactcggcagcagcccagccaaactgagcagtcagaacttcagcgatggcattagcaccatcgaacgggaacgcatcgaatacacggctgattgcaaccgcttcttcgaggtaatcacgctgacgctccagcagatcaatagcctgctgagctgacatcccgttagggatcatcagagcatcatcgtggtacttaatttcggcaacttgtactgcttcggtagcttcggtcagattgcgtggcataattttactctctcctgagaatgggattgagaggcttcccaaaacgggaaacctcaagatttgaacaaccaaaaaacattttaacgatagggcagcactggcttagccagttgtctccgcaaagcctcaaaagactctgcttcaactccggtgccatacgctttgagaaaggtacgcaccattttctttgactggttctcgatacccacaatgacattgcttgggtatttggtgatcaccagatccagaagggcatacttcagggcattcagtttgatgcggtcagccatgatgccagcacagttcctcagtgcttgatcggtatcacggccttccagttcagcctgccttcgggccagttttaacgtcacaacagcatcagggaactcaccatacactgacgctgcaatgacttctttagccaagaagtgcatggcttacttctgacgggcagcgattactgctggatccatcaggtaatcgccgacttcaaacagctcatccacttcttctttgctcagacgcaagctgttgccagcatcagtcacagcgcagtagacaacgccttgaggttcttcgtggacacaggtgatacctgcgttaccacagcgacgaccgttacgggtcagcagttgtgcacccggcacgagttgcagatcagtgttcagaccaacagcccattcaggcaattgctgttcttcctgctggctcttacgtggctcaacgtcgatgacgttaccgcacacggtgtgctcaacattcagagcacgcagtacagcagacacacggtgagcctgctcgacgtgggattcctgcttatcatggtgatcatagatctcgatagcagaaccacgagcagccgcacccatcgcagcctgagcctgtttcagagccagactggtagaacgacctgtaccacgctgactatcttgctttggctcgctctgctgacgtttagccagttcagacataacgaccagtgcagccagcaaaccacctaattcacgattaatcacgatttctccttttggcgtttagcacgcctacgttggttttcgaggtgagtcaccagttccagatgttctggattaacgcagttgcgttggttacaaaggtgatccacatgcattcggtttgggatatacccaaagaaatgagtgtaagcgacccggtgcacggcagacgtaatgcaattgatattgatacgtccataaccaccaccacgcccactaccggagtgtgcaccctgccacaagtgacaaggtgacggaacctgtttaatacgataaccagtatccacaaccttcacgagtttgtagatacggtcaatgatgtcagtacgacgatcaggagctttactcatcatcatcttcctcatgaggatgaggaggtaacggcgtgagatccaagccgagatagataagctggtgcaccttattacccagacgttccacttcagcagcaatgacggcatcagcagcaatacgggcaagttcattgcccagttgtctatccgcgtagaacacacggaagaaatgcttctgctgcatgtgatgcttgatggtaagggcaagttcatcgatctctttgctcagcttgtgagcatgatgcaaattttcgatgttcattatttcagccccataaagtgcaggtgaatagccgtgttcatcagacggataccaattggagtctctttgctttgggcaatgagaatattggtgatccctttgatgtgactggattcggtgccatcaggatacagcttgcgatactcctgatagagttccagcttattgatgtgcttcttcagttcctccagaggcactgcctccgagaaaaagaccaaaggtacacgaccaagaaactcggtacgcataccagtttctttgaggtcagtaagcgtgtgaatcttctggttgctgtacgcaccaccgaagatgaacagagagttctcaatcatcactggctcgtacttgccatagtctgtgaagacactggcgtacttgctttccagattcatgaggaactcatcctgcacctgagatcggaagctctcagtcttctcaccgttgttctgaaacagcttgtcaaactcatctacgaagatgatgtttggctcgttccagtgctcacggagttgacgcagggacttggacaatgagttaccagacagcccttcagcagtaagctgggctgcatttatctccataaacttcaggctcagctcgttggctaccttgtttacgaggaatgacttaccggatccagatgggccagtaaggtggaaatgaggacggatttttgcatcagactgtttgaacacgctcatgacgtgagacatctgacttaccactttttgttgctgaggaaacagcatgttttgctccttggttcaaagaaccgcatctgatgtaagtgagtgaaaattcaaataaaaaggccaccccgaaggatggcctttttactaaaacttaatctaactgcacgttggtgcaatttgaccgggatgacgcccatttagcatattaacccccagcgatgttcgcacacgcatggagtgaatacgctcgaccagcttccattcagccagtggcacaaccatcgcaatggttgccgcagccttatcgaccacggtacgcagaacgtacttcaggtcatggtagaaccagtcagactggacgtagaagaaagagctaataaagccccagatataacgagttaatgaacgcatttttatagccctgtgttgacgaggatgttacaaccaaaaaactttaatgcttaggcagcattgacaatcttgatacgctgcatgttccagatcttcagaggatatagaagatcacgtactttatggaacagtacataggagtttggatacagggtatcaggtacggtgatgctacccaccttggtatagccagtctgtgcagcagagccagtagcctgtacacgcacagtctgtttcagtgtgttgtcgatatgaacatctaatgaggccatgagtattctccataaaaaataagccaccaagaggtggcttatagattatgcaagaagacggattacttgtcttcttcttcgacttcaggttcctgtggttcctgtggttcaacaggttcctgtacaggctgctcagtaggctgctgttcttcttcagtgttctcagtcacaacctgagcctgctcatcttgagctggctgtgcagttgcttcttcaacagtgtcaggaacttcagtcactactggctgaggctgtaccggatccgaaccagtgagaacctcaccattgttcgcagtctctggcacagtaccagcttcacgagcttcctgaacttcttcagccttttgggcttggttgttctggaattgagtgctcaggtctggatcaacctgaccaatgctaccatcataatggatggtgatctggctcatgtcggtgataccgtacttgtcacgcagagcttcacgagctgcttcgtagtaagtaccagcagcaatctggcccagatcggtgtagccatcctgaatcttatggccttccggttgtaccagaacttctttagtctcttcgttgaaactgaggtttgcgatagtggtcattgcattttcctttagtgatgatcataaccaaaaaaaaataaacgcctacccggttaagggtaggcgttctattatgacaggcaatactctgcattgagaatatctttgtacatctctgggtcagccttctcaatttcgataggcttgcccagcaactggcttaacataaacgccagaaggttgctacgagcaatgtagtacagttgcaactgatactgcttacgcatatcgttcgcatagtttggaagacaacggaagcagtcatggattgcgataacctcaaatggtttagctggcagagaagccaacagttctttcactggttccagttcaattaacatgatgttgtcatagtctagccagtgcaggatagcagcagacaggtagcctgacttctgatagtgatcccacaggatacgaacctgctgggttgactcatgttcaacaacagcaggctgatagccagcttctacttcaccgatcatacgttcaatcaattgaacctgagtacggttatagttgcagcgacgagacatctcacgaacgatcatgccatcaatactgtgagtagtgttggcacccagtgaacgaccttcctctgttggttggttcaccttacgataagtctcgtatggtgcgttctggaagtgtactgtttcagctacgctgtcgattactttcacatgaacgtggaagttatctggcagtacccatgagttacagaatgcttctgggttccacatattcagataggctttgttcagttcccatgctgctggcgctgagtcatccatagtagactcgaacacttgcagcagtgcaccttcaccgaatacctgctttggaatagcctgtgagccatacaagctggtcatgattgcctgcttggtgtcttcacgtttgatcttaccttgctcacccagcttacctaccatgcgatgatagataatggtgtaggcatcagcacgtactgctttgccagctacatcatagatgttgatgacattgcacagttcagcagctttacggtcgccagtgagacaggccagaatctgcaagccagatgacgttgcatccagtgatacaggatagccacttggctcacctgcatgtgcagcgttcagtgctttgatgcctgcatagaacagagcagggttatcagcctcacgcatgaatgtgtgaagctgttctttattcttctcgaaccattcgatacgctgatcccacgttttcttgtccagaccaacgttggatgcgatgtcgattttcagatagtctaagccattaaattgctgcatattcgcctcttgcaattaggttaattagtgaaggttctttttgagatcttgcatcagggaatcgaatccctgttcacttggttcattatcaatcttcccctgtgggtcagactgatgatcttccagacagtgcactaagaagctaattagctcctttaattcttctgggtcagtagagagtacaacgccagttggctgaccagtacggcagtccaatgaactcatcaggacagtaccgtcttcgcctacctcaaataaacctctattgttacccatctgacatacagctttgaacagtacagcttttggtttactgaacattggttacttcctcattagcaaattcgatgacagccttgttccatgcattaccttgataggtgacatgatgaccttggcagtatgtacgtccacgtttgtcgtaacgatgtgtcagatagaatacgtctgactcctgcaacagtacgcccattacgtccttggcagtctcatcgtacttctggaatgcacgtacacgtttctgaaagtcctctttagattcaccttcttttggcttatcgagattagcccatgagttctgcaccatgttggcagtatccatgttcagtttaagaggaatacggttcattctgttgatatgatcaagacatacatcatcatcatgatggttgtctttcagaatgattgacttatgactggtgaagtagcctgcttctttgttcgaggttacttcttttggttccactaccattggtaatggatactggaaacgatctaacagtgcttgtgtgtcagcaccgatagggaattgcacaataaagatagaccaacgtggatcatagatgaccagttgtgcatcgatagccaactgaatgttgtctaccacttcctgtgctttgtcacaatggtgacgtagtgtgcctactaacgtaacgaggtcacaccgtttgtgcagagccatctgcactaagaggtcaataccgaacttgagttcaagtccagcagcttcaatgtgagccttaaagtcccagtctgcacattcttcaaactctttcctcatacgaggcatgagctggtgattggaatacagttcttctaaatcaatttgatgttgttggagcttattcattcgcatctttccttttacatcggttaaattaaatcaacaggtgagttaggttcaccttcgaagtcacttgcaggtgacttgacgtacagagactcggcttctgttaatacttcagcaggcttcataccgttgtcccataacaggtcaacagtgcagaagtaggcattcttctctttgtgtttccacaccagacgatcccattcgtctacgcctttgaactctaagttctcacgcttaacagttggattactcattacttggttccccagtaagtagcttcatcgcctaaccacggcttccatgcttcatcgaactgacagttctttggagcacctttgaacagaggagcgatttgctctggtttaaagccagccaaaccgcaaccaatctgagttacttcaaagaccagcttaggatgaccaacagcgtaagccagaaagccgtacacgtaagcagtaacgttctccaagggtaacgtttgaatacgttcgtctttggttgggatggcgaaggagtcgccatagtgtccatacgattttccataacgagcacctctttgtttgtaagcgaattgagctgcacctgcaccatgcattccagcttcattggatccaaatacgaatactttaccagccatgattaactccagaattgagaagccaccaatagctggtggcttaaattacatgcctttagctttatcagcttcggctttctcttcgacttcctgattatgaatacgaaccagaatgtctttgcactgttcagtgacagtttcacctacagcccacattttacggtgaggttcaaagcgttctttgtccttcaccacacgatgcagtgctgtcatcaccttgtgcagaccatgacggtctatgagttcttctaactcgtcgtccacttatgctccttggttcccagcaattgctgctaacaccagacgtttaatgacatctccatgacattcttttggagaacaataacaaaccaaaagaactggaagaccactgccatcgagcacctgctctgcaatcttattgagagcatttgcgatcacaggatcattggcatagatcttacgcttgaggtaaggctcgaacgcattgataacatcaatacggtcaacaatatggttaatctcaaagggattacctaatgctgacggtctgccaatataatggtgacgatcactcatccccactttgtggtgcttgttcactacttttagttcgttcacgttgtgacaccttgaatggataaacaggtttacgggactgccactggttcatcatgatttcataagcacgaggctctttatcagataagaacacaacgacaatatcgatgacttcaggtaattcagagacaagttcaacctcaataccagcacttgccagtattggttcgattacattctctacaccttcagcacgagtggtaataaccttgaactgttcaggcaatgccttcactttaaataaatgttcaagaccactcataataccatcggtatctatataccaactgtcacctgttactaatacagttttcatttgtgtttgtttctccatgcagtcatgtcatagacagttgcactattaagtacagcaccgttgtgatacacagctttcttacgagcctgctctaatttcatttcagtgaaacgagcaaccacgacatattcaactccgtcatgactgaacttgagttctttctggataatacgcatagatcaccaatgcgagcatttgccaccgacaggtggcaatagcgagttagagttttgttcttccacgaatgcgaatagataattcacgctgcatagactgcttcatatcataaagccgaatggcatcatgaatttgtttagtctcttcgggattgtgcatcttttgtaatatgcgagagcacttacgatgcacacgtttatttcttggttcaccacagatttcacacaagcaattgagtttattaagcaacatagttacacacgtagacaggtttattgagtttctccatgtacgctatcatatgctgtgtacccggtgatttaccatcccagaatgcaataagaatatctgcgaagtaggccatttcacggttacggatgaatccagcacctctgccttgaccgtcccagtcagcaggaaattcatgaatacgaataccatattctgtgaacaggtgatgtgcagtaatatcagcacctcgtgccataccacatactaattcacatggctcggtgatgattccatttttaacgaggttctgcataacattatgcattccctctttattagtgtagtcacgaccaccagccacaattattcttaatactttcttacgagcatattcttcagcagccttacgctcatttttaccgcgacagtttgcacacaagtgatctacacgcgacatgtagcctttgccgcaaagacaatgcttttgaaatggatgccttgggttcaacatttaatttatcctctatccagcttatacgcttcttgtttagatgacataacgagtaaatacattcttttttgtattcaccacaggtattgaatgggaaacgataatctaagttatcgtctttaaacatttccactaactcatttgctactctgtagtagatatgagtcagtttatttttctcacaccagcgtgagaggttttcacacagaccagcatgtctgacgaatacgccacccattactggatcttttagccagcgataatactcgctgaggaatatttccatgagtccactcatactggctgatccttttcttctgtgattaattcaatacagatgacttccatgtcctctttaatacgaggaactttgggatgatatacacagatgccatcttcccattcctgacgatgcacaccacgtagccacattctcaatgatgccagtgcatctttttcagatgtgaataaacgaggagttgcatatttgttgtcgcagtcaatatcaatttgagtatgaccacgacctttaggattagcttttaacagcttacctgttggtatatgtcttattgcccaaaggccactaagcactgtttccacgaggatgtttctccatcataaacatggttaattcctgaagacgtttcattgtctcctgacagcttctgcccattgagaactcaatagcttctactggttcaccttctttatctctggctccccagttcgcatagcagatgaagttgtcattggcagtgccatcatcttccattgagacgatgatattgttgttgttgaagaaatcagcttgctctttatcaatctgagtaatttcgatttctttctgacgaccatgaggtctttggtagaaaatgacttttagcatttgataatccccagtacgttttctttctggatcacagttttagacaggtaatccagtccatgttcagctacatgaacaaggtcattgtccacaatgattttgatgccttgtggtgttgcaccagcaaatgttccccagaaccattcgcgtttaccactacggctgagcacacccagtttcacgaaatcacccatcatgagattggctatattttgctcacttggttctagtgcttctggtggtaatttgttcgattcatatgacttcacatgaacgaattggctgtcattctttaacataggtttatacccgtttatagtcggatagctcgtaaaatcctactttagtatttagtacgagactatccgtattagaaataagtagaggctcccgaaggaacctcacacttgttagcccagcagatttacctgacgagcaaatggattatttgcagggtcaattacctgttcagtatcatcgctgacacgacgaacctgaacctgaatgttgaccagtgtttcatcgcccggttgcagagactgagctgctgcaatgagctggtcgagcagaccattacgagctgactggaatgctttccaatgctcgtttttaccactgattttcagatgttcctgagtatccaatgggataccagttggcagtgagacgaatacgtcttcaccatctttgccagcaccttcggctacatagcctacgttcagccagaactgagcttttggcaggtctttgttatcagaggtagtctgagcagatttgttaccaccgaactggaatttagagatgtctacggtcatgatttcacttcctatttaagttgaggtttgagggattatcttggcgaataatcccattaattgcggagcaatttctttttcgaggaagaattaactcttcctatttatgtcgtctttatcgtattcaaaaccatcagttttggatttaggataaggacagaactggatgaatagtccaaacagtccagcaccgataaacacgttaccgattgcaggaatatttgttaaccagttgaacaggataccgatgatgagtaggactgttgagagcataggattatccatctgttagaaataactttgggtatctcgaatgagatacccttttgaggttatttagatttatcgaacaggttacgaagacgagtctggtttgtcttatacagttcagcagtttcttcatcttgcttgcagaaagctaagatcttcttctgacgttcagtatcttcgacagcagtgtcttcaatgagacgttcacgatacgtttccatatcgatagttgcgcggtcagcttgtttagtagctgcgttagttacgaatacatcaagcatagatacagctttagtacctgcattgagtacagtagatacagtggtagctgcatcagatacagttgacagtacagcaccaaaggtcatacgagtagtagccatgagtaacactccagttagattgaggcaagacgccataccatgcggagcatgtgtagacgtgtaggagtgtataccgggggggtacttagtatgattgggagctgcgcccccaagtgtagtgctgaagtgggacatacatatcagcaaaatatctatatctacaaagttagttctaactttatattgaggtaatagaaaaggactccgaagagtcctgtctatgctgaatcaagtcctgtggtgaagcgaagtgtccaccagaatctaaatggtggtaggaggccagaactcttcagttgccagtgttatatgccaccgctggctgggctttgcagctatcgtacctgtggagcacagtaccatagttaaaattagataggtaggattattctcatccttggttcctgttaaggaaccataggggggtgcctccaattccaatagggaatagagtagacaagagactaaatataccctataaggtaacttgtcaatccaacatatatgagagatttctaaatgactgtaccaactgaagaagaattgcaggcagcagcagtggctccacgagttaagcatgaagagattcatgcagaagtgaaggatgtggagtatgcctatctaggcttgctgactgtatgtgctctgacactgcataacggattcaaggttgtgggacaaagtgcatgtgcttctcctgagaactacaaccgtgagttcggtgagaagtttgcctaccgtgatgctgagcgtcagattggtgctttccttggcttccgtatttgcgagcagcgttataaggatgagcaggccaatgatttggtagccggtctgtcagagggtgattgcgaaggttgcaagatttaatctctcttctctggatctaaatagggggagccagtggctcctctttttatatgaggtacaccatgcttactcagcagatgattgaaaaggctttgccagccaacctgaagaatgctgtcaaccagagtttggttgatatggttaacaacgcctctactgacgatgtggttgctgagcagattcgcaataactttgtcagctataccggggtgctgaaagacggcaagtataaggcagaggactatgtgaatgctgttgcgtttgtgagttacaaactcatggggcaaagcaatcaggatgcttacatccgtaccttccctcagcgttatcagaaattattggctgaagggcgaaccagtaaagacattgcggcttacgtgagtgcttatgcacgaggtaagttagtgaacgccattctggaacagtcactggtgccttcttgggtactgaatcaggacttgcaccagaaggcgattaaccgactggctgatctgatggtcaatgctgtgtctgaaaaagtgcagagtgattctgcctcggcactgctgactcatctggctaagccaaaagaggtaggcccactgctgaacattgatatgcgtgagcagtcaggcattaatgaactgcgtgacctgttgggcaaaatggcacaaggtcaggtacaggcactccagaatggtgagtctattaagagcatcactggttcccgaatcttcgagggtgaaaaagatgctggctaaaaaggaactagaccaatggcttgatgaggtcagttatagctatcttaactctggggagtatatccccactgagtttgctgtaatgttcatgaacttcatcaagctggttaatggtgtcgaaggtgaaagccataaaacacctcctgttcaccttgctatgttagacaaagtggtaggtaagtcccagtacattgctaacttatgtttccgtggtgcagcgaagactacgttgttcatggaatactttgcaccattcgttgctatgttcgagggactaccgggctttggtcgtattgatgggatgatctatgtatcagactcaatggataacggcgttaagtcagctcgtaagaacattgagttccgttacaaccaaagtgagttcctacaagagtggctaccagaagccaagttcactgataactacatcgagttcagaaacaagagtgggcatcagttcggtatcaagatgtttggtgctaagacaggtctgcgtggtacgaagatctttggtaaacgtcctaccttatgtgtgcttgatgacttggtatcagatgatgatagtaagtccaaggtatcaatggaggctattaaggacaccgtatataaaggagtaaaccatgcacttgatccaaccaagcgtaaggtaatcttcaacggtactccgtttaacaaagacgacattctcattgaagcagttgagtctggtgcatgggatgtgaacgtttggcctgtatgtgagcgtttcccttgtactcgtgaagagtttgttggtgcatgggaagaccgtttctcattcgactatgttagcgagcagtacgacatggctgtgaagacaggtaagatctctgccttcatgcaggaacttatgctgcgtatcacctctgaagaagaacgtcttgttcaggatgctgagattcgttggtataaccgtgctcgactgttggcgaaccaacatgcctacaactattacatcaccacggactttgccaccagcaaaaagcagaccagtgactactcggttattgatgtctgggcatacacttccaacggtgactggctctgggtagatggcattgttgaacgacagacgatggataagaacattgatcagttgttcaagtttgcccagaagtacaagccacaggcagtgggtgtggaaattactggtcagcagggtgcctttattcagtggctccagcgggaaatgattgaccggaatatctggttcaactttgccagctcgtccaaatctggtgagccgggcatccgacctgagacagataagctgtcacgctttaatctcgttgttccttggttcaaagcaggtaaaatctacttcccagaggagatgaaacagtcacgagtgatcgggattactatcggtcagattcgactggcaactcacagtggcctgaaaggtaaagatgactgtatcgatggcatctctatgctggcctacctcaaaccattcaaaccgtctgagacacctccgattactccaacggaagtaaatcgctgggatcaggaagtctcaaacgatacgggtggtggactttcttcttatattgtatgaggtataaatgaacatcgaagaactgtttacgaacctgtcctatggggaactgagcaacctttctctgtcggctgatggttctggttcgatccaagaagagtcacagcccaagatcatcctctatgccaatgagggtctgaacgaactgttcaataagttcgtgctgcttgagaaagacgtgattatcgagatggttgcacacatcaccaactatcactttaagaagcgttttactgagtcgggctttgatccagagaaagaacattacccctacatcaaggatttgattaatgagccttttgaagaggacatgatcaagattctggcggtgtataattcctttggttccaaagttcctttgaacgataatgaacgtgccgactcggtattcactccacagaatactgttctgcaagtgccacgtccgattgatcgggcagccttgagtgtgctgtatcaggccaagcatcctaagttgacactggatgatctgagccaagaaatcctgttaccggattgtctgcacggcgcattgacagcctacatcgcatataaggtattcagtcacatgaacactgaagtaagttccgggaaagcacaggaacacttccagatgttccaagctgtttgccagactgcggtagataatgacttggttaactccagtgtctccaccacgaatactaaattccgcaaaggcgggtgggtataaactatgcgaacagtcttcgataatccgtactgcggcccagatcatgtgagccacacagcactggtcgataagatgatcgggaatgcgtatcagatcgtgaaatatgtagccatgaacatggtctacgtgaagcatgtatctgatcagcttgagaatgtgtacaacgtttctcagcaattgcctgcaattctgtcggttaacatgaatggcttagccattgccacattagccaacatctcagccgatgtggttgtcttggctcagcaggcaagtgctattcaggcactgaacactaaccttacgaaactcttagatcttcagagtgtgcagggtcagttactgttgcttcagccatacgcatcgaaacttgcagatatgcagtctcaccagacgcagtatctggcggttgcagatgctttacctgcgattaacgctgtttcatctaatttgcagatgctacagactgttttcgacaatgttgatgcgttagttgcagcaggccagaatgctcaagctatcgtggcagtgtcagaagctatcccggctattactgccgtgaaccagaatctgacaatgctgaagtcgatcaacgataacctgaccagtctgacgccaattggcaccaacattactaagctggtggcagtggcagatgacctgacagctatcaatgatgtgcaggcgaagctggcagtgattgagtcagtgaactctgacctcagcaacatcaatgccgtggctctgaacattgccagtgtgaatgcagtagctgcaaaacttcctcaattggaaaccatcgccaccaaagtagatggcctccagtcgcagaagacagttacaggcgtagcaccagcagtatctgcctcagtgaacattgcaatgggtacggctgctaccacagtcaaaggcgtgaacgtttccatcactggttcagatggtacggtttacttcccaagctcaagcacattctcctattctctcactggttccaatcttgtggtgacatctgctgcaagtgctccagcgaatatggtaggtggtgcagtcaatgctctgctttcttacaccccagcagcataaggaacggaaatgacttataacgaccgtaagtttttccgtctcagcgatcagtggtcaagccgccgtatccttgaccatgctggtaagcctgccctacgtgggcagcttaaaccggatgctctttcctttggttcagtcacagcaggaaacctgtctgtgatccagaaagctattctgaccaacactggctatctgccattgcaggttcaggaagtgaagctggttggtgattatgtggtttcacataacctgcctgtgaacggagtcattccggttgatggatcagcggagtttcagattcaatttgcccctcagcgtgcaggtattgcaacaggtggcctgtatgtaaacacgttggactctgatggcgatgaatttgttgctctgcttggtaatggccttgcatctggtgtcggtgttgctaccgtttcgccaagctctctggcttttggtaacgtcaccattaacacttccagtgctaatcggactgtcaccattaccaactctggtactgaagacctgtatatcactgggatcactgtcacaggtgagttctccattacctcgacgagtccgattacgttgggtgccggagaatcgacaactgttactgtcaaattctcaccacttactgttggcgataagactggaaccattaccctcgctcacgatggcaacggtgctaccactattgggctgactggtaagggtgtgactgcttcatcgctgcctacgctgagtatcagcacgggtgtgatcgagccatacacaggaacagcttcagtttcggcatcaggtacatcaatgagttttgaggatacgactgttggcagcattagtgctgcccagtccgttaccttaaccaactctggaacaggagcagcccagattactgggctgtctttcgatgcgtctgtgtttaaactggcaagtgacagtgcgaaagtgggtgattcaattccggctggaggtactgcaattgtgaaagcaatcatgcagcctacctcggctggtgatttatccggttcactgaccatttccactgatgcaaccgtaggcagtacgtttatccttgctctcactggttcagccttggctgctccagtggtcatgaaacgtttgagtaccagcggcaatcagtttgtagactcagatggtaaaaaagtacgtctgaactctgttaactggttcggtatggaagatacgaactacacgccacatggaacttggattcgtccgtggaaagacattatcgatgatattgcttctatgggttttaattgcatccgtattgctttttctggttcagctaccagtgccggacgtactccaccagcatcagccattaacactgaggctaatcctgatctggtgggtgtaagttctctggatattctggatatgtatgtcgattattgcaccacgaaaggcatctatatcgtattggatcaccatcgtcgtacagcaggttctggtggtactcagggatctccgattgccagtgactacacacttgatcaatggaaagcatcgtgggctgttatggcaaaccgctatggcaataaccctacggtagtaggcgcagaccttcacaatgagccgcatgaactgaattggactacttgggcaggttatgcagagcaagtgggtaatgccacactcgctattgccccagattggatcatgtttgttcagggagttggtgcaaatcttgatggttcaaatgcgtggtggggtggtgcattgaaagatgttgcaacccgtccggtagtgctgagcaaaacaggccgactggcgtactcaccacacgaatatggtcaatctgttggctctcagtcttggctctcaaccgattctactgccgtacctaactacccgaataatctgtacacaatttgggataccaactggggttatatctttaaaaacaatattgctcctatctggttgggtgaatttggtggtaaatttggggtagacggttctggtactgtaaaccagccaaatgcgacccctgagaaacagtgggtacagaccctgatcaagtacctcaatggtgatttcaacggcgatggtacgtctgatctggctgcgggtaacaaaggtatgagctacgcctactggagttacaacccaaacagtaccgacacaggtggattactccaagatgattgggaaactcaccaaaccgttaaactcaacctactcgcacctctgttggctgcataaggaaacctaaatgcgacaagcacgatttactgtaacgctctcaaaggcgtctacagataccgtgactgttgattggaagactgtcgatggtacggcagtcgctccaagcgactatacggctggcaatggtaagctgactttcctacccggtgagctatccaaggacattattgtcttggttcgtgattatgctgccggaaccaatgatgagaagttcaccattgagttaagcaatgcttccaatgccacgattcttgcaggcactggtggtggcgtaacgattccgggtgatccggctgcactgccttcttatctggatcgcttcaatacgatttatacggctgtgcacgataccgacaacggttatttcggcccagaaaatggggcatctgcgaaaactgtaccgtatcactgcatcgaacgtctgatctgtgaagcaccggactggggacaccaaactgtgtctgaaaccgcctcattctacgttggtctggaggcatttcatggcctgctcaacaatgattgggctggcttcaacatggcgtggaacacgatcaacaatatctacgtgccgagtgctgcgaaccagccaactcaggtgtatctgccagcaaaaccagcagattacacgccagaaggtgacactccttcggcatatccggtattgggtgactcgactgctgcacatggtatcgatccactggcagatgaactggaaaccacctacggtgacaagcaggtttacctgatgcactggatcatcgacgtggatggtcgttatggctaccacaatggtgataaatctaccctgaacgtgtacatcaacacgtatcagcgtggacttcaggagtcggcatgggaaaccattccacagcctgagtgggaagacttccagtttggtaatacctacggctatctgccgttattccagcagggtctgccactgtatgcagcagcagagaacgaatacggtaagcagtggcgttatacctgtgcaccggatgctgaagctcgtgccgtccagtgggcatactttgcgaataagtgggcattagcaggtggtaaagctggtgacgtatcaacgtctatcggtcgagccaaaaagatgggtgattacctgcgatactgcttatttgacaagtatttccgtaaaatcggcccggatcgtgcacaaggcagcacttcagcagacgtgtattcagcatgtcactacctgatttcttggtacgtttcatggggtggacaggtgccaacctctgctggtgaagcatattggggcttccgtattggatccagtgaagcacacttcggttatcaggctccagacattgcctattacatgacgcagactggtgggggcatggttcctctgtcaccgactgcatctgatatttggcttggctctctgtaccgtcagcttgagatgatccgttggttgcagactgaagctggcccaattgcgggtggtgtgtcgaactcatggcatggtcgttatgaaacgcctaacgatggtcgtgataacttcaccttctacggtatgcactatacctatgcaccagtctggcatgatccaccgtctaacaactggtggggcttccaagcatggggcttgggtcgtgttgctgatctgtattcagagacagcaagcaaagctactcagttggcttcagacgtgaactttatgtgtggagtcatcttggatcgctttgtgaactgggtgatgaataacatctcggtagacactgacaacggtacgttcgtactgccggatacaatgagctggacatctccaactcagaactctggcacaaccaacaaggctaaccttgaaggtgtgtacgaatacatcccgtcaatggcttgggacggcacaggtgatcatactgctttctggtctgagacttctgtaccaaatccaaagctgcactttactgttgtggctactggtcaggacttgggtgttgcttcttctctgtcactgttgctgctgcactatgcaaacgcaaaacgtgtgcagaacaagttcgaccaacccatcttcactggttccactatcacggctcgtgatgtgtacctgaagaccaagagcctgatggatgtaatgtgggctaacaactgggatggcatcggcctgactcgtgaagagaagcgttcggattacaaccgctataaccagcaactgtatatccctaacaactactcaggtacaatgccgaacggtgacttgatcaactcaagttccactttcatcagtattcgtagttggcagcgttccgatccagactggcctaagatccaagcctatctggatgctcagagtgaggccacgattccggtgttcacgtatcaccgattctgggcacaatgtgagtacgcaatgtgttgtggcactttgcatcactacttctctgatttaaactaagaacgttcctactaccgaacgggagggagtctgaataaggctcccttttttaatgccacggggatactaagcaatgtcagataaccttgaattacacgttcaaatggcccgactggaagaacgtatgaaagtcatgtcagaaggtctgacattggatcgtgaatctcgtaagcagcaatatgagaaaatggaagagatctcaaagctgattgtaaatatgtccggtcgagtggagtccgtcgagcaaggtttagctcgtagtgcaccaaccatcgaagaatttattaccatcaaacacaaagtggttggtgccggattagctggcaaatggatgtggttagttgctggttccgttattggattcttattcacgtttcgcaaagagattatcgcatggctttcaaagtgatcgacaactggaagcgagcacataagttcgcatcaatctggtggagtatcgctggtgtagtggcaatgttgctggagattttgaataacacttggttcagtctgccgaaagatattcaggataaagtccctaatgcctcttacgtcagccttgctctttttatcgcaattgctgttgcccgtgtaatcaaatgggtacgtccagaggaaaatgtggatggcagtcagtaaaacggtaaagacaaccacaggaatcggcagtgttgctgctgcaatcattgcagcaattttcgctgtcgaaggtgggtatgtgaatgacccaaaggatccgggtggtgaaaccaaccacggtatcactaaaacggtagcagttcagaatggttacacgggaaccatgaaagacctgactactgagatggctacctcaatttactataaggattacatcgaaaaacccggctttgttgggatgattgatgtgtctcctaatgtgacttggaaactggtagatgctggcgtgaatgctggcactgctcgcccttctcgttggttccagacatcacttaattccttcagcagagggggtaaggactacccccaaattaatgttgatggtaaagttggtgcaggcaccattaaggcatacacctcactccagaaagtacgtggaaaagtgaaagcctgtgagttgatgctcaagtctcttgatgctcagcaagccgtttactatatgtctctgaccaatctgtctcagtacacagttggctggatggacaatcgtatcggcaacgttccttacgctaactgccaacaggaaaagtaaatgccaacaaccaatgcagtacggtatgtgctcattggtctggtagttgccctgtttctcggcttcctttactggatctggggacagggtaacgctcatggcaaggatgcagtccagacccagtgggataaagaaaagaggctgtataatctggcaattcaggctaccaaagaccattatgcagtgttggaagccgcaaatagagccaaaactcaggaacttgaagatgagctttccagccaaaatgcccaacatgaagctgccattactgctgctaattacgagtttgctgaccgcttgcgccagtcagaagccagagccaacgtatataaacgtatgtccgaaggtggatccactcagtgcacagctctcgcaagccatgcagccgaactcgacagatctcttgaacaaggccgatctttggtacgagaactcagggaaactcttagattccgtgacgagcaactccgggcagtaagtgctaaattgctcgctgaccgtaaactattaacttcggatgatgcagatggacgaaaaaatcctaccacgcaccagtgaagaagcccgtgagaagctgacggattgggacaatgaacccactttacgccagcttaaaacggactttgataatgccaaacctgcccatgatagtcaggttggtaagatcgctggttggaatgacctgttaaatgtcaccaatggtcagaaacctccaaaggttaaaggccgttcacaggtacagcctaagctcgtaaagcgtcaggctgagtggcgatactctgctctgaccgaacctttccttggctcaaataaactgttcaatgtcagccctgttacctttgaagatcaggctgctgcgacacagaatgaactggtgcttaactggcagttccgtaccaagctcaaccgtatcaagctgatcgatgagtacgttcgttcagtggttgatgacggtactggtattgtgcgtctgggctggaaacgacagaccttcccgatgaaacaggaagtgcctgtttattcctatttccagattcaggatcagcagcagttacagcaattgcagcaggttatggatttgaaaaatgagaacccacgagggtactcagaacaggttccacctgagatgcaggcagcagtcgattacttcgaggctaaccaagttcctgtcatggcacagcagacaggcaccgaagaagtgacgattgatcaggttgttgttaaccagccaaccatcgaaatgatgaacccggaaaacgtctatatcgacccgtcatgtaatggtgacatcgataaggcaatgttcgttgtgatctcttttgaaacctgcaaagcagacctgaagaaagagccaaaacgctacaagaatctggacaaggtagactggcaaggcaatggcccaaccacgaaacctgaccatgcaaccactacgccaacgaacttcgagattcaggatgaacttcgtcgtcgtgttgttgcatacgaatactggggctggtacgacattgatggcaacagcacgctgaagcctattgttgctacttggatcggcgacaccatgatccgtatggaagagaacccattcccggatgagaagctcccgtttgtcttggttccatacctgccagttaaacgttctgtatatggcgaacctgatgcagagatgttggaagataaccagaagatcctcggtgctgtaactcgtgggatgattgacctgttaggccgttctgctaacagtcaacgtggcttccagaaaggtatgctcgatccactgaaccgccgtcgatatgacaacggtgaagactacgagtacaacggttcaggtggtaatccggcacagaacatcattgagcacaaatacccagaacttccacagtctgctttggcaatgctgaacttgcagaaccaagaagcagaatcactcactggtgtgaaagcattctccggtggtgtatctggtgatgcttatggtgatgtagctgctggtattcgtggtgcactggatgcagcatctaaacgtgagatggctatccttcgtcgtctggcaaaaggcatggtagagatcggtaacaagatcattgccatgaatgctgtgttcctgtcagaagaagaagttgtgcgtgttaccaactcagagttcatcacggttaaacgtgaagacctgaaaggtaactttgatctggaagtggacattgccactgctgaagttgataaccagaagtctcaggacttggcattcatgcttcagacacttggcccgaatatggatccacagatcagcatgatgattctgtccaagattgccctgctgaaacgtatgcctgatctggctcatacgctggcaaactggaaaccaactccagacccagtggcagaacagatgaagcagctcgaattgcagaaccagcaacttgagaaccagaaacttcagtctgagattcagcttaacactgcccgtagtaaactggctgatgcacaagctgataacgctaaccttgagttcgttgagacagaaactggcaccaaacatgctcgtgatatggagaaacagaaagcccagtcacaaggcaaccagaatctggaaatcaccaaggctatgctgaagactcagaaaaagcctgacggtagtgagactaaaccagatgtagctgctgcatttggctacaaccaacttagtgataagttggatagtgctggacaaactccagtagctcccactatcatcaaccgcaatgcacaagctgctggaaatcctcagctatcccttggttcaggtcagttcgatcccagccaagatcctgcgttaaacccaaacctaaatatgtaataggaagattaaatgtctcaggtacaagctcttgaacagcaattgaagaatgctaaggaactcgttgcacaacgcgacttggcaatcaaactgtcagagaacccagatttccgtaagctgattctcgaccaattctgcaccactgaatgtgctcgttacgttcaggcttctgctgacccagcactcaatgctgaacagcgtgcagattctctggcaatcgcacaggcatctggtcatctgaaacgtttcctctctgtgatcgtcacaatgggtaatactgctgcccgtgaaatcggagaactggaagatcagatcgaagaagcacgagtagaagaggacgcataataatgagtgatccgactgagaaccaaggggtaactcagtcggacatgcttgccatgtccgatgatgatttcctcaaacagaacccaccttcgtcttccaagccagatcctgaagaagttgagactccttcaactgaggaacctgagccagcaccagtggaagaagaggaaggtaaaccagcttctactgaagataagtctacttctactggtaaagtagaagaaaatggcgataataagcaggtgactgaaccagttgagactgagcagaaaccagctaaagctccaagcaaatcgccagcagcttcgacggaagatgataaggcgaaagccgagcaggatgataaggctaagaaagagccagcatccacggaagcaaagccagacatcgactataaatcgtttcatgatgcggtgatgaagcccttcaaagcaaacggcaaaatgattgctcctaagtcagttgaggaagcaattggcctgatgcaaatgggtgcgaactacactcgcaaaatgcaggacttggctccgaagaccaagatcctaaccatgcttgagaataatggcttgcttgattcagacaagctctccttcttaatcgacattgagaagaagaaccctgaagcaatcaaacgccttattcgtgagtctggttttgatccactggaatataatccagaggatccagataaataccttaaaggcaatcacgaagtcagcgatgcagaagtaaccttccgtaaccatctcgatgacctacgttcatctgaggatggtcagaagactgcaacagaaatcgcttcttgggatcaggccagtaaggatgtgctatggaacaacccagagatcatgggcattatccataaccagcgtgagaacggtatgtatgaccgtatcaccacggagatggaacgcttacgtgtgatgggtaagattccggctaaccagccgttcttgcagtcgtataagacagtcggggattacctgacttctcaaggtgcatttgctgacatcactggttccaaacctgaagctcagactcctgctcaacaggaacaacctaagcctcagcctcttgaaaccaaggctgccaagccaaagcccactgtaacgaacagcgataaagcgtctgctgctttgcagacaagtggcacagccaccaaaaccgaagggaaatccaaagactggcttgcaatgtcagacgaggatttcttaaagctcggcaaataaaacgcctttaaggaaatcgctgaatgttaaactacaacgctccaattgacggtcagaaatcaagcatcgatggtgctggctccgatcagatgaacacgttctactggctgaagaaagctatcatcactgctcgtaaagaacagttcttcatgccactggctaacgtaaccaacatgccgaagaactacggtaagaccatcaaggtctacgagtacgttcctctgctggatgatcgtaacatcaacgatcagggtatcgatgctaacggtgtaaccatcgctaacggcaacctgtacggtagctcgaaagacgttggtactatcactgctaagctgccgactctgaccgagaacggtggtcgtgtgaaccgtgttggcttcacccgtctgcaacgtgaaggctctattcacaagttcggcttcttcactgagttcactcaggagtctatggacttcgactcagatgatggcctgatggatcatctgtctaccgaactgctgaacggtgctgtgcagttgaccgaagctgttgtgcagaaagatctgctggctgctgctggtgttatcctgtacgcaggtgctgctacctctgatgcaaccatcactggtgaagtgaccgctgctgctggtggcaatccagaaatcccagcgtctctgattacctatcagaacctgatgcgtctggatcagatcctgaccgacaaccgtactccgactactaccaccatcatcactggttctcgttatatcgataccaaagtgatcggtgcgactcgtatcctgtacgttggttctgaactggttccactgctgaaaggcatcaaagacctgttcggtaacaaagcctttatcgaaatccagcactacgctgatgccggtactgtgctgaacggtgagatcggttctatcgataagttccgcatcattcaggttcctgagatgctgcactgggctggtgttggtgctgcggttaacgataatccgggctaccgtaccactaccgttaatggtactgagcactatgacgtgtacccaatgctgtgcatcggtgacgattcctttactaccatcggtttccagaccaacggtaagactgtgaacttcaccatcatgaccaagatgccgggcaaagaaactgccgaccgtaacgatccatatggtgaaactggcttcagttctatcaaatggtactacggtatgctggttaaacgccctgagcgtatcggtctgatcaagactgttgcaccaatctaagtgaatggggaaccttcgggttcccctatttttgaaccagataaaacaggacacgctcatgagcaccctagaaaaccagaacgttggtgataattcagaagcactggcaccagaagcagaacgcaaagcattgatggaacgggctaccatgatgggtatccagttcagtaataacattggtactgacactctgcgtcagcgtatcaatgacaaactggaaggtaaggactctactgagtctcagcctgaagtgcaggctaaccctctggttggtgaagctcccggtaaacccgtgaagaaacgtaacctccgtcagatgctggcagaggaacaactgaagctggtgcgtattcgcatcacctgtatgaacccgaacaagagcaatctgccgggtgaaatcttcacagttgccaacgagtatctgggtacgatcaagaagtttgtaccattcggcgaagcaacggacgaaggctaccatgttccattctgcatttatcacatgctgaaagagcgtaaatacctgaacatccgtaccgttaaggatcgtcgtactggtatcgaccgtgtagaatctaactgggtacgagagtttgctatcgaagttctggatccactgacaccacaggaaatccgtaacctcgctacagcacagaccgctgcgggcagtgttgagtaacagcactcattaaaaatacggcccttgattgggccgtttttatttagggtaaacagatgagccaataccagttagagacagaagctaacgccctattcacatcactgatggacggtgtggattacaagattccagatattgatctctctggatctgagttcgacctgcctgctgatattaattccgaactgtataaacagattacgaagctgagtgacggtgatctcgtcaacactttcaatgccctgatggctggtatgaaaggtctgcttcagaaggaatatgagacaggtcgtatcactggtgctgaatataccaaggcatatgtcgcccttgttggtggcacattgcagaatgctacctcattcctcttgggtcgagatcaggctttctggcaagcacaacaggctcagattgctgccattacttctcgtgtgcagttggcaacagccaaagtacagctcgtctctgtgcagctcgaagcactgaatggacaggcacagtacgcactgaccaaggctaagctgggtactgaatccgtgaactacggtatcgctacttacaacctgaatcagatgctgccattgcagaaagctcaggctgatttgcagaaccaaatgctgacccaacaggttaaaactgaaggtgtgaattacagcattgctgcatacaatctgtctcagatgttgcctgctcagtatgctcaggttcagcagcagacttcactgactggtcgccagattaaactgaccgacgagcagacagaagctcagcgtgcacagaccctgaacactcgtactgatggtcaggttgttgctggttcggttggtaagcagaaagaactgtatgaccagcagatcgtttcctacaaacgtgatgcagaagtcaaagcagcgaaactgttcaccgatgcttggatcaccatgaagaccatcgatgaaggtctgacggctccagccaacttcgccaacgattctgtgaacagcattctcggaacgctgaagtccaacaacaatatcggtgtgtaagtatgggatttagtctcggtgcgaagaagaagatctatgtttccagcgtggtgtataacctcgctggggatgaagatgatcgcgtcaactatctgaagactactgtggtcggcaaagttattgccgacacaaacccagcagttggtatggctgatgccattcaggatgctctgatcactgggccgggtatgcgtaaccgttcgttcatcaaatggtgcgatacctctggctacagtgacctgatgggtatgcagcctgccaccttatatctgggtgacagtatcgacgatatggagttggcgaaccaaatccctcacgatgctgataaacaggtgcaggtactgaacagtgagatcgacgtagccgattatggctggtgggctgacaagttcatgtatgagaaccatccagaccagatgaccactgcttacaccgtggactttgatgacaataccaaagaggtaattgtcacactggctgatggtactgtttaccgtattactccagagaactatgtggaagacggtcgatacctctactccacgtatagcctgattggtggcactgtaacaggtgacattgttccgggtgatactgttctcattggctccaatgaagagtttccaactacctctggatggacgactaacagttatgatgctggctctgccaacgtcactctggagcgtcacattactcaggtgaaatcgtactcagatggtcgccctgatgagacgacaacaggagaatcctcttcgactggcacgtataccaagatcactggtgagtttgagcgtactgattatcagggggcaacctctgatggaaccaagcaggaaacaactgctctgcgtcaaatcatgtaccagaaccagttaggcactgccgtagacggtgatcctgaagtgaccactgagactgaagttgttgggggagtgacagtcactactaccacgacaacggtgcagcaggttattcaggtgcaacggtcataccggattgataaacagacgaatatctcagctactttctatggctcagacgtgttcatttatctctttggttccggcaacagtgtgctggatgcaatgttttctccacaggtatctgctggtcagttctcacctccgatcccgattcgtatcaataacgactcgattacggataacaagtttaagcagtattatgagccttctcgtaaggcatataagaagctcaccaactcgaagttctcagagatcatcgacaaggttgaggacaatgattcgatcaaggatattgactatgcctactgtgttcttggtgtgtctcttaacgttaaagagaatgcctgcaagaagtatatctataagtggttccagaccatgttggaaacgtcaactggcgtaaccacagcttatggtgattacaaaacacagatggtactggcacagtccagcaatgagacttggcatatctggctcgatgcacagcaggataaaaacaatcctctgtacggtactgctgaaccaacgaagattccttatccgactcttccagtatcaggtatccgcatcaagtcgagcagtctgattaactatgacatcggtatctcgtggtcagctatggctgaaaccacaggtacagggatgcatgatgctacccataaagtgggtgactgttggtttgtgatcaatggtgatgataactacgagcagatcgtttacaccgggggcaatgctgcaccaatcaatgcattctcagtaagccatatcacgctgtattaccaagagacagcgaaccgttggcgagccatgaatgtctggggattgcgtcaggttaacaagatctacggtggtaagtcggttgatacagatgccaaaagtgctctgaatgacaacgatgaatcagggttcatcatcccattgcagagagatatttactcttctatctcactggtggatgcgactcagatggctacggcctgtatgttcatcgttttcaactgctatcaggttgttaagcagaagtggtatcagacgggtatcttcaaagtcattctggtcattgtgatcatcatcatctccatttacacagggggtgctgctgctggccttcttggtactgctgcctcggtaggtgcagcagttggcctcacaggtattgcagccattatcgtcggtacgattgctaacgcactggctgctatgatcttaatgaagctgattggtctggttgctgtgaaagcctttggtgcaaaggttggtgctatcgtaggtgccattgcaggggtaattgccgttgccgttggtggcagccttgcatcagggggtacagtgtcagcaggtgttgcctcgcttgcagatccaaagaacattgcagctctgaccgttgcagcaggaaatgggtatgcaggatacatggcagcagctacgcaggagataattggcgagacacagcaggtattggaacagtacaatgagcagtcaaaagaaatctctgctcagtacgctaaagagtttggtgatcagagtcagggtatgattgatcccctgaaactgaccgaggcaacccagtacatctttgaatcgtctgactcattcctgaaccgcactctcatgactggttcagatatgatggatctttcgctgtcgttgctgactaacttcgttgaagttacaacaagtaccgatctttcctattcaggttaaggaactgatatatgtcagatatgctgaatttcggtggctatcagccacaggctctaggcatgggggcgaacatcccccagttttcgagcaacaatgctctgggtgctgtagctaccaacagttggcaaaacagcaatgcctataactttggtaacggctataaccctgtagctgggaaccaagcactgaataaccagtgggctgactaccaaagcactaaaactttggatgatgctggtggtgctcagactggtcagttgggtatgaacattcctactttccaactgggtctgtcaggtctgtctgcaatcggcaacctctggggtgcgtatcagtctcagaagctggcaggtgatcagttcgactttgccaagaatatggcgaataaaaacttggctaaccagactgcttcgtataacactgcactcagtgatcgtgctacgtctcgtgcttcgatggaaggctggtctgatgctcagactcaggactacatcagcaagaataagctgtctaattaagaggtaatcaatggcccaaattacttggcgtaacgttgattctcctaacctgtcgggtgccacggatggcattcggactgctgctgcgttatttggcaatgcaaccgatgcgatccaaaagggactggcaggctttcaggattatcagcatgactctgctgctgccggagctatggctaatgcactgaagttcaatgatcctgctgcgtaccaagctgctctggcagatggttcactcatgcagggtgttgatacctcaaagctgactgctcaggatctggctaaccttggtgcacgacagggaaccctgttacagaaccaagagcaacagcagcgtaatgacatcactggctatggctttgaccgtactaagacacagaatagcaatctggatgctgcgtctccgttcattgctcaggccaacactgcttatgcccgtggcgataaagcaactggtgatgctctcatggctcagcaccaagatgctattggcaagctgacaccagaccagattatgtcgctgaacaaaggcaacgttgatctgaccggagcaaacctgctgaacacaggtcgtggtatcgataacaaccgtggagcatttgaactcggtcgtgatatgacgaactatgaagtgcagaaccgtgcgaaccagttgctgcaagacatgaccagtcgtacattcagccctaacgataagctggcttatattgaacaatatgccaactcaccaaatgctgatgcaagagttacagctctcctccgtggatcaacgccgggactgtacaacggtggtgctctgccgggtgctccgggtgatggtgcaggtgctgtatatggcaacggtaaatatggatctcctgctaccccattggacaaaggtactatgggtcaggcagtggacttcggtaagaatacgctgattccaaataccaaaggccagattggacagggtgatctgggtacatctgcaactggtacattccagattacaggtggcacgtatgagcagtatgctccgaaggtattcggtgatagctggcgtgataccccgaacactctggagaaccagaccaaactggctgaagccatttacaatgaccgtaaaggtggcgacttaacccagacttggacaagcctgaagaacgtaccgggtgcaagcactccgggtgcattcaaagatgtgcctttctcacaggtcatggcacagattgccaagggtgaatcgggtgcaagtttgcagcctcgtactgaccagcgtaaccaaggccaagctgctcgtgcagccaacgaggttattgatctggctcagggtcaacgtggtggtggcatctctggtgatgcaatggcgtctgccgtacaggacaacggtaaaacgtctcgtgctcaagttgttgatcagctccttggttccgacctgaagggaaccaataaaacatggctgaacaaccagcttgaggatattgctcagcagactggctacaacaacaactacaagatggcaggtgagattcttaaacagtctctggcctcatccgatgaaggtgttggtggtggctgggatcacttgttccgtcaggtgggtgaaacctttacgccgggtcaacgaggtgtgaacctcggtaactctcagcgtcttgaccgtgacaagctgaacactgcgattgcttctgttaagtctggctccttcctgaaagaacgtctggcaaatgctgacgtacaggatcaggattctcagaacagccagttgcagcagaaggcagatgccgatgctcagcaactccagcagttgatgctgcgtgctcaagctcagccttcactggctccgctgattccacagtatcaggctcaggctgctcaaagtcgtgcactggcaaatgccagcttgcaacagacaaaccagaacccgaactataagccagatggctttgatcctttgggtgcacagcgtgcagcacagcaacgggcagagcaggaagcaatgattgctcagcaacgtgcacaggctgctaaggtacaggcacagcgtaaagctaaccctgtcggtgattatctggatccgaactggcgaacggcagatgccgaacgtcgagcacgatatttaccatagtaagccaactaaaaaagccctatcctagtgatggggctttcttgtttcatcccctcaattcctgtaaattacctcaaacttatatcgtataaaggaaccagaaatggcgagtgtgtctgatctgttagctcaggctgccggaggcggagacttaccgcaaccagcaagtgctgatagtttcctgaccacagcagcaccgtattcctcaactgggatttcagaccaagtacagcagagtgttgctggcgtatctggatccaaacaggaatcgttagctgctgcgtctgctgctaaacagcaagcgttgggtcagtctgataattaccagatggcagagggtgctctgaccggaaagggtaataattcctccagtgaactggagaatgacattcgtacaatggatccactgagcatttacctgaaatacggtaaggatgcccagtctctgatcaatgactctgccgcaggtttgcgtcaggttactcgtgaccgtactgctcaacgcagtggtggtgaagctgcacaggactttgctctcggtgtaggtcaagggatcgttaactccattggctcaatcggtgcattgggtgctggcctctttgatgctgatgcaggccgtgttgctactgacatgatggacgaaaccaataagtggtttgacggttccaagtcagagggtgcacaggctggcaaacgtatttacggtgctgattccacactggacaaccgtgataacgaacagcaattcaagatcgatacagccaatgatggtgcctttgttgccagcatgaagcgtattggtaatgacgcttgggatgctctcagcaactcactggaaaacagcacatctttctcagatggtatggctcagggacttggttcactcgtcactgctggcccactgggtaaaggtattggtgctgtcgctaaaggtctgtcagtcgaacgccgtactatggctgctatcggtctgatggaaggtggtggtgcattccagcaagcctcttccgaaggtaacaatatgtccttcgatgacctgcgtaagaactctcctgagtttaatcgtatggttgctggtggcatggatccagaagaagcccgtactcaactggctaactctgctggcctgcgtgctgctgctattcaggctccactggctgctgccactggtaagatcgctgctgagtttgaagctgctccactggctacccgaactgtccgtggttttgctaccaacgtgggcaaagaaggtgttgaagaaaccattcaatctgccactggacaactggcacagaacctcggtatcgagagcactgtaaaccagaaccaatccttgtcagaaggtgttggtgagcaagctgcgctgggtggcctgtatggtcttggttcagcaggtatggttcaggctccgggtgttgtactgtccaagtcaatgacgggtgcactgaaaggtgttcagactgctgttaaagctggtcaggatgctacccaattcgtcatggatcgtgctgctgctgtacgtgctgccaatgagaaagcctctcctgtttccaatgagactgtttctcaggctgcaactgaggcacatgctgctgcaccagaggctgctactcaggcaactcaggctgttgatgagacacctgatctggctccagaacagaagacagaagttaatgaatacattaacgaactggcttccacactggacttcgatcattcgactgaagctactcagatgcctccggctgctgctcgtgctacagagggtgcaaccaaccgtgttgatgctttgcagaagatggctgagtttgccaacgatccaaagaacacggtgcaggatcgtctggacgtagtgaatgtgctgaatgcttatctgccagcactgggtgagttcgttaacgagaacccagaagcacttaactctctggctgccgatcatcctgctgtgcagtttgttgatggcttgcagcgtgtcgttgccggatacatgcagtctcctgcattccagcaatcacagtctgttgcagagaatatcgctaccaatgctgagaaggctggcttggttcagcctgtgactgaggaaaacatccagacgccagagggtcagaagaatgcggagaaccacatcgcaattgcggatattgcgccagagaaggctaatgctgctgcgattacggagatcctcaaacactcagacgctggacgtattcagctttcaccaaagcagattgcatcactcaagacagcagccgcactcctgaactcagcacgtcagtatgacgaggctgctaaagctcagggaatgaagccgcaagatattgtctcaatgcaaattaagacggacgagaatcgagtaggccaaggtgagcaatcggcgttgcaacacgcgaaggggattcgggcggcgtataacgcgggtaatctcgacactgctcgtacccggttggatgacttcaagctgtttgcgcaacacatgcagaacaaggtcggtgcgcttaatacccatctgctgactgccgacccgaatacgaacagtacggttaagtaccaagctcttggaaaggatcgcaccttcagggagtccaagaatggcctgtacgtcaacacgcgaagcactggatccattgccactgccaagcaggtgggactggaagctgatttcgtcgccgatgtggtgaacagtctggcctcggcctacccagaacttggtgttgaacatatcggtaaaactcctcttgacgctgcactggtcaatggaacccctgctgaaattgtcaaaggtttccgtgatggaactcgtacagttggtcagccaactcagcaagacactacggttaatgatagccctattgtcgctgaagaaaatgagaagacttctcaaactgatccagtaagcgaagccgtgcaggaagataataccgtagaggaaccagtaaaggcagaagaagaacaagctgttacacaagaatcagaaccttcacaggaagctgaaaaagaaccaacaactgttgctgaacagtatccttctttggttcaaccaaaggctggtaacaagtttcatgaggcattcaaactgcctaagactccgatctctcgtttgctcggtgccatgaaccctgtccagtgggtgaagaatgctctggcctctgttgagtccatgcaggaaatcacgggtgaaaccaagaatgctctgactaaaccagtggcaaaagcctatgcagaatacctcagcgaagtacctgccattgcttctctggttcagcaagcactgacaactgctctcaccaatgagaagaatgtcggtcagcgtttccgtgatggtgccgaagccaacacttggaaggaaatgcgtctgctgaatatcgcagaggatgacggcaaaggtggctataagctgaatgatgatctgctgcataccgcagtgatcgctgcttatcagtggctgctggaaaagaacaattacggtacaacctctgattcagagtctgtatccaagttctttggtatcagtgaagccgatgtaactgacgacatggttgaagccatgaaccaaggtctgtctcaacttgaggccgtatcttccttggctcagaagatctctaaatactggggtctgcaaggcaacaatgatgcatcgttgggctacgttgaaggcattccacaatcgatggctgctgagattattcaggcaatgatgaacccagaagtgggtgtattcagtgtgaaacagcttcgctttgatccggtgcaaggccgtctgctggaagaaggtgaagaggctgttggtaagcctaagctgttcaaccgtttgatctccagtgatctggctgaggataatcctctgctggcattccctgatgcaatcgaacgagttgttgcccatgagccagataacgttctgtacctcaatggtgatgagccaccaatgcctaagagccagctccgtaactctacggttaagctgacagctcagcagaagaaagcagttcgtactgtgcagaaccagaaatactacctgcatactccgatgctgaatttgtatgaagcactgggtaaagacggcatcgttaacctgctgggtgaaggtgatctgactgaccgtaaggatctgctgaacaagaactaccttgccactctggaaggtcgtaacttgtctatgacttctgcatttgagcagttgcagcttgtggctgctgcctctcgtaatgctgctgaagtagcaggtactgacgttggtgatgtgtctcaccagtatgcgtttaacatgactcgtgttaaccgtctgcaaatgctgggcaaacagaatcctcagtcttccaaactgatgcgtgaggttatgctgcctacttggtcaactctggatatgactaagccggagaaccattcagcattcatgttggctgttggtcagatgctgggcgtgaaagttcacaatatgccacgagcacaggccgtacagcaggcacaggacattctggataacctcactggttcacaggatgtactgcgtgatttcatggaaacaggtgaactgggatccaatgctgccgatattctgaagtctgagaataagggtaagaaactgactccaatgcagcttcaggctatcaacgaatacgttcgtctgatgagccaagatgaggcgggtcagaaggctttccgtactccaatgtacgtcgaggctgatggtatgactaacggtgttatcaacgccattggtctgctgacaactggagcatttacccaagaccaactggataacctcggtcgtggtggtgtgcagatcggtggtaacgctgagactactgctaacttcctgcgttcacagggagccaaagaagtccgtgttgatatgtaccaagcaactactgacgctttgaagtctcacctgtctacgactatgccaatgatgtctggtgacttgcagaagcaatcccgttctcttctctggttcatgaatgagtttatgaacggtgatctgactctgaacagcaatggtgacattgacactctgagccgtaacattgccaagaacccactgaccattaccctctatggatctggtgcagagggtattgcaggcaagatggttaaaggtgtgatggataacctttaccaacgtatgtctcaagctgctgaagcacaggctgctgatccaacactgagcaatgctgaagcaatgttcggtgctcgtggtgacgttgcttggaatgagttcctccagcacatgagcaatctgaccaactttaccgttgggaaagatttcggtcgtatggtgatccaaaagaatcaggccaagccaaacaatgacctgagctggcagggttacacgatgaatgcgtctgagctggcaaacttccgtggcaatatgcgtcacctgtttgttgagccaatgcgtgatgctatctctgacaccgttggtgaatcagtgatgcagtctgctgacattattcgtcgtgcaacacaggcacaaagtatcgtgctgtcaagcctgttcaagaaggctgttgatgccaaagttgctgagaagaaagctgctgataatggctacaagtcacaggagttcctgtctcagaatgagctgaatgagattctggcttcactgagcaagtatgctccactgattaacaccggtactcagaccttctacattgcaggttcagagaacagtgaagtgaccaatgtttcctttggttccacgctggatgggaagatggttatcccagccatgatcagtggcccggctgactcaggtgtagcaggtacgccattcatcgtcatcggtactggtgatgggcagatggttcagaacatctacggtactgaggatgctccagaaaactcaatgcctgtgtttgatggtatgaactttgctctggatcgtatcgttcaggatagccagaaggctaaccagtctgtgtacgatagctggctgaataacccgattaagcacgttcatacctcggtaaatggaatgctggctaacatgacaatggatgacttcccagctgatcaacatgctgcgtttgtccgtgctgtgtatccagataacctgtcagagtctgatgcgaaagcaatcagccctgctgctgcaatgaatatgctgggtgctttggttcaacgtctggctgctgatgcagagagtgttgatcgccgtcatgctgttatggacggtgccaatatgtctgtggatcagatggctgctgtgggtgctccgtatgtgacaaccggacgtgcacagtacaccggatccaatgcagacattgcccgtcagatgaatgaccatctggatgcgatcaatgctgctgtgggtgttgacgagatgaacccgatcttcacacctcgccctatgcctaagccagcaactgttgagcaggctaagcaggttgaagcagtcgcagagaaaactccgtctggtgccaaggtactgaccaaaaacgctctgactaacctgatgaaatcaggcacacgtactcagcgtttactgttcaattacctgatgcgtgttcgtggtatggaagcgttccgtgttatcactggttcccgtcaggaactgatgcagttcaaccgtgagaacggtaatactgtgccagaggaacatctgctggataaaggaaccaacggtttctataaccctgctgatgctcgtatctacctgattaacccatctccagaagtaatccttcacgagatgatccacgcttcttcaatgaaccaagtctggtatcactactcaggccgtgaccttgggccactgtctggcattgtgggtgaatcagttgaagcactggaaggactgatgcagcagttcactgagatggatgtttctcatctcactgatgagcagcagattcaaattggtcatgcccgtgcagagatccagcgagtatctgcttaccctgatgcagtcggtaaaacctatgccctgaatgagttcatggcttggacactggctaacaaggatattgcagaggctgctaaagacaccaaggttaacgtcttcagcaagatggctaaggatgctatccagtggatcaaacgtctggtgctgggtcgtaaacgtgtgccggagaatccgggtgaagacctgttctcgaatgtgtcattccactcgaccattctgatcaaggctaccccgaacatccagaactacatggctgataccgtggcacgtcataacagtggctatggtaacaatgcccgtctgcaagacgtgactgagacgtttgacaaagctgttgctaattacctgtctaccaatccaggtgacatcttccagcagtctaaacgtcagtcagagatcgatgctgcttaccagtctggtgctcgtattcaggcatcctttgctgctcatggtttcccaatgacagcacagcagaagactgcgtttagtatgatcgtatctgccatgcagactcaggcacaacttgagccaaactctatggctgcattgcaggaactgtatagccacgtcactaagacgctggactacacagcattcctgccggagaacccgcagccacaggatgattactatgctcaggaaaagtacaacgccattatgggtaactacctgacagagaaaggtgcacagggtaaatcaactctgctgcctgctttcttggctctggcaactgtcagcgatgagttccgttctgtactggctgaactgccattgccgaagggtgcacgtaacgaagatggtaacgttgatgctcgtctggaaaatgctggttcattcctgatggagaaactgactaagcacttagctggtcagcgtggtgacaacgtgaatcaagcagtagatgctctgacccagcatgtgatggaaactatcactgactctgaatcgttctttgaccagtacgctcagaaagctggtggttacgttgatcaggtaaacagcttcatggttgactctatggataagctgtctgacaaagtgatcgacaaagctgagcaggttaaggctggaaccaataacaaatacgttaaggctctggctacctctgccaaggtaatggcttcaatcgtcactgaagaaaaaggtgaagtggttgcacagggcatcatgtcagcactgaaccgtacccgtggtatgcagggttggttcgattttgtgaatgacatggttggacgtaccaagtccaatgctggtgtatacgacatgattaaagctgttcatgccttggttcagcaagaccgtcaacagttccgtcagcacctgccaactgttatcgctggtaagttctctcgtgaactgactgctaaagagtggacgctgctgcacaagtctatgggcaagtctgattcagcttccttggttcagacattaggccatgaggctgtacgcaatatcatgaaaaaccctatcgctatgcgtaaggcaatccgtgatattgaggctcgtatccgtgctgagaatccaccaacgttccacctgaccaaagccaagatggaacaactggctgagtacatgatgactggcaaaccgggtacagacctgtaccgtaatgctgagatcattgcactcaaagcaggtatcaccgatgagggctttatctctgacgttaaccagcttacttccctgtacgccatgaataaccacatgggcgtagacgagaagatcaatctggcgaacttggttgagaatgaggcagaaggtatcgactttgcccacagctacctgatcggtcagaacgttgaggagcaacgtaagatccaacgcagtgctggagccaagtacaactactacaagggctatatcccgtctaccaatcagccgggtgttaacctgattgtggcagacgatagtaactttgaccgtctgcgtcagatgagttatgagcgtgttgctgattatgagcgttcatctctggatgccgatcagactaagctgggttattactttgcacctgtctccggtaaaaacacgttcaaccaaggcattatgcagaacgttcgtgaaactgctggtggtgtggataccaactctggctatacccagtctctgactgctggacgtatcgcagatgagaaggtagttaagcagatccagcaacgtgcacatcgtggcgaaacaggaagctctctgctgcccgtattcgatgatcagggtgtcatcgtagcctacgagcgtagcgtggctcctgagcagactgagcgccttaatcgtgataccaatctggctaacatgattggggtatggcgtggtcgtcaggctgaagagatccgttcggatgcagtgaacatgggtctgattcgtgcgttgcacgatatgtacaaaaatgaccagcttcacaatcgcttctctgatgctgagtacattgatgttctggatcctcgtgagtgggcaaaagatcctgttcttggtgacgcaatgaaactgatgccagttcacatgcgtgactatgccaagaccaagtttggccctaacttctgggttcgccgtgacatgctgaatgataccttcggttatcgtgaggcttcagtcggtgatgcttggacaggtaactcacggttctctgaccgtacccagaatgctgcgaagcagatcgcactggctatgttcggcaacgatgcttacaaatacttcgtcaacactgagaagaaatggcagaacatcattcacgatgcccgtaccatgatcgtggtgaaatctgttgtggttccaatggctaacgcaattggtaacgtataccagttgatcagccgtggtgtgccactgttgaacatcgctcgccagactccacgtaagatggctgagatcaaccagtacactaagagccgtgtacgtcaggttgagctggaagcagagttacgtgcagagcagggtgtggtgaaccagcgtaagctgaagaacgagatccagagtattcaggacagccataagcgtatgtccatctggcctctgattcaggctggtgagttctcagcgatcaacgatgcttcactgccgggcgatgaagtggaactgacatcaggccgtctgtactcataccttgaggcacaggttgataagctgccaccagaagcacgagatgctggtcgctatgctctgattactcaggacactgcattgttcaaaggtctgcaacgtgctgtggaatacggtgacttcgtggctaaggccatcctgtatgacgacattaccaaacgccaaggtaagacttcagagtacgctctgtctcgtgttaccgaagagtttgttaactatgaccgtctgccgggtcgcttccgtgggtatgctgagaagatgggcttgatgtggttctataacttcaagatccgttcagctaaagtggcaatgtccatgctgcgtaataacccactgcacgcactgatgggtaacttggctccgactccaacactgttcggtaacatcggtactccggtatcagataacctcttcagtgtattggctaacggacgcctgagtttctcactgggtgtaggccaagtgttacacgctccgatgcttaacccttgggtcaacattatgagcaactaaccaaataaaaaatcccctcgaatgaggggatttcttttacttagtagtctcagtgtaacctttctcgaatacgtctttcggactccagctaatgtagccatcaaagtcgtcatggttagctgggccaccatcgatatactctaccagataacccggatctgccgggttctcatctcggggtgttacccaaccacgcagttcgttatactcaccacgagtcatcggggcagcataaacttctttgtggcagacataacgcttaacagtaaccattactctggttctccaccaagtgcttcgtaaatttcctgtgggtcttcacccatagacgaagcatgatcttcccagcgtgaccagttctctgcaagaaattctcgcagaacacgcatgtattcatcgtccatactgactcctaatattctctttggctcaaataaaaaagccacccgaaggtggctatcttatgctatttacccatagctggaaggcttgtttgagagcagcgtctaaacatttctcaggcattgtcactacggcaggtagaacaatttggatcacagtgcagagtagtattgttatgacttctcgcacccctgcgggatctttcgtctcatggaacttattaagttgaaagaaattctgcactgtgaatctggtaggtcgtactggcctcgaaccagtgacacccggattaaaagtccggtgctctaaccaactgagctaacgacctgaagatggtgggggatggtagattcgaactaccgtgtgggataacagatttacagtctgccgtcttcgaccgcttgactaatcccccgaatttgaatgggcttctcacccaattgaacatttgatctatccacgcaccttacccccgaagggatgtctcgtcgcttcaatgccagtgtcttctggcaggtcttccggtagcgaatcggaattgattgatctattaagcacgccctctgacaaaacagcacatcatcgtagcttttagctttcgaccactagcccgcagcaggctccgaacgtgggtatcgctgaacgatactgccaagtggcttaacagatcaaactggttgcttcaactggacttgaaccagtgacctaccgcttatcgggcggttgctctacctgctgagctatgaagcaatctggcaagggcaagtggattcgaaccactgacactcaggatcaaagcctgatgctctaccaactgagctataccctaactatatggcagtgctaacgggactcgaacccgtgaccactcccgtgacaggggaggattctaccgactgaactatagcactataaatttggcgactcagacaggacttgaacctgtgacatatggattaacagtccaccgttctaccaactgaactacagagtcttggtgaaatcgatactacctaaaagatatatcgggtgtcaagcctgtgcatcttcatctgtttgccatagacgagcgaatagtgcttcaccagttttaatcttgtgtcgcagatcttcgatctcatcttccaaccgggtgagttcttcgttccactcatacaggttgtctgtgtcatcacagtgaaaatttccactatctgtaaaaccactccccgtactgtcggtataaccacaacggtggcaggtgtggtagcagacatactgtgcaccgataaacggtgacgctgaatactgggcgaagaaaggttcgctgactttgtggtgattactgatggtgccacagtcgggacacatcaatcgtgttcttggtgggaacagcagattacgtgtcaggatgattggcccatcttcttctgggtcgtattgcatgttcatctccttggatcgattgattgggtggctggtgtgtgcgccaacacctacgtggcctataggagagtgaaaaattcagccccgtagccagccatagaaaagcccccttactctgggggcttattgtttttgtcttcagtcaagctgaagtacgcagcaatagcaagaacaatcactactaatgctatgtaaggagcagccgccataaccgctgctgtgatcgcgaggaaagcaacgattatgaggatacctacggtcagtatcctcattggctaccttactcgtttactggcttttgcagattaccgaacagtgatttctttggctcggcactggcagcagcatcaccggaagcagcttcagtctgtgctggttcagcagcggcagcagtttcctgtgcagcaggcttagcttcagccgcagcagtttcagttgctgctggtttgctttcaccagccgcagtcgcagtagactgtgcagccgtctgtgcaccaccattcgagtcgcttgctgcctgagtctggttcgctttctgctgatcggctacagcttcctgcttttgctcagtcggctctggctttttcttttcagccggagttgtatcggctggtttggtttcagcctttggtgctacagaagcagtaccaacggttgatttagccggagccagtgatacatcgatctcagcagtcacgccgtctgcaccacgagtgtttttcaggtcaacaacgacctctgcacctggattaacggtgatcacggtgccgatgtagttgcgaactgccagctcgatttcagactgtacgagagtgaatttcatgacttaacctcagcgaataaacgcattaaatttttgaataccggggtgtgtaccccagcatggatactggctatggcatctgccacatgctcagctttaccagcaatctcaccacggtgacgtgggaagtttgcagcggggtacagctctacagccttttggatcataacagctttggaagcattcttatctccagtgaagatcttctttgattccattgctgtgatctcaatcacgggtatccccagtgctctgattgatccaagtatgcctacgacaatgccgtaagccttcatgccagaggcagattgggaaccaacaggacactctatgaagatcaccttgcagcgtctagccacggcaatgactgccgtagccagatcttctgcacgttgcaggtcatcgctattaactctgacctgctttgcctttcccttggaagtctcaatgacttctaagttcaggtcttcaaggaagcctgtttccagatccaatgtaccttcagcaatgccccagcttgctaagctgggatcaaaacctgcaacacggatctgcatggcttacttgttgccgaagagagatttcttcggctgaccatcagacgcaccctgctgtggagcagaacgctgctgaggtttaccggcttgaccagcagcaccatctttgatggaacgcttgtcacgagtctgacctttgttcttctcaagccattcttgagcgaatttaggttcttcagcaccttcacgcacttcggcgtaggtgaagccggattcagtgtgaacaactttttcgatgttgttcacttcacgggtatcggcagtaggcacatattcgttgccttctttaaccgatttgttttccagtgatttctggatcgccagcgtgacagttttgccgataacatcggtcgccatctgcacgtttttcggaagctctttcttcgcgtcgaagtcgtagacgttgaatactttctcttcaaagtcctgatcgcagagaggcttctcagtggtgcacaggcaaatgtcatcaatgacagtgaagcccggcagcggatttttcagtgcagtgttacgtgaaccatcacctttcttcggatggaaccagttattgccgttacggtcagtaacgtacacggtttcacggtactctttaccgttttccagtgtggcgataacggtgacgttctgtgcacctgatgcagctacgccagcgtacattgctttgataacagctttgtacaggtcagtttccactgcaccaaaaccactaccacccagacggtcttcagatttttccagaccatcgttattcagtttaccgaaaggattacccattacatttctctctttggttcaaataaatttacagccttgcctgacgacaaggccacttactacttgccgtaataatcttcgagacgcttaaatacctgctgcacatcgttgtcgatatacagctctttgcgactccaaagatccattgccgaacgcatcttgccaccagcagtctctttggtgactcgcgtttggaagacatatttcacgccatcttcacgctcatcatcagtgatatgcagcagatcgttttcaaagccttccagcttcttaactggcatctgcatggtacgcacgatggttgtgaagtcggcttctacaccgaccttgcctaccgcacctttaatcggtacacggctttccatcatcattgattgctcattcagactttcatcttcgtgagctaagatggcatagcttttgcttcccgatttgatcttgtggatcaggttacgataaaagttaccgtagtcaccccaagcagactggcctgttttggttccagcatacggggcaacatactgacgctcatacatttgcatgaggaatgtcagcgtatccagcactgctccggtaacgggttcagcaccttcgatttcgtctacaaagctgagcacatcacatgcgtcagcgatttcgacattggacataaagcggtcacgaaacggaatgtctttcaagtccgtgttcagatagaccatgctttcctgtggcaagttacgcagagaggttgatttccctgtgttgggcttgcccatgatcattaagatctttttgttctgttgcactttggttcctccacagaagccctaacccaaggaaagggcttaccgtgttaaacgtgttgataacgcttggctacagtcaccataatggtcgaggagatttcatcctctgtcagactgttagacagcttcgcattgaaagccagcacctgttgctggacagtcataagatcatgaccaccatcaacgagagctaacgcataacgcagcatgtgcttgttacggttgccttcggcaatacgctgagcgaaccaacgttcgaggttatccatcgaatcaatcttggcgaagtctttcttaaactcttcgttcttactggttcgtggaataaacggcagcacatccagagtctgaccttcgtgattaaagtgaacctcactatcagcgaaagtctcccacttcttagcgatctgctcagatgcgtcatccgttggttcttggaatggcagccaagccagaacgttcttcatgaactggcgatagtcctcaacgtccagctccagaatatagttaatcggcatcacgatacggaagcgatcaccatgtccttcggtctggtggcgtttggttgtataagtcatgaacttataaccggacagcagctcatgtgcagtagcgagagaggttccactgtcaacgtcaatgacgatgcagttgaagccctgaatgacgttctctgtagcacgatgaccgttcttgaagtggtgattcacccagtgcataccatcggcctgagccaattgatgcaactcctcaaacggaacttcgacaggctcaaattcgtatgcccagttatcagaataggacagacggatcttagacaggtcagtttccttgagtgtctcgccttggaagagttcgatgccactctcaaaacgcttcttgataatgatgtgtcgtgtatgcccccaagaggtagccatagtgatcatctcattacgagcagcctgacctgacttatagaacggtaacgcttcgttcaggtcagcgtgagtcacttctgtgccaacgttagcgatatacttcgccagtttcacataggctttctcacggttgagaatacgctggaaggattcgccagactcttcaaccagcagaattgctgacatcagatgccccatctccacttcattggatccatcaacgaatgcgaatgcacccgctaatttcagagccttgaagtaacggtgagatagctcagcctttttgatctcttcatgctcaggcagaagatcagaggctttctcgcactcgattttatattcgagcagcttgataccaacctcatcctcaacaaccattttccagccatgcatggcaggatcagccagtttgtggaactgtgccttccatttctggatcgaagcaccgttacttggctgagtcaggttacggaagatctcttctgctgtctggctatggaatgccttacggtcatgttgaccccagccaaacagacaacgacgagcataaccagtatccaagaaggaatagaactggtcttcattctgaccaccatccagcagcttactcggcgtaccgaacagcagcatattggttggggtcttgccgtctacctcttcaccacgggtattctccgcagtgtttttggtcagcttctgcttaaccaaaccttgatcataaagctcaaggaacagagtcagaacatcagtcgaaccaatgaggttagaaccgacttcatcgatctgaaggttaagggaaccaacgtcaccaaggatcagcttgtgacgtaactgtttaacggcaggtggagttgcagagtcaaaggtaaatgccagcataccagcacggcgatattcgccctctaccttttcaaactcttcgttgggatctgtaccctgacgagtggctcgttcattggcgataacccagagctgtttctcggcaattaccggaacagtgtcctccatgaaacgctttttgaatccacctaaaaactcgttctcaatgatattcactgagtggcctttaccgaaaccggatgtagccaagcacaaggcatagatatttacgggaatgtccccacgatctttggtgacaatggtggcacgcatattgctcgccaccttaccaagaaagtaagccaccgtagttcggaagaatcccctatcagtgttctgggtcttgttgcacagtacctcaacgatctcttcaatcgctgggtggtgctcgacccctgttaggtcaatcattcgtgtattccaatctctgttcacacaccggggcagcgtcacagtaggcacaccgtttcacttctccggggatggttttcacgataccctttccacctttttcaaccttccagaaatggtcggctgcttccttcgtctcgaagttcttggtggatcggccctctgtttttgctggatcagcgtaatacttatacgctggtgcagaacgccacagttcttcgtcagtacaacgaggcagttcagactgcggtgagtcccatttcgtttcgagaatatcgatacgatttgagatccattgctctgtctgacgggtatcccacagtggtacgtttttataagccaaacgcttctggggatagttcggattcgtcttcgccatcatcttctgccagtcggtgaagatgaagttaatgcgaatgaaatcctcggtgataatgtccgggttcagccatttgtacagcgaaccttgggtacagtagtcatcgtctttatcgccataaacccacgtccatgcggtcgtagatttgttgtcgtgtacgatgccctctgccaccatgtcgaacttcccaccgatggtgtagcctctgaactgtcgtttggcacgctgctccagatagaccggaatcggatcctttacagcagccagttcttccggcgttgggttgatcagcactcggttaataacctcctgcggataccccatctttctgagtgagatcttgtaagactgcttccatgccttttcaatggagtcatgtaacgagtgacccaaggcacgggaaataaagtcttcaaggtctacaacttgttgttccttcggaacgcgaacggcgaggatggttgacttcaatggcttcatcaacttggtagccgaaatgtatttcggatcgtcaatgtagtcatattcatcgtgtaataaccatacgcccagagccagcggtatatcgctgttattggtaactttcacgaatgatctctcctgagttgataaagggactaacccccacaaaaagagggcagtcccatgtatcaggcggattgcagttgagctaaacggtgaacacgtttggcatagtgcaggatcttctgagcatcatagagagccttttgatcaggctttccattgcccagacgggcattcgcagtacgccatatggctttgaaaatacaaccttcatcgaaggtcagattcagtgattggattatgtcctcacactcagccatatatgctggctggtcttcccgttgtgggtgagccacccatgacaggtaataattgaccagcccacctgttagcttactctggcttggaagggcttggctcattggaagcctctgcctgttcttcttggttccctacggagccatcgttttgcacgacttgcagatcaggcttgtacgcatcagcttgtgatgcagccatgtcagcaggcagacgagagaagtcctcagtggtttgcagaccgaggtaacacataccagtgatcaccacgtcaacaacgttgacctgtgcaccgtccatgcgtttgaagaagtgcatttgcagagcttgctgagcacgaccgatgtgaacaacggacaaggtttgcgtttcgcttaccagtgttgcgttgagatccagagcagacaattgcatagtctcttcagtctcaccgaccttaaagataatcttacccgctaccagataatgatgaagacgttgggcttttttagccatgtaacatgctcctatggagttttggatggtcttagcatgtggcccacctacaaagttaggcagggggaacacatgataaaacgaccagacgaaaaaggccacatcactgtggcctcgtttacaaaacgtaacggttaagagctgatcagtttacccagtggggtaaatgtcagatgtgagccagcaaggatgttagtccatgcaccagatacgagctgacaggtcaggtcgataccagttgggttcacataattcaactgaacaatcccttcaattgtcaccatgttgtcaccgaaacttgtggcattaatcgccagagaatcttggttactcatgacctgcttaacgttgccattggcatcagcagaacggacaatcatacggaacaggcttgcaccttcagtaccacctgtgaatttaacgctgaatacagcagcagcatcagttggcccttgggtcagcagtacgcctgacatcttatacagagcagccgtagttgaatcacccggaggtgcaccagcagatccaaaggtcatagccagtggagtagccgaactggtatttaaacctttctgtgcagattgcactgaggcataaacggtagttccaccaccaccggatccaccacctgaacttgggccaaccagtttccacgttgcatcccaagtaccagcagtctggtagcgaacgtacaccttaccggtatcgttctcgattgccagttgggtagcatagccatcaccagatggaatacagataccacgcccatatgtgccagcagcagggatatgagttgtgccaccagatgcagcaccggaatagttaaagaactggcctttaacaatcaggttcagatccgtagcctgagtggtgaatgatgcagtcagaccgaatgactccatgtactcacgtacacgagcaggtgtcattgcaacagtgttcagcagagcagcaacagcttctgggttggatgcccagttgatgccacctttcttcgtccacgttgtgcctgaacgactccagataccgaggccagcagcagttgtgctcaatgccacggaaccatctgcaccgtcagtgctcgttggatcagcagtcaataccagtaccgttgtaccggaaccagtaccaccacctgtaccatcctgaccgtagtagcccacgctgtaacttacagcagtagcagcactggtcagagtcagtgtggtacgagtccacagatactgacctttggtaacagcaggtacactggcagaccatgtaccagttggtgcaatggtgccagaactggaggcttgataggcgataaccaccgtatcaatacccacaccgttattcccgttggttccatcagtagcaaagtatgccactgagtagctggtgatagcagatgcatcagtcagcgtcagaactgtacgtgtccagaggaactggcctttcgatacagcaggaatggcagcagtccatgaaccagtaggagtagcagtgccggaagcacctgcctgataagtcacagcactggatgcaatgcctcgtccagcagcacctgctgcaccatcaatagcctgataacttacagagtattgggtgacagttgtgttgttggtcaggctgaatacagcacgagtccacaggtatgcacccttggctacgccgaccggagttgatgaccagtcagaggtaggcacgttggttgcagagccaccaccctgataggagatagtgacggcagaaatgcccacaccatcgttaccagcaggagcttggaactcgatccagtgagacaaatcctgtgacggggtaacggttgatacataatcttccgtaccggacaggatccacatcgagttattaccgtctgcgttatctgcaaacacgtaatcacccggcgaatatgtctcaccagtttgccattcctgacggttgttcaggccagtaccgtccttaccatctttacccggcttaccttcgagagacgcaacccattgggcttctgtcttctttggatcatccagtgtggtgtcaaggtatgactgatagctagacttgcccggatcacctttaacggattcaccgggcttgccttgcagcgaagcaacccactgcgcctcagtctttttgggattatccgtagtcgtatctaagtacgattggtacgttgatttcccagggtttccctccttgccatcgagagatgctacccactctgcctcagacagaacggggttatcagttgtcgtatccagataggactggtacgaagacttgcccggtgcaccatcgttaccgggtgggccttggtaaatagttcccttgagatcaagggtcagacctgcaagcagagttggtgtactcatttagtgattcctcggacaatctggatctgcaccgtagttgatcgcaacgtattgccatcgaccgaggtgaatagaacgtctaactcagccagaccaacaggccagttttcggtcatattatgatacaggcacaatgacttagttgtctttggatcaccccagaaacaattcaggtcagcgattaaaccgttagcctgattgcttttatacttgcgaagctgtgcagtaggcacccagcttttaaaaaagccgttgtccactgtgtcgggaatagccattaaaaaattaaatgtctgtcccttaatgaagttcactggctcagtcatttccgatccttaactgattgtacaagcaaggcttgacgtaaggtttccaatcgcagccgtcagtgttgctgtacctgtcttggtgacagacgttacctgacctgtagctgagacaggcgtgttaggcacaacagcagcattggtagttgtccagttggcgacagcacgagcagtggtcgcagtgctaggagtaaacgcactgtcatcactgaatcgggtatagaaagcagaccagtaacgagtaccaccagcagcattgtgggtatacgttgtattggtgactttcgttgttccgttggcagtaccattccctgcactcgcatcattctgaatgcgaaggtatacggatacaacatctacctgattggaatataccggagcagagttgccattgattgcacgcagacgataagtggctgtggcattagtggcattggcaatgctcaggttgactgaagtctgtcctgctacatcagcccagcttgtgccatcagtggatcgttgccattgatatgcagtagccggagcaacagcagcaccagtgattgtgagtaaaccattctcctgatacagagactggacttgtggctgagccgagaacactggcagcggatcagcagcccctccacgagagaaggagctacgtgaactaaacgaccgagtattccctaaagggaatcggatcattgtttgaatgcctcccctttgatggttacggcagtggcattctggtctacacggcgaacgccaatggcattagcattggtaatgcctgtgataagacgagatgagccagacggaatggagatagctacgccagcaccattacgacgatattcgattgcggttcctgtgtcgttcacaaggtcaaagccttcgcaggcttgggaaccaaagacagcccagttagcaccattggatgcaacactgacagcagtaacgctggtgaaggttggcatcttgatctgagcttgcaatgcagcaatggcattgagaacaggggtgaggtcagtacctgaaccaccaccacctgttgagggtttccccgtgacgggatcgatcagaatagctgcaaccagctttaccgattcggttccatcgttgttacgaacatctacgtttacattagtttgtgacatggttgcttccccagtgtgttatcttctggggaagtataccctacttatgccgcatttaatgcttcgctgattgcttcgtgtacgtcctcttcattggctccattcttgatgccaatttcctcattccaagtcggatagaagatagagaactcaccaccgagtttcacctcttcgtgccagatgtcaggatgatcctgccagttgacggcattaacgaggtgttcgttggcgaatagcagagcaccaatatcgtcacgcaccagcatgtactgagcatcatggatgtgtgcacatggacgaatggcggtacggtactcttcactggctctcacatgccccataaattctacggatgcacgagagttcagcagacaccatgactgacccaaggcattaccagcagttctgccttctgcctcagcttcgtatggagtcttactggttccacgcactacctgcttcagcagcggagttctcacccgcagaccgaatgcagcagtgatgtaaccagttttggtagcctcgtccagcttggcgttaacccagtcgatactgactttgtaaagttccttaaatcggctctcaacgagctgtgctttctctttcgggaaaccacagttcttcatcagagtatggtaagtaccctgataagtcagtgcgaatgtcggagctttggagtcctgacgatacggcttgtacttcttctcaatggagttaattgacgccactgagtttggatcaatgtccggcatattctcaccgaagtaagcatgtgcacgaagacagtgaccatcgtagccatccgtatataccttgatcttgttgggatctttggtagtcaacgcagagatacgatcctctaacgaggcgaagtctaaaccacagaacatccagcccggtggagcttggaagcaagacttgatgagcttggcatagccagagtttgcaggcaggttctgtaggttcggatcagatgaactgagacgaccagataccgtgccaccaaggttgaagttaccgaacagataatgccagccatccggcccctcaccagcattcttcatcgcagggatgaagctggtaaggatcttgttcaccgcaccgtaatcctgaagtgctttcaggaaatccagcacatctggatcagtggtgtggttaagcaatgcctcaatggtgtccccgtcagtgcttggttgcttgctgtcagtcagactgataacaggcagatccaatacattgaacagcagatcctgcaattgcaggttactgtttgggttgaaggtaatttcgtcgataactttttcgttggttgaggaaagcacctcttccaccgtggtacgtttctgcttccacttggcgtgcatcttctcgatatagcgttccaccaatcgatagctgtactcctgaatgattttagagttacgcatacggctgaccgacttgtcatagtcgatctgtaagagagcctctacctcaaagactcgcttcatattcagaggcatacccgtcaactgcatctggataacatccagagtagctggcttgaataacgtctcgtaaatatttagctgctcatcctgcaccatcgtgtcgtagtgcttctcggcaacatgccaagtagcaagaccatccacgaggttgtacttcagcagttgatccaaaggaatcttggttatgtccttgatttcatcttgggcatagttaccagtgaactcctgagactggcttttaagatcgagcttattgccagcacaactgtttgttgcaaggtagctgatcagcttggtgtcatcccagtttcgcaacaggatgcccatgcctttcagcagaccttctgtatccagaatatcagacatatagagctgataaatcagcacatacgcatcataggcaatgttgtgatacagagccgtttccagatactgctcgaagaaagcacggagcattcttctcactggttcattacgaacgttacgcccgtaatgtttaccttctttttcgtcgagccactcctcttcgacataatcgacagggaaggcaataccctcatgcttgttccagcagaaggtaatcgtaccgatcccggcagtgtgatgtttcaggctgaacgcctcaatatcaattgccagagggcatttcatctcaagcagcttgaccagccactcctcgatttcgtggagttgctttggataggcagcgtatttgatgatgtccacacccggcgtttgatactgaccagaagcatggtcatacagagcattcataccctgagcaatcttgctctttaccttatctggatcatagaaaatggcccgatagttaggaacatagatcgctttaacaccatattcggtgtccatcacatagccgagattggcctcgacttttgcagctttggtcagagctttgaaatactctgagtcagccaccagtacatattgcaccttgaaatcctgccacacaggcacgagttcttcggttatgtactgacgcatctcagccattggggttttctttttcccctctgcctgatgcagcgtaagcaccatcacatgctctggatcgactccatagtctgtgaagtatgctcgttggatctcatcctttcggatgcttggaaccaagaggcaaacgggatattcgttagcgtctgcgaatgttaggtaagccataggttccccgttagtaaatcatgcgagccattgcgtacacagcaattgttggttccagcttcttcagatgacgcagcacacgaggctcttttgggaaagcctcttcaattggcagcgttcgctgaagttttgccacggtatgagcaaaaggaaccagtaactcaggcatacggttacgaacttcctgatcacttccagccatcatgacgttgaacagcaactgacgaatctgttgtctgtccagacctaccttcttgtaatctttcaggaaggcttccatgcgatcattaaggctgaagtccagcattggcaatcgaccgatttgagtagctctggtatgacggtagtaaactccgttgtacataaagcccatctcagctttgcctgatacctctctgtgagcatcgaccaactggtcaatactcttgaggatacgacgatcctcagcctcgaataaggtgtcagtgattgcttcaatttcctgcgaaagtgttgtcattggatcctcatggaaggattaagccaccgtacttttcggcaaggttgccatagagcactacacggttacgagaacgtgtgaatcccacatacagcagacgagccgcagtatccgggttgtgacaggttgacagattggcaaggtcgatgaacgttgtgccatacgagctaccctgagacttatgaacagtctgggaatcacgctggcggagatcagggaagttgttcttcaggaagaagtaacgttcaaaattacgctgctgaccgaaatacttcatcagcttcgtaaaatactccatatccactggcactttcacgccggggataacttcaccgagacttgtctccagtgttgtataacggaagtcaagctgggtgtctttggttacatccagcgtctctggttctgactggctcagaatagtgacttcctgctccacacgtaacatgcctttgccgaagcgaatggcattgttgttgatcaggcgttcgcctacggtgaagctgtgaggcagaccacgcaactgacggatatacgtgttgtaatccagtacctgtcggttggtgtaggcgaggatgcgagcatccacgttctcatcgataaaatgcttatcgacctctgcttgcatctccgatccagaaaggaaatcgatgacgccgggaatgattttgattgggttgaatacgccagttctcactgtctcacgaagctgtgtgcacacctctatcagctctggctggcctgcatttcgcattggctcagtcagttcaaatagttggatgccacgcttgtagataggcgagattgtctccatgaccggagcaagctggaacatatcacccacgtagacgattttgcactgaatggtgccttccagaagatgctctaacagagcacgatctatcatggaacactcatctacgaagataatcttcttgttataaacctgccaagagtggtttttgctgatatagctcttaccagtgttgtagtcgtctttgactttcaggttcataaacgagtgaatggtgcctgcatcacgctgggtactaagtgagagtacctctgctgctttgttggtagtagcagtcatcaccacctgatcatactcaggttcgatgcccatgatcttacaggtctggaaatactgaggcaggatcgtatcgatcatatgccccatgagaaacgttttaccgtacccaccagcaccagagataattaactctttctccgggctgaacaggaagtggaaaaatccttctgccgcagcctgttgaccttggttcaaggttgcggtctgtggtgttgccagcattggaacactcctaagcaaaaagccatctttcgatggctctgtggaaagaccgcagtggctttagctttgcggcacgtaaggggaaaggttagctacgaagtattgtgggccttttttgatcttccgattttcatcgaaaagaggctcaccatcgacaaacttagagaagtttgaagagtttacttccatcatgccaccatgaatttggtagcccagcatgtgtgctgtacctacggcagtaacgatctgatcgcaaagtgcgtccagcatttctaccccatcaggaacaacatacttgagacgctcatcagacttcttcaggtgatcggcgaggttgcccagatagtcagcagcctgactgatgagaatatcagtcgtatggtctgtgcctttcatggctcgcagcatctcgcatacttcctcgaaatgcacaccagtctgaacgttgatgttcttggttcccggagtaggcacagccttctcgaaccaaagaacagtatcaaatagtgggtttggcattagcatcactcttcatgtaagcctgaaccagcaggttcttcacgaagtctttgactgtgatatgtgggccgagttgatcggctaaccattcctgctgattcggggtcagtgttacgaatatgtcttccataaaggctcgacgtgtatcggcaggaggaacacccatagccttgaggcgtagcgtgatagttgttgggtggcagcccgccaacttacctatagttttgagtgaaaggccaacgctgttcatgcggatgagatcgtcgtcttccacctttctattggcacggtatacatttgacatgattgttactcccataaaaaatacctctagtctatacagactagaggtattatggaagtcagcaattacttgcttttggcttcgatttcagcttgctcgtcaggagtgacgcccagtgcctgccaacccttcttggctttcttcttgatcagaagaattgcctgatactgaatggttgtcagaggacgctgatccagcatctcacggatgagagcagacgggccagaaccgcctttacggttgttctgcttacgtgcttcagctttggcattatctgcctgaatctgatcggcacgttcgttggactgcttcggcaggctacccatgatctgattaacttcagtcggggtaaagccgagtttgtcccagcctttcttggcaccggatttcattttcagcagcttctgggcagcagcactcgctacatcgctggtttgagcagcttgcaactcgtccatcgcctgagcaaatggcagagtcttactgacaaccttggctgtcttagccttggttttggccttagctttcgctttagccttggctggtttcttgaccactttctcttccttcactggttcagcaggtttagctggagccagatcattagcgttaatcgccggggcagagttctggactggatccagtgcctcttccatatccagcgtctcgcctgttaccagtggagacgctgccagttcgtcagcagagccgacatcaacatcggtgtattcgatcttggtgccgttgtgaccgccaaccttaacgtgctggcttacacgaacgtgattaccagcgatgatgttacccagaatcactgcaccctctggatgagaggacagtgacttaccactgttcacaatgtctgccagatgacgaggcaggtcgtaaacgatgtggtagccggatacacgcatcttgttatggctgtactctggcacagcgaacacgtcttcagggcgaaccttaccaacgatggtaacgtcaccactgaagccgccgatgtaagagagagtcgctacgtgcagaccgttggaacagtcacggcgacgatttggatccaccagctcaggcagcaggaagacgtaagagccgaccttttgcttgatgttgccggagtgaacgtcggtgaagtaacctgtcttacggttcagacgcttgtagataacgatacagccgtcatctgcaattggcaggtcgccataagcgatgaacttcatcagatcttcaaccgagtgagcacggtctttgatgatgagttccagccgcttgatgaagttggtgaagcctttgtaattcttcagcttctccgcacctttcaactggcgtgccagattgtgagcatctgggatcaccgaaccagtctgcgtatttaacgcaacgatggtttcagttttctcatccagtggcttatggaaatcagcgtggtcagtgcctttaccattgccgatcagttgttccatacgctcagaggcgagatcaactttctggtcattggtcagttctggttccacttccacaacaggtgcaactggtgctacagtctcaaccgcatcaggtttggactcggtttcctgccccggaaacgtaccgatctccagaggagaaatgtgagcagcttcgccgtccaccttctctggagattcggtatccagcagatctttgacgaacttcttcgctacacggaagaatttcaccagaccgccagtacctttctcagcagcactgtattcagtacgctcagcgatacgtggagtcacatcgacttccaccggcagattcttgctcagtggttcctgagccactgccacgatttccggcaggcgaagatcgccctgtggaatcgtgatagtgttaccgtccaccgtatacagcgtggcgttgcgactgtcgattgacagtgcaacgatggtcacgaattgttttttcatttcttggttccgtttttaagtgcactcaaaacgagggttttaagagcggattttcgctccgggaatttagccatcagatggatgatctcctgaccgttaccgagcttgcgcacgataggatcgtttctgaaagctattacctttttcacaaaaggtaatttgtttgcatcgagatgaagaccttccagatcatcaaccaatgcactcacattggatacttccagcccttcgatgtattgatacagatcccaatggttattggtttcatacatacgtctgtaggcttccagtcgcacgtcatgacgcatcttgtcgtaaccgaccagcttaaccttgagaatacgcagcagagccagatcagacgaggtaacgccgatttccggcagacctgcctgacgatactgcgtcatatactcacggtattctgtgctggtgatgacgtcatggaacttctgtgcaaaggcactatcaatgtccactgcaccacgcttgattgccatacgctcctctgtgccgttacggatgataacggtacgagtacgctcatcggcagtcataagctgtatgtgagcaaatttgccaatacgaccagaacggaaagtagactgataacgcacaaagaacagagggctatcagtagtgataagaccttgtttatcaacgttcatttccttaatgtcggaagacacggcaatctgcttattcgtcactggatcaaagatattatccagtgagatcatcagattcttcggcttcgccacaactttatcgtcagcggttagtttcttggtctttgcacgagttttagccgcagctttgatttcctgtgccacaggatcccagttatgtttctgagtcagatccaccacttccagacctgcatcctcaaagagcttacagatctctgggatgtttttggcagtaggcgacacacgatagaaccagcaagaagcatgaccaccacgtccaccatcgtcataacgagggaacttgttgatacttctgctcagacttttcacacgagtggtgacgaagattgtcgggcgatcaatcattgccttcagttcgtcgaactcatggatctctgacacctgattaaaggcgtttttgatatagtccttgcggtcatagtagtgacgctgagagaagcctaagccttccagattcagcacatcacgattggcatagaagaacttgcccatcggtttgatgatgtactgctttacaaacttctcagcattggattggttataccaagtgctgtgaccagtacgacgatgcgaggtacgatcccggaaatggaaacgcagtctgtgcaatttagtcgtagcaatcttgctgtttttgaactggtgtacacgcttaaagccgatactctcagaaccaaatagatgcttctcatgcttgacgtacagagcagatccaaggtgggatgacagatacttacgcagagcactgtgacggatccattcaaggggattcgcacgacgactcattgtggcttgatcttttgttacctgagtacgcagacgcacatgagcctcagcaatggcggcaggagccatagcaatcagatcatcttcgatgcgttttaccagtgacagacagagatcggacaggccatcctctgtcattttctggctcgataaagtctcacgacttggtgataacgcaagcgtacccggtgcagcttgcaccagcattttgccgtagccaatcagctcgacaaaacggttaagcatttgcaatgccttagcagtaccgggagtctccagcattggatacaccacagcaccgtaacgcacgaacagagcagtaccacgtcccatatagcgagcgtaccacttttcatggtcgatgctgtatgaacccggctcttgagacatacccagtgttgggaggatctcagtgctaccctgcatgttgaactgaacgttcatctcgccgtgcatcacgatgtacttgatgtacatcacgatttcctgcacgtcttcagggttcagcttcagcgatacagtcagaccagtg

SEQ ID NO: 5 - DNA, 22 bp, synthetic construct
  source 1..22: mol_type = other DNA
agtctttgttgccagtgagtgc

SEQ ID NO: 6 - DNA, 20 bp, synthetic construct
  source 1..20: mol_type = other DNA
atccgaaagatggccgtaac

SEQ ID NO: 7 - DNA, 22 bp, synthetic construct
  source 1..22: mol_type = other DNA
ccgccaccatactgtactgcca

SEQ ID NO: 8 - DNA, 90 bp, synthetic construct
  source 1..90: mol_type = other DNA
agtctttgttgccagtgagtgctttcttaccgccaccatactgtactgccatgtatggagtcttgatgaagttacggccatctttcggat

SEQ ID NO: 9 - DNA, 20 bp, synthetic construct
  source 1..20: mol_type = other DNA
ttcgtcaagggatgatgctg

SEQ ID NO: 10 - DNA, 20 bp, synthetic construct
  source 1..20: mol_type = other DNA
atcttgcggattccatcacc

SEQ ID NO: 11 - DNA, 25 bp, synthetic construct
  source 1..25: mol_type = other DNA
cgctgagttccttgaggcacatatg

SEQ ID NO: 12 - DNA, 112 bp, synthetic construct
  source 1..112: mol_type = other DNA
ttcgtcaagggatgatgctggatagcgcacaaggcgaatcagagatggtcgctgagttccttgaggcacatatggagcgtgaggtgatgggcggtgatggaatccgcaagat

SEQ ID NO: 13 - DNA, 20 bp, synthetic construct
  source 1..20: mol_type = other DNA
accacgacatgatccgtcag

SEQ ID NO: 14 - DNA, 20 bp, synthetic construct
  source 1..20: mol_type = other DNA
gtgtctgggaacggacaaca

SEQ ID NO: 15 - DNA, 20 bp, synthetic construct
  source 1..20: mol_type = other DNA
cggtcgggaacgttgtttgc

SEQ ID NO: 16 - DNA, 162 bp, synthetic construct
  source 1..162: mol_type = other DNA
accacgacatgatccgtcagctgattcggtgtgtagttaaacgtcgaacctgaaccgggtaaatcggtcgggaacgttgtttgccagacacgcaggtgcttcttctggttaagcgttccgtcaaacatgacggtgtagtatttgttgtccgttcccagacac

SEQ ID NO: 17 - DNA, 20 bp, synthetic construct
  source 1..20: mol_type = other DNA
gtggatccactcagtgcaca

SEQ ID NO: 18 - DNA, 20 bp, synthetic construct
  source 1..20: mol_type = other DNA
cggtcagcgagcaatttagc

SEQ ID NO: 19 - DNA, 20 bp, synthetic construct
  source 1..20: mol_type = other DNA
ccgtgacgagcaactccggg

SEQ ID NO: 20 - DNA, 154 bp, synthetic construct
  source 1..154: mol_type = other DNA
gtggatccactcagtgcacagctctcgcaagccatgcagccgaactcgacagatctcttgaacaaggccgatctttggtacgagaactcagggaaactcttagattccgtgacgagcaactccgggcagtaagtgctaaattgctcgctgaccg